European Patent Application EP 4 186 977 A1, published May 31, 2023. Title: PLANT REGULATORY ELEMENTS AND USES THEREOF. Applicant: Monsanto Technology LLC. Application US PCT/US2012/036955, filed May 8, 2012. The sequence listing filed with the application follows.

SEQUENCE LISTING (212 sequences)

SEQ ID NO: 1 - DNA, 2611 bp, Cucumis melo
  source 1..2611: mol_type = other DNA
atctgaaaggaacacctagcaaggggctactctacaagcatactaagtctacaaagctagagttgtatggttatgcagaagacctggacaaaagaagatcactcgctgcttttacttttatcctaagaggaaatgtgattttatggaagtttaacctatagcctgtagtggcactattcacaacaaaagtaaagtttatagccatgactgaagttgttaaagaagtcgtctggctaaaaggactacttgaagaacttggcttcttttaacagtcagtaaacatcatgtgtgatagttaaagtgcaatacacttgtctaaaaatctgcaatatcacgaaagaactaagcatattgatgtgaagctatatgtcattagagaagtcatagcaaagagaaaagtaacagtatcaaaggttcagacaaaagaaaatgcagcagatatgttgactaaaatagttactaatgctaaactcgagcactgcctacagttgctcaaggtaatagactacttaaaagaatagaatcagaagaaatagtcattggtagcaataaaattcaaggtggaggattgttaaaaagaagagtgaattttattacttaaagaaaatctcggtgaaactcgaaagatctcgattcgaaactctattgcttaagaacctggtgaagctcgagagatcttgatacaatcccagtgccctaactcttcaacaagctaagcaagttgtactgtggggctcaatctcggttcaatctcgacgcacctgatgctttgttccctgtctactcgatgaagaagcaattacttctcaggacaactcggtacccctaaatacagattttgagcttcgtgatcctacaactgaaatcaaatagaaaaactaataagttagttagagtttgttatatttactgccattaaataactctgtaatgtaaataataaaccatttaactcaatatgaaatatagaatgagaaaaagaaaaagaaaaagttaaagagagagaggaagaaaactcattttcaaattctctatacttgtttgatccttgaataagttgaataaaagctctatggcggcttcaaagtggatgtaggcactattagtcgaaccacaataaatttgttatgttcttttgctattccttgtaatctccataaatattttcttactaagctctagaaatctgcttgtcaagagattaggtatcatttatgccttttatatttcctttcggttgcatatcttgagctagttaagatcgagaggttactgttgttgaaaccgagattagtatctttggattaacacgtgcctaccaaaatttgaaattttgtatttaccccattcattggataataagcaattcttatagtgttatcaattaaactcctataaagtgtaataattgaatccatgaactattttcatatgtaatcttaataaaatgaatttagaagtttaattaaaataatatattttgtatgctatttttcaaagtttgaagaatgtgttaattgatacacatacaaaaaatctaggttttacatgaaaaactatggaagtgaaagatagcatctaatattttatgacacaaaatgcaaactaatatataaaggatttaattaatttttataggtttcaaatttgttagacttgtcaaatacaaaattttattgaaccaaatacatacaaacatcaaaattaagaacagaaaatctaaattcaaatgaaatttattaatagaaaaattagaaaaaagaaaaagaaaataaaaggaatcgtattgttttttccttcctttttcccatttgagaggtgaataaagctaattgagctgctctaacttcctaatctttatgctttccccataaagctttcccaactgcgcgtaatcgtataaatggaaaattgacctttccaactagattcttccagaactaaacaatacgtaacacgcaagtaatcaaagacacgtttcattttcctatagaatattatagttattcgtgattaacggaagtcggcaattttaggtataaatacgtgaattctcgagcgctaattttccatacagactcgaaatactctaaactttctcatcgcgctttattcctatttcgtaattcgctcttcttcaacctctcaaggttttcatcttttctctatcttctgttttcagattgcatcttttccccctcctgttcgattaattgatgtttgaattttcgagaaacgatttgaagtctttgttgtatttttcatttctgttcgttaggtaggtcgatttttaatcgtgatgtccgacgttgttcggatgattcacatttggtttttgtcatcttctttctatgttgtgattatcatgatttttatctttttttcttctcaagatttgtaatttatcgattccccatggttcttggttttttatacatgtattgaatctggttactagaattatgttcttcgacggacgtctttcagatttaaattgcattgtaggaaatatgatttgctatctgagtaacgtttttccagagtattcttgattgcgcgatctatcttcaattgttaaattgtttttgtttaattggggtcatgacaggtg

SEQ ID NO: 2 - DNA, 2068 bp, Cucumis melo
  source 1..2068: mol_type = other DNA
atctgaaaggaacacctagcaaggggctactctacaagcatactaagtctacaaagctagagttgtatggttatgcagaagacctggacaaaagaagatcactcgctgcttttacttttatcctaagaggaaatgtgattttatggaagtttaacctatagcctgtagtggcactattcacaacaaaagtaaagtttatagccatgactgaagttgttaaagaagtcgtctggctaaaaggactacttgaagaacttggcttcttttaacagtcagtaaacatcatgtgtgatagttaaagtgcaatacacttgtctaaaaatctgcaatatcacgaaagaactaagcatattgatgtgaagctatatgtcattagagaagtcatagcaaagagaaaagtaacagtatcaaaggttcagacaaaagaaaatgcagcagatatgttgactaaaatagttactaatgctaaactcgagcactgcctacagttgctcaaggtaatagactacttaaaagaatagaatcagaagaaatagtcattggtagcaataaaattcaaggtggaggattgttaaaaagaagagtgaattttattacttaaagaaaatctcggtgaaactcgaaagatctcgattcgaaactctattgcttaagaacctggtgaagctcgagagatcttgatacaatcccagtgccctaactcttcaacaagctaagcaagttgtactgtggggctcaatctcggttcaatctcgacgcacctgatgctttgttccctgtctactcgatgaagaagcaattacttctcaggacaactcggtacccctaaatacagattttgagcttcgtgatcctacaactgaaatcaaatagaaaaactaataagttagttagagtttgttatatttactgccattaaataactctgtaatgtaaataataaaccatttaactcaatatgaaatatagaatgagaaaaagaaaaagaaaaagttaaagagagagaggaagaaaactcattttcaaattctctatacttgtttgatccttgaataagttgaataaaagctctatggcggcttcaaagtggatgtaggcactattagtcgaaccacaataaatttgttatgttcttttgctattccttgtaatctccataaatattttcttactaagctctagaaatctgcttgtcaagagattaggtatcatttatgccttttatatttcctttcggttgcatatcttgagctagttaagatcgagaggttactgttgttgaaaccgagattagtatctttggattaacacgtgcctaccaaaatttgaaattttgtatttaccccattcattggataataagcaattcttatagtgttatcaattaaactcctataaagtgtaataattgaatccatgaactattttcatatgtaatcttaataaaatgaatttagaagtttaattaaaataatatattttgtatgctatttttcaaagtttgaagaatgtgttaattgatacacatacaaaaaatctaggttttacatgaaaaactatggaagtgaaagatagcatctaatattttatgacacaaaatgcaaactaatatataaaggatttaattaatttttataggtttcaaatttgttagacttgtcaaatacaaaattttattgaaccaaatacatacaaacatcaaaattaagaacagaaaatctaaattcaaatgaaatttattaatagaaaaattagaaaaaagaaaaagaaaataaaaggaatcgtattgttttttccttcctttttcccatttgagaggtgaataaagctaattgagctgctctaacttcctaatctttatgctttccccataaagctttcccaactgcgcgtaatcgtataaatggaaaattgacctttccaactagattcttccagaactaaacaatacgtaacacgcaagtaatcaaagacacgtttcattttcctatagaatattatagttattcgtgattaacggaagtcggcaattttaggtataaatacgtgaattctcgagcgctaattt

SEQ ID NO: 3 - DNA, 82 bp, Cucumis melo
  source 1..82: mol_type = other DNA
tccatacagactcgaaatactctaaactttctcatcgcgctttattcctatttcgtaattcgctcttcttcaacctctcaag

SEQ ID NO: 4 - DNA, 461 bp, Cucumis melo
  source 1..461: mol_type = other DNA
gttttcatcttttctctatcttctgttttcagattgcatcttttccccctcctgttcgattaattgatgtttgaattttcgagaaacgatttgaagtctttgttgtatttttcatttctgttcgttaggtaggtcgatttttaatcgtgatgtccgacgttgttcggatgattcacatttggtttttgtcatcttctttctatgttgtgattatcatgatttttatctttttttcttctcaagatttgtaatttatcgattccccatggttcttggttttttatacatgtattgaatctggttactagaattatgttcttcgacggacgtctttcagatttaaattgcattgtaggaaatatgatttgctatctgagtaacgtttttccagagtattcttgattgcgcgatctatcttcaattgttaaattgtttttgtttaattggggtcatgacaggtg

SEQ ID NO: 5 - DNA, 2002 bp, Cucumis melo
  source 1..2002: mol_type = other DNA
tcggtgaaactcgaaagatctcgattcgaaactctattgcttaagaacctggtgaagctcgagagatcttgatacaatcccagtgccctaactcttcaacaagctaagcaagttgtactgtggggctcaatctcggttcaatctcgacgcacctgatgctttgttccctgtctactcgatgaagaagcaattacttctcaggacaactcggtacccctaaatacagattttgagcttcgtgatcctacaactgaaatcaaatagaaaaactaataagttagttagagtttgttatatttactgccattaaataactctgtaatgtaaataataaaccatttaactcaatatgaaatatagaatgagaaaaagaaaaagaaaaagttaaagagagagaggaagaaaactcattttcaaattctctatacttgtttgatccttgaataagttgaataaaagctctatggcggcttcaaagtggatgtaggcactattagtcgaaccacaataaatttgttatgttcttttgctattccttgtaatctccataaatattttcttactaagctctagaaatctgcttgtcaagagattaggtatcatttatgccttttatatttcctttcggttgcatatcttgagctagttaagatcgagaggttactgttgttgaaaccgagattagtatctttggattaacacgtgcctaccaaaatttgaaattttgtatttaccccattcattggataataagcaattcttatagtgttatcaattaaactcctataaagtgtaataattgaatccatgaactattttcatatgtaatcttaataaaatgaatttagaagtttaattaaaataatatattttgtatgctatttttcaaagtttgaagaatgtgttaattgatacacatacaaaaaatctaggttttacatgaaaaactatggaagtgaaagatagcatctaatattttatgacacaaaatgcaaactaatatataaaggatttaattaatttttataggtttcaaatttgttagacttgtcaaatacaaaattttattgaaccaaatacatacaaacatcaaaattaagaacagaaaatctaaattcaaatgaaatttattaatagaaaaattagaaaaaagaaaaagaaaataaaaggaatcgtattgttttttccttcctttttcccatttgagaggtgaataaagctaattgagctgctctaacttcctaatctttatgctttccccataaagctttcccaactgcgcgtaatcgtataaatggaaaattgacctttccaactagattcttccagaactaaacaatacgtaacacgcaagtaatcaaagacacgtttcattttcctatagaatattatagttattcgtgattaacggaagtcggcaattttaggtataaatacgtgaattctcgagcgctaattttccatacagactcgaaatactctaaactttctcatcgcgctttattcctatttcgtaattcgctcttcttcaacctctcaaggttttcatcttttctctatcttctgttttcagattgcatcttttccccctcctgttcgattaattgatgtttgaattttcgagaaacgatttgaagtctttgttgtatttttcatttctgttcgttaggtaggtcgatttttaatcgtgatgtccgacgttgttcggatgattcacatttggtttttgtcatcttctttctatgttgtgattatcatgatttttatctttttttcttctcaagatttgtaatttatcgattccccatggttcttggttttttatacatgtattgaatctggttactagaattatgttcttcgacggacgtctttcagatttaaattgcattgtaggaaatatgatttgctatctgagtaacgtttttccagagtattcttgattgcgcgatctatcttcaattgttaaattgtttttgtttaattggggtcatgacaggtg

SEQ ID NO: 6 - DNA, 1459 bp, Cucumis melo
  source 1..1459: mol_type = other DNA
tcggtgaaactcgaaagatctcgattcgaaactctattgcttaagaacctggtgaagctcgagagatcttgatacaatcccagtgccctaactcttcaacaagctaagcaagttgtactgtggggctcaatctcggttcaatctcgacgcacctgatgctttgttccctgtctactcgatgaagaagcaattacttctcaggacaactcggtacccctaaatacagattttgagcttcgtgatcctacaactgaaatcaaatagaaaaactaataagttagttagagtttgttatatttactgccattaaataactctgtaatgtaaataataaaccatttaactcaatatgaaatatagaatgagaaaaagaaaaagaaaaagttaaagagagagaggaagaaaactcattttcaaattctctatacttgtttgatccttgaataagttgaataaaagctctatggcggcttcaaagtggatgtaggcactattagtcgaaccacaataaatttgttatgttcttttgctattccttgtaatctccataaatattttcttactaagctctagaaatctgcttgtcaagagattaggtatcatttatgccttttatatttcctttcggttgcatatcttgagctagttaagatcgagaggttactgttgttgaaaccgagattagtatctttggattaacacgtgcctaccaaaatttgaaattttgtatttaccccattcattggataataagcaattcttatagtgttatcaattaaactcctataaagtgtaataattgaatccatgaactattttcatatgtaatcttaataaaatgaatttagaagtttaattaaaataatatattttgtatgctatttttcaaagtttgaagaatgtgttaattgatacacatacaaaaaatctaggttttacatgaaaaactatggaagtgaaagatagcatctaatattttatgacacaaaatgcaaactaatatataaaggatttaattaatttttataggtttcaaatttgttagacttgtcaaatacaaaattttattgaaccaaatacatacaaacatcaaaattaagaacagaaaatctaaattcaaatgaaatttattaatagaaaaattagaaaaaagaaaaagaaaataaaaggaatcgtattgttttttccttcctttttcccatttgagaggtgaataaagctaattgagctgctctaacttcctaatctttatgctttccccataaagctttcccaactgcgcgtaatcgtataaatggaaaattgacctttccaactagattcttccagaactaaacaatacgtaacacgcaagtaatcaaagacacgtttcattttcctatagaatattatagttattcgtgattaacggaagtcggcaattttaggtataaatacgtgaattctcgagcgctaattt

SEQ ID NO: 7 - DNA, 1507 bp, Cucumis melo
  source 1..1507: mol_type = other DNA
agtcgaaccacaataaatttgttatgttcttttgctattccttgtaatctccataaatattttcttactaagctctagaaatctgcttgtcaagagattaggtatcatttatgccttttatatttcctttcggttgcatatcttgagctagttaagatcgagaggttactgttgttgaaaccgagattagtatctttggattaacacgtgcctaccaaaatttgaaattttgtatttaccccattcattggataataagcaattcttatagtgttatcaattaaactcctataaagtgtaataattgaatccatgaactattttcatatgtaatcttaataaaatgaatttagaagtttaattaaaataatatattttgtatgctatttttcaaagtttgaagaatgtgttaattgatacacatacaaaaaatctaggttttacatgaaaaactatggaagtgaaagatagcatctaatattttatgacacaaaatgcaaactaatatataaaggatttaattaatttttataggtttcaaatttgttagacttgtcaaatacaaaattttattgaaccaaatacatacaaacatcaaaattaagaacagaaaatctaaattcaaatgaaatttattaatagaaaaattagaaaaaagaaaaagaaaataaaaggaatcgtattgttttttccttcctttttcccatttgagaggtgaataaagctaattgagctgctctaacttcctaatctttatgctttccccataaagctttcccaactgcgcgtaatcgtataaatggaaaattgacctttccaactagattcttccagaactaaacaatacgtaacacgcaagtaatcaaagacacgtttcattttcctatagaatattatagttattcgtgattaacggaagtcggcaattttaggtataaatacgtgaattctcgagcgctaattttccatacagactcgaaatactctaaactttctcatcgcgctttattcctatttcgtaattcgctcttcttcaacctctcaaggttttcatcttttctctatcttctgttttcagattgcatcttttccccctcctgttcgattaattgatgtttgaattttcgagaaacgatttgaagtctttgttgtatttttcatttctgttcgttaggtaggtcgatttttaatcgtgatgtccgacgttgttcggatgattcacatttggtttttgtcatcttctttctatgttgtgattatcatgatttttatctttttttcttctcaagatttgtaatttatcgattccccatggttcttggttttttatacatgtattgaatctggttactagaattatgttcttcgacggacgtctttcagatttaaattgcattgtaggaaatatgatttgctatctgagtaacgtttttccagagtattcttgattgcgcgatctatcttcaattgttaaattgtttttgtttaattggggtcatgacaggtg

SEQ ID NO: 8 - DNA, 964 bp, Cucumis melo
  source 1..964: mol_type = other DNA
agtcgaaccacaataaatttgttatgttcttttgctattccttgtaatctccataaatattttcttactaagctctagaaatctgcttgtcaagagattaggtatcatttatgccttttatatttcctttcggttgcatatcttgagctagttaagatcgagaggttactgttgttgaaaccgagattagtatctttggattaacacgtgcctaccaaaatttgaaattttgtatttaccccattcattggataataagcaattcttatagtgttatcaattaaactcctataaagtgtaataattgaatccatgaactattttcatatgtaatcttaataaaatgaatttagaagtttaattaaaataatatattttgtatgctatttttcaaagtttgaagaatgtgttaattgatacacatacaaaaaatctaggttttacatgaaaaactatggaagtgaaagatagcatctaatattttatgacacaaaatgcaaactaatatataaaggatttaattaatttttataggtttcaaatttgttagacttgtcaaatacaaaattttattgaaccaaatacatacaaacatcaaaattaagaacagaaaatctaaattcaaatgaaatttattaatagaaaaattagaaaaaagaaaaagaaaataaaaggaatcgtattgttttttccttcctttttcccatttgagaggtgaataaagctaattgagctgctctaacttcctaatctttatgctttccccataaagctttcccaactgcgcgtaatcgtataaatggaaaattgacctttccaactagattcttccagaactaaacaatacgtaacacgcaagtaatcaaagacacgtttcattttcctatagaatattatagttattcgtgattaacggaagtcggcaattttaggtataaatacgtgaattctcgagcgctaattt

SEQ ID NO: 9 - DNA, 1022 bp, Cucumis melo
  source 1..1022: mol_type = other DNA
tgacacaaaatgcaaactaatatataaaggatttaattaatttttataggtttcaaatttgttagacttgtcaaatacaaaattttattgaaccaaatacatacaaacatcaaaattaagaacagaaaatctaaattcaaatgaaatttattaatagaaaaattagaaaaaagaaaaagaaaataaaaggaatcgtattgttttttccttcctttttcccatttgagaggtgaataaagctaattgagctgctctaacttcctaatctttatgctttccccataaagctttcccaactgcgcgtaatcgtataaatggaaaattgacctttccaactagattcttccagaactaaacaatacgtaacacgcaagtaatcaaagacacgtttcattttcctatagaatattatagttattcgtgattaacggaagtcggcaattttaggtataaatacgtgaattctcgagcgctaattttccatacagactcgaaatactctaaactttctcatcgcgctttattcctatttcgtaattcgctcttcttcaacctctcaaggttttcatcttttctctatcttctgttttcagattgcatcttttccccctcctgttcgattaattgatgtttgaattttcgagaaacgatttgaagtctttgttgtatttttcatttctgttcgttaggtaggtcgatttttaatcgtgatgtccgacgttgttcggatgattcacatttggtttttgtcatcttctttctatgttgtgattatcatgatttttatctttttttcttctcaagatttgtaatttatcgattccccatggttcttggttttttatacatgtattgaatctggttactagaattatgttcttcgacggacgtctttcagatttaaattgcattgtaggaaatatgatttgctatctgagtaacgtttttccagagtattcttgattgcgcgatctatcttcaattgttaaattgtttttgtttaattggggtcatgacaggtg

SEQ ID NO: 10 - DNA, 479 bp, Cucumis melo
  source 1..479: mol_type = other DNA
tgacacaaaatgcaaactaatatataaaggatttaattaatttttataggtttcaaatttgttagacttgtcaaatacaaaattttattgaaccaaatacatacaaacatcaaaattaagaacagaaaatctaaattcaaatgaaatttattaatagaaaaattagaaaaaagaaaaagaaaataaaaggaatcgtattgttttttccttcctttttcccatttgagaggtgaataaagctaattgagctgctctaacttcctaatctttatgctttccccataaagctttcccaactgcgcgtaatcgtataaatggaaaattgacctttccaactagattcttccagaactaaacaatacgtaacacgcaagtaatcaaagacacgtttcattttcctatagaatattatagttattcgtgattaacggaagtcggcaattttaggtataaatacgtgaattctcgagcgctaattt

SEQ ID NO: 11 - DNA, 716 bp, Cucumis melo
  source 1..716: mol_type = other DNA
tcgtataaatggaaaattgacctttccaactagattcttccagaactaaacaatacgtaacacgcaagtaatcaaagacacgtttcattttcctatagaatattatagttattcgtgattaacggaagtcggcaattttaggtataaatacgtgaattctcgagcgctaattttccatacagactcgaaatactctaaactttctcatcgcgctttattcctatttcgtaattcgctcttcttcaacctctcaaggttttcatcttttctctatcttctgttttcagattgcatcttttccccctcctgttcgattaattgatgtttgaattttcgagaaacgatttgaagtctttgttgtatttttcatttctgttcgttaggtaggtcgatttttaatcgtgatgtccgacgttgttcggatgattcacatttggtttttgtcatcttctttctatgttgtgattatcatgatttttatctttttttcttctcaagatttgtaatttatcgattccccatggttcttggttttttatacatgtattgaatctggttactagaattatgttcttcgacggacgtctttcagatttaaattgcattgtaggaaatatgatttgctatctgagtaacgtttttccagagtattcttgattgcgcgatctatcttcaattgttaaattgtttttgtttaattggggtcatgacaggtg

SEQ ID NO: 12 - DNA, 173 bp, Cucumis melo
  source 1..173: mol_type = other DNA
tcgtataaatggaaaattgacctttccaactagattcttccagaactaaacaatacgtaacacgcaagtaatcaaagacacgtttcattttcctatagaatattatagttattcgtgattaacggaagtcggcaattttaggtataaatacgtgaattctcgagcgctaattt

SEQ ID NO: 13 - DNA, 2000 bp, Cucumis melo
  source 1..2000: mol_type = other DNA
cttattcagcgctttcctgtaaaattaaagacttgatgagggagaaaaagaaaaccggttcgcagcttcaagaagacggcttccgaataagaatcagatactcgatgatggggaaacaataacaaagatatcaaaagaaatcatgaaacatagcataagaacgaaaacccagaggtgaagaacagtgcccaaacgcaactttacccaaagaacatgtataaaacgtcttccagacgttcaaaataagaaagtggacaaaatcaaagctacaaacgatctccaataactagatggaaaacactaattgcactagagattttgaatgctttgttgttgatttataatcctcgacttccaagaaaaagtaacaagtagaaatgaacgaatcagatccgcaatcgaagatctgaaggcaagataaggtaaggctaaagaaccataggaaaacggtaaaaacgtccaaaacagtgtgagaaatatcgcagattcaaaggtccgaaccctaagaacggtgttatgcagctataaaggtgagaatcaaaaccctctatccataacgtggacggcgcggttgaatcattgtcttgttccttgaaactgaaggtatgcgagacatagaattcgatctcactattatcttctaatcaacgacgaagtaaagaagtgaaatccagaacaaagaatggagaattggaaatgacaagaaaaacggcagaggaaagtggaaaagtgaaagcggactcacctagatcaatgcccttggctggtcgagcttcaggaacctgtcgtcggagagaaagagaaagagaaaagagcaagagagagagagagagagcacaaggagaagagaacgaggacaatggaggcttttgtttcgatactccctgatctggaattctataataacataactataaacttctctgggttggcccatcatcacgtatattgggcttttagcccaattatttgttcactgctcatgggccggtgattttgggctttcttctgggccttggtacataacaacccagtatatgacgtattttcggtgatagctattttcaagaacaccaacttttttgttcaacaatgtggagatcaaataacagtatgtatatatacacaaacatatgctcatttatgaaaaatagaaagaaaaagaatgttggtaatttgttacaaaattataatttctctctctttgtttgatttcatgaacggtgtgttctatataaaacaatgaaataacataattattaaaatgattcttaaaacatgatgatttcaatattcatggtttacatttggtgggatgattcgtttaattattattgataatgtatagttattgtgtgtcccgttttctttttctttggtggaagaaaagaaaaaagtaggaaggcatgtaatattgcgatccttcacgggacagatccattttccaatgtgatcgagtactagttaggtggagagtggaagaatcttcgtgcatgcataaatcaagtcacaacttgccaatttggaaagaatcatgttatattctacctttactttcaagtagggttaagtgaattagaccacaacgaagcaatcaagtccaaccaaactcacttaggtcaagcagtttagtgatatagacaggtcagtggtcgtttttttaatactaagaaatgtcaattctatctagttgactattattcatatagaaggagaaaaatgataactatgattgtcccacaaacaacaactaccgatcgatctaaaccaacaagtcgatgattggtgccactttaaatttaaatctgacgccactcaattgatgatcacccctattcaagcacacaagaacgcatgctcttaaaacatttggtaatatgattggaattagtacaaaatgtttattcgatctatacaaacaactcctttttaacacaaatgttttattgtactttcccgtgaaatggggttagtaaaactatggagttaataaaacataa

SEQ ID NO: 14 - DNA, 2000 bp, Cucumis melo
  source 1..2000: mol_type = other DNA
tataacaaaatatgtgaaattagccattatgtttgtcctttcgttcttcttattcacttcgttgcgatttctttctatcgtctatcgtctttcttcttttttctgttgaaatttattttcatcgtttttcttctttttccatcgtgaaaaaaatagtcaaatctaaatgatcgtgtataaagaataaacgatcgtgtagacaaatctaaatggtcgaatattaagaaaattgataggaaaatttattcattagaaaaattttagtaagaaaaattagaaatgaaagggttgaaccagaaagaaataaaagtaatagacaaatgaaaattttaaataaaaagaaatttgggatgggtgcatttactatttagtcttgagttttaattcttttattactttacataagatgtattaaattaaagaggtaagatagaatttttttttaaaaaaaactatcattagtaaatttaacaaaagtgacatagcaccattttcgttaaaagaataattgttttatgtagtaaaattggtagaaatattttttaagtatagcaaaatatctttgtctttttatatctttcactgacagataataataatttattaatatatcatttatatagtcccattttcggtaaattttaatatttgaacataaaacactatttaaaataatgaaaaaaaactttacaaacttttttatttttattatatttgtaaatatttctaaaaaattttacatttaaaataatattttcaaggttaatacagaagaaaaaaaacaaaaaaagaggaaaaggcaatttaagaagaatgacaagaaaatcgggaggtggtgtggctaagaggaagaagggaccggttcttcaagatccaacgctccacattcaatctcacttccttcttcaattccgtcttctccgtttcctcctttatatgcttctctctttccctccctttctttctctccttcaatcaatcaatcaatcaatcaatcaatcctcccattcccattacattgccaaaaggttctattctcattctctacatccatttccctttctttccttcttcttcctctgtttcttcttcgtttccttgattcatttctctttgtacgttccttccttccttctgcattttgattattttcttttgttttacgtccggaattgcaatgtggtttatctttatttctgtttttggacgtcaagatgcctgttgtttttaacattttgatttgattcatcgttcatggcgtaatcatgtcttttggaattgtttgaaatccaaggatcacattgatttcactattgtttcatttgttcttttttgttaattttgtataatgaatcgtataggggatcatttttccattggttctcttgaaaatctttaagagttgcattatgtatactaagtctctcttatggcgtctgtttgagtgagaattgataaaagatccatgggaggaagaagttttctttcatgaggcttggttttattcagctgtttcttctcgttgcaatttgttgaagaagggacatgggtatcttttacatcaaagtataactaactatataattcaatttggttgataaagtagatacatgtaggagtcaaccgatttgagtgtataataatgttgttatgtcccttgcaacttaatgtagtgcatatttgggagtgattataaaattgtataaatcattttatgtttagaatcatcttgaaacacgttttttagtatttaaaaactaatttaatatttagttttgcacttttaaatgaaatttttgtttcactaatattagttttgattcattaaatgcatgctccatcgtaatattaaaagtaactagtgattttaaccattttataatcacatgtctgtgatatagtgaagtgtacggctgccttgttgagaattgttaccctttagaagaaacacaggatgtatttgatgtttaacttgcattttcttctggcaggcttagaaa

SEQ ID NO: 15 - DNA, 1990 bp, Cucumis melo
  source 1..1990: mol_type = other DNA
tatttgtacaatgaaaatatttatttcttttctcgattctttaacaaaagttcaaaatcttttatcataaatacaaatatttagtaatttaagtttagactaggtgtatcagatgtgcaccaagtgtatattacgtgcatcaagtatatatcaaatgtgtaccaaacgtatatcacgtgtatcaagtgtgtatcaagtgtctatttgaagtcaagtgcattaagaatatatcacatgtgtaccaaatatatcaaaataaatactgattgagcatcaagtatgtctattagtagtgtatcaagtgtattaattaagtttgtagcaaaggtgtatcatgatgtataacgtgtattatgtgggttggtttttttttttttttgtcatttttgcaaaagtaattaagtttgtgttatgaacctaattttttaaatttctttttgtcacgtataagagacttgaaaataggtttaaaaggtcttaagggtattttagtttgacttttttaaaaagtatttatatgatatttaaaaattagaattttttagaaagaataggagttttataaattattcttttaagaaaaattgcatcagatgacaaaaaaaatttagaaataagcagcccataataactctttaaatttgctatcagacgactatccgagggttatcatcttttaaatttgctacttttacaatttagaaaatgtagtgacatggaccctattatcataagatttttttttgctatttttgcaaacacatgttcttttaaaatgacataattatttaaaataaaaatataaagttatttgatggatcttttgaacctatttttaaaagctaaagtactaaaaagatacatattgaaaacttgaggtcaaatgggctattattataaatatgtggactaaaaatgtacatttctaaaacttagagactaaatgcacatatttaaaaaagcatgtgaactaaaaaagtcgtttttcctaatatttttttacaacaatgactaaattgaacctcaaatttgaagggtggaaaaccatactaattattcactaatgaactaaactcatttgatgatttcaagacatatgaggttcattgagtagttgggtttgaggggatgaaatgagtggtggaagaaagtttatgtaacgacccaacgaaataggaaggtcatcccaaggaagtcgcacatccaatgagtaattaccacaaaacaacctctccttttttctcaaattcccttttaataaataatttgattccccattccttcctttctcccttggcagccttctccttttttcaaaggtttttgttttttcttttcttttttaaatttcattcctttgtttctctctttctttcttcattaacattcttcttatttcctcattactgatcatctccttttcttggtattattcttctttcttttctcaaagttttgtttttcattgatgtagatgtttttgtatcaatcaatggaaatttgagtttttcttatctcattgtatcatcattgagtgtgtgtttatgttagggatccattattaggatggatgagaatcataatttcattgctaatctatgaaccatgaataaagaaatctaaatccaacatagaagatagaacatttgcattgtgttatgagtaaccagctctgtcacttcaattggttcttctacacatttgatggcaatggctttgtttgatattcgtgatggcatctaagcattggttcttcctatgtttttcgttggctcttggtttgatttgcaattagtgaagagcatgtttggaatgaatgagttgaaatcacctttaacatttttaaaatcactttaaatattaaattaattttgagtgataaaagtaattttaacaatgataaaattactttcaaatgtgggccgaatcaaattgtctagaatgtttagggttctccaactaatagcaatttatccaaacagggtaaaaa

SEQ ID NO: 16 - DNA, 2005 bp, Cucumis melo
  source 1..2005: mol_type = other DNA
ttgttagaggagttagcttttcagggagtcggttacaacttacaagacagacaaccatactgtacaatcaatcactactgcctcaaagtcgaaaccatttaataccagttgagcctcattgtgactgcataattttgacccctaccacgaggtaatttcagttcaaatcaattgtatctctcttctggatatcagtcaagaatctcatgttctcaagttatagtacattgataattactgtgcatttttattaatttatgagttaaaatcctgctgattaattcaactaaaggaataaaatagttattggcatttggatgagaatagaatgtgaatcccatcattcatcgctagattggaccgtaattataagtgagagggagaaacttctgttgctattccctttttatttcttaattcatttataaattgtttttaggccttttatatatatatatttctaccatttttacatttaaaattcttttaactttattatgtatggactcaaactaacaagctttatttgataaaattgttcaaactattatattagttttatatttgtaaaccataaaacaaatccataaaattccacctgcatcactcactcatgttgttgaatggtacgaaataaacaatacatgtgaaagatgaaaataagaattgttctcttattaaatctaaaatctagattttctttttagtacatttaacacttcaatgaaaggtctaaaacattattgaatgacgtcacgaactattacaaaagattattccgatttatctcaaaaggggtctatttcactaattttggtgtcccacatctgtaaagagaattttcgtgatatgtgtagatatttaaatataattgaattcgatgaaagcaaagcaagaatcgatatccgtagttattttgatatagatcggtgataaataaaagacaatatgcataaagtttgtgggtacagagtcggctagttgcaatgaggggtatggccccaagacttttccccaaccccaacggtcaattaatcaccccaatggggcatcgaatcttccccaccattttccttttcttcgccgactcttctacccatctcttttgccgactctttctcacaggtttgattaaatcccattcatattcagatacactatttcaaaataactcgcaaattaatttgttttttaaatattggtataataataaaattaattataaattgtgacctaaaaagtactttgtggaagaggggatatagtctgtctaatatattattgattaaatatataatagaaccataaatgcaaaccactagaattgttaataaaaatcaacgctcttttaagtctttccatagaaagaaaggcaaagacgcgcaacgtctagaattttctttataacggaagctaactctgttataacggccgtccacataatatggtagatttaaaatgacgtcagcatgtcgcttctaaatttgggtccaaaggggggattcatttatagggaagggaaacggcaaatgcaagcatagtgagtaaatacgtggcggcaaagtaatggataattctgcctctgccgtgacgacattgcccttccatttcactataaatacacctcctctatccctcgatttcttcgcaattgaatttctcttctcatctctgtcgtagcaaaccaaatcgatttcttcaaaggtatttcttcctttcctttttttttttttttttttttttttaaatcatgttgttcaaactttgagagatgaaatgattaggggctttcaaagtggttttcgtttgatatgtttcttagatcgatagggtttagaatcgagcatccttgtaggtatcctgaggtttggtggttggatctgcttaatttttatgtggttgcatggaaaattgggattttttttttctaattacgtgattctggaaatattgatctgtggttcagatggaattgaatctgatctttctgttttgttctgtatag

SEQ ID NO: 17 - DNA, 2004 bp, Cucumis melo
  source 1..2004: mol_type = other DNA
tagaaaaaaattgaagatcttcttaatgctaataataaaagcatatataaaaaggcttcatattacacaagcatcttaaaaccaaaccgaacttgatttgaaattatcccactaattctgtagatttcaccaaagtccttaacctttatactaacatctgcatttgactctttcatttgacctccaacatattctttctcattttccttccattcaccacaaaaaccaacaaatacaaaaaaccacaaatacatagaaaattaataaaaaaatcaaaatttcgagatgaaatcattataaactcatccgataactttgagatttgaaaccttacactatataaagaaactcatccgataactttgaattcgcatcgaaattacgtaagtgaagacgaaaatgtaaatgattagatgcgaataacaaaaaaaacataatttctaaacgtaaaacactatattcaccttattatacttgattattttggaaaagtatgaaatttgagtgtgggagaggagccaaagaattggaaacttgttattaggagtcgttatgaaacattttcaacaagccaatattctttcacatactataatgatatacatagaaataatacaataatatttttgaaattgaggcatttttgtcgtaatttatctaaaaatgtcagggtagattcatcatgtatacaaatctctcgctatcaaaactatataaaaatcttgtgaatgatttcaatcgaaatggaccgagaaaaaacatcgtaaccacctctaaaatcgataaatttgtttcaatttcaaatccctaaaactaaaggtgctactttgtacaatttcccctgattagggtgctaaagttaaaccctaaataaaggtgtgtacgtttccggaagtttctagaatccccagcgaagttctccaaatcgtggcttgcagaccaaggacccccattaaaattcgtttcttcctctaaacctcctcccttaattttggcattttggtattttggctcctataaattcaccccctccttatccctaatcctttgtcttccaaattttccttcaaagcctgcttttcccatttcgtcgtgctttttcttcatctaaaggtatatttcagttctagttttctttctctgttgatctcttggatttgagggacgtttgaagttggctttgtttaattctttgttattcaatctctttttttgttagagttgttgtttaatcgtttcccttgttgtttttctcccttctagttcgattttagaacgctttttgtgggttgattttaatttctccgttttcttacatctttcacaaagaaacgattgaaatcgtgtttgttttttttcccacggcatacgttattagatcttgtagataatgatctcaatctattgtttagtttttgcaaataagaagttggttttttatctccaacttttatatattcgattcgatgagatgttctacaccgttaggatggaaccaagaagtgaggtaagggtgtttgattgaaaaattgaactgagaagttaaagttccttcctaactttttaatggattgtataattcgttcaattccttgtcgttccatttttatttctgtttcgtttttcgtgttgctgcgtatcgcttcccttgttgttttcctcccctattgattttgcgtttcttggagtttctctgttttctctcttcatttttctacaaaaatcaattctatttttattcgttttcaattcccgagctccttggaatgttatccttttctcctgtgtaaataagaacccgtattcaatcccagttcatagtttggctttcccaaataagagcaaaaagattgtactgagaagttgaagatttcaaaattttgtacatgatttcttctaatttatcaatttgattggactttttgtatatagatttggttcttgagctatttatgttatgacgttttcatattgaggccatgcgttgaattggtttcttaacag

SEQ ID NO: 18 - DNA, 1935 bp, Cucumis melo
  source 1..1935: mol_type = other DNA
tatacaaatgacaaaatatcgttgaagtccaaaaaagatttattgttggtaaatatcgttaaagttagtaaatagattttagagaaaggagatatagcccttgtagtagaaacacacacacaaattgaattagatgtgtttaatgtttaattaaattagatatgagtcaacttatatctaatataggacattattaaacaaataagaaataagaaacatgaaacaagaaaaacaagaaatagaaacaatatcaaacacattcctatttcttgttctaaaaaaagaaaaaacatggtacaagaaataggaaacggaaaagaggaaacaaggaacaaatgctaccaaacgggcctaagtttctaacaaaatgagctaggtgtagtttattggtatagatagtgactttcaattattttaaatttttttatccatacctccacgtctttagaatctttcttatttatatgtgatcttaattcattcatgtctcaatcttaaaattagaacattacatgttcatcattttttccttttgttactgtgtttaatctttcctaacaagacaaatagtttaaccttaatccacacattattataaccaaattaaaataatctaccttcaaagaaaacattattataatcttatattaaccacaaattataataccaaactctaacgctccaacccaacctaggaagaatgacaaggctgtcataatttagttggtttggcacgttgttggaagttctcaaaattatggaaatatttatttccttcttctttatccatcatcctccttgggagggtgaatttgtgttaaaaaagaatagaaactaaagtctaagtggcaggacttacattatgtgtgtatgtggaagtaaaattgcagtaacagtttacaaaaacaactcatccatgattcataaccaacttaaatgaatataattttttgcctaaagattttaaattaatatataagcggaagaattaacctataacttcaagtttaacaacacaaatattatatcatactgattaattattggaatgatgtttaggctttaaacataaagtattgagaggctaatttgagtttaactcactaaactatcattaccctttcaaaatagatccaatcatccatttattataatactcaatgaaataaagcaaaagatgagtaaaataattcaccatgaacattgataattaattttcccactaagataaactactactcctcaaatcttcatatgtgtttttcctttttgagttgcactcaaattttcatagttgaaatttacccatcaaaacaaccaacaatctttcaaattcaacaaacatttgaccttacaccctttgatgccaaatccttaccctctccctcttccataaaaattcttatataaaccaccatcactctcacttctcaattcactctcttctctactcccaatcacctgacttgcctcttactccaccgccaggttccgccccaacttccccggtaagttccagttcttcagatctggttaccacatttgatttcttgcttgtatttgacgtgggaattttcatatcggcgttttttcgaactgggttttgctttatgatcatattcttgtagtaaaatgccatgaatctgttatttgattccgttttttttggagatcggtctagctttatggccatattctggcatttaaatgccatgaatccgtgatttggttgaatttcacttccgatccaatgtttatgctgatattgacatctttgcattcaatgcagaggagttttgtttcgatttattactgatctcatcacactgatcttgaattttttatacttttatgtgtgtgtgtgtattttctttaatatctatgccaattgaactatgtggttaacttcagagtgttcttgtgggcagtgagaag

SEQ ID NO: 19 - DNA, 1606 bp, Cucumis melo
  source 1..1606: mol_type = other DNA
atatattgtatcgattctttagttgctctatgtttttgtttgcttcatttgtcgattaaactgtaaaattaatttctttgacaaggaaaaagatataatttaattctataatttattacaatctaatccatatggtttaataaaacactgaaaattgtttatgaaaattttatcgaactacaagaactattaataaagtttttttaaaccgtaaattgaatgaattttctccacggtgtaaatttgaaaacattaattaattaattaattaattttaatttcaaggttttttctgacccatgaacctattttatgatataagttgttcaggggttgcaatagtaaccaaataaagttgatcagaaaaggttaacaactcatgaaaacttccaaatgcatttgtgtttcaattattttcttaaccctctttttttggtaattttagtttaaaaagtgagtcggttgatcattattgttctttaatttcttgggagaaaaatattaatgttgattatggtgatgagttaagtccaattcttcatcaaatcataccaaattaggaacaaaaaaaacatcaattttaaggtgcaaatccatttctaatggctaaaatgtcaagcatcccaccaaaccaacaatctctaaacccatttttactccactaatctaatgtttaataataatcaacaaggttttgctcattccttttttagttaataatcatttaacaccaaagctcaaaagtacccacccaatggatcaaaatcgagaatatatagcatttaaggatataaagactagagataataataacctagcttagagcttaaagggatacactagccatcaagtcaatttggtagacaatctaaaaacaaataattcgatgaaaataaagttgtatttttgtgttttcaaacatgttttaagacgaaggtttttgataaatttgatctcaataggtaaacaatggtaattactcgattataattactcactaaataccaaatcgaatataaattattactaattaattatgaacatgttttacattttaaaaaatgaataattttttttttagaatttgtgttattgaaaataattttcaaaacaatattgaatgaatcttaagtgaaatcaatgtattaaaagaacataaaacataatctagatggtctatcgaacaagctagaaaatatcttccataaatccaatgattaagacaggcaggcaggcatgaagataagaggattggattaattggtgattttaagttatgaataaagacacaagaactagcagctctcctcttcttgtcaccttcctttgtcatccagctcacacaactccaacttggaatttgacaggtctctcttcactcatacattcccacatgaaattattaattgaatcttcaacattgtctttgattcttcagctgcactgtccttttccaccatttttttcttcaagataaagactaataaactccttatatattcctctcttcccattcacctgtgcatactcacaaagcaactgccatttccttcttgtttatctctgtttttttcttacacatttgttgaactttccctctgaaaaa

SEQ ID NO: 20 - DNA, 1487 bp, Cucumis melo
  source 1..1487: mol_type = other DNA
taatgaatttgtatttgttagtggattgagtttatatgatattaattttgacccaaacagttgagtacgtaattaatgtggcttgcattgaaagtgatatgggcatatagtatgtgtagaatgtagctgacacaacacattaacaaaacccaattttaactttttctttttctttttcttttaattttatatggatcagatcacatgtcattttccattacaactcactctctaccaatcatcccatcccataggccataccccataacatccctttctaaatatctaaatcatctccctaaattattacattttttttctctcaaatataactattcaattcataaatattattctttttttagctcttattatttcaattatgattttaaatattccttttcaatttacgaccttttatttaccatatcaacattttaattctactcaattaaagatcattataatgaaatttcaggtataacaaaataaataggtgtgatataatgatggactactaatttcactaatttcgtcatctgaaataaggacaagttccaactatcactattgtgaaaacctcataactcctaaaagtgttaaaattggaccctcaagtttataataattttgcaaattgaatcccaaaattaaataatcagtataatttatacgttttgagagtcaaatttaatatttgaataagcttgaatacttaacttctaattttgaaaatttaaaaatgcaactgcgagagtaacttttgcaattagccgtcgaaacaattaattatattggttaatttatgtctcattctcttttgatgaccataaagataaacccatttataatataaatatcaagcaaagctaaaacaaaatcttttttttttcaaattagatctaaatatgaataaaagcagaactttctagaagtacaaatttgattatttttcttgagataaaattttcgctatgaacctttttataataggaaaaagagaaaaaggatggttttatataaatgtatgataaaaaggtaataatatccattgtaatagtaaaaaagaaaaaaagaaaaaaagaaaaagcaattttctttttcatgattaggaaatataaaaacaaaaattggctcccaattgacatctttaatcttctttttctttttcttagaaaataaaattagtgagagaaggaaaaaaacgaagggttgagagatagagagagaaaaaattgatttttaatttagtttattttccttttttggagcacaaaataaatagataaataaaatattagtttgcaaaaaagcccctcgagtttatcttatttgctcaaaaaagcaaggataaatacctcccgacatccctgtttatccctctcagtttcataattccattggttcgataagaaaacaattctcccaatattcccgctgtagatctcgtcgattttccgtttgtttcccgggaagatcaatcaaag

SEQ ID NO: 21 - DNA, 1448 bp, Cucumis melo
  source 1..1448: mol_type = other DNA
ggtgtcttgttgtaaggaaatggaaagaaaagagaaaggctcttgttgttgtccttgttctgtgtatcgatgaaaatggatcgacgcgaagaagatgaaggacgagagtggggattataagacagagaaactccgaaatttgagggctaatatggtaataacaaatggcgggatactttcaatggacgtggacccattgcttctttaactcaccgtctgatctttattttacggtcatgatttccctctttccccaatatttttgggagggaaaaccaactttgtttttgtaattttaatcatttttcctcaaatcgtaaaaaaaaaattatagattttttcaaaaatagaaaaaattcatataagaaaaccaagataaaatattttgaaaaatatcctattttttacttcttaaaaataattcataaaagaattattataaatattaaaaaatatcagtaccactatagacaactatttatatagcacatatagatatatttgttggtttttctatttagtatttgaaaacaactccaaaaacaatacatttcaatatacctacgaagcatacaaatataattattaattttaataagttcaaaaatatctaatggcatccttatttaatcaattttttcatcgacgttatacacggtaaggatgtcctaatccttgaccattgaaagacgtttgttttgataattatatcttttgatatatacaaacatttatctcatgattagaatagtcacctttttatttgatttaacgattatacataatatttgaaaatttttaaatccatcaacacaatcaaaccaaaaatttcctaactacataatctacaagagatttaccatcttctttaaacaattggtcattacgtttgttaatgtttaaaattaaatgcaaccatattgggtgtaaaagccaaacattgatttgattattaaagttttttctatatagacttgatgtgtaaacctaataaccaacttgagctaaataactttaatttctaaaattcattaaactgtcctcatccaaattataatatcaaagatttttgaaatatttaaaaattccgaacatgggaactactggaacttggcaataaattcaagcaagaaagaggaaaacgatataatcaaacaattaaaaaacaacagaaatttatttaatcaaaggaataatctcatcttttatttattgggttttacttttaatactgtgagtgatgattggaacattaattaacatttaagacattaatttgcaacaatcaatcaaaattgtataaatccacttgttttgatttatttgaaccatcacttttttttttatatatatatataatatgggagtgaaagatcaaacgtataatcatgaaatgaaagatgggatatcattgaacttaattaaatatcattgaactgcaatttttt

SEQ ID NO: 22 - DNA, 1235 bp, Cucumis melo
  source 1..1235: mol_type = other DNA
aaattttaataattaaaatgaacaatttttcaagagtaatagagtttgagagatgtcagagaagtttgaggaagaagataacaagtgggagaagagaataagtttgttgtgtgaaagagaaggggaaatttcattcaagggtatattgaactttttactcaaattttgtaagtctattttttccgatcaatcctaaaatcacacacacccttaaaaaatggattatatttggcaattttccatgataaactcatttttaatttagagttattttttcaacgagatattaacagttttagttcatatactaattgtaagaatagtttcttttaagttgaatagaatttttgaaacttttaatagttcaaaaggtatttttgaaacaaaataagaatgtttttgaactttttataaaaagaattgagatttttttgaaatttttgataaagagaaaagaaaagaagaaagaaaaaagaaaaacaagtttgtagaactccgtgggaaaatcgtcgagggccctgtgaaggaattttgaaattataatgagggtattttcgtcaacaagggaatttagacatcgtatataagcatcctcaaaccctataattaagcccttcaatccaattgccattctccatctctcgccgcaagggtttaagagcagcttctctcctcaggttggggtttccccctatcttcttcattcttcctcttctcgatttctttcttctatttgctcgatagtctcttatttcttgagcttttgctgtttttctcctgtacatcctaacatgaattataacttggttttgattttgtcttttacttctgtattaaacaacttttcttacccttttattcttctcttcttcttcgtgtccctgcccttttgtttttatgctaattttatgtttctgtttatcaatctatcgaggcgtgacctgtcgttcttccaatagcgtagatctgcacttaatctattctagctgattggattggtcgtttttcgtttttttaatttattttctctgttctagttccgataaatttttttatatataattaacaagttctccagccaaaagggttaatattgcgttggatattttaatttttacgttatttagatgtgtgaatctaataaaattagggttattcataaatttcagtaatgatattttggttatctgttcttgctgttcctgtttcgcagttcttttacctaatattcaagc

SEQ ID NO: 23 - DNA, 2003 bp, Cucumis melo
  source 1..2003: mol_type = other DNA
ctagacatttttgtctaacctttcaaatgttttgttttaatcttccctctcccaaatagtgaaggacatccagtgtcaaccgtgaacgcatactgtgtcattcatgaaacaaatcttttttgtagtgggcattgtcagcatacatagcatgtagaagctatagacagatgttgctttgagttgtatttagttctctttaaaggaactttgtacaaagtactgaatgtactctgttatttgaaatatcaatgaagtcctcttaattcttttgagttcccattccacgtttaagttgttagttgtattcattttcgcttactaggtgttctgcatgtatctcacagagagactcacgtgaaatgtttaggcggtcacatccctaatgacttttgaaggggtgtgacacgatcatttgaatatatcacttatctaatagtgacagtggtctatatctttgtctatctgtatagatcattggttgtttagatattggtacactattgtgtagtgaaaaaagaagaagaagaagaaaaatataatacttgataatgagaaaagaataagaaaaaatattgtctttatgaaagatgaaaaaatgatgctgaagacgagaaatgacggaaaaggaataaattctagatgaagagatgaagaaattctagaagaacaaatctagaatttataaatgggataacaataaagataaatgggataacaaagaaaaaaaatcaagaaattacctaaatgtttcaatcttgctacgccttaattagaaaaagaaaagaaacaaaaaagaaaatgcacaaaaatatctatatatatatacacacacaagcacaagaaaaaaatgaatattggaaaaagacgaaaatgcattattttttatttgcgttagcgagttgttgtgattttgtgagcaagaaaaggatatgcaggagaattaagataaataaggaagattgaatagagattaaaagagaaatatgggaatagagtggggatgaaaggtttaaagatagggagggagggagcgagagagaggagaaacaaacataccttgagaaagggagaatgagagagataataaataaatacggtgatttggaactcataaaaagattaaaaaaaaaaaccttagagtaaagacttttccatgcatttcgagaaaatggaaaagaatattctattctatttgcttggacaccaagttcctttttgtcgcatgcatacgtctatttatttctgcttgcttgcataggcagtttttgtccaaggaaattcagcaaaggcggtatcaatttcgtcaacttagaatccactcagtactatttgaagttcctcactaccaatttgcaccatccaatctcttctctctccaacttcctgccagggcttaacctctcttaattccttatccttacttgttaccttacctggttccactcttcacgtctctctattctatattgtttttttttcattcataattttgttactctcttctctgtcccctttgtcttggattttatctctccatatattcattggaataatttaagttctttgtagattttatgaaattaccaatttaatttttcaaacagtttttggatttgtttaatttctccttctctaaatcgcgttgactttatgttatttcgcccttgctctgttttctctgatcataaagtatgtacttgattttatggtgaatgctttcttgatttaacaaccctggtgctgaaatcttttttaaatcctacttttgttgttttacatatgttcttactctaaaatgagcgacttatttccttttattcttccttcttgattaaggatttaatcgttgaagtatgcttatattgtggaaatttggttttaattgatcatacgagctagtattactagcttctcggtttctttggatgagttatatgcatatgatgatttcaattccaatttttattttgcaacagattgttttttgtggctgaaattcaagt

SEQ ID NO: 24 - DNA, 2015 bp, Cucumis melo
  source 1..2015: mol_type = other DNA
gatcagagtagcagttgagcaaacccaaaccaaaccctttatctatacaatcctctcaaaataaaattattgtttaattattcccatatctattatcatttttccataattgcattgagagaaaaaaaaaaaattctaggagacctaaatacaacaacaactatttaataatagccccatgtcacattaaataaaactaacaaaaagtttaatacgtcaagaaacgatacttgtggatattgaggcatgggtccctccttctttgtatattcaaatctgtggtctgccatcagataaggcctttaccatataataagttttcaaaaaagtaagcaccacttgctgcttttttaatttaattatatttaatctaattattgaaacttatagttgttttctatccttattcttttcttctcttcaaacaccctcctattaatttaaaataaccaaacaacctttttctttacatagacaaacttaattagattaaatataacttgtaattagattaataatatagtttaaaaagaattttattttaagtagaattattagtaaaaatgaattttgtggatagatacttggaatttaagagaaagttaaaagagagaaaaatatgaaaaggaattaaatgattaaagttgaatgtaagaaatcaataaacataaattccatgtattaaatttttgtcggtgtgtgaataaataaatatctattactattagattacccagctttgtttataaaaagaaaaagaaaaagtttttaaaatattggaaaattttgtataattattgaagaaattgcgtggtctttgcaatttgggcatcgttcttatcgcttccaatgaaggggccgtttacctccaccactatttccaacttgtttttgtaccattctctatatttctttgacacctatattacacgtgtctttaatccattggaccttcgtcctactatatttttacccgaaatgacgaatctgtccttctcatccacctataaattcacctctccggctccttccctttcattcagttttcctctattcttctctctatacgtcatattcatttcttccaaggttcgtcctccttttatctttcttctttctttcactttttttcgcttttttcttttctttcggtttttgttcttttaatttcattcgtttctttttgttatatggtatgtggtatttgttgaattgagatgttttagggtttcgatttaggttttatttcttatcctacttaagggctattgtgattttggagaaaggagttcttatttgtttttttttttttcctttttcttatctggcagatgcaaatcttcgttaaaaccctaaccggtaagacaatcacccttgaggttgagtcgtctgatacgatcgacaacgtcaaggccaagatccaggacaaggaagggattcccccggatcagcaacgtctcatcttcgccggtaaacaactcgaggatggccgtaccttggccgactacaacatccagaaggagtccaccctccaccttgtcctccgtcttcgtggtggcatgcagattttcgtgaagaccctgaccggaaagaccatcacccttgaggttgagtcgtctgacaccattgacaacgtgaaggccaagatccaggacaaagaaggcattcccccagaccaacagcgtcttatcttcgctggaaagcaactcgaggatggccgcactttggccgactacaacatccagaaggagtctaccctccacttggtcctccgtcttcgtggtggtatgcaaattttcgttaagaccctgacgggtaaaaccatcaccctcgaggtcgaatcctctgataccatcgataacgtcaaggcaaagatccaggacaaggagggaattcccccagaccaacaaagactcatctttgctggtaagcaattagaggacggccgtacccttgccgattacaacatccagaaggagtccaccctccaccttgtgttgcgtcttcgtggtggt

SEQ ID NO: 25 - DNA, 2006 bp, Cucumis melo
  source 1..2006: mol_type = other DNA
accaccacgaagacgcaacacaaggtggagggtggactccttctggatgttgtaatcggcaagggtacggccgtcctctaattgcttaccagcaaagatgagtctttgttggtctgggggaattccctccttgtcctggatctttgccttgacgttatcgatggtatcagaggattcgacctcgagggtgatggttttacccgtcagggtcttaacgaaaatttgcataccaccacgaagacggaggaccaagtggagggtagactccttctggatgttgtagtcggccaaagtgcggccatcctcgagttgctttccagcgaagataagacgctgttggtctgggggaatgccttctttgtcctggatcttggccttcacgttgtcaatggtgtcagacgactcaacctcaagggtgatggtctttccggtcagggtcttcacgaaaatctgcatgccaccacgaagacgcaacacaaggtggagggtggactccttctggatgttgtaatcggcaagggtacggccgtcctctaattgcttaccagcaaagatgagtctttgttggtctgggggaattccctccttgtcctggatctttgccttgacgttatcgatggtatcagaggattcgacctcgagggtgatggttttacccgtcagggtcttaacgaaatttgcataccaccacgaagacggaggaccaagtggagggtagactccttctggatgttgtagtcggccaaagtgcggccatcctcgagttgcttttccagcgaagataagacgctgtttggtctgggggaatgcctttctttgtcctgggatcttggccttaaaagaacaaaaaccgaaagaaaagaaaaaagcgaaaaaaagtgaaagaaagaagaaagataaaaggaggacgaaccttggaagaaatgaatatgacgtatagagagaagaatagaggaaaactgaatgaaagggaaggagccggagaggtgaatttataggtggatgagaaggacagattcgtcatttcgggtaaaaatatagtaggacgaaggtccaatggattaaagacacgtgtaatataggtgtcaaagaaatatagagaatggtacaaaaacaagttggaaatagtggtggaggtaaacggccccttcaattggaaagcgataagaacgatgcccaaaattgcaaaagacccacgcaatttcttcaataattatacaaaattttcccaatattaaaaacttttctttttctttttataaacaaagctgggtaatctaatagtaatagatatttatttattcacacaccgacaaaaatttaatacatggaatttatgtttattgatttcttacattcaactttaatcatttaattccttttcatatttttctctcttttaactttctcttaaattccaagtatctatccacaaaattcatttttactaataattctacttaaaataaaattctttttaaactatattattaatctaattacaagttatatttaatctaattaagtttgtctatgtaaagaaaaaggttgtttggttattttaaattaataggagggtgtttgaagagaagaaaagaataaggatagaaaacaactataagtttcaataattagattaaatataattaaattaaaaaagcagcaagtggtgcttacttttttgaaaacttattatatggtaaaggccttatctgatggcagaccacagatttgaatatacaaagaaggagggacccatgcctcaatatccacaagtatcggtttcttgacgtattaaactttttgttagttttatttaatgtgacatggggctattattaaatagttgttgttgtatttaggtctcctagaattttttttttttctctcaatgcaattatggaaaaatgataatagatatgggaataattaaacaataattttattttgagaggattgtatagataaagggtttggtttgggtttgctcaactgctactctgatc

SEQ ID NO: 26 - DNA, 2017 bp, Cucumis melo
  source 1..2017: mol_type = other DNA
atggataaggcagagcttaccactaaccttctaagatattttcgtcgctcggcatttattcttggagggaaccacaccaactccaaaatacccatgaaacataggaaaaaatggttcatagtctaagtttccatttcgattcggtttggttcggtcttttattttaaaaacaataaatataaacctactaatttgatgatgacaagtttactaatgttaagtaagaattcatcaatacctaagaatttgcaagtttttcttaagtttgatggtaaggatttcgtaatccttgaaatacaacaattgtatagaaatgaagcgttgcatttttaacgtctatataggaacactattttactccaatcaagttgtaatttgatagataatagtttgtataacttaatgatgaagagcttttttttttatatataatttttattaatacgtatagttcaaaattggaattagctatcactaacacgtgcttgcgatagaaacaacaataaattcaattagtgtcgcatgtatttcatatggtattgatgacataagagtagtttgatacgatgggttacatggagtgacatgataattgtattaaatttcaatagttatgatctcaagtttgggttgtgtctcactttgagctttttgagaaattggcctcaagactcgcctaatttaatgttgcttcaagctatagatgcttacatcgtgtgtatgaaacatattgcactttgatgcttaaagttaatatagtgagtaactaaccagatattacacgctactcttttaaaatggtcaaataagaacatttattagtatgtgatataacacgtaccctccaattacatacaataattgatcaacccaaatcttgaggtatttaataataacaaatacaaaatagatggattatatatctgaatagctaaagaataaagaatatgtgttatgttgtagttacatagtacaataagtcctctcaaaattagaatggtataataaaaaataagaggtacattcttaaagaaaatgttatcaaaactgttgcatcataggcattttggcaggaagaatagtggaagaaaattcttaaacctaaattctatcgatattaaatagattttataagggataattgcaaatgtagcaattatatttaaaataattaagtatatagcaacattttaaaaaaatggcaaatatagcaaaatttgtcaaaatctatcgatgaccgatagatcatgtaagtctatcactgataaaccataggagtttatcaacgatagaagtctatcaccgataaattttgttatatttataatttttttaaaatattgctacatagttaataattattctaaaaattgctattaccaccggtttttaaataggacctaaatttaaggtatttgacataaattttgatgaaccaaactagcccaaatcaaagaagtttgggcccaaagcccaacgaatccacaacaaacaaagcccacacaacacttcatgaaaatgattttttcaaattttagaaaaaggttataaaatataaaaaaaataatcaaactatccctggtagctaagtagttattattatttttatggatacgaattgagtagtatttattttaaaataggataattgatcttagtttcacttgtgatgaactatttcactttattatttgtttgtaattcaataaaattagggtttgattgtcaatgataattattacaacctcaatattatactcagtaaagaaaaataaaaatttaaaattgagaaattaataccaattttttttgtgaaataaaaggaaaagtaagtaaatattataaaattttggacttggaaattaaaatgcattaataataatatttagtattattgaattaaaatggacaccggaaaccctaaaagagggagtggccacctataaaagggaagcactcatctcacccaaacccttgttattcccaattggccgtgcggcaaagaagcctctcaacc

SEQ ID NO: 27 - DNA, 1353 bp, Cucumis melo
  source 1..1353: mol_type = other DNA
tgagggtcaaaggaggaggaagaacaagaagtaaatgaagtggagtcatgggaaaaggaaaacaaatgtgagaaaagaaagaaagccagagagggaacataaaattattagtcagaattacaacagaaaatttctgaagaattgagtttgtatgcagcaataatatattgaacaaataaggagagaaggaggaggggaaattcaataaacagcagaggaagaagaatggcgaaaacccaatatctaaaactagttaattcaacaagaagcaacacaatcatttcattaaaaaaagaaaaggtaaagagaaattcccagattcgttactctagattggtccaatggagtggaaagggatgcaatgaaatcagtaatagaaaagaaaagagttaaagtagtattggtaggtaccgattaaaaatggaaggcgtcggaaggaaacggagagttcaataaaaggaagattctttgcttcctccggccatttgatgagaaacaaaaactccgcacctccaagttccttccgggggaaggagaagactcttctattctggggtacacaccctcccttcctgctacagaatcaaatctaaattattttggattggaatggcatgggattggtctaacttccaatttctcgacacacaaccccaatctacccgccacctgtacccagttttcccaaaacgcaactcacattgcaattgcaattcttgtctttaataaatacaaattgatttttctttttctttttttttttttttaataacgattaaccctaaaaaaaataaagaaaagaaagccgatcctaaaagtagaattactttttttttgtttttcaaggttcacgtctgtgtttgcatagacgtgttgtagtcggtgggtgtgtaaattagagtttgtttttctcatctcttgttctttttaacgaaatttcaaagatacaaaagcataatgaagaaaagtatacaaagcaacgtaaacttagcattttgcacatgatacaaatttagtcaaactcaaaccctggacaacctagcactctcttgggcacgtggtagatttatgtgaatttccctatttttcttttgaactcacaaatgggcaaataataataataaaatttattgttgatttttcttatatttcaatttattacctctagttttaacctaaagtttagatgtatataattataaatgagcggtgaaacgggcactgattgatgaatatattgggccttgggttggcccaacaaacctaatgcccaaatataaaactttggcaaccatagttaaccctaatctgtcaatctactctcctcgactcggtaaacctgcgactcccaca

SEQ ID NO: 28 - DNA, 2005 bp, Cucumis melo
  source 1..2005: mol_type = other DNA
cagtgtgctggaattcgcccttatccaaggagattaatgtcgagagattattatcgaggtttgaatttattttgtccaatcatatgattccaagagctgaccatcaattcaacagaacatgaaccggaacctcatacctattgtaatggttcacagcatcctaatacagaacatgaaccgaaacctcttacccattgtaatggttcacagcatctttatacgtattataggtagtaccattgaagatgcatttaaatgctgtccatgctctgttctctaaaaagttggacttggacttggacgtcagctgaaagtatgaaatgcactgtagccaacgaagctatgttttcaggcttcaacatggttttaggaaagtggaggctctttggttgaagggttgaatgaatgcttttctaattccagcatgatcttcaaatttcgacacaaaaagcttaagtattttgttccgttattcttttaatccttgtattgttatatattcttttctctgaactgaatgtacgatgattgcaggggtcgagagcaagtccgatataatgaaacacgtaaggacgtgattgaatgaaaaactatgagcagagatacaaagtctaacttacgggatgaacgatgagaggtttgaccaagagctgtgacgcctgtatatttcaacaaaagttgatgactaacatcacatgtcagagtaatcaaagaaatgcagccgcacatatatatatctatatatatatcgtttagtttttttttttttttttttatttttttttttatctaattatattttaattctattttcctctgccctcctccccctcctcttcccccacccttcttctgcacatagtagccaaggattgatcggtttcttttgattcggggggaaaatgttgtacaatttttgcttccatagaagcttgaaagttttgcagattatgttgtaaaattacccttgtgtactcacactagttcttctcgtggaaacttatattacaatggttgagttttaaggggcatattcacactggtaactaccattttctaatttatgaatgccgagtttctctccatgaaagacctttcaaatgccctttcctccgcggtgcgtttgttgttgtaaatgtgcagtgtcgttggatacacgattgtgtgaaagggaaaagggaatacgattaactcttaaattcaacccctatctccatcagtatcaatcacatttcagcaactagctcttgaataacattgagattcttgtttaatccacgtactactactactattactactatttgacagccgatatctcaaataacatccatatttatcaaattggtattttaaggacttttaatttcttcgtacatatttcattataatttaactactctgaccatcattgaaaatttcacaaagaagacattttaaattgaattgagttgaattaagttgatataatggttgaacgttggatttaatttataatttagtggtgtatgggtccattgtaataattcttaaaaaaaatatcatattctgaattctaaagaaccatctaagaccaaaactaaggggtcaccaatgagtatggtaaagtcaacaaagtttgtctacttttcttatccttatcatcaagagtgcaatatgatatcaaagataaattgtacgtgggcgtcatccattgggtaagaccaagaagcaaaatatcatagagaagttgttttagtagccataggaaggaaggaagcaaaataataatatagatttgaaattgtggatgataaactgccaaatgggaattcaaaataaactaaataaataaaataaaaagagaaatcttgggagtttccattttagccaatgaggaaacagatagagatctcatcaagataaggaccctattctcttcttcatctataaaacaaaaacaaatcaaaccctcatttcactcattcaaaacaaaaagtactccaaagtcaaactaacaaatacg

SEQ ID NO: 29 - DNA, 1445 bp, Cucumis melo
  source 1..1445: mol_type = other DNA
tcccttcagccacttaacacttaaaaatcttaggaaactccattggctcctctttctccaatgaaattttgacatctgtgttgttgatagctcctatatcctttgagaatttgatatacacctgtcatttgctgatttgtggataactgttagccttttgatattgatacgttccttttttatgaatttttgtaaatccattcaattttaatgctgtcgtaaatgaaaagccctttcattaatgttgtttatatacatattttaaaattaattcaataacaagtttagttctgttagcttctaggtttgtatctattttatctattaaaggtatgtttgggcttcaggttggaatggagtagaattgaatgggttggggagtaaattttccattcaacaagttcaatttcaaaatggctaataagttttgaactcaattttattttcaataaattccttaattttttgttccttgtttgtaaactattgacttattcgatatattttaaaattgaggtattttaaaaaaataatacaatattaaaattatttataaaatataacaaaatttatgtatagtttatttgaaaattttactatagtttcatttttatattattcctaaccatttccatttaaaattatttcaattatttcttttattaatataattgaaatttcatggatttattagacacatgatttgaaattttatgggtttattaagtattttctaacacaaaatcgcttccgcatcgttttcaattcattcagtaatagaagtaattttttaaaagaaccaaatttgccaaattttgagttccataaggactctgaaaactcattatgtctattactcttcactaattgtagagacttaaattcaagataagagacactaattgatgataattgcccaaaaaataaaaataaaaatgtttcttccccatcctcaacctccatgaattcacagagcccaaagattaattattgggccccaattcctactcatatataccttacagtccctcaaagaaatcttaggaagtaatcaatttctgtttattcaagatgtagcctcccaaaagaaaaatacatcacatcaaattcaaacaaaaatatctacagctagcaaaacctcaaaccgttaaaatttcaagccacataaatgaaattttcatctgaaaaaaggacaatctatctagacgttagatttcagccctaatatgaatctgaagcatttggtggacgagaaagagccatgtaggaatgcatcaaacaaaggaaaaatctttgaactccaatgggattgaagatacagataccaatggataagaatctgttctctttgcccactatttaaactcaccaaacccaccagtatcttcctcaccacaaaatacattccaccgttgatcacaagccttattccaccacctccaaca

SEQ ID NO: 30 - DNA, 1282 bp, Cucumis melo
  source 1..1282: mol_type = other DNA
tgcaattaagaataagctaatcttaatgaagaaaagaaaatgttctttgtatttgataaatggtggcgttttgggggactttatatgctttttttttcccatgagattggttatcttcatttccgtcatgatgtcgccaagtggcgcttcattgatgatatcttaaaatctataatgatcatcctctttgccaatggtgtggtgacacgtggaaggactctccatcttctaaaagattcttcaaataaaaataaataaataaagaaaaaacttgtaagaagatacatatgtacatttttatatgaaattaatatgagaaataatcgactttacagtgacttgatcaaactttcttatttgtttcatatgttaggttaaattactaatcaattcacgtactttactagatgagatttcacgtactttactcattgagtccaacggttgattaacttatttcaagaaaattgattcattcaaggatgtttccaactctcatataatttccatgttgttccacttctatcaagtacaatcctatcgaacacaagtttgtttaactgaagttcaataatcgagatcaagataggccttattatttcttctagaggttcaagtgatcaatcaaaaaaggtttatcacatgattcattccaattcaactaagctaataagtggtgttgcatgatagagtatcggactagctcgaacccctatcaatatgataaatgtctatgtatataaataggtacttaacccaacgaacaatgtgtcttacgtgagaaagcttttttctaatatacataaaaagcttgcatgactttttgatgaattgtgttttgataaaacatatttgtgagtatattatctttataaatttaagttataacaacaatgtataggtgtgagtatgcttttaaacttaataaaaaaattagaaaaaattacctttttagtatgaaagttttaatgatatatcaatttgtgtctttatgatcaaaatgtatacttttagtctcaaatgtttataagaattaactccttaataattatcctaaacaatcatgttcaaacttggattcttattgacacatatttcattttaatctaagtttagaaatgaagataattaggataaggatctttagcttatgatatcttatccaatatcttaaataaatcttcaacaccaagaaatttccctattgcggatatttcaatatcgaatgccttggagtatcaaaggcattggataacaagtgggacataattgcgataaaaaa

SEQ ID NO: 31 - DNA, 2002 bp, Cucumis melo
  source 1..2002: mol_type = other DNA
ccgtagattgaacttatggcttcggtcagttattgagattttaattctctttaacattaggctaatccatgagtttacgtgtgctaacatgttaatatgaaaagtatagtagaaaagtaaaataatataaataaataaattggattgttttgaaaagttgaaagattagaatatacataagattctgaaatatctcaaatttttgacccagcaaactgaaattagccaaagtaggttgtgttgtaaataattatactttatattgttctttttgtataagcttttatgtgtcaatgacaattttaacagctaaataatttaaacagaatattgccaagatgggtggctacaaaaataattgtaaatagaacccaataataattagtttaatcaattatgtttttattaacttgtaaattaaatttacactgaaaagttgaaagagtttggaaaatattttatttgaataaatcaaacaattgaatactaatttgcgtaaaatacgtagtttaaaatatatatatatgtatatatatatatatagtgtaattttcaagtaataaataaaatgaaaattaaaggtttaaaaataagctaatgggtgcttaaagtatctacggaaacgagattgcattcgactcacgtacgacatgaaaaagatataaatgaattttacattaaaactattaaattgcacatatgattgtccaacaagtaagaagaatcacaatcaaagtaaaaagaatcacaatcaaaagagaatgtatctaatggatgatgacaatttacttaagatttaagaattaatctaaaaatttagagagaggggtaaagatatcaacttttatttaccagaactaaaaattatccttaggcctcaattgctttagtaatggatatatatatatatatatacacatctacctaacaaagctttaataatagtaataataaaaatttaaataataaataaaagaaatcgaccaatataaaaacatataaaaaatgtatagttaaaaagaaagagagaaagagagaaagagagaagagtacatgcaagagatttgatttggaaggagcacataataggacaagagaagggtaattttggaatttgggtcaattattcttagtccaagggttacactacaaaaacctaacagccttcacaaatttttccctctttcgctcgcttcgctttgcccaaacactcgcctccaactccacggatcagatccgaagagtttggcaaaccctagcttcctctcttcaatctccatctttttcttctctaacaatccacaggtttgtttttcattcctttctctttcgattttgccttcctcttctacttattcgactgcacgaatatggttgtatgtatgtttccgccctcttttcatatccctttttgttcctttagccttgaactactctgggttttcttttctttttttacttttttctattattgtatatctcaagatttgacgctaatctggtctgtggttgtgggttgagttcgtttttattcgtttgtttgtttgtttgtttatggccatggcttgtaattgcttctgtaatctacgtgaatctgtttttgctttggaacgtttttgttgttcaactcatacgagaatcgtcgtctatagttgggttgggttttttttttcagtagcatcttgctttgggaaaaggttaatgcggtgtcttttttttttttttggagaaaaaaagttattagacatccctcaactccttttcctacattgagacagaagtttaatgcttgttttcctctttatctggattgcaagtttggcttttctgttacagatttcctttctcaggatagctttgaacagatttgtaatgttgttctgtttattccttggtggggttgataaaatggttatgattttttgtttgttggcggcataattctggatatttttatctgtttggtctgtgttcatatttgcattgttttccacttacagct

SEQ ID NO: 32 - DNA, 2003 bp, Cucumis melo
  source 1..2003: mol_type = other DNA
tggatcgaccatgacattcaaaaacctttaagatatggatcttataaaataaatgtaaagggtaaacaattcttccttgcttaacccaagctatatattttatgcactaatttaggtattagagtatattcagctgaacaccacctaccaatgctagtactttaatcagtcaattctaacttcgataatatatctcaaccaaattagtgaaaaagagtcgtaaatgaaaaactatgtaccaagatattctatttgttttttttatgtttaaatatctcaaagataatacctaaaacgttttctcctcgtacaaagattcctcatttactttttattgtcgtaaactctaatacaataaactaaaacaagtacaaatacactagctttagaaatctactttttattgaaaccaaaaccaataattcaacatttcattttcaccgacaaacctttgtaaacaattgaagtaatttttgttggtactatgaatagtaacatcaagtcttcaagtgcatcatatcaaccaagacatgttcttaaaagcgacactaaaagatttaaaaccaaaagcatttatgaaatccgaacttaatcaaatcctaaatatttttcacttaaaaaaaaaaaaataggaagaaaaattgacataaatgggatattttcgttttcaaactggcaagccagcatgcaccacgttgttgacgtgtccttccacgtcggaaaaaaaaatattaccacagtaaaaagagaataaaatgaaagtcgttgactctcccttagtcggaggaagcgcgtgaagctgaagccggattagaaatcggcaataaccccgacacgtcatcgaaatgctagtatcaaatattgtccgttggatcttccttcaccaactctatttgaacggccacgatcttccaggtccaacggttcggaagaatcttttcgaaattccatggctagtccctacactcctccctattggctccctagggcatcccgaccggttattccggttgccgggaaggtggctggacgctataaatacccgctttgttcatctcgtagtccttgtaccgttgagcttcgccttctaatagagctctggttcggttggcgtattagctcgaattctttctctcttccagatctacgctgccgatttcatcaggtttgcgagctctgttccaccatttttcttttcctgaagctttgagcatgcttgtgattcttcatttcctcatttctttgatggtttatgaaagaatttaggggaattttctctttttgtattctagtggtactggtagatttgtttgaagtttgtttctcttcttctgagaagtgaattcttccagatctgacagttgcttttgattttttctttgggaattagtgaatgatacttcgatactgttttttgctctctgagattctggatctcgggccttggggttttctattgtcttttggtagctatgtttcgtttgtcagcttgtatttgtcattgttgaatggttcgatccggtttgtaaataaaataaattttgtaggcgcacttgttttccacggttttcgtgttacggtttcatgattccctagatctctggttagaactaagttttttgtcggtaattggatttggtaagggactgttactgtggttgaattgtagatccagtcatcttctacatgagtgtagggttccttagggcagatcttgtgttttataattttaattttgttgtttccctgattttgaacctgtttggttgttcagattcgtcgagtcatttccattcattaaaagtttctataattttatttgaatcttctgaatctgtgcttgtattacccagatttctataaacctatcttgatttcaagtgtgctatgtggtaactgttgatattttcaagcttaagcaatactgatgtgactaaaacttaactaatgaactgaatgttttttgtacacgaactaatatggtgttttgttatgtttcagag

SEQ ID NO: 33 - DNA, 1372 bp, Cucumis melo
  source 1..1372: mol_type = other DNA
aaataaaacgcggagacaaacttggacttccattcccttcttcttcctttttcttgtaggaattcttctttcttccttataaaattctcggaccctttttttttcctttttaattttatttttccttctgtagttcgtttcttgatttagattttcgacaaaggtaccttttacaggtttgttccttctcttcatcgtttactccgattgatgcatttcctctattttcacttttggattggaattattacgatctatgttcaatatcgtttgatccattccctagatggaaattatgtctctgtaattatacatagtgtttgatttgtttgggaaattttgtttctttgtgataatgtcttcatcgatttgatgatgtatttgtttttttttttttggtggaatcgatatgatttatgatttgggtgtttttttgcttttgagaattatgatttgatcagagtttttcttattatttctgttgttttgtttcatttcctgccgtttttaaagatgtgtttagattctggttgtttttgtccttttgattatgtttttatttttcatgtagttggaaatcaataggatttcagataattcatttggttgcatagggatttgaggattggaagttcggcactctataactttgcagtgaatgatttgggtgaagtttttcctcttgtttgtgctttcatgcttcagttgcctcaaccaatatcgctttttggaagtcttgaaaatctgtagctttgagcttgtgtttagttcgcaactgaagcttcaaggaaaaagtaatttctttcgattttcgtaaaaggggggaaaaaggaagtaattctactaaaattttctcctatgaactcgtaggtcacatagttgttatttggtcagttgacactctagactatcttgttaccattccacataactcaaaggttttaagaataaactcaatatgggaatggtttcattaggattgcagagtcaggaacaagagaggttgctttgcacaagttacatactttctattcttagggagaaaagccagttgtcattgttcagggagaagattaatttggttggaaagatttattgtccttctgtctttaggttgtcattggtttgttataattaaagtttcttgtttcctagaaaatagaagtttttccctatgagtaatgttatacttcattgtcttttattttgtgacaagcaaacagtgatttattggatgaactacagttaaattctgaatccattaatttttctgaaatccattgtgattagaatcatgcaatgccaactgaagaaattttcaccaattattaaatgaatatgtttatttgcagggtgttttaaatagatcaag

SEQ ID NO: 34 - DNA, 1122 bp, Cucumis melo
  source 1..1122: mol_type = other DNA
atatatttattgctagggttttccggttcctgtttgctccactatttcagccgcctagggttgaaacaactcattcctccgatttcaggattactatcttcctcctcgaccttctccggtaatactttctcttcacaccccttttgttgtttgtgatttttaacttcctttggattgaaatgcgagatctgtgtgtttctaccactcttctttcttaacttttcgatagtattgcatgttccttacttatggagaggataatgtgtacttagggatatcaattttcgttcacagtattcaatattcatgacttactgaggtgtgaggagttttcatttcatagaccgactgatgctatgatctcaagccgagtttgacccctgtttttctttttatattctttttcttatttttgtgtcaatatattaggtgatcaatgacatcctaatctattattagtgaattgagtaataagaagtaaagtcttgtttatccaattttttggtttggatttattactattttgttggaatgcttgaatgaattctaatggagtccgtagaaatttgtttcaggcgtgcgccttttcttctcactaaatttttcattaggaatgggtgtatttattttcaggagaatttgtcgattggcgatagttgtcttgttctttttcatttcctttataaattctttatggaaaaaatgtatttgctgcaacctctgtcttattacccctatttgaatcaatagagttcctgatccttcctacgatgtggtttctggggatttctctctgggttcgtgtgatagatgggtgaccgagggaacaccctttattggaaatgctcctattcttcagagtcggtttctcattttctcacctttacgctttgctgctgctctcattgacagtcgaaccgttttggaattcgtgatattgtgtgtattttggggatgaaagttttctttaataagactagtgacagttcattattgattgtggagaaatttatgaccatctaattttaatttgaacaagggaggatgaaaatgattgggcgcattgcatgttttatccaactagtactcattttttctttgttctgatattcttcaggaaca

SEQ ID NO: 35 - DNA, 2017 bp, Cucumis melo
  source 1..2017: mol_type = other DNA
actattggagacgacgaaggaaaactctaatgtgagcttagaattgaagatggtgaacaattgggagtcttttttaaaaatctttcgtcggtatattgaaatttccttttacactcaaataaccccccttttcacgcgttcaacgtcttcaaaccttcctttttcaattattttttcgtttacattaatgacatttaggtaataagataaattagtggattcttttgtgaaaaatgttagcccatttaagacttttatgaaatatattagaaaaaaatcatatagcaatttatattattctagttaaaagcccataatagaaactaacccaacctaaagtaacgtaaacattcaataagagagacaaattttaaaataatttctaattaaaaaaaaaattgtcaagaccgtccgggtcggatccaaaatataacccgaaccggccggtttagcatctatataaatacacctttagggtttttattctctcaagacttcaccgcatttccacttctctgaggccacggtcagccattggagcagctcaataatcctttgactccctactacggtaagtcgaccttactgctttcggcttctagttttttcaatcctgtcattagtcctttggagttcttctgtacatttatgacgttttcggctcgtgttttgtttcgcctgtatgtagtgggtttttcgagttttgtttttacttttttttatacttgcaggaattagttgaaatctatgtacttcatgccttggataatactcttgatctgttgtgttattcaaaaatgaattgttttaagatggtatttgagaatggtcatgtgagttttgcctacttggttattaaaatgaattgttttaggatggtatttgagaatggtcttctgggtatttggttggaacctttgtgctctgctatgaattagggtgttctccccgtttttttttttttttttcttttggttattaatatatcttttatgactacttattcatatatgatatcttttactcgtaaattttgactcatttgaaagttttatccttagtcctttctcattcagggtgtaaaggtatgttgttagggttaaaatagcctatgcaggaaagttctgtatttgttctaattattgcatttgtgtgcatttgtatctagtttatttcttgctgagagtatgcttcattttttagtacacatcacttgtgccactttattatagttgcacatttttgtttatggagaggatgaatagcatttagggatgtcaattttttattgagaaaaccctctctcctacttaagcttggggaatttttgttctaaatgtggtaaacataatacttcttcttattttaatttgaatggaaggggaagacgaatactaatattttcaacgaaccttcacaacttttttttcttatttaggaagccatgtttttcaaaattgtactgtgtgatccacatatttatcgattattagtgaatcgaataataattagagttttattggtataattttgaagttcagacttattacatttgtggaaagtttggttacaattttcaattttattggaatcctaagaactttgtgttaacatatattgagttttcttctctttttttttactcattaagttctctattaggaatgtttggttcaatgtcacatagtcgatagctaagaccagtgacccacaaagctatgattgaacgaaaaacaagcctttcacatcttggtaggaatttgttatttctcaatagatttacagagctgtttcatgtgatcacaatttttttctatttttctgaagttctctattaggaatgggctatctggttagttgcttttgagagaacatgtggattggtgttgctcggtttccttgcctttgtaattttgtccttggaaaaagcaaaatgattaggtatcctgatatgcataacatgtttaagccaactagttctcacttttttagtgcaaataattgatcttcaggaatc

SEQ ID NO: 36 - DNA, 2000 bp, Cucumis melo
  source 1..2000: mol_type = other DNA
aagttgttgaggctttcaatccaaccaaataattgtttcgttttccactacaatttcctagtactaaggtagcaatggatcgatccatagagaaccatttgatttttcactaaaatcaatggttgctaagtaaccaagggaggattggttgaattgattcctaatttcacttcaataattaaagcaatggcaataaaacaaaaattggaagattgttgaattaaatttagcaatgagataaatacctaggccaagacttacgtaggttactttagattcacaactcaattattgattcataatgatattagattccttgcaacatatgaacaaaatcttagttgaccacgtctagagaagctaatgtgatgttctataaatcaaatcaatccttatgtctagattaaaagcatcctagagatgaaaatcaattggcattaaggtttgaggctaaagctaagtcgatcaaacaatttggagttgtctaattgattgttcgatgtgatacaattctaaactagttagataaacgtaattagaatggaattgtcaattcaataaatgattctaacttagcttatgttatcttgcagtctaaaaataacaattacatattagatctagatctataacaattaattaaacatgcttggaaaatcgccaatatttccgaacacactcaatcaaagaaataagtccaaggaaagaattcattaaatcttaagattcacaggatgaaaatgttcataacatcacacaagtgtgtgaatcaaaagataagactagaatctcgagataatagtaccttagctatgatacatcctcgaaaacatccaacaaaatcaatgaaagtcttgagtcaattcgtctagtaaaatacgaagagttcaagagaaaatgcctaaaatttagtgccaaaaattgtgtaaaaagtgttggcggctagggtaataatgcaaaattaagtcacagcaccgcaacaacgtgcaaaacacatgtgctatactctcgaaaaactctatagcatcgcagtcaacacgataccgctacacaacacgttgtagggctgaggtgtttgcatgaaattagaccattctaccttacagcatcgtgccttcttcgttccatttcaattttcttgccccagttgacacactaaacctccaattaatctcgtttaatataaaagataattatgattttctttatctacgaacaacattattgtgaaaagatataaggatgatatatcacaatttttagggaaaaaaggaaaatatattggcatttattatctctatcaaatagatgattttacaattatatgttaagatgttttaatccttgctaatgtgaatatttattttatttttgttcacatgaaacaatggtattttgtacactccaagtacaatagtttctttaaaaaaatttaaaatgatacgtaaattatctaaattgacatcttaactaagcaaacaaaaatagttgtttgaaaactagacttatttagtttacaaaaacatgcaccagatatcctcacttaatcactagctctacacccaaaatatagactaaataacttcacatataatatacaaatttaccaaactcaattcggcatctcaattggcgaaagatctttttaacccaaaagaagacgttggggcattaacttttcaaaatgaactttggcttcatagtaggaaattgggagtgaaacatgaggctgaaaaagggctaacaaagagagcgatcgtccacgtggttggcagtcaagaggtctttatagaagaggatgaagaacttgtttcccattggtccgaaatctatccaacaccctcctattagatttcccttccagattctcatcttcatgattcctacttggctccatttaaacccacaattcaattcacaatatctcccacacatcctcttcttcatcatatcataaaacacagtccgttacatacctgaaatcttccatctcaaaaacc

SEQ ID NO: 37 - DNA, 1760 bp, Cucumis melo
  misc_feature 1..1760: note = n=g, a, t or c.
  unsure 1..1760: note = unsure at all n locations
  source 1..1760: mol_type = other DNA
ataatgaatagcaaactacgtaagttaagttttggttactcaaatttaaacgacgtaaaaaaaagaagaagaaaagaaaaaatacgatggaaagaaatcacagagaaaaaaagaaaggaaaaaaagaaagacgatggaaagattaaacgacgtatagaaagaagaagaaaagaagaaannnnnnnnnnnnnnnnngcagcgaaaaaaaaagaggaaaacaataaagatgacaaaagaaatcggagcgaagagaagaaaaagatggaagaataaacttgaattggacaaattttatggactttttacatagacactaatttggtttttttgttagcttcctacaaattttcctcttttattttatttttgtaaaagtaaataaatatgtgtcattagtctaattttttgaacttattttgggagagatagaggaagactttaaaaaattattattactctccattttaattttgagaagagattgtgttgtaccattcctcttattgcttccaatttctttgagggcagccctagcctttgtacaacgcaagcttcctgtagtatctctatctctctctctccctcttccgacggtgatctcttttctctctctcacattcatcacccgccgccgccggtagcttctctttctctgacgccaccgccgccggtaatctctcactcgtcgctctcaacacagagaaatttctgattgagcatcaccaggtccggcaactaacattccttgcttctgcatctctttttcttcaatttctggtatagttttgatggatggattgtgtgtattcaatcatttattgtgttttgatggatgaacccgtttattattcttttttatgacttcaagtaattgcaactgggtacttctatctgcaacttcttggctgaagtaatttttagttaagtgcaaacggacgggctgggaccgagccaatctaacgcttattttatcgaattttgaggagttggttttgtttgggtttatagcttaggaagggtttttggtttcgaagaacctaccatttgaagggttgggtctaaaatgtcgcttaattcgacccaatatgactctgaatgttaaatattgaatagaaaagaaatgaaatactatccctaacctgtctgccaatttcgtgcaaaaaagcctaatagccagttttttctcgccggcagtacattcgccttccccttccaagcgctacggactgttgctcaatctccagaatctctcaattcgcagggggcaagttctttccatcaatcattttatgtatttttgcttctgccctagatcgttcatctaaagttctttacctttttcttctgttttgttttttggtgtataacttatttgatggtgatggattatgattcagtatcattttcttattttatatcagcaacaaatttggatttgaaatcattttttaaataccttttgatgttaagggtttaggcttattattatgattcagagtcattttctacgtgttaaattagtttactttccaagtatgcagttatgttcaagcagttatgcagtcattttctgatgtgggagatagtgctgttttccttaaatgttttctatttaaaccattgtgcgcttggttggtggccgtgcagataattgcatttctttttttggattggggcaggttggttactctctggtttaactttcacaaagaaccaagacagacatccgtaacttgtttgcataaagacattcaaccaag

SEQ ID NO: 38 - DNA, 1767 bp, Cucumis melo
  misc_feature 1..1767: note = n=g, a, t or c.
  unsure 1..1767: note = unsure at all n locations
  source 1..1767: mol_type = other DNA
aatataaataaatctcattactctttatgagctagaaaggatgcctaatggacctacagactagaagctacaacgatatgagattaattggctaaactcattaaccacattatgatatatttgttaactgtgtgtacactccactaaagactcgcagctgaactcttctcactgtagatatatttatgtgtccacggatatagaccaataccaataagttagtccttcacaagtgttcataacactagctgggtcaaattactgttttccccttgggttacttctagtccttaaataccaatgctcctctaatgaacaacctgtttaatgtccaaccactaaacagaatcctttctcatgccatagagagggtaagaccttcaagtcctggatacaccatttaaaggagcgcttatctatttaccataaagtcaagaaggagtgaattccatcttnnnngattatgttcccagctccccacccggttttgtcctcaaaatgataaatatattgagttgacaatctgaccactctcacccgtacaaatcaaaagacaatccctcgcgaataggagttcataatatactcataattaagactaagttatccatgtcattctaatgaaatagaaacccaactagttaatggagttacatcttgtggttactatttcgtggtcgggtcttatgcaaactcattacatacgataccctcactcgcatgtcgcttacttgaacatgttgaataaatgcatttatattagatacaaagtaagtcgtatccatagtgttaccaggataagttacctagccttaaccctatactatagacnnnttaagctgatcttgaacattgtttcctgtatgtctctacatactgttcaagactcatcaaacaactcaagatgttaatttattggatttaggttattaagataaaacgaataatataattaataacacttcttgaaattataataatataacactttattaataactaccaatgaattatatttactatatacgagttttaagacataaaatccaatataagggtgtatgaactgttaaagatgatgtgctattcttgttggatattataggaggtatttagtggattatttgtgaaagaataaggaggtacttatgggaagactgctggaggttagggaggatctttgaaaattaggaagtagggatcaacaaaaaaaacgaaagggaaagcttaaagcttaaaaaagaaacgaaataaagaaaaatgatttagaccagcatactaaaatggcaatgtaatctgaggctaatgtatcaattgagaactttgtagtcataatgattaatcccaaacaaattagttttcaagaaatcaaccccaaataaaatgacttaaatattgaagagtttaaatggtctaaaattattgttactgttttttatttttggaaaagagacgaaaaaggaaaaataagaaacgcccaccgtggggctcgaacccacgaccacaaggttaagagccttgcgctctaccgactgagctagacgggcttggtgtccaaaaatccaataatattgaaaataccatatagtttaatgaactgggcaattggaataggcccaatatattagatatagcgacccaattgttaggcgtgtcttcttccaaaaattggaggcaaaacacaaaccctagcatccgcttctgctcctttatcgtttctctcggcgatcaattttcacggagctaggtttaatcaagcttcaagca

SEQ ID NO: 39 - DNA, 2000 bp, Cucumis melo
  source 1..2000: mol_type = other DNA
tttaaataaaaataaaaaccatctctttattttaagtagttaaatgattgtcgtttactaaattaactctagcctattttaagacggtctggtcaaaaaatcgattacgaccgaccaatattcatctaacggtcttattatttttaaaagatatagaaatgtatctcgttaataaagccacgacggtctttttctaataaaaattcaactaaaccatataacaaaattattgtaccatgaaaaacactttcatacataatgcaaaacaacaatagcaaaaaaccaaagaggaaggggacaatttggggaaaagtaatctcaaatttccctttttgactttgttctaaattagtttattgaaataaaatctactaatttcccatttccaaattaaaatgcttaatctttgtctcattagcattgctagaacaaattgtcttctcaaaataaaaataaaaatacaatatcaactatttatacttaattatctaacatttctccaacataaaaagagttatatatatatcctattttgttctctaatttttcctctttttttggtaattaattataatattgtcctaacatattatattagatagcttcgacaaaccgttgcttaaaaaaagaaaagagaaatccaacctaactcaatccgaaaatatacaaagtacaaaataattataataaggtagatggtatatgcatcaatgaaataatattgtcaactttcctcgatgatgatggtaataataataataattttatatttattaggcgtaatattttcctcaattttagtgtttgtatatactttcatatgtttaatttaagttttaaaatttagtccctcaattaacttgaaattaattaaagaatgtgaaaatgttaatgggtgaaataaataatttagagaaaaaccaaaataaattagaggtagggagtaattttagaagttcaaaaaaaaaaaaaaaataaattagatgtttgaaagtacagatttgtttaaatatgaaccaacttcgaatagtctttccattttttcttataaaaagtctttctgatgtggatactagttagagtatcctatcaactcatcgatccaaagaacatactttcaatcgtaagtcgtccattctacttcgatctaaaatgatgctaggtttgcttcaccttcacccttcacaaagacaagtgcaggtgtgcttcgctctatcacatgattttgattatgtcttcaagaacttcacagcggttttaaaaaaacaagaaagaaaagagtgagagtgtttttatgtcagaaacatatgcccaagcttatgaaacttgttgatcttgtagcgattgaataacaaatggaaagtatctcatacaatttctctatttttcacttttatcgaagaactttgtctcactaactcgtaatctaaaatacaaactcttcgactctaatatattaactccaaacttcatttttcacatctatggaacagataaaggtctaattttttaaaaatatgatgggaattaaagtatagtaaagagattagcttcatcaatgggcttggattggagtccaaagggttagcccaaacccaaaacatagtaaatccaagccctggaacaatgaatagcacggaaagtttgtgctgccggaggagcgtattggaaatgaagggtttaggatagttatggagcagaaaacgacaccgcatcattaaggacggatttgggattttaagaatatattagggacagaataggaatttgaaaagtagccctagccactcaatttggtaacagtagcacaaaaattggaggatacctaaggtaagcgacatggggtaatacacagaattgtggctatggcagaattggatagaactcccatttgaggctctcttttctcttaccatttctacaagataacactactcttcttcactctccaaaaccccatcttcttcttcttctcttaggttcctctctcccttcctcca

SEQ ID NO: 40 - DNA, 2000 bp, Cucumis melo
  source 1..2000: mol_type = other DNA
aattggaacctgctgatatgaaatgcataagagaactgaacctatcagtatcatgcgaaacctgcagcatagacatactaccgtgatgtttcaatttttcaagcaaacaaaatatccaaaaacacacaaaatagaggaaaataaggcgaaattacaaacctctctaggattttcaagatcttccatattcctctcagatccgggtgtaaagacaaccagttcgaagttccaaagctgttgcaatactacttgtctaaacgtcatagcaagtatatttttggacgaggtacttgaatggaaatcttgagcgagagactttctgagcttcgtggccttttccttgacttctctggcaggtaaaaactgttaacacagtcaacttaggaatgacaaatacaatcggatagctaaattttatctaacgacaatattccagagaggggagagagacacattgttttataacaagactcccaatttcatgagatgacaacatcgcacgacagtcaaacaaaattctaagagaacatcaaataatactagaaacggacatattagtgaaggagctcttaaaggtagccttgaaccagagatgggaacgccatcaaatcaatctcattcatcaatcatggagttaattgttccgatggtggaattcaaaatcggtcatagatttttattttaagaataaaaattaaaatggaggctcctgaagctaacatgccaggtgcaaaagtttgggagaacgcgttcacgtcaacattcgaattcagtctcataaatggaaattgtagcaatgacgaaaaatattcatagttgttagtcacggaaatcggttccataatacaccaccgtcgaatgcgagctaaaacgagcaccaaattacgcagtcaggttaaaaaataactaaccagccgggtcgagacagtgctgtgttcatcagaaattcccggaaatacagtctccacaaccattgcaggcatcccagaatcaaggtgctcagtggcggtttcaccgccatcagccgcagccgcagtaacagactgccggaaatcgacgcctccgaccagagaaagccgagacaagtcattctcgtacgtccggacacagggaagaatcttctcatcggactccagcacagcttgaagaacctcttcctcggtcgtcggaattggcctcccagcagagcaagagaaggtagaaaagcaatgccttgagtttttcagaacaattttgggagtataaattaagggtatagcaaacagttggcgagctggtatagcctgtataggagaataatggataaaagacaaactcaacgccattggagaaatggccataaacctctgagcgagtgctagggttttcgttttatagtgctactagctgtgcgtcgccggagaagcgatgtctcgtgcccacatctttttccctccatttcttttcggggttatttctctatataccctcccaaaatattacaattaaaacagttccattttgttttaaaaaaataataaaaatttatttctcaataattttttttgaaaattgaccgtcaatttcgtacaatctacttttaaagaaatgattacttcatggatggtttctaaagggaatccaaaatttaaaagtttaattaatttagattatgttttatataacattgattaaatgaaatatgaaataaggtgtaagttgatattagccctaatatcaaagatgagggtaaaagtaaaataatagtgaaaagatatccaactgattcttgggtaccggttcgggtagggtttgggggaatccggttggcgttttttgagcacagagagatgtaaacgggacgggaagaaataaaggccaacacaactataaattctcctctcggcggaaaggcggagcagcgtccaacttcgcctttcacaaaatttactaagagggggcttccattctacgtcgattctgctcctcttctactttttcccttctgctttttgtcgacg

SEQ ID NO: 41 - DNA, 2000 bp, Cucumis melo
  source 1..2000: mol_type = other DNA
ggtctcagacccataggaatagatcatttattgccttatgaattagtttatgagtacataataattgtcaaccgtatacaaatcaacatgaaagaatataatgttgtacatagtcattccaagtttactaatattatattttaggagtgttctacaccgaacctgtcacatgtacactgggtatgctacccctgaattcaatatcataaagcaactttaattgtcaagcattctcttgaccatttgtgacccatttgctcctactttttcaatcaataactatcacaaaaagctagataccacatgtgataaactcactgaaatcaggtatatggttacctgtgcttggtcagcactcaatcagattcgaaggcctagtctttgtatttccccccctctgcacactacaaatagtcctccacgtaaagacccataacaaaacgcaaaccaagtacagaaaatctagccgaaatccagaccactcaaacataacaaatcttctggtaagtttgaataaaatataaaactaacctaatttaatcaaataatacaataaaatggaagcaactaacataacatatctaaatatgatcacgtagtaggaaaaaaaaaaacattccaaaactattaacaatcattcttaatggtatgggtcaatccccattatttaggactataacaagaattcctcatacctaatgccacatcctatgtccaaccctcgagattacctcgtgagtaatcaatcttattcatccttatttcaaattatgtgaaatttctcatcaggttgatcatattgactttcaatacaacttatgattaatctttcccttgatataatttcgtatgaaaaggaagttgacattatgtgattttctcataaggtaaaccaagtaaacttgacatgacgtcttaacaagtcttggtttctaagtgtaatttactgcagaaaaaatcctaaattctatgacttttcctatgagattgaccaaatcaactttacgagaaatcttgggaagccatacctacaaagtcttcccccaagaaattacaatttctagtaaagattgttgaaatttaccctccaatttttccgtgaaatttgacaaacttgtaagaatatcaaatttgggttggatattgacattccaaaataagtagttttaaaaaggatttatccaacaataatagaagaaaaaagataggaaataacatacccacgtaaatggaatgtaaatatttatatattaggtgtcttgaacgaccgtcaaacgaaaataaattgttcatccgaagttgaaactctttaagtgtacatttatcttttcgtaagaataaaatgtaaaattaacgtgtgaaaggttgggttaaataagttatgtagagataatattgaagatgatagaataatcacgatcgatgaattagtatagtcccagagcggatttaaacctctctcactttcatgctttctatatatatcaaaataatttcaagtagttggtttagtcgtaaaaaagtcaaccaatctcttttagataaaccttgagttattaaaaaattagatcaaagataatcgttgaaattgaaattttaagagtataattataacaaattggaaagttctaaagtagtttttgcaatattctccatcaaaatagagtagaaaaatattttagtaattttcttatcttaattttagttttgtaatagttattaggatggtcctaagttctcaatccgcttttagtccataaaaagaaagaagagagagaaaaaaagtccccgatccgcgacacataccaatccaaccaattatgcacaatccatgtgatatcgaacggtcacaagaataaatgctttctacacacggatcaccatccaacggcttttccttccatctcatcctctatataatctaccaactctgtcatcttcgacacacttcaattatctcagcttttatttcatcggattttccatcaaacaaggcaaca

SEQ ID NO: 42 - DNA, 2000 bp, Cucumis melo
  source 1..2000: mol_type = other DNA
actccattatttggtttgattaaagcttccatctgattaataaataataataattataaaataaaaaaaagcgagagttccattaagtaatattatctaccgaaagagagcaactatcacctcaaacttcaaaaagataaaatagagacgaaacttgaccaagtcaaacacaaaccacaaacaaccgatctgacagaaagtttgccagaatcttcaatgtacacgcgaagataaacaaataattaaatctcgttcgtctggataacataacacagcaaatgaatttttttaatacatattttaaaaaagaaatttaaaattggtagattttataaatcatttccaaagggtttttcttgttttaaaatgtttttttgtttaaaataggcagttcatcaccacttgagaagatccaaactgggcggcaccggttctgcgacgcttgagggccgtctccgactcttcgccgtaggaggccgatttacgcaaagaataaccggacaatgttggacagttttgacgagaagttaaaccgagtaagggcttatgcttcttctcaatgcgctcgtcgtcgtcgtcggcgacggcggcagcggtgatggggacttgctctgttgcggggtgaacattgggattccgacaagaaggtgggttcttagggttggagggaaagtggaaagcgttatggggttcttgatgctgttcctgcaacttttgctgtttgaggaagcgcttttggagatctaaaagagaagggcgaccctttttcttcttcttcttcatggtggatttagaaacctcgcccattgttcttcttccctttctcgcaggaacgaagcgcagggaggttaattgatttcagttttcacggcggagggtgcaggatttctaggcacgtgcgaatcgcatgaccctatcacgtgcgaatcagtgacggtataacgtgcatgcaaaggaatagaaacacaaaccgctcttacaattataaaactctaaactaaactacgaacgcatctcataatgggcccactccatcatcctatgggccttttgaattttatgtatactattttttttttttttttttttttctttaatcacaatcaatttttctggtatttttttaaatattcaacaaactttttgttttaatgttgtgtatatctaattaatttagttttattggatgtcattttttctatttttgaaaaaactcttaaaaaaaatataaacaaaaaaagaatggaaaaagaatatcaaacaaagagaggagagagcaaccatacctaaaaagtttgaaagtaaaattgaaaaaaagaatatacattgagggcagtgttgaaaatgaaattaatgaaaaaggaaagggtacgtaacaataaattacattttcttgcaggcttaaacgaaggcccatatatgaaaagggaagcttcgatttgggttcagttatgcgggcctggggttggtattgggcttaattttataaagaaggcccaaatgttggaaagacgggctttgagagagggtgttcggcttttgcccgaggggggtgggggagtggcaccgccaagcgaagacaacgaatattaggagagaaaacacaaagaggcggagagatggaagagaatgaggtggaccaatgagataagagtgcgcagattattgaggtggcaataaatttagaatcccgcctaaatcccagctttcatttcatgcgcaattgaatttcaatttgccattcccctccatagggacttaattatccccttttttttactctcataactccctctcttcccaccacgttcgcttcttcctcccccttcctcttcaaaccctaaacctaacctaacctaacctccttccccaacttcttccgtcggtacgtttcatccatctcctcccacttttcatctttttttccttctaatttcatctcttttctttgtttttccttccaattgttgctgatcccatactatactgcaggattcgaa

SEQ ID NO: 43 - DNA, 1115 bp, Cucumis melo
  misc_feature 1..1115: note = n=g, a, t or c.
  unsure 1..1115: note = unsure at all n locations
  source 1..1115: mol_type = other DNA
aaagaaatcaaagcgaaaaaacgaggaggaaaagaagaaaaacgannnnnnnnnnnnnnnacataaataaagaatagaaaaataaggaagatgaggaaagaaatcgcagaaaagaaaaagagaaaagaataaagacaaaattgcagggaaagatggagaagatgaaataataggaagaagacgaatcgcgagaagaaaataaagatgagagggcaaacctgaaatatttaaaaaattgctaactttatgggttttgttacacgggccgtaaatagttttgttacatttatgtaaatttacaatcaattaattatacaattaatcaaatttccacaaatacaataattggatattttcccaaaatatctaataagtttcaatttctacccatcaaatatttcaaccattattaacaccaaaaaattcaaagattaaacttaagataattacaaanaaattaccttaaatttggggcattacacatttacattgaactatacaattgtttaccataatcaaaacgatcgtttttttatgatcgacatgataatttcctatgatcaacacgattttttatcatatcaacaccttcatttaaatttgaagtttttttcccatcgttaaaaagaagtacacgatcttttagaagaagattacttgcgcgggctgattaatcgtctgttgactgtgacattttttatatttttcatcatgagcctgtatgtcttttttgtttttataattgttttacatcgtgtaaatagtttgccgattagttatatttgttagaaaacactttttcaaatgtcgaaaatttgattttgatttattaaaactttagtaaaggatagtgtttattacgtatagaatcccaaattttcacaataatttttcaaaagtaatccaaaagaaaaaagcaacaataataaaaggctcaaagcgacgtcgtttagggcaacagctggggagaagaggacgatctgaaaaatcatttcttgagcgaagggaaaaggagctctactaaagcagtcgaaaaaagaaaactcaaacctcgctgcgactctcgacattgattctgttttcaattcattttgccaaagttaatcgatccgaac

SEQ ID NO: 44 - DNA, 2000 bp, Cucumis melo
  source 1..2000: mol_type = other DNA
tatagtttgtaacaatctactctatgttctttcaattttgatacatttgaatcttaaactttattgagttacacaatatagtccttgtattttaaaatttataatgactctatttatattaatattatagaaatttttgttaaggtttaataaaaatttttctgtataaataaatcgaacacgaagtctatatttagactgcaatatagtaaaacctgacatctaagtttggtgaattttgttttgctttaaaaactaaactattacaattttaaaaatattttaatttagttaatgcacattaactttacggagtaaatttttacaagattgaatatacatagattaaatagttataaaaccaaagattagagtaaaaacatttaaatagaaagaactaagatttttttaaaacgaaaatgatactagatacatatatatgtatctatattataattactcattttaacatatagttttgaaagaacaaagattagttgcatgtgttgattgtttttaagaaggaaataatttttgaatggaaaattttcaaaagttttaaatttgacaataaactcatatttaaagtgtactacaaattttaacttttggttaaactccttgtttagttcaatcatgtaataaattctcattccaagaatcgttttagaaaattttattgtgcatttaataaaatatagaacatatatggcatataaaaattgattacttttttctttttttgggacgaaaaacacattagatataatcttttttgaaagtttatgaactttaaaaatgggttattttatacggtggtcaactttattttattgaaattattgagtttataaagattgttatatcattttcttcttctctttcactagaatacaatcaaacctatcaaactctctatgacttatttagaattctttttgttatatttttgaaattaataaatgaaaagcttagagtctaaattataacaattaaaattgaaaattttgcaataattttatttttagcaaaatgacgtttggtttttggggattgggaatggatcgatactatcccgattccggacaaagaaaccgacccgagattcgaattttttccattcccaaacagagcacttaaaatttaagcaacgttataacggcgtcaccgaactaaacggaaaaatatgaagaaaattagaaaaagaaaaacggaacagtcaaacgttacttcacgtcaatggcaatattcatttttttttttgtttaaataattgaatttaattaatttggtttataaaaatagagtcctcatatatcgcgaatgcgcatttgatcgtgaaggacagcttctcccttgtgttcaagagagagagatctatcattcttatttggggccgatctctctattctcctctcttctattccgtaagtttttctcattcattctcctctctcatttctctccgagatctgtttacaatccttttgattttcatttttcctgcttcgatctgtgctcctggtgattcccttttcctgttttatcttttgttgatcttggaattgattgttcttttgtgggttttcattgatttgtattttctgatctgggtttctgttttctcgccttgatgttttgtatttggatctgatctgacgtaccctttttttttttttttatttgaattgcttttccaatgtttatacctggatttttattgatgcatgggtttaaccgattggttggatgcgttttctttgtgctggatctaggtgtccttgtttttaatttgaattgtgggtaaaaatggcattattgtaatgtgtttggagtttgattttgaatcttggctagttgatttttgaattacaaagatcggatcctcttcttttttgggttgtcttaagatttttggctggtttaagtatttgatgtcgttgtattttaaggggtaactgatgccggcttgttgtgtttgtattcagtttacttgaaaa

SEQ ID NO: 45 - DNA, 2000 bp, Cucumis melo
  misc_feature 1..1115: note = n=g, a, t or c.
  unsure 1..2000: note = unsure at all n locations
  source 1..2000: mol_type = other DNA
attatctaaacattaactgcaactaatacagattacagtaaatttgaattatgatgttatctagagtcatttgtcttcaatgatattgactcagattcaaactttatgaaaatgttaccctggaaaatattctaccgcaaaatttcaatccaaagttaaaggttgaataatttagaagttttctgcgacttccacccacttattatttagaagacctgaaatcaaaatgatagaagatgaatataaatatatttttttgctttaaaatttataaatcaaacatttgacctagtaattgataatacataatattatgtgactcgtaagtaaaaaagaaattgaaataatatatatatacggagatcgcaaaaaataaaaatgaaagtaatataaagtaaacgcaaagtaagaaagcaagcattttcaagtaagattgaaacccccgtccctgggggctccaagataacacgggtgcccaattacccggtacacgacttttgttgaacaacattgaataattagcccaaatgaaaatatttgtcgacatatctttcttataatatgtaaattagataccaacacaaacacttgtaacaatatcctaactaacttggttttaaatatatatatatatattatttttttttctatttatttatttnnnnnnnnnnnnnnnnnnnnnnnnnnntagataccaatatttagtggcgggtccataaattttatatagggttattatataataaacactaaaaatttagatattattattttcaaagttaggccacaagtaaaagtggggatataattattatactataaccatattttggtaaaattaagtattaaatatactttaaaattaatattaaaatataaaaatcgataatgtgtgggataaatttatggatgtaaatatcaatgttttaatgttcaaataaataaatagtaaatagaaacaaaacaagaagtcagtctttactactaatcgggactaaaatttgaatttgatttaaaatttaaaacttaaataggactaaaaatgttaggacaaaatagtaacaaacacgaaatttaggcaaagaaatataattttatttatttattatcattttttttatatatataattgaaaattgattactaaaaaaaacaaagaacggtaaaaccctagattaaaatcaaaatagaaannnnnaacccgaaaggagaattttgatttccagagctaaacataacacgatccaaacccataaatcccgcatcgagtggaaccgatatcttctccccttcgaagttccaactctccgtttccgtctttcttttcgattctccttcaaaccctcttttcttcgtcttcttcaaatctctacatttcaaaatcttcgctaatctcttcttccccttctcttccgatctgaccgtgaccccattcgaagcttcttctttcaccaagctttctctccgctatcaactttaactttcgtcctgtattccttagccttcccttgcttttgcagtctccgccaccgaacaattcctatcccgagataatcccacttttgggtcgtgtttctcacttattcaaatcgctggttctttgattttgggcttatttcactctgcatctgctgcgacttggaggttataacatctctctctcggtcttgttaggtatgaaggatttgagatattttctaatctatctgaactgggttttctttcgcttccgtttatgagatgtaatttgttgttctgggaagttttcagatcctttctaatgggcttctttaatttaatttaaagcttctttgtttgtacgagatgtcaagtcttaatttctagcaatatcagtatctgggttggtggtatttaggatgatcaagtcttttgttatttaatggatgagaacaattattgtcattgttattattattttttggaaaaaaaatcaatgggttttcactggttttgttgatctttttagataattgaagttc

SEQ ID NO: 46 - DNA, 2000 bp, Cucumis melo
  source 1..2000: mol_type = other DNA
cttctcgatcgcagcaattcaacttcataaacaagtccaagaacgaagagtttgattcccctaatttaacttaattttctggtgaaaatggaccatacttttaattacatattattttggttattgccttttaaatggtctattttaatctctaattttttttattaaacaatgatggtgaatcttttctaaaagaaagaaaaaacttctttacaaactatccaactctaataacaacactaattataaactagtctactacctttattataacagcaattaaaagaaaaaatcgtattcactgacaaaaattcgttcttttgaatgcttatcgaatgttttaatttttttaaaaaaatatataaatatttgtaagggaaggatcagaattaaaactctctcccctcaatgaaattgaattatttgtttttcttgtttttctttttttaaaataaacctatggatttagttggtcggtcgaattaaaatcgtgaggtcgcacacgcggtgtcttgtggattcaaaattatgattatttccatcaccccttggctttttcgctccattcggccatgccttacaaatttcgctccactcccattcttctcttcctctcctctttcaactgcattgaggccgatcctttaggtaaatggttctctcccatttcatctctaattcctctgtttctttttattttacttgttctttttccagccggatcctccatttctgtggtgaaactgaattgttcttatcgatttcttgtttgaattctgtttttctctgtttgtgtctgtgtgtgtttttaatttgttttggcatgttgaagtttaaagataccaaaagttgcgcttcactactttccagtttcgatggtagctgctagttgtaacgcttacgttcttggttttttagttaaaatttttttgcttcttgttgtttactgtttagcaaaaagcatggggaatactaccaaagtcccgaacttaatagatagatgatcatgtgctaagaagtgcgatactttccgtagctgatacgtgacacagtgtctgacatttgtttgacacatattagaaacttgttagtataacatatgtgttaaacaggcatagaacacctgttgtactaaaaaaaatatttgtatgataataataataactttgaagtgtaaaatatatccagctaagttttttcaagtatacaagtgcattaactcatttcctcttgattttcttttggtataaaaattatatatattttgaaaaccgtatactttaataaatgtatccttgtgcattatgtcctagatttttagaatatggtgtgttgttgtgtctatatcgtgtcgtatcaatatctcgtattcgtatctgtgtttgttagatcatatgtataagcgaggacagctatttctgatgttacaagaccttcttcaaattttacaggaaatcattcaatttgaaaattcaagattacaaatgcaatctaaaccaaacttcaagaacaaaaagtgttatttgttaatatccttgcgacctcacccaaagtatctattacaaacttcagaaaaaacttcataataagggttgggttgaaaaaaaacatgaagaagtcccaccccaacctaactctaaaaagcataaaaaattcaacccaacccaaaccttacaatttgggttgggtagtccgtgttgttcgggttgtcgggttatttgaactcctagttttagctaagtgtaaacttatttaaggatgttgaaggttagcattgatctttctctctcaaatttggtcaagaggaattattttttgagtcattcatatagttccattttgcttttgagcatttgaattgtttgttaactacttctttgattaatatattcgaaagtgaaatttccttggtttactttattgatcagtgtcccattttaccagttatttcagttctcctaataaccttcattggacttgagttcggttaacacaaaaca

SEQ ID NO: 47 - DNA, 2000 bp, Cucumis melo
  source 1..2000: mol_type = other DNA
aatgtatcgtgggcatttattatgacaatagtgtaaaaatgttgttaacatatctgtgtattgtcgatgatgtagatctactacgccaatagttatagtttccatcggtatatctatgaaatgtcaacgccttaaaatagttgcatgggcatagacttgtttttttagaaaaatatgttttatatttgtatttttttcactaacatccttttggttttgtatctaaacacaactcaaaatatatcaaatactgaaattcatttcctaaaaaagttacaattgtttcaaatataagtcacctgaatgaagttcttaaaacacaaagaattgttccttacaaaattaacataagcaaaatagtaagatcgtccaaaataacaaacattacataaactttagaccaacttctaatttgtttgccaggaagtgatctccattgaaagtttgtcttaaaaaacaaataaaaagaaaataatagaaacatattcaataaactagtacattttgcaccttacatatatatacaaaaactttacctactttaatttcttgaaaatctaaattttgaattaagaacttttcttacaacgccaaaacaataataacttataaatcttagtgatggaataataagttataattcattggttgattgtatcattaaccatttctttcttttggtgtgagaaacttatccaactaaaaatattcacaatagtagggcgggtttgtcgtggctttgtctgaatttctacaacatgtgtaaatattttcaactgttttatcctctaagacaattttcctaaaaacaatcatgttgttcacacgagatttccaaggaaatttaattcaaggagttgaacttgtatttatgttgatttgatgcctatgcttaattttaagatttgagaaagcacgttatatttgtaaagttggagtattggaagaaaagtttgtattttcaaaagaacctcaatattcgagatcgacggttggcttcaaaagttaggaagtctttgactcataggagaatcctatctagactttatgcaatataaagagagttctgttttatggacttagttggataaataattaatttgattcaacggtcataatgaaaacatgtgacatcattataattaaccaatttatatctttaatacacatatcaacttttaaatagttctaaattcaattatttgtatttatcatcattaattaaataaataatgtgacaatttgtgattgatccaaaaatttcatattcaatctatactatattagttaagcttaaaattttactaaatgcttaaagttttggattatcgagcttcctaccaaacaaaagcctctattgcacatttaaaatatagaatagtaggtttatataatatgaaagattgactcttaagaccatactctatgacctaatgaaatcgacatttatgtaattgataattaataattaataaaaaaagtgtgacaaaaaagtggacataataaaagaaaggaaattgtgaagcattagcatccgaatttcgaagaaaacaaagggcgccctcagatcaaagaggacatactataaagtctccacgctatttcaagaattggcgtgattctcaagcgacatttccgtaattcaccacaaaaattaaaaacaaaaaagaactcacagattctgatttgacttttgaaaccccaacccccatcatctcccaatttaattttccctcgatatttatccaaattcagaaacataatcttgacaattttatgctccattcttccaatctcagccgtacgtttcattcaaactccaattctcccccactgcgccttccactacctttttcctttctattaaagtgtcctcacaaactcacctcctctctctgtttctgtctgcggtaggatcgccgactccggatttacatttcaggggtcgaagatttgttctggggtttctttaatttctttatatatatacacacacaatc

SEQ ID NO: 48 - DNA, 2000 bp, Cucumis melo
  source 1..2000: mol_type = other DNA
gccaaggaaaatgaattgtctaagaagaagaaagaaaagaaagaacattttttgcaaggctacaaatcaaaacttaaattatccacgtgacacaacaagttcagagaggaaagaaccctctaaaactcccatataccttggcaataaccatgacaatagcaataaataaacaagtccatgacataaaataaatattgttttcattaaatctcaataattcatatgtagtccgctccgattatgccacagtcatatatcaagttcagtattttaacaattcaagtagacatacataaagctactatggaaaacataaacaagaatggaagaaggagggttaaggaaacctttatccctgatggagtttcagtaaaactgagcttgtaggtattagtacgaaagctgtgaaatgaacaaccttggccaggtaattgaggcaccccaagatttcctttatcaacactatcaaagaaagtaaagaaagttatcacttcaaaacccaactcccaaaagcagctcatcattttccagtaagttaatactttgaaagatcaaaatcaaatctacaatcaaattagacttcttaatagttattgccacgaaccatgcatttgtcacgttattaagactatggtttgcaataatctcctatctggttggatcactacttatactaggcacagcataaactaaagtagtttcccagagaaggaagaaacatgaacctggttgggtccatcttggcagtaaaggatttaagggagaagagcaaaccaaacataagtttatggtcttgctggggattcaatgtccggagaggccgattccactccctgtagaacaagcaaactccattcctattgaaaatatacatcatatgcacattgtttccagtcgctgtcggtaccggaggcgagggactaatttctgacccaccaaagaactgcatggtttctggaataaactaaactaaatcaaatcaattgtcatataaaatgatctacgaatctaagattctaacaaacccaacatttcactcaactctacaatcagtaacctagcaaagcaactaataattcaatcattcctaataattcattgaggttaaaaataaaatagcgaattgtcaacaggtaaaatctaacccgacccaaatcaggaatcactaaagcaagaagctgtatgactcgatcaaaaataacccagatgcatttccctttggcctctctacagaaccactcaatatagttagaaacaaatctagtgtaaaattgggagtcctattcatacataattccaaggaaaatggattttacttatgcatcgtataagagactgtgagcaggggaaaatggagagataatcaccaatgagctggatggtgacagattcaagaagaagcatcaaaatcaaacaacggagagcagaaagatacctcaaagagcagagactgcaaagtaaaggaagcgatcaattcaacgacgaagctcttgattcgtcaggcaatgattgccggcgacaacaacgtcagcagatcggagccttacggcaccggagacccctccgacaaggacagagtgaacgaacgtcgtttgtgaacggtgtaagcaaatcgatctctcggagtccaactccaaagtactgtttcgatatgcattaatacatttgatttttgttatatcaaaaataaatattatattaaaatttataaacattaacaaaaaaaaattaatttcacataatttaaaggaccatttggtaatatatacaaaattgcaaaaatcaaattgggcctattttgttgttattggaggcccaagatgggtggtgataaatatgggcctccaaaagaataagcaaaaaaccctaatttcctctcttcctctctttcccaatactataaatcttcaccattttcctgattagggtttttgttcgttcttggccgtccccttcatcgttcccagagagagggagagagtaagttgcaatagtaaaac

SEQ ID NO: 49 - DNA, 2000 bp, Cucumis melo
  source 1..2000: mol_type = other DNA
aattagcaaattgtatgtaacaacgtcatgaagaggcatttcatcgaacaatttaatagcagagtcaagatggcccagttttataagtttattgatttctcgattcttaaggtaaatgagatcgcgagcatggaaatgcagacccaaacgagaatatgggtgtggtaaatggaccggtgatgttgtggctacaaattcggattttacagcagtaatagttctgacgaaggaagcgaatttagtgacctttcgcatcacagtttaagcttatcagagacctgaacaagggctctagctctacaacttagaaaggtttgatatggtccgtgatcgggagggaccgaataacaggcgcttaaattgttgttcataaagaagaggattgtcgttgatgtattttaaccaagagatgattagttatccacatccacagagagaacagaagacggctttctaaatctacaccgataaaaataaccctaccactttgtttctttagaaaagggtcacattctttaaaaacattagcgtcgaggattaatagggtatattgactaatgctctgtttggatttcgagaaataccaatttacaattgatttcaaattaattatgttttgttgttgcacgaaagataaaaagaatttaaaattcaaaaggatctcaaatcttatttttaacttaaaaacttttatgacccaaacggtttatgtatgatttaaaagtagaatacctctgtgaattcttaatttttttttctttccaattaccacataaatatgaaattttaaatacatttattttaaattttatatccgaaacaaaataataatttaaaactatttctcatatatgaagtgtgattcgatctaaattataaaataataaaaatttacatctagttttgattattttttttcgttagatactaaattgttaagaaaataacatttttaatccaaagttttgaagaatatatgacttttaaaatggtatttatctttttagtgtctgatttttaaaaaatggatttcaaaagttcatcaaatagcattgtatttttattttaaataattttgacatttaaaattagagtaatggtttataaaagacacttgatctctaaaactattttcttagatataaatacgtatgattatttttaaaaatcaatcaaaataggtaaattgtaaaaaaaaaaaaaaatcacatgaatagtagttgtaattatgctctcaaactttcggttatgaaaaataaacattttaacttttagacgtgtcaaagttgagtcaagttggaccttcaaagttatgtagttatataaattgtaatatatgtataagcttgtggattcaattttatcatttatgggtccaatctctacaattatcgtaagtctatgggtcaattgtaacacatgtggagtttaagagctcaattttggacgtggatgtgttttgcaaccaactccacaccttaaaaaggtgtttttttttaatttatcaaaaaacaagaatttagaatctttaagtttatctttaaaaatcaacggacattttgaaaaccaattgaaactactgttataaacctaacaactaaaagtatattttttaagaccgaaagcataaatccataaaaaaaaaatccagaactgaaaatgtaacttttatagttgaaaatttagctaaattatacatattaaaattcaaggaccatataaaattaaagtacctgattaaataataacgaattaatgtttggtatttttaacctacattagaaaaaaaaaacaaaagaaaaacggcatactatttgtcaagcgtccgatgggaagaaaatccaacggtgagtgttagtattgaaatacgcagttctcgtgaatgagcctggcttagatttgggaacaagagccaacccctttcgaccgagaagccgtcgtcttcaccatattcgcctcaaccattcgatagccacgtttgaagaagaattaggattgcc

SEQ ID NO: 50 - DNA, 2000 bp, Cucumis melo
  source 1..2000: mol_type = other DNA
agccaatggttcaattaacagctctagttctagcatggctaccgctggtaacctttctatgactagagacgtcttggaggtggagggtagggcacgaggattgaaaggtgagggtttggtgaaaactcaagcctttcaaattcaagaaagcatgcttgacctagtagcatctggtgatcttggggaatttgcaatggatactcatacccttagtcggcattcgtctcttggttctgctggtatatatttttttctcttgttttctagtgatattttcttttatcaatttccattatgaagatggaatcttatgttctattttttcatttggaatgtaggctttcacaatgaaaaaattgctaatacgtttccagaagaggttgctaaagacccgtaagttcttatttcttaacaatttcctcagtttaacaagttttatttactaacatatccttagttgtataaatatgaatctattatattaactatttcatttatctatcttttaacagggtgaccattcacaacaaagataatacttcattgaaacgccctcctgtctcacgcacttcggcatcccaggatggattgtctgtcctgattcctgatccggttgttagaggaaagaactcagatggtaaataataagtgatccattctgttatcttctttattcattttcaattttgtattttgtatatatttatataatattttagaaagataaaagatccatcctgaaactttgtttcaggtggaagaccggacccaactagtatcttggtgaaccaagaaaacatggcagccatgaagaaagagatgcgtttccggcgctcttcttcttgtagtgacagcgacgtgtcagagacttcttttattgatatgctgaagaagacagctccacaagaatcccatttgacaacggcgggagttccagagccatctgatggaatgcagggagggaaaggtgggaaaaagaaagggaagaaggggagacagatagatcccgcactactcggattcaaagtcaccagcaaccgaattatgatgggtgaaatccaacgcttagacgattgatccattaggcaagatatagaacagaaattgatttttttttttttttttccaatcatttttgtagattgtgcagttatttgttttcgtgtttgtttaaccctcttgtaagttgttgtatataggtttcttagagttgtcagctgcgttgaaacatgtggccggtatatgtattccaattcttttcttttttcccgcagttgtaaatgatcaaatttgagttggtcaaattaccaaacctttgtacaggaacttcgaagagagttgaaattttattctttttcttttttgttcttttatagagttcgagattatttgtatgaatataatcaaaagcaaagcatgtaaaaataaaatgatttgaaagggaggttttctatcccattcaatgtgacgaatccaacacttaaagtaaatttgaaaactgtctaatttatatgtatggaatgtaatgctcttcaagaaattatcttatcttctaatatttaatgggattcacataaatatgaaatttcaacgtttttcttttcctttttgttgtgagattaaggatactagataataaccgacctcaaccttttaggccaagaggtctggagtctttatacttgaaaaaagtttacacatattctaaaagattaaaaggttaattgtttggtaaaacattaatgatgacgatacttaaggtttcattaaaaaaatatttggaacaatttgtttataatttaataaaattgtaactttgaacattttgaattacattttgtttttccatttttacggtcctcgaactcatcgatactcacaatggagaaaaatatcacaatgccgaaaatacccttcttgttcccttcttatacaaaagcaacactattggccttatcaacggagcagcagctactctcctttagcacaaatctccatcc

SEQ ID NO: 51 - DNA, 2000 bp, Cucumis melo
  source 1..2000: mol_type = other DNA
tggtgtacccacttggttttttctctttttttcttttagctttttgctcctaaatttcttgccttagttttcaaaagcttgtttttatttttgaaatttaaccaagtgaatagaaaaaaaaaagagaaaacaaaagcttttaaaagcttgtttttatttttgaaatttaactaagtgaataggaaaaaaagaaaaaagcttataaaatttgacgaaatttgctgtattttgtacattttactatttttctattttaaaaaatgtgtctgaacgaaaaacttatattatgagatttaattttcaaaataaaattataccaaacagactttagaattgtcaatcaaatttgacaatgattaggtgcattttttaaagttatcctaaagtttttttttttttcgtagtcttgcccttgcttttatcgttaacaaataaaattttccttatatatatatacacatttaactactcaaggtctgtattttttccacctgatttatttaatattttttttttttgcagaaaatctatttgtattttaggggaaacaaatgagtgaagagatcatcaagcaacggttgcgatgttgcagcggaaaaatctttggtttgtcatttcttgtgatgggggtttatagggtagtatggttattgtattttaggatgttgatttttattttaatgagccaagagagagatgtggattctaaaattgatgattgatattattgatgtgatataaatatataattttgtgcgaaaattgctattttattttctgtatgctcattcagatcacacaataatatttgatgtagctttacttattgacaaaatataggttttaatcttgtgctcatacaaacaacagctatgggtgaaattattttctgattttatttggcaaagatgatgtcagcattgtgtaaatttaatgtgaattacacttctgatttcttcccaatgtgccctctcaaatattggcaccaagccatttaattgtaaatacggaaaggtcataaatttccatgcaagatttatttcatgtttaaaatgattgtgtgaaacaaaatgaaaaacaagaaattcttacctccaacctcaaagtagtcgatatgtcaaggttcaatatcaattttaaatatccatgaatagctttgatatcttttataaatgcttgtaatatatatatactaatagcaatgtctataagttagttttgagagtaatacttgttatagataacaatgttactctatttaccactctactattgaaagcttctttttcttccatttatgaattaataacggtcaagatccaattgcatgagttacttttaattaattacaatctaaaatgttaatataagtctaaaattgtccaatatatgtgattttttttttctctctcaaaccttcccttcttttcattgaacttgtggttcaaatttgatggaggacactgggaaacagcacaattcaaagagccaaagattgagtaattttttgatttcagagttttcatctcttcttcattctacacctttcacttctcatccacaactatccaatcaaccattgccacgtggcatcaaaaatatccaaaactgaatgagatccaccacaaagttcctctcatcactgtttgtcatcaactcatcaagaacttcatcatcaatcagaaatccaacatttcaacttctcttaggaaatgacatttttaccagtctccaatgtcaaaaactcacacaaaatccctctttccaatctaaattttacaaagataacaggggtaattgaagaaacttagcagtaagttaacatattatagctttcatcaacccaagtttttttggttcctttctaaactgtagtttgttttcttgatccattctaaatatttcctctgcatgaaaagaagaaaggaaaagtgaaggcgaaacctgttttatgcttcagaaaaccaattcagagtaaccaaagatctgaacttcagacc

SEQ ID NO: 52 - DNA, 2000 bp, Cucumis melo
  source 1..2000: mol_type = other DNA
cgctcaaattactaacatccttctctttcttgttcccattcgactagagagacactatcttatccacctcagttggctgggtgaaatcattgaaactaacggttgattgtccagattgttaaactaccctatgttttatcatcttggttacatttataggattgtcagaataataattccttttgaaatcatattctaattggcacaggactaaaataatgcctttcttaagctgtaataattagaatctaaacagtgaagttagtaactgattgatgacatttccacgattttcatttatatcctgtgcagctattctgacatcacaaaacatttcttgattttcatttttacttgtcatccatcagtcaggacgatatcggcgcgcttgttgacgaccttgtcctaaatacaaagaggcttatccgagctacttcaagggagattgacaagtggaaaagatgaaattactcatttgttattacattgtacaagtgatctattaggaagaaccacaatcaaaactgaagaaaaaagaaacgtgctggctgtctacgtggcttttagaggtagaatttatgtacaattgtttagaaagatgtatttaattgctctaaatctcatatgcattggattttgagcaatcttaaaatgccgaatacttaatgtattatcgtaggggtccctagatggcagatttatcatgtccattctccagaaagaaagaaaaaaaccctttttattatacttgttcattttaagctttttctggttgattataatgtcagtaatttaaaaaaaaaaaaaaattactgtgtattggcatcggttatatgttatatacaaccctagttaaaaggtaaagttttgttcattcggtcattagtcattcctatacgaacgtcacattgtgctttataatttcaataggttaaaagtattcaatatagttttttaagttacctagtagaggtgatcattggttgatcggaatcggttttttgacaaaaccgccactgaaccgatcatagtcggtttagtaaatgttcaaatcgaccttgacatcgatgagtaaagatcggtcggtcggtttttgtcggatgggccggtttaacacttggaaatactattttgaaatttttcgaaattaatccctcttgttttcctaccgaccgattttgggtttggtcggtcagttcgattttttcggcctatcttactcactcttattacctagggattgaatttcattttatccttagttttagggttctttttttatacttttgaaatatttatgtcgatgtctagagtttaaaaataacacttgaaattataatataattttttataattgttagctataattttacgtccaaatatcaactcactcgcaacttgtttaatcaaccaataatatgtgtctggaatagtaagtatataacttgtggaaaatgactttaaaagacttttttaaagtatttatttaatgccaaaatatctatatttatgtttatacattaacatacatatccaaagttacatattagatttgttaaataattcaaaatgagctaaagaaaaaaagaagttccatataccaaaataaaatataaaaagttgaagactaaaatagagattttgaaacaaggtaagttagatttacaaattgcaatatgggagaccaaaccaccacataacaaaaatcccaatgtccaaatggcgcaattttgtttaggatagctcacgttatccaaatcactcaatcggagagaccaacttaaaggccacatctgccacgtcaccatactccaccaatcacaacacagcattggatttctcagcttatgagaccaatcacaaacctgaatccgacgtggcatgtccacatccaccagtaccaaccatatagcttctacgttctccacatctaatcttcaccatttacacaatattcttcattcttctttcctcccttcaatccttcatcctctccgccc

SEQ ID NO: 53 - DNA, 2000 bp, Cucumis melo
  source 1..2000: mol_type = other DNA
aattctaacaactccggaaccaaataatttagcatggattgaaatataaatcttcttgacttgcaaaaaaatcattgtaatggtcttatgttggttatagttagggtatcgaaacgccatacaggaatatgggattaaagttaacttttgttcatcaatttcagcttatgaacttctaaaatatcaattttacctttgaacttatatgttattacccctttcgattgtggtatgttaattaatatctgaatctcagtccttatgaaacttttttatactgtcacaaacatatgaagttttattgtaagttcttagaaatcatctaaaaagagtagtttgttggactatttattttattttttcttattaagttgttttcacgccatttcagtaaaataactatagtgaatagagaatcaaacttctaatcttaagttaaggtagtagggtatatgctaattcaataagataatccgtgatgcttgacatctgacttaattgttataagttttaaattttttattgtaatatttaaaatactagtttttggtttctaataaagaaataattgaacaattacaaatatttatacaaaattaaactagaatatatgatcattttccttcgtgttagaaaaagggaaatatatgtgtgtatttatacatattagatattgttttactatattccattttcctcacgggaaatggaggattgagtgggagataaacattgtccccaagagaattgggaatggaaatgcaaatgacatggccctccacaaaattgttcgcctaaaaatgggctttctcacttctcactccgcaagaaaaatatcgtttcccttcgaattattcgggcggcaagatctcaaaaccacatgtttttctttctttatttttcaagcctacattatttataaaaatataacttaagcagagaattatgtaaattcaagtccatttttcgcttcacttagctaaatcattaacaaatctgtaattttgttcataaattagctcaccaattatgttttagcccactaaggcccattagacatttttattagaaaaacatgaaccgttggatcaagatgtgtgttttcttttctttttctttttattttttttgggttttggtggggttttggtggatcatggtggatcaattcgtagctttagcaacctattattatatggagggaaagggcgtattaatctgttagcgccgtccgggagtttagctttcttccccgagcctcggtcttatcccctaactccaaaaccctagcccaaaggtaatccactccttccccctccgctcttcatctttttctattcatcatctttaatctgttctcccttttggttcttagattcttcttttgttggattcttttaatctttactcatggttggccttgtaagtttagacgacgtttttatacattggttaatcctgcttctctatctattcgcacgctagggttttcctattgttttctattctgctctacttctgcaaggttgtgttcttcttcgttcaggtccctttttttaaccgaaattaaattaatgcaaattcgtttgtgcttctaattaggaagccttttggaacatctcgacattttgattgctgcatttcatttcgggtatatttctatgattgaaggatgtgggtctgttcactgcatggtcattacttatgcagctatgcttatcgagtccattatgtttgtgcaatctgtttccggattcataattttttagtaattgatcagtagatgaaaaaagatattgtaatattccttgagtgttgcaccagtcttggtgggtatctgctcctgctctttgcttgtggattttacttttattatatctgtattattcgaaatgttctgttcttgttataacttatacccgaagatgtgttcctccccgcgtctagcgttgtgggttacttatgatggacatggttttgattctgtttggtttgtgcag

SEQ ID NO: 54 - DNA, 1547 bp, Cucumis melo
  misc_feature 1..1547: note = n=g, a, t or c.
  unsure 1..1547: note = unsure at all n locations
  source 1..1547: mol_type = other DNA
ataatgtgttgatgttgatgatcatgcatggtatattaatctcatgattaaagacgttaagattaatattcattccatgtttatgatgggtgttcttagggttgtacccatatgggtgtccctcgggatcaccaccttttttatgactgtatggttctacgagaccaccagtctgtcatgatatgtttatgaatggtacgacggggtcacttacagcccaattgcttaagtgttccttcgggttcactgaagacctatttttcctaggttttcctttgacttcagcaaaaatcagttttgtcctaggtgttcctcgagttcactgaagactagttttgtcctaagtgttcctttaggtttatcgaagatcagatgtgttcctacagaatcattagattgcaagtgttcgggaacacatcggtttaggggtacttctttacatgaaccctaatggaaaattaacagacatctagcggaattagtagttggtcccttactgagtatatatttatactcactctttttatgtttaatatttcaggcaaaggttaaggtagaggaaagttgacgagtgatagaaaaggatctgtgacatgtcatatggggactcagtttcgtttctgcttctatgtatcagtgtttcagtattttgtttnntaatgaaaatttagtcttcctctattcaagaaagtgtctcttgttattgtttatttttagtaatgatttcaacttagtataaatagttggatcattacaaataatatattggtgatatactttgtaatgatacattgagttatattattcatatgtttaatatacaaaactgcaatattaaaaaatgaaaatcacgtaataagtatatcaacaaaataatacatatattacaagcacgtcacaacactaatatacaaaactaatataaagtaagatcaaagcaaaaccaacgtaaaaaataaaacaaaatcatttgaaattaaatttaactcaaaatacacatcgaagaaagtggagaaaaatcacaatagagttaaattactttgattaataaccattatatttcatattgaaaataatatgtcattagtattttaaaatcaagattaagataggaagaatgaattgctcttttcgtataaaaagggatgattggggccttacgaaaggagaaaaatacatatgttatcgaaaaaacaaattatttttcttgtaagagagaatgattatatccttaaaaaaatgaaagaaagaaacaatcatggcattaaaaaggaaaataaataaattattaaagggcagttcgataataataacaaattcaacgagagtattaaaagaaaatgagaatttgcaaaatttaaacaaatgtgtatattaagtacagccaatgcaattttcaaattttaatttatttggtttacccaaaattcaatttctaaattgagaggaggatatagtaaattcacacgcattatccccttcgagtttcatcatctcacccattcttgcatacagtgcagttacaattccttcattctggatagaca

SEQ ID NO: 55 - DNA, 2000 bp, Cucumis melo
  source 1..2000: mol_type = other DNA
aaacacttatcatgttatgtatcccacatcgaaaagataaaagagacttcatgatctttacatgatatatgagttactccttcgactaccattggttttggagatggattcaacccaataatatgaatctgacccaacaatggtcaactcaaagagacaccatcttgagatacatgttgtgtacccatattagatgaatgactatacctcgcaatatttataacatacatgaattacttctcttactgtaatttggttttgacgtggagcccatgattatctaattaaccataactggtatatgatatattagtaggtaacccgaagaggttctaagataaacacagaattcaatagaatcagagcctttccaatgatatggctttagatgggaatgatttgaagtataatcattctaccacaccctttatatttgtctgtcaccagaaatctcatcttttcttgaggtattattcactcgaaaagagggaggcatttttgggttacccatctaatgcacgatgaactaagggaggtcaagttctgggaatacagctaggcaaccttcacagtggatacattcgaacaaatgataaatgtgaaaatgaatcatttcatgagtgtgactaacccaatcattcctccttctatatctttgaatcccacagtgagtcagagtaaaagttccagcaacaagtcctacaacccaaattctttagctatttcttccaccagaacaaaaccaagcaaaaaatcagccacaaacacagctcaacaatctataaaggccaaaatactaagacagtcaccattaccacattgaaagccgtattttccaacagactttgcctgcaaaatagatcacaaagacacgatttcacattggacagacgccacagctccacaatctcaatttcaatcaaataaaagtaaatcaaagctaaatagcaagtgtatggtaccacgaaagcagcatggctgacgccactgaggcctgtaagagagaaaacaaaataagtgtagaagataaagtgaaatagaaaaatcaatcgataagatagattttcagattaccatttttacgggaattgtacggacccaaacacaaaccccatagagcgccggcctgaagatgaacaggggcaggaaattcagaggaagaaattaaagaaaatgaatcatagtttgagaaattattcgtaaagtttaccgttccgacgcgaatgctggattcgacggcgagggaagaacaaggaacgacgccgttgagttcgtcttccatcttccaattctcaatttccttcggaggtccgtatgctgagagctctgtgtctaccaagttccaaccatactacgtcgttttggatttttatttttattttctttcctctcttttgccaaaaaagaaaaaaatagtattccaacctaaaacctcaaaataacatatttgttgtacaaattataattagtaaacatttgtcattgtgagcttggtatgtaatattaacacgaactttatcgctaataatttagacgttaatgaataatttgagcattgccttcttatattgttattgtgtttataataggattgcttacaatgtaacctagtatgttgttgagctcgttaacttttttgtttttcttgaatattcaaagttaaaaaattgtacaagtttttggtgacgttttcttactacattatcgggatgaagatcaaatatagcttagattagagaagataatcatgttgatttatcgttaaactttgactacaaaatccgtttaatttttttttggatgaattagttatacaatttaaacttaaaaggggtgaatgaagaaagaggatagttttacaaattcgaagtgaaatgagttatttctgcttaaagaaaacaaatctccttcgtgctttaaaacacaaactcaaaaccctaaattcagcgccgattcttcaatacatctctgcaggaagttagggcaaagcagaagcaaaa

SEQ ID NO: 56 - DNA, 2000 bp, Cucumis melo
  source 1..2000: mol_type = other DNA
acttccaaaaatcagcctcatgggatatttaaagaaaacgtaaattaaaattagcatcatttcatattgaacaaactacaaaaattaactctaaaagatgatggtaactacaactaaaccttcaatttttcattgtaaaaatcgaactcttaaacttgttcaaatattaaaatttgaccctcaaacttaaaagagctaaaaaaagaccttcaaatagtaaaagtagaactctcaagcttatagaattattacggttatgattatagccatagatgattcaatcgattttcctccaagatgatggagtataattcttcaaatctagctgcttagatgttatcacgataatgaaatcatatgggaactcaacaaaaagaaagcacttaatgttgaaagacattattctttgggtgttgagttgggcgaacttgatttttattattaatccgcaaaggaccttttgagtaagttgtggcaatctttattggagtgctaagatttgttattcgaaatttcttgttttgatatttttccaactaaaactaatttttttaagaaatgcaccttcaactgatttcatgcgtgtccttttgcaagactcgcatgggacataacacatcatcttatatggcaaggcctatgtgtcagtggagatttgacgtcaatttctttccactgagagtcgtcctctttgtgatggcagaactttggagagtcatcaaaattggttctttgaaaatgtttcttattttgatttttttttttgaaagaaatgagaggaataagatatttttacgaggactctactagtgggtcaatttgcccgcatatggatatgcataagagtccttttggagagaaagggtatgatggaaagacattgcaaaggcccgtccactaactttctattatacaattaggtggaagccacccatagcaatgtcttggttgaacactgatattacttgaaaccatgcatttaagatgtgaaatctcgactagatgctttaggaatttggattgtgtctgttttgttgaattcaagttcattcctaaataccatgaagttaagatccttgaagcaatgaagaccatttatttagatccttaattcaaatctctttactaaagatgattgtttataaatgatcaatttgttgaatgatgttctacttgatatctctaaagcatctcttttcggtgagaagcccacaacttgaatagtattccataaatcatctatttttagtttctatcatgttctttaacatcaaaacattttagcgcactctcttataactaagacttagaaaaacacgaatcttcctttcttacgatatatatcctaaatggttttctatatttgtgccttacaatataatcaattctttttctatttgatattgtcataaaataatactgataacatagtttttatgttttattaacacctaacaagaaatatggaagacgttaatatatcttcaatgtcgatattgaatcattttatttatgaatatatccacgcgtcaaaaaatattttaatcattaacttctaggactaaattcaaacattcttggaaccatagacaaaagaacaaaatttgcaacctcaacaaacaaaattttatctttacatttgcggctacaattcacaaattcccaaaccatgatagaaaggccccaatctcccacgtgataaacacacatatggcacgtgaccaaatcaaaatcatccacatgatgaaaacttaatggacagctcggatcccaacacccaataaaaagcagccatgaagctgacgtggcagatttccccgaaaaccttttaaataataaacaataaaaaaatatatacataaccgttggcaacgtttttccctccacacattttcccattgccttatctttctttccctccaaacagcgagggaagaagaatccaatcatcttcttccaataatttctaaaacgaaattctgctcgattttccctctcca

SEQ ID NO: 57 - DNA, 2000 bp, Cucumis melo
  source 1..2000: mol_type = other DNA
tgggtaacattatgagttttattataatttaaatgaagatcaaactttaagttgtagggtcaccataggaataaaatataatcaataagttagggccccttagtcccacctcgtaaaggagttctgtcatacatatacattatgatattaattctatctccatgagtcatacatgtgattttagtacttgtaattttcattctttttcctattataattcattcaagtactgtcaatatggttaggtattgaaattaattatagactcagatatcatcttcattaatggaaatggaatgttatattctacctctcatttttacacgttgatgataaattagaagaaaaaaaattattatttatattgttttaattgtgagatattagttcaaaatgtaattaataaaatgatacgtgtcttataataaaattaaacaagtataattaaatataaaacaacatacacactctttaactaaaagacacaactcacctaatgctcgacttaaaatcactttgtgtcgtaacttaaccatcaaagcatgttagggtaaacacaataaagatgatttttgagttatgcatgtcatataatgtcacttccaatttgacttatcttgcttgcttgattcatgtatataaacaaaaacatgaaaagtagtgtaaggataccaattacctactgattttttttaaaagtagtttgtctaagacgtgttaaattactaacttagtcacatttgagttttagttctaacttattaaacataaagtaggtatctcccttactcatgtgtgtttcgataatgtcaaattccaatgtttgattaaccaaattgggtaatttaacataaatattcataatataatattttttatggaataccgacatctaaaaagaaatcaaaatgaatattattaggaggtgagtttttaagagagaggaaaataataaaatatggcatcaacaagaacaataataataagaatagaaatccgacaaaggaagaagtggatgcgtgttagtactattgacattggcatatgaacggttgggttgggcctcaaataatttgcatttctaacttccaaacacctaattcctttttttttatccatacttgcaaatatatatttatatatattcaacaagtagtttaatttatttgatataccactttaagttttaaattgatggtagtgtataaataaataatttaggattaagcatgtctatgaaccttttgaaatttgatggagtatatataaaacagaatactcatgggttcattataaaaatctaatagtaaatgtattttttatttcatttaaacattttcaaacttttaaaaattaaaattatcttaaaaaacacgtgtggtttcgaaccatatggttaaaaatattgaggttctctattttgcaaaaaatttggaaaccttcatggaagttgatataaattgttgtaattagttagtattttttctttatttgtggcttaatcatgctatgattgatcattttatcatcatttctataatgtaaaacaatatatttgatgtgtattgtaaatttttatgcaagagtagaaaattaataaaaaaaaaagagagaaaaataattataaagtaatataaagctattaacattttaagaaaaataatagtgaaaatgaaagtttcggacaataattcaataaagaaatttgtagatttcgattaaaatttccaaaattaagattttcattaacacgtgtgcctcgcaaccgtctcctacgttatcccgtaagtagcccaatctatcccattcttacacaagccgtcggcccaaattgattgtaggccatcggcccactcaacacccacaaaccctagccccttgctcctcctcctcctcttttcacggctgctcactccctctctttttacaccttctccttctccttctccgtccctcttcccttttctgctactatcttcagcacttgctgagcttcaacc

SEQ ID NO: 58 - DNA, 1591 bp, Cucumis melo
  misc_feature 1..1591: note = n=g, a, t or c.
  unsure 1..1591: note = unsure at all n locations
  source 1..1591: mol_type = other DNA
aatgttgatttacccttgctttgtttgaatttcgtcctcgtggacttgacctttggtctgcttcgtataggactatttacggctgccctcatagtccaagtccttgtccgccttaccctatactctctatctctagacaatgtgaagcgggcccttctataatattgggccttgaagttttgggctttggatctgccgaattgtgttgggtttctctcccaatttatttcatttctttattcaaataattataaatatggaattttattttatttaaaatataaaagttaaaattgaacgaatccaaaaataatggaatcaaatcgacgttttaacatatttttcaattatgtttttacattcattttcgtcctacaaaaatattcccacctttatttcctcgatatcggaggtcactttgtatgtttcattcgggtgatgtgatatagatcgagtttctatgcttgattgactatggaaatatattttaagaagatgttataaaagtaaaataaatgttttgattgtggatataattatattttaaacaagatgaggaataattagatccgaaccaataatcttgagtcaagagtgtacattgaaagtcgtatattaaataatggttgagtttataataatattgatagattgcagttaaccatattttctcaagttgttgaccaaagtacttattttataaacagtttagggaatgtttatgaagttttgccaagtgttttgaacctatatgagtattgacttaattggtatataagtgcattaacaatcaagaggtatttaatttgaatcgtcctacccctatcatgccaacaaaacaattatatgtttgtcatattttattgaaagtgttttcagcgcaatttagtttgatttgcgtacaaaacatgtctacacgtatcgagttagtagtaatggttgctagttaagactgtgaactaaaactttaaatttacattaaaaanaaaaacattatggtcgtttggtcctcatatgtgattgatagatattgattaatgagtatttgtggttgttgccaacaataaagatgtagacaagtgaactatgttggttgtcaaatcttgtttgtatttgttatgtgtggttttcaccaccaatgttgtagagtgtcagatccagaatagcttgatcatttttcatatatatctacagactcaattagtagataaaaactataagactttgacttatttctcttaaaatgtctcctcgttctgtacaatcctcaacaacgtttggtgactttaaaacatcacaagaatctaagaagaatgatgaattagatgcaatgcaaagatttggaccttaattttgttactttaaactttatatccgaacattggaagaggcaagcaaaaagcgcgctttagaatcgcggtttctttgggccgagtgggttgctcataacagcggaggtttgcttttctgccaagaaaacccctcaaagaaaaagggcttaataagcagctgctccatttctaagtgggtttagcctttagcacggaagcgccaattcgattcaactctgatacactgcaaaaattccgcc

SEQ ID NO: 59 - DNA, 2000 bp, Cucumis melo
  source 1..2000: mol_type = other DNA
aaagaatggagcaagctgatattgctaagcaaaagcttctgcatgattgtgaagttcttcaccaccgccttcaagattctactgtcgactttttcattgagcaggaaaataaactaattttggaaactgcttcgacagctgacgacgcaatagatctgttggcaacatctgataatcacattaaccttcttttagcagaggtacttgcgtttgtttccattgaaatgcatttgcatattgaacttcttcatcctgaatggcacaagtttttgtccatacaaacaggcaaagcttctggctcatgatgctaacaacagcgatgacactgctggatcagcccgtccaaatggaactgataaaggggcagctgaccaagtattaagtaacatactagcaaatatgcttgtcgaaaatgcccgattaaggatgcagatgaacgccgtcatccgctgtgttctaaatgcaaatgggacaagtgagaaagatgaagatgaatctctcaaggaagaactgttctaagcaagtttttagaggaagagattcctgaatgcacatatacaatgaccttatactgtcgtggcaagaaatgggagagctgtagattttgaataaatgcaacagatgttgcccattaatttgcaagtcctgacaaatttggttgtcggaggtgtagaaatgatgtatcaattaaatatttaacaaagtgccttttggcttggctaatcatgggcatttgaagactttgcacttggtaagagctcaaacaaaatctgggtggctaaatttagtgttgattaaatggaatttcactgatattcatgatctgtctcttcttccttcattgatatattatcttctcagtaaactcctgggcctgatgcagaattgcttttaaccatctgcatacagagaagaagtaaaaactagctcacgtggataaagggaaatttctactgacatgttggcattagaagaaaattttgaaagagttctattaccataacatcatctacttccgtgtattattgaaactattatttctcttacccggagatattaaattaataaatttctatttacattttgaagatgctcgtgattattgataaaaatgatgaatcattattttgattacgttacaaaaaagtcaaagagagtaacaaagctatcaacaaaatattagtaatatatacaaaaaaagtgtaaatttaatattaacactgagaaatatacacttaagctaatgggttaaaatatttatccattgaattaaatatggtttttctgtatttgtgatattccaataaatatgaagctgttatactgtcaaattcatattctgcctatacaatcaatttcaagtcactcaattttgcaaaaccatatcatattgagttcaaataaaatttcatatctatatacataacgaaaatgttatgtttttgcttttaatgttttgggtatctttctaagctacaagaaaatgtaaaaatgataataagaaatagattatattaaaattattttacaaatcaaattgcggggatagctcagttgggagagcgtcagactgaagatctgaaggtcgcgtgttcgatccacgctcaccgcaaatttttttcttcttttttttcccttgtgtatcattttaaatgggctgttcttactttgaactgcggaagcccatgaaagctaggcccaatttagaaaccgaccatctcaagggtcggttcgtcatttatcaagatccgataacccgattcgctccattttagtctctgctctttcatctccctcacccattctcgcttccactgagcgggcaagggagcttaacccctcaaagccctagaaaccgccattggagaagctccactagcttcttcttctatcagcgaacgtattttcgtcttgtatagacctttcatctctggaaccgatcggaagtttggagtttcttggtctcagtttgtagattagttttatcttggcgtctcaat

SEQ ID NO: 60 - DNA, 2000 bp, Cucumis melo
  source 1..2000: mol_type = other DNA
gtgcatttaaaataatctagttgcatgttctaggttcgatttattatttggggatttagttgtgtctgtatgattgaaaaaattaatgttgatcttgtaacacaattgtttttccctcgatgatttgagattatttcaacaatttagatccaatgtttaaaaagccaccttggcatcttgccttcctcattcgcaacctgcctccagttgaagcctcgaggctcaaagcccagtgccctaggacttctttattaattttacttaaaaataaagtttgtatccctaaatgcataaaatacccttgtgtttaaggctttctgtttcttcgcgtttcacgtcaggtcagaccatgctcagctatttttccaccattcttcttcttctctcccaaagtctatcaagtattttatttccacacatatattcacctacgccaatttctttttaaaattttatagatatatacagtgcacctcacgaaaacaaagtttgcacttcttcagttttttgtttcgcctcacacttaagctacaaaaggttattacgttttagtaacccactactcagctttaaaaacactatttgtatcatatgacgtcgcccttatggaataatttcacttgattatcgggttgtttcataaacaatcttactctgttgtacctttgacaggcctggagagcatgcaactcctctcttgcttgagtttgagtaacaataaaatcggaaattttactgcattggagcctctgagactgataaaattcttaaaagttttggatatatcgtacaacgagataggttcgcattcgatcgacacaaccagatatctcttctcatctccactgtcgcattccgaagaaattgatttgagcagtgatgaaatggcaacaaattttactgatatggcaagttactgggaagcatattttctattcaaagatataagcttgatgcaattggatatagaaggaaacacaatatctagtgaaagtttcaaagcatttctggtaaagattcttcccaaactccactggcttgatgggaaacgggtacaatagatatggcttaatttatctacatccaatcctctgtccattgtggttgttcatcccctgaatgtaaaaaggtacgctacgaactagcattgatcctaaattgaagacattggttttgatttcttcccaatgcaaggttaagaactaaggatttgatattgcatccaataagcataggttatttaagattttggtgatagtgaaaattaggtgacatgtctcgaaagcttaaagggatacatgaggtatggagatggagatggatgtggttacaacatggaaatgaatacggtgcccagttttttggactgctctaaatcaaattttatcatatacattatgatactgtgtgccaattgtatttaaaaaggtactgaactttacatttttgttgtcccaaattttgaaggattgtagttttaataattcttataataactatcaatgttaattaaaaacttcagtatatttacaatttttctaaaaatgtttgctatacgtttagttattatcttgatcaattgccccaagagaaaaattaccctggactatttcccaaaaacatcttctagtcgtccatcagctatagtttcaaatctgtgtgggcccagtcggcccagttcattgggcctgagaatagagatcatgaaccggacggcccaaacctttttcaggccccagccaagcctggcctacaaacttctaacctaaaaccttatccgttgaagcaatccaataaaacaaagccacgtaagcacccaggatctaaaaatgtatccaaatccaccaatctgaggccacaaatttagcctctgtggctgaatggatgtcgaattacaagaatctctcgatttcttcctcttaaatccatttacccttcaaacaaataaacacaaaataaagaaaaggagaagaaacaattgtcgtaattagcagcaagaa

SEQ ID NO: 61 - DNA, 2000 bp, Cucumis melo
  source 1..2000: mol_type = other DNA
acctagaacttctaaacgataatctcggaaaaaaaattggaacaaatcataataatgacaattaagaagcaagaaccgttgacaaaagcaagatttagagggagtaaatttgcatggtttggtgatgattatttagttgaatttagcctactcttaggaagtatccaataatcatacgcaaatttcacgtagcatatgaagcaagtgcatcataataccgcataacctgcggggttttgtcatctcgattaaacacaatgtgaacatgatgatgtctatgtgtttccagcttttgttctaatgatgatagacgatagtgtggtatagttcatatccttgatttaattgtttccatgtatactatcgaatttttaatatataattaatgtatgaaatcaaatatcaaataatgattgtgatttaatggaataagatcatgtctaaaattggtaatagtaataacgaagaaggaagagaataataaactacgatttcttgtgaatctcctagataaattaggataaaaactacgagtaagaatagaataattatactatataaaataggagttacaaattttgtttcttaaaataccaagctctgttacaagaaaaaactttaggtattatatcttcaacattttgttaatttgttagagattttaggatagtttgtcaactatgggtcttctaagaaacttggtcatcaagcaaatctaatgactcgaattgtccttgatcgatgtgaaagatccaatgacttcgaattatctttatgcaatgtgtaagatctaattgtcataaattgatctcatgtgcaaagtgtaagatccaatgatccaaaattgtctccaacaacttcttgaacaataagataactctttgaagaatcttgaatattaattttgacatagatagattgatcttgaatattaggaaataaggaaattttcttatgtacatgcctgaactccttcaacatagcattttgaatcatatctcttctctagtaacttgtatagttgcaatatattttgcttctgttgttgatatatcaacactgattgaagttttgaaacccaacatatagctctagtggcaagagttaagacatatatgtggtgaatttacttctatcaagatcacaatctaagcagatatactttgaaaataaagttagattatccattatacaatgtaatatttacggaccatttaactcgcttagaaattagagttattttgcaaactttattgacaaatatcttcaaaaatttcatacaccgtatagacactatcataagatgttaaagaaaaaaaaaaggtgaattttccatacaattaaaaaaaatcttaaactataaaggtggtttcgatacctttaaactttgaaaagtttcattttaattctcgcacttattgttttaaaacaaacttagtaaaattttcgtataaatttagaaagaaattttatatttacaggtggggaaaattctaaacacatagatgaagataaataaaaacacgatcaactataaactatacctattattaccttcatccttaacaccatgcactcaaatattcattaattctctatatttttttctatcttagcctcaaaatttactttcatcctaaacttcgagccctcaaatttgcgttatttcattcacgatattccttttttacgttctttcatttatggtattcttctttacgttcttctatttacgatattcttcttgcttttatagtgttttagatttgttcataaacaacgtataaattgaaaactttataaatttagggcattaaggtataattgaaattaaaaccatatttatagtcattaaccacagtattatttatcctttatttattaaaaaaaaaatctacttttagttttaaatttaggcattttacgcaaagctaattacgacataaaacaccaaaaggagaccccgttcgatcttcacatcttctcggccagaaacgacc

SEQ ID NO: 62 - DNA, 2000 bp, Cucumis melo
  source 1..2000: mol_type = other DNA
gcaatggcggaaataacgtagcagagggcacaaacaacgaagaggagcttcgttcttcggtgcgccatctgggaaagtgagaaatggtggacgaaacacaaacgggggaatcggattggatctctcagaaaagaaatggttggattcgatcacagatcaatgaagcacattactcggtttttcaagaagattacaagaacttgcttcttgaaacctctcttcttctgtttgaaatttttgggcgtagaattgaggaccggagcagtcgcctgaatttggtcgtcgaatcgattccacggaaacaaaaatatgaagaaaccaaatgaatgacttagcccactcactacgcttggcgacgtgttcttcttacgaacggaccaatcaaatgcgagcctgatgaatatgggccaatcatattatgccacgtaagactttacttttgcccctgacctatgggaagaaaattgtggtcttttcttatgtcaatagaagaaaaataaaattatatgaaagtcttaaaaggaaaaaaacaaaccatgttaatattactgtttaaaaccataacacaaaatcaattattgtttatgttttgagactcccttatggtgtttgctagatagtgtggattttgtttttgaaaattgtttttgaattttgttattcttaagtttttttatccgaaaatttcattctagaaaacaaaattatataaaaccattttaaaacataatatatcgtgttatagttttttaatgtaacgggattacacggcctattatcaattatataataagatagattaaataaacaaaaatgatttatatggcttttttaaaaataaaatttaatctctaccgcttataactataattaagtcattttggtttaataaaatcatattatatagtctcactcgtatgtattatttacaaaagatgtcgactttttatcaaattatagactaaactataattttcttcgaggctaaaattataatttaaccaaatttataaatgtaaaatgtatttataaataaacgaataatagcttgtcgtcaactatattttagtggataagtaagattagttttatgatttataaatatatagtataaaacacatttaaacatgttttgttcattgcgtttggttgatatttaaacctagtaacgaaaaagtattaggtattacattaaattagcatccacctacaatgttaaatttttaagtcagttaataatttaagagactctcttcaacattgacttcatgcaacataaaatggtagaaattttcacaccattgtttatcgacattactacgtaggagaatggcaaaactttcttatatgtatgtgtgcttttagatgtgtctttacatcccttatcaaaacgaaaacctaattctaaccaaatcaaaccaacccgggttgttgggttattcttacaagccatttgttggattaaaaaaccaaaatagaggatgttcggttcaagcattttaaagttttgggctatttagttcgaccactggtttgttcaaagtcgggtcggaccaaaccgtgagcgatgtaaacaacaaaggtctaaattgggccgggatcagatgggctgaagatccacgattctggtttccaacccaaggcccaatgaattacaacaaaaaagcgtactcaggaaatccgaatctggatctcaacgtactctaacctctcacagttcgccacgtcaagaaaacacgtcaatactttaggcgaaaatcaagtgaagaattccccacaataaggaatcgtatatccacgaaactatccaatcagcttacgccatcggaagattcggaacaaagcaacagttcaatggtatatcatagggtgagaataagtcggttccgcagactagtatttcttagtcaaactttacctgcttcaatcggccgccgatttcccgatatttacaacatttagttccgatttttccctcgaagctctgaagtatcgtaaaa

SEQ ID NO: 63 - DNA, 2000 bp, Cucumis melo
  source 1..2000: mol_type = other DNA
gatcaaccttgaaattttcccacatactgtgttgtaaagttgtccccaatttcattcacaaattacctacttgaggaatcggcagtaagaagagatcataatgtatttttgctactacactcgcaagtctaatcagaggatttgattacaatatcttgctgctgtaatagattcgttcataaattaatccagattgaaaagtcaagctttacttcattttcatcgacaatgtagaaattttgtttataactttgtactattgaatctattgctcctcgatttgcccccttggtacgatatcaagccattatttttccaactcttactcgcaacttcaacgcatgaacttgaccagcttcaacctataatcttatgcatgtttttaatgattaaagctgaaatagattgtgaaacgtaccttattctcactaccgctgccaaagccaaccaagcttccacgggtacccataaggtccacaatcatggcactcttggatgacatgtattggttcctactgtctcttccgggttctcttattaatggccccgaaagcaacctctcccggcattctcgaaattcggctcactaatattctttagctactaaaacacatgtcctcaaatttctcatttaaatgtgatctgagaaagtcattcgacccattttagtttaaataagcatcaagtcaaaaaccatttaacgtgggcttaaaaatttacagcagcgcagcgtacactaaagtttatgaacgatgaaagtgggtggcagaagaaagcaagaagtccgagagacatgccaaaaagagtaaaagtcatttgttggggccttgacagcaaggttccatatgcatcggtccattgcagcatggcggctcaaaattaaattttcacccttgcttttgcttctctaacctacccttctacgcatcgtgtctatcttccttcacactcattttgtggtaagctttaacgcaacattttcttaatgtaatttaagcttggcccaccaatccctttgaaaagtttcctctagatggtgcgtgtcaatttcaaattaacaatttgaacttatagttctaacccccatattgtctgccctttttctcttcttcttcttcttcttctagttttgttctggtttaatctttttcggttttctctgtgcagggtagtagcttttaagcttagtgattttctcttgttaacaactctaagcagtgaattgttagagacctattatttcatataaatactagatgacttcgactcattgattaggctggaagctgtcaaaattaaagagtttgacaaatacccactaatttggtaaccaagagccagcaggaacatttgtatttattgagacaagtgaaagtttgttattttctttactcaaaatctctctttaattttatagatatagacattacttggataagaaagggagttcaccggccggaggttttccttcaaatttaacagtgactgaggtctctttcagctttgtttttttggtgttattactgtttgctcaatcctttgaacgagtggtgtaacttgttaaatgcccacaaattcatgggacgcaatcctttaggagaaaggttggccactagttattggtggttaccgtggctcttagcaacttagcatcagaatttgtcttgaacttctagtcgttgaaaattctcttcatacaaagctaagtctgcttatttgtaggatccataaacatgagatgataagggtgatgggcctaagaatgcttgatggaaacatggtcattggacttgcttattaattgaaaaaaccagccccgtctctggttagaaccctcattaggattgtattgtttcaattctttcagcttgttctggattttaaaggctccaatggtttgagatgatagtcatggaggtgggaaggaatggacaatacagttttgaagaactgggttatctcaaatgggaaggtgaaatgtttatgtcagtatttgcttg

SEQ ID NO: 64 - DNA, 2000 bp, Cucumis melo
  source 1..2000: mol_type = other DNA
atcttcaccgttaaatcgccgtggttgttagcggcggcgaggagagagagtgctctttctctgagaactcctgccatagtagacctaaaggaagaaagtggtagtgaaacaaggaatggtgaggagggtgagaattgaggaagtggttagggctttgaaggaacggggaattttatttccgggaagggaaacaacaggggagaacacagccggagcggtgtggttgtgagaaaatttaagcaagcagatgagacgacggcctggcgccgaggacaggcatatgaatatcacgtggctatggctatgggaaattgaacgtaggccctttctcattcttataccaatcttcatttttctattttctagggtttcttttctttcttttttctttttcctttttcacatttttatatgtcattgaatttcgaagtttggagttaatatgttggagtcgtgtatctatttagcttcatgggttataacattattttggatgatgtatgatatttaatctcaatttaagaaggaaacgagtaaccaaaaaatcttataatgaggtttgtccatcttttatgtattattctccacttatcacatttgtttgaaataaataaataaataaatgttgtgtcacctcaaacacaaccatatggttcaaattgaaatttaacacttgatggtccctatgttccatacgacctaacaaggtcatcttttgattgtgaggttcatccaacataaagttgttataaactaagaatatttcacttatgagtgtttatgtgcacgttgttggtataggccataattttcaatcatttaaaacttttattaaccatgatttcacattatcttgatctctcccattcgaatatgattttggttcatctatattccccttataaactcaacgttacgtgcctaccagttttcgcttggctcatccccaacccatatcttactgtggaatgttttttctctgataccatttgtattgtttcacaccttcgaatcatattttagaatgttgatacagtacctaatgcatgtgatattcccctccatttgttgtgacatggcagcatttgttcttacttgtgtttgaattgttttctaagagaaaaaaatgatatctccacaaaccaacgcacatcattttagcatatcatgtgtctcattcacgtggttcttaaaaaaaaatcaggacattatccaataagacgtggtcaagggatgaaccaaatgaaaattaaaagggcatgtaatggccgagttcatgaatgcgtcataaatgaatcaatatcacactaaaataagaccgatcacaagggtgtgaaagcatagttaacaataatataaaaaaaactaaaagctcatatctatgccaacaacatacacattattttcgattgcttaatcgtatgaactttaaagttaaacgtgtttattttaaagttaaacgtgcttatcttaaaacaatcttatgttggacgacctccacaattttttccattacgcatgtgagaaacacattgaaaggactcgaattagcatgtagagaatggtgtagcccccattctataaaagcaactcaagatctgaacatgcattgaaatttcactcttcattcctgacacatacataaagagaagcaagtacgagaatcatcctctactttttattcacaagttttaagtcaaatttcaacttgatttgtatgtttcaaaacgacacacctactcatttaatcttgagcgttacttcaattgtttttatgtttcaaaatgttaaaaaagaaaaaaaaaaaaagttcaatagttttgtaaattgcaaaaaaagagaattacgagtatgcccctgtacatttagaagaagcgtaaggtccatatgggaatcagaacaatcaatcgacggccacatctcacgagacataaacagggggagttggaggaatcgacggagatcggaatctggtttagggttttagcaaaagaagaaca

SEQ ID NO: 65 - DNA, 2000 bp, Cucumis melo
  source 1..2000: mol_type = other DNA
aactcagtgaatacgataagaaatttaattgaagttaacaaactcaaacttaaatattttttaacacggacaatttaaaaccaaattcatagtctccttgtatagtgtttagagtgtgtcgcttcattaaacctttctatcgtggaacaaatctcttctaatattttgtcaaaaacctatcatcacccaaaatatcatgataattatttgatgaggatcaaggcttagagaggaacaagggaacttttcacaagggtggagagatttagctattaggtttaactcgttgcttctaatggtggatgaataacgacaaattttaaacaatgaacgttatcacgttgaaactatctacttctctcaacctactactttatcataaggtttgaaaagttctatcgaaaattttaaatacataaaacataaaaaggaaaattttcattggagaattttccatatatgtttacccacaaaactaaggctaattaaaaagctaaccttaagactaaggctaaaatggtatcttatgctacatttttcagttgctatgttttgaagcaaaagctaattatttgctaataatgagataggcatgtgggtgagtgatgagcttagcctggcctgcctttgtgtttcttcttattctcttaaatatcattgttcaatcaaaatagttttgttaaatttagcccatcctcacttcaacctcttatatttggattggccttctttgttttttgggcttttgatatttgatgtaatggacttcaatcatttatagaagccttaccctacagaaacaaacaaacaaaaagaggaaaaaaaaaatggtgagttggttaataacaactttctaactcaaccaatatatggtgtgtgtatatatatatatatatcgaatacaaaatatgaatatgatatgaccacataaaattgttgaaagggttgaaaattagtgaattggacttttaaattttgtagtgtagtggtttacctatgatgctcgtaatgttatttaattttaaatgtgttttttttttttacaaaaaaaagtctcgcggtgcaagttcaataagttgatttaaaaacaaatccatcaaaataatgttcgcttgatatgatcgagtatagagccgaatgtgtatcaaacataaattcaaactttaatagagtgaaaaataaatgctacgcaaacaaagtttttgtattagcttcttaaatgtacatatatacttttccgattcaaacacctccaaaataaaactcaaaagttaaaatttagactcagaaaatgagagaaaaagaaaactaaaaacgaattctaaagataagcattttcaaatataggaaaatgaacaataaatatttacaaaatagaagaattgtaaaaaacgacaaattgacataatacttacaaaacataacaaaatttcagattctatcaatgacatacactgatatatctttattagtcatagaaagtctatcatttataaaatccaaatttttgttatatattgtaaatatttaaatttgttttaccatatttaaaaattttagatttatcaccaacaaataaccatagatttcaaattttgctataaatatttttaaccgtttatttaccataatttttctattataaaaacaaaaaaaacaaaaaacagataaaagcgaagaaaaagtaagagagcagaaatattttttgatttaggtttcatttggtaaaaaattgttattaaaaaatacaaactaatgggaaacaataataataatttaatttttttaaaatctaaaaagaaaatagttgacaacaataatttaataatttaatacacaagccagtgttattaatctctttttttctaacaacgcctttcacgagacatcctctcaatcctcgacatccagtggaaaaacagtatccctcaaccctcagctttccccaaccgccctccgtcgttcttctgatcgtcgccaccctactccgtcatcggaaa

SEQ ID NO: 66 - DNA, 2000 bp, Cucumis melo
  source 1..2000: mol_type = other DNA
catatatttattatgttccacttgataaccattttgtttttgaaaattaagtttaaagacgacactaattccatcttcaactttcttcttttgttatcaacattcgaccaatagtccagaaaaccaattaagttgttgaaaactaaaaaaaaaaaaaattcttataaagttgttttttttttaaatttggttaaaaattttaatcattatacttaaaaaatatatacacgaatcatagtagaaaattgaaaacaaataaacttaattccaaatctactttaaaggctcactatctgtcaagaggctttggtatagttgtctgtactgattaagtgtgagagttcttttaatatttgtagctgaccaataaattctttcctttctttctaattttgctttaactccctatcctattcatacacaataaatatacaccatattctaattgacaatattgtttggatttgtttgttttctttacggtaggcaagaagttgcctagttgttgtctgacctcaaaaccctttgttgataagagcaaacaaagtctagttttccaaaaaaaaaatcaccaactcaaccaaatcttgagccttttactaatttccatcccaaactaatatctaatcagtgcttacatgtttgagccttcaactcaatttaacatcaaaacatcttgcaaccacaccttgacatgagtatgaaaacaatataggagagaactttagtattacattgagttccattatcattgtacattctcaaccaacgaaaccaacccaaaacaaaatagttttttgtaacatatgagattaggtatcgtcctagttaatgattttacaaagttatatgagtattcatttgttgatatagtttgaccggatcggacagttggctacaatggtatatttctataaactaaggtatacaatttttcatgtatgttgtttgatattgttttattattggcacatgtcttttgtgtccaatagtaataacaaggttgtttcttatctaaataaaataaactcttgccagataattgaagttagacttttaatcaaaacgtaatattaaatggggatgagaaataattgattattaggtaaacctaacaataaaatctttaaattgtgttagaatcatttagttagtcgagttctacactaaaaaaaattaaaaacactaaaatcatttataaataaaatattcaatatcttcaaaatgtactaaaacattgaagctcataaaactaatcatttttcttttgattaaatttctctctcatattaccaagaaacctaagataacattaccaacgattcataccaaaaaaatttattatcattgaacatatctcaaactagtgtattcaataatggttagagtagtagttatattaaggtgccatgagtttgatatttttcttttttgcctaaattaggttaagccgtagctagcttgaacaatgctaaagatcttcttaagagtttcgtagtttaacgtttatatgataaattttattacatccgaacttgatatttaatttttgtggctcttatctgtgtttagtttttcttattctcttttaacttgtagtaatcaaatgaaagccatttgcaaatgaggacaaatgcatctgcaagatatatattagccaatctcttgatatttttatgctctatgagacaatatattctgccatttgcccatcaaatggccataatttctcaagatttttccatttcgagtttgtttcaatcttctactccttttgtttttcctttgttcaattttttggacctttgatgaaatatcttcataactcctatgacgtgggcaccatccattggttgtcatttgataagaaatatgtgtcaatggcacaattcccattccatttatatattatatagttcctaaagccatatccccatgatttatatccttcttcaagctcacaattgaactttaacattacttcttccctacacaaagat

SEQ ID NO: 67 - DNA, 2000 bp, Cucumis melo
  source 1..2000: mol_type = other DNA
aaataatttgtggattttatcatattatgtaccttagactttgtaaggtttataacacaagatgtggagaaatcccatgatgaacatggacgttattatatcctttgaaactaaaaacaaaggaaaaaaagacaaatggctgagtataagaaaaagagaagaaacaaccaaaaagctaaaatgtcatgctctcatatgtaacatatttgaattgggattgatttcaagatgtattttaaaataatttaacacacgataaaataattctaacaaactcaaaattactcttaaacatttacttgatatcttcgacataatgacttttgttttaatacaactcaaaacataattaaggttggttttaaatgacaacaaacgaaaaactcgattctaatttcaatactagtctttgaaagccctaaggagcgtggttttgaattgtatagcaaggtttcgaaaattttaatcatcaaacaataggtatatttacctgttcctcaagtacagttaattcatagctacttgtcgtgcttcctacgacaacattgtaagacttgccacacactaattgaagccgttgttgaaggtagttttccatgtatagcttgaatcgacggatgaccaaagaggttgaagaaggtttgaaaaataggggaagggatatacaaagtttgagagtgagagagggagagaaatagaaatagaagagactgaaaaatgtaaaagaaaggatgaaaaaatgtggggtaaacgcaaattggatttttatagtagtattttgaaaatgctatagaaaggctatgtatagtagtgcttccaaagttctatatgaatgagacaaatcaaaatatattttttttgattaattaaccccaaaaagactcataaaaaaatcttataaatcccactaagatattgcatgttatatgtagtaaaatttatcgttcaaataaaccttaaacataattcaaacgaagaaagtaaaaatttgaatttcttatcttacatcattcaaccaaacaatttccatataagagattaaacttctaactttaagagagagatatccagcatatgcaacctaaaccaacagtgactttgctatatatttgcacaaaatgtgggggacaaagttgtaatttcggaatatcaatgattaaagaaaaggtaaaatttaaaattcggaagcttgacgtggcaacacggaatggtgatgatatttccaactcctcgcgacttttagaagttggcctcaccaaccgcatatccgcccctttgccacgtgtcagactacaacaacttccaacaatttcctttaagaacaccaaattatatcaataaatatttaacttaaattaagaatatatttgttacaattttcctactgagttagatagatagacagacttgtcaattaactaataagtccaaagtcaatttactcaacatagatacaattctaatttgagtgtgaaatacatattcaaatcaaaattattattaagaggaaaaactgatttgctttctcaatttaaaatataatattttgaaaaagaaacacacatgtattatggttttcaatatatttactttcttagtcacctaatctcaaactaatttttgaagaaattaaatatatatattatcatttttattttcttggttatgatattggtatagaatcaacaaaactacaagtgtcctctcctctgctatcgatggggattagactctaaacttgtttagcgattagtaattatatattagaaaaagtttatgttaatgtggacccgacaatctcaccaataggctcttcacttcaccaacccccgacccattccctctaataattcgacacggctcatccccggttcgaaccgggccgacgtcttcctatttaacacacctccatttcctcttccctccgcaacacaaacagagacctcaccggaaaatcaagttaaagcaaaaccaaagagaagcttcatcactctccggaa

SEQ ID NO: 68 - DNA, 2000 bp, Cucumis melo
  source 1..2000: mol_type = other DNA
taatagttgcaggtcttgtttaaaatactaatctaggtgtgtaaaacatagaaagtttaatgtggaatttcttatgagaacgattaaggctggtgaatctcgcttggttaaatttgaagtagtttcacttcgatggagactagacgtttaggcattcgtaatttcagagacaacataacgaggctacgttgggaaaatagttatgtcattttatcataactgcatactttgtggtaaggatcatactgattagtaagtacggtttccactctatagtgtttgagtcaacttctgtgcccctttactaatctcacgagagaatccgcctggtcctgtaacatttgggtgtcaaagaaacttgtaggaaagattccgaccaccatggattgaatcataagtcaagggccattagtaaaaacctctaacttgctcttgctttaaattttcctctattctccttattcgttaagcattgggtgtgggtgctatactaacttttgtgggttgttaatggcctttgtttctgtagatagtaaggacttctactgtaaacttgctttttgtttgcactttctcactctttcattttgttaaaaaatataagacaacataacagagcgacagagagaaagagagactaaccatagcaactggagctccttgtgaaatttatccaattcctcagaagtagacaatataggcttctttacagcaacttttctaccatccaaccttccttcatacacagtactctcggcccctgcatcaccattcgataaaaatccaatatgtcaacagaacctctcaggcaattgaaccggaataaattagtgcagcgttgagtgcttacctcgggcaattggagagagcagcgtgaatgcggaaggttgaagatgaagaggaatcgaattgctggagcagcagccctgatgcaggtgttcggatccataattcccaaatccatatccgttttcgtgaagaaatgttgaggaaaaattcattatgcgttcagtttataccattggagagtgggaaagttcgtattgttttgctaatttcgtcgattctcaggtcttggagtaaaaacgttgtacccgccacttcccattgggccattgtccaatattgtttgggttgggcgggtggatgacccaaattttggggaagatatgagatttgtccaactctgttatcaaatatgaccaaatgaacaaaatattgacttttttttttctatatttttttgaatgaagtataagtagttgttttattttgtttattttaactcaaaattaccaaatttggatttcacaaacataaaatagattttatactttttataattcaatcgaaagttgatcgtatatgaaaagaacaatgaataaagaaagaaatgtaaaatttatatcaacttaattaaaacctcgcaatacaaaaatcgagtgaaatagagggtggaggatgagaggaagagggagaagacatccataccctccatggacatgggtagatgtatgggttgggttgggttgggttgaattgggtcaacccatccactcggttcatatagacagcattcgttttataatttatccaaaataaaatataattaaaagaagaaaataaaagaaaaacgaaatctccaattcgcgtaggaaattaaaaaggaagagttaattcaattcgattctctcccatcttcatcataattttgcgaaaggatcgtaagttgtatacttctctccttgctgcttttcgaatcgggataagaatattttctttttgtcttccccattcctactcttcaaaattctctgcattttctacccatcacttttacttcaaccatttttgttgttgggagttccatattttgatttcctctacaacgcctaaactcttcttcttcttcttcttcttcttcttcttggagtgatttttcagttcaattttggggatttcatctatttctttgatctgcagcgttgctggaagttgcg

SEQ ID NO: 69 - DNA, 2000 bp, Cucumis melo
  source 1..2000: mol_type = other DNA
agtttattctgttgtagcaattcaaagcagtgtgatccagatgagtacatatttggtagtagactcaattatcattttatggttgaaaaccacatcctcttctgtcattgttcatattattacgaggaaaaaagccacgtcctctttcaaaatttcttccacaaactctttcttaaaaggaggaattagagtttgaaagactaattagatcgagaattattcatattcagattggtacctaattgagtagcaaccatcgcagtaggttgaagagaaaggtcctcttgtttacgatgttttgcaagagcaaattcttcaaatttcaagagagtatgaagttcttcaaagattactgattgtgaacgagtgcgcatagagatgtgaaaatattgtattcatctagaaatcaaatgagagtatagatcaacaaatcttcatcgtttactattgaaacacacatttgcaagtttatctttgatttttttgcccctcctcatgtatgaattaatagattcatcaacttctttgaaatcgattgaagattagttttgagattaacaatatttgatcgtaaatttgagtagtgattttcaagtgcgacccagacttcctttgatgaagtacaaccaacaattagggtttttacagacatagtagcactgatcaaggtcataaaagcttgatctttagcaatttaatctttatatataaaagattcaacattgtcgtcgattgattttgtattgtagatgaactagtggtcgaagaaatcaaaatcgattttgaaatcaaaatcgattttgctagagctgtacttatgtcatcaacaaatccatataaatccatatagcttgtgtgctctcaaaatagtggagaattggaatttctaagaaacataatttgttgattcgagtctgataaatatgaggtacatatatttgtgaggaagatcaaaaaattgatttcttttgttcaagaagactcagcggaagccattgatggagagaacaaaaatcggaggggatggttaatcatgggtctttgatctgctctaataccatgtgatctttaccaagttgtgaaaaaataatctctcattttctcattaatttacaataatagaatatgggtatctattacaacccaatttacagaggaaatactagctgattacaacagaatcagtgccaaatcaattattaaaactaatactcaacactaattaccaaagaattagtggtttttttaccacgaatttatggggtaaaaaaagtgaacttttaccaaattagtaaaataaaaaaagaaagaaaaaaaaacgtaatattcaaatggatggtgaggcatgaagaagagtagcctaaagtacatgaagagctaaaagacttattatcttccattggtcccattgaagaccacaaagaaaatatcagtcctttttctctttagagacacaaacccaaagtagaaagaatctttcacaagaattaggaatttaatgcaatttttctttttaaaaaaaatctccaattttctatctcattatccaccctttccactctaaacttcactacaatttgatgaaatctgtttccaccaatcagattgcaccaaattccatcaaaaacgccccatcagataattatggatgtcttcttcttcctctcttctttcgtggctgaaattgaagctcaactcaaaaatacatttcattttcaaaattccctgatgacccaattcgccacgtgtcccttccactcaccactacccacacaaaacaactgcttctcttcctcttcctcttcttctccattaaattcccagacccatccctctgcaacttcgaatgcaacagaaagaaaacggaccaaaaatcccttgaggaatttctcatttttgaagcataattcaaagattaaacccgtattaaccctcttcatcttaccagaggtttgatttattgatcgaattgttttattggttttttttcaaggtcacca

SEQ ID NO: 70 - DNA, 2000 bp, Cucumis melo
  source 1..2000: mol_type = other DNA
gcatcttatggatgtagtcacaacatatttatatggattttctgataatgatatttatatgaaagtcccaaaaggatttaagatacctaaaacatataaatcaaattcccataaactatgttcaataaagttacagagatcattgtatggattgaaaaaatcatgacgaatgtgatacaatcgcctgagtgaatatttagttaaaaaaataatatcaatataattcaatatgtccatgcgtttttataaagaaatcaccgtcaggatttgctattataactgtatatgttgatgatttaaatataattgaaattttgaagagttttcaaaggcaatagaatattaagaaagaatttgagatgaaagatctcagaaaaataaaattttgtcttgattttcaaatcgagcatctagtaaaagggatatttgttcatcaattaacttatacagagaaaattttaaaaagattttatatagataaaacacattcattgaacattctaatgcaagttcattcattaaatgtgaagaaagatatttttcgacgtcgagatgataatgaagaactccttagtccagaagtaccataccttaatacaattggtgcacttattttgtcaataatcaagaccagatattgcattttctataaatttattagctagattcagttctccaacaaaacaacattggaatgaagttaaacatatacttcgttattttcgaggaacaattaatataagattattttattcaaataaatcaaattttaacctagttagttttgcatattcttgatttttatctgatccacataaatctagatctcaaacaggttatctattcacatgtggaggaactgctatatcttaacgatcagtgaaacaaattaccataacagtcaactcttcaaaccgtgctgaaattcttacaattcttgaggcattcatgaggctagcggagaatgaatatggttaaggtcgatgactcaacacattcgaaaattatgtggtttgtcttctagtaaactccttccaacaacattatacgaagacaacacaacttgtatagctcaaataaaatgaggttatattaaaagtgatagaacaaaacacatctcaccgaagtttttctatactcatgatcttgaagaaaatggtgacatcacagtacaaaaaatttgttcaaaagataatttggtagatttatttacaaaattattacctactgcaacctttgaaaaattggtgcacaacattggaacgcgacgacttagatatctcaagtaatgttacatcttacttgccaagttaactatacatagtgacatttggtggagttgtaagaaacactaatattggagaaaaatcgaaagaaattggaaaatatggagaattgaattttttttagatttttcttattttctaattttaggtttccgtattctgattatgcctcattttcacaacattaataactttaataagatgatttcttgggttaagggaaaaaatcatttttttagagttgcacgtacaaaaatattatcataacatatcgattataataaaccaattcaccgtcaacctaacctaggtagagtttgagttaaatgttaaaagaatatccacccctcaacattgtaatcccaactaataaatcagcaacctaaagttttttttaaaaaactaaaaagaagagcaatatattttttttactattatttttttaaagagtggatttatttattaaattaaaaaatgaaaagaagaaaatttgttagtttgggtaatccgaaaacccgattatttgggcccgagaaaccgacgttttgtttattgttcctcacggcaataagtaatggcgtgaatcgaccgcgtgcgcttcaagctatctagacatttttatatcctccgattagaaaccctaattcagattctccgtattacccaccctggaacatctttgaaacgcgaaaaggtgacccgaagaaacttgaa

SEQ ID NO: 71 - DNA, 2000 bp, Cucumis melo
  source 1..2000: mol_type = other DNA
taataaagtcgatgatatgaattaattagacggatgggttatactatagttattttattgtcttttatagagaatttaacattggtagcggggaaaatccgatagatattggtgaagaggaattcgttggtggatgtaaaggaaagttagtttcgccttggcacaacgaagggtttgaatggaaaatcatgataagttcgactgcctgttcaactaaacgaaagataccaagtcaaaccttagttttctttaaggatttatgatcttagtagtgtatctatttaaagattcaaaggtatcaatagactatttatttcaatcgttgtgttgaaatctaggagtatatttaacgattaacttaaaagattttgctatcttgttttgtgtttttcatttttttgggaaaacctagtgtctttttattttatttgatacaataagtattataaaaatgactagaatgactatatacttgatcattattttgacatatttgcaatatattaaaaatgactacttattttaattaccttcatggtctttttttaatttatgaaggggtgggctcgtgtggcagatgaggcctgtcataattagccttaccttaaataattgggccggttctttgggaaatatcggcccaacctaacttttcatgggctcaaatgatgctttatctaatacccatactttccattacctttgtatattgaattagaatgatagaaaaacatactacacagttgagttaggatataaataaatgcattgaactatgtattacatagttgagaaaaatgagaatgaagttttgtcttttgaatatatattctgtgaaagttagatgtatatagaaatgatgatacttcggcgtttgttgaagattgagtggggtgtcaacctaatcatagttggtttaagaaaagttttaattataagataaccgttttaagtgacttatgccatattttgattgcaggttcacaatgaaatgttttaatttggtgattagactttgacaatgtggtaatttatgttaagtgagttgttgtctcgtttaccttgatcatttgtctctactcatttctcattttgtttcatcccttgttatatggcatccattgttgttgtatttgtcattgttcacattcgatgcttaactaggtaagaacaacattttcattttagaattggaacgatagaaattcataagttttatttttgaggcacttggttcattttaatcatagaacattagtccacaatcgtttggaataaatttacactctatctagatatggaactcttgacaacctctaccaaggaaggatgaaaagcaaaaaaagagtagaaaaacgaaagtagacactataacaagccaattagcccattgacaaatattaccacgttattaaagttcattttaatcatcgtgtcaattatcaaccttataggtcaaataccatttataattattttcaaattcaattaatgaaacaagactcaaaaaaccaaacaaatatccaaacccaatatttgagtttagaatataataatttcatagttagacttggagacagatttgtacgtatatgttaaattaaaaatttaatcaaagtataaataaatgatttggagtggcaagaaaatattggccaaaatttcataagaaaaaggaagaaaataaaaaggtgtattggctaacaaaaacccaattccatggggaggagaaaatttgagtcctcaaaaaaggatttcagatagggaaccaaccaatcaaaacgaaggacgtctccacgtgtcgctacaagaggccatctttccaaaatgagatcgcggataaacaagccttttctgagcatagaaaaatggcgaattttaacaaaaagaaaaatctcagtaaagtcatcagctacagctgctctttgacggccacttgattcactatttccctctctttccggcgctgattctagtgtggttgaactttctgcaaagaa

SEQ ID NO: 72 - DNA, 2000 bp, Cucumis melo
  source 1..2000: mol_type = other DNA
attacttgaacttaatccacatttatgtctttatataaagttcgaatactcataatatagccaagaaaccttgtttattggattttgagttttatcataagcaaatctcttatccaataacaaattattaaacaacacttcaacaataactttattcaacaatatattagtttaacattcacaaatcacgagtattagaacataaaacgcaacaaagaatggactaaggtactatattctaacttaggttgtttaggatttccatatgtcaatgcttttgtgatttttgaactagattttcttgttagattaattcaattctatttttaaatggcttaatatcttattttcggatgcttggggattgctagactaccgctttgttgaagcaataagttaaatttgtttgttacaggtattgatcaatctaacatagaattgaatttgtatgaatatttagttagacgcttgaaaactaattattctaccaatgagccgtagatcttaatgcaattgttattaatttgaactttgtatgcttctcatcgattaaatttatatcaagtagttaattaggacaaatctattggctttttcatttaattttgttaagtaaaagcaacttagaattttgaaaatgatgaacccatgatccaatacattgaaagagaattttgtttaactcaaactaggattcttctcacattgatttcgtataatttaactttttcaatttatatcaatccccccagggtgaaaaaaatttgtttgaagaattcatgtgctttctaaatctgatctagacttgccactaaaattaacttttgatatgtaatttggttaaatatttgattcggatttcgacgacaaacaattgatcaatgtggtattaaattctgatctccatgtaagaaatttacacattttcataagttcaatgttgacacaaagagagtaagagcattttaaaaaaaaagatacttttaatcttttctaaaaaaacaccaaaatgccattatgtaaatgtaacctaaataataaacatttaaacttagaattcatgcaattaggctttgtatgggacattgaattgattattaaaatcagtagttatagaccgtgagttataatggtttgtattagaagcataaattattttaattttgatcgtaatagcatgtatttgagatataaattaatttagtttgggtggcaaatagtaaacagtaaagcaaaatataaaaaaatgaatttaaaatagtaagatttgtaacaaatgattaatactataacaaacgtggttttaaaataacgttgatcgtagctaattgaacattatttattgtaaaattgagtgtttttaatatttggagcctcaaacttcgggtggatcaccacaatataatcatattcaaatttaaaattttattttttttattaattataaatattgattgttaatagatgctcattatgggccatctgtcactccctccgtgcatatcctacctgaaacatcatatatcttaaacaatgtccattgccatgtgtcactatttttacatcccatccacttgacaaatatgttgaagatgcctacttttttagggatcatgtaatctatctcatgcttgtcaaattgttcgataatagtgttacaaaaaatttagtaattattattattatatttcttcgatatttatgcttcatatgccattgtgctctccatttttaccatacttaaaaaaatttcttattataaattttttcaaaaaaaaatttactatatagtcatcatctttattaaaattaaaattgagaacctgatatttttgatattaataatttaaaatttgaattaatccactttaaaattattaataatttattcgaatttgggccttaaggaagagatacggaaacaaaccctagatcccatctatatataaatcgccacaaaaccctacctttctctcagtttctcgttttagccggcaaaa

SEQ ID NO: 73 - DNA, 2000 bp, Cucumis melo
  source 1..2000: mol_type = other DNA
tgaaaaactaaattaaattgtccttacatgtgtataaaagaaaccttcggacatttgatctgagaactatgttaaataataagatccaaaaaactgaaccccaacatcttcgaaatcgatttgatttcaattcttaagataagctacattcaagttacctagatgatctaagaaactaatgattggacaaagttagaaactcccaataaaccaatgatcttcaaagcactctacgatcaagacagattaatttttagtttgaatgctttgaacactcgtgcattctatcacaagaacaaaaattatacgttttagaattttcaaatatcattcatcccaatttttattttaaacgtgaaaattacaactctatttatactaattaaaatattaattaacatgttacaatatttaattttatgtcatttcaactaatgtaataaataaaaacaaataagacaacgtaaatacacaatttcataaacatttaatttcacgacttttaagttttctaaataaattttcaactttttcatttgatttaattatgatttctcggatcatatctatatatatatatatatatgaagctgagttttagaaattgtaaattcaaatttctttaaatggtacaaattcaattagtaagaggaaaaacagctaattaaataatgtgtgatgccccactccctaaaacagtgggtttggatcgattaatcaactaaaactgaccacaaaacaatattcttctacaaccccattgatttttttaatcattaagtgccgattcaaagaaacaataaacaaaagaagttgaaaagattgagacttttaaattaaatctgcaagattctctccaaactcatgttgtattcaagtgtttaaagcttaaaatatcagtaattatgtgttatttaacggtgaaaccaatcaaatcaagcaagattcttcaatattcaattccaaatcctcaagtttccatgaaaacttcataacgcctttatccctcgaaagccaaaattcaatttcctccattcatcttgcagccctatctactttccaaaagccaacaaatacccttttaagcagtagccttttgtttggttgtagtaggatctttgtttctcttccattttaacacaagccacaggagaatctctatctctatcctgcaaccttcatccccacattgttcttcctccattatcggaaaaacccagtacagggtttgctttccggccactatccggttgttctttgtaagttttttgggttttcattatctgggtttgtggctgcttgtggattcagggtaatgtggccatgttttatagtccacagcctttttttcttcttttgacatgggattatttctgattctatttgtctattgttactttgtgctttttctggtttgttcttgtggtcatcatttcttatgcttggaagttcgaacatgaatcaattcaacaactaagttgagagtgttcgactctctcatctcattgaccctgatggtatatcttggcttggaagttagaacatgaatcaattgaacagcttacttgagactcgagagtgttcaactctttcatctcattgaccctgatgatatatcttggctttggagttatgaactatgagagcttggaggatgaactaaaaagaagggactattttttgagatggatatttagttttagtaatttagctttttttttttagtacatagtacattaactttgttcgcgaggaaatagtggtcttgttgacgagcatttcttaaacaatgtagtttttgtctcatctctttaaaagtttatggaggggcaaacaagtgagatcaatagttatagtatttcaatctataactttggaacagctgatttttaacttttcctttgtcttttttttattatagaacacattagagtgcgttagattcttcagttctgagattttgatctttgagtgctctcttttagcagtagaggcaaaca

SEQ ID NO: 74 - DNA, 2000 bp, Cucumis melo
  source 1..2000: mol_type = other DNA
actttcagtagattttatctcataaaagagtcataaagataattagtaatgaataaagctttgtttgaagaaatgtttcattgcaactgatatttgtcattgatgtacaaatggctttgtaactctccactttttctaatctaaccatttacatacaaaatatctacgatacactaaaatgaataaagaaattttttttgtcaaaaactgtggggagaattgctccttgttctcaaatcattcatgaactttgcaatttagaagtaacatcaatgaaggcttcttccttgcagggaattctcaaacctccagttgggtggctgaatccaaactcttcttcagccttgttgagcaagtctatgaatgaaggctgactcaagtacgatattggaacgaaaaaccgctttctgtcggtttctcccacgtacactggaatgtggcctttgggaacaatggactgacatcttgctgagacagactgcatcttgagaacttgcttggcagcggaaagaagaaccgaaggcaaacgaattcccatggctaaattggattgaatctttttggaagtggtaaacttcaatgcttgaatgagaatatgtgaaagatttgaagttggagattagttgtttgtttagagtctatatatagaatgagaaaagagaaggtattgtgacatatgaatagaagatgggaaaccaagaaagttgggttcatcaatggctcacatgggttgctccattggttaaggtacattcattttctcattggcaccaatttctggtaagatggccccatatgtcataatacgtgaagtcatattgatctaaacaaaatgggacacaaaaattgtaactatttcaattagcattaaaatcatgtcaagaaaactacattaaatatagatatattagttaatgatgtaataatagtttcatgtgagatcaaactacgatttttttttataaataatgttacttttaaaaaaatgtcaaaaatatggtagaagaaaagctattacaaaaagttaagtcatctactcggttcataatgcgttatcgtggatcgggtacacgacaaggcaatgaagacatagacccagtctatgacttcgatgtaaaatgtgggtttttcctaattactcgtaaaaaaatatttttgaaaacttttctttttaacaaacttaaattttggttaattatatatataaataccatctttactttcttattatccaaaacaatttaccatatataattatatttattcaataaataataatataaaatatttagataaacaaaatcaattatttcaatcttatatattttaaatatacactaagctaatttaaatttacattctgaaaattttaattatatttctatctaatttaagattttaattatatttctatttaatttaaaattttaatggaaaattaaattgtaaataagaataagagtacaaacttactatttttatttcatttttaatttataaacttcatctcttttttcatatatttttaagaaatccaaccttatatttcgaaatttatttaaaaaaattataaaattttttaaactatatataaataaaaattgtaatttttgaaataatttattaattcttacaacaaacttataataataacaataataataataataatgagggtactcgattctcaaaaaaaccgaaccgatcaaacaacgttagatcaccaacacagaagtagggtttttcatcggcacataaaaaccctcacttcttcttcataaaaaccctcacttcttcttgacctaattcgcgccgttgatctccggttcgatcggtttctacgctgtaatctcaagctatctcctaccttatccttccctctctttttcttcttcttcttcgtatatgcatatcttcaaatttgctgctttttttgtctgattattcatctgggtttgtttgcaacaggaaggaggaagaatttcaaatcaagaagaaaa

SEQ ID NO: 75 - DNA, 2000 bp, Cucumis melo
  source 1..2000: mol_type = other DNA
tttattaatctgaatcattctgtttcttctgagagttttattccttttaagattctaattttattttggatagttgaattttggtgtgctctctttgccccttctttattatacattcctttatcttaaaaaagccaaaaagttaaaaaacaaaaactaatcaaaattgtaacatttacaattttatgagcatgacatttaaaatatcgattttgaagttaagacgttgtattctcaccatcggtttttatctcttcccattccattagagtgataggctttatctttcatcactgtcaaaattcatccaacgtccaagatctcttctgcaaagagttacccacaattctctcagactcattggcccaccggataccgagtggatggatagaacctccaagattgcgagagcaaaagctcagccaaaacttgcacaaactcacccatggcttccctctcttgtactacctccattaatctcaccccaagatccttcaattctcgcccccattcaaattagcttcccattttcttggtcttcagtccaaccttcgatggctctcacccctctccattggaccctccaatgggtctagagcaacttgctggttcaatttaaggcaaaatgccgagggtgcaggcatttatggcagccagtcccgagatgatttcaacagagatgatgttgagcaggttcttttactaatttctctcttctttctttgtattttgttttgtgactttgattgttgaagagtggtgtcttttgtttaattgctggtttgggctgattcttatgggtttggagttgaaattgttcttaccctctggctgttctgttttcttttaagtattgtgaattttcaatggctcctttagtgaagatagatgaagaaatttaaattagtaatttttcgtaccgatgactctcttccagtggtgttaatgtcaaactaaccttttctttacgtcataaagcacttaatcggttggaactcagtagacgtctcactcatgtttgtagccctaacctaatgccatggcaatcgaaatttatatcgtatccctattgcgattattaaacatcaccataggtgagacattcctaacgtgatatactgagttctagatggttaagtgctctgacatttcacattaacgcctcatccgcactggttagtcgaaagaagaaggtgtttctgttatgagattgtgagaaaggacctccttaaacattataaccaacctcataacttgtgcatttgtgtatcaaactctgctttcacataaagaaactaaaacaaggtatcacattgccgttatgaaaagtgcatagaacttcctgcttccctcaaacaaaacttgcaaatattactgattggccttagcctttaggtaagggaagaatcaaaagtattccttcatccttctgctttaaaaatgtgctaaatgacgttgtccatagtttaaaaactcgaccaaatcgcatttgtcttacagtctctcaaccctttttaagcactctcagagtcaatccaaatagattcctagttcctaatatgtaacaagaagagtgatactatgaaaacccacaaaaaacccacaaacatgtgacttgagttaagatgactcccaatcccactgtatcaagcttttcaaatagaggaatcacgatgagatgaacaataatatcccaacgtgctgctatcccaaattagatacagaagtctacttgtggtgttcttaatccaataattcattatgaaattcttatataatttcttaatgagtatcttagaattaatgttacaacttatctcttattctatatgatagaatcttaacataagtattcatattaagagcaagattatgttgatacttctcgaatcataccaaaaacttggaaccatgacattaacttcattcgtggaaacaagttttgaaggaaaaagaaggattgacaaatgaacgttatggttgtgcagtattttaactac

SEQ ID NO: 76 - DNA, 2000 bp, Cucumis melo
  source 1..2000: mol_type = other DNA
atctaaaactgcattttttactacatacagattcacctttaggtgctggggcttcccctatttcattttatcaatgaaatgtttcttatctagaaataaaaagaactacatacagattcacaccactgcagaaaggtcaaataaaacattcatcataattcaaggtaagtaagcataattttgtgaaacttatgtgatgcacttaatatatgaacgattgccccttgttctctcaaagtcagatcttctttttcctaacaattgaagaaagtggaaataagttaattaccacggccacgcaataatctcctgatggcctccaatgaaccccccaaacataatgctgtagggaatgtcttcttgcaatccttcaagacgcacaatgtgagacatgcaaaatattaaaaagtgacatcttcaaatatagcaaaagaaatcaaaatatttacaaaaaatatagcaaagtttcatattttatcaattatacacactgatcgacatattttgtaaatattttcaatagttttgacatctacaataattagttgagattttgtagtcaacaggatccagatttgtgtgttgaaagttgaaacccatgataagataaaatcccggttaaatatttcattttcattcttaagtttttgaaaaaggaatagcttggtaagctacattccgcatggtaaacaagcatacaacttttgtttcaaagaaccaacaagtactacaaacaaaagagtaattgatttaatccaagttaacaatgacaaattggtaatatttataggatattagtgagataatacaatcaagttccaaaagatgttatatttacaactatgagcattcatcttgttactaccaccaagaaaaagtagcggttttccaatctctgtcaagtatccatttgagttatgatttcatattcaagactgtcacaaaaatttcattaaaaggtgcaagtgcaacatttccttaagaaaaggataactgagagatcaatgactggaattcacaagttaaaatgaacacaacttcagaacatcacaagctaatacctccaaacggtccaataagttttctgcaacactgtcaacaagcgaatcctttgggcgcatcaaccaagcagctcggtcccgctgttaccaagaaacagcaatttcagcaagaacaaaatatagaaatcctccaagaaaaataaacaaacaaataagttcgaaggcaccacatatcagaaagcttatggaggagtacatgtagtacaaacgctcttgccatttagttttacttgttaaaagtgatttgctcagaataaacataaccaaagcagaatccgaacatatgaaccaatgaattaataaaccccatcacagaaagacaagtaatactcccagaattgtactctatacagacgaccactacaatttagccacacaatatcaccatgttctctccaaatatatttaaaaaaaaaaaaaaaaaccctcctattgttgcggttaacacaaatagatcaaaaagaagaaagaaaaaactaaaaggagacaaaggtgttaaatttggtttacctgtttacgcttaagatcacgatcaaaaaccttaacctttgagctgtgcattccatcaccgattcttccgtcataattatcatcaccagtagagaaagaacaacaaggaattgaatttggaaaatctcgccatcttgcacttctcaacactgagaacgatcttatgatcgtagacggcgacagccctctcatttcacagtcaccgattgaacctcgccggagagacggagggaaattttgtaaatttttaatgggcctgggccgtaaagtcgtgtccaaacactccttaaacggaccaaaaccggcgtagaaatgaaactatccagataagggacgtgctatacatttatccaaacgaggtctcttatcgtatcttgtacaagttcgttgcttttcacggctgtctctagaattttgggttgggcgaaa

SEQ ID NO: 77 - DNA, 2000 bp, Cucumis melo
  misc_feature 1..2000: note = n=g, a, t or c.
  unsure 1..2000: note = unsure at all n locations
  source 1..2000: mol_type = other DNA
aaacctactctgtaaatgaaggtttacatctcttaaggcagtaccatttctgccattacttctaccattcccacgaaaccacctcttttctctttcattctccccgtcaggtatgcatttctcatctctaagtccgcccactgttttccgactgatttttcgatttttaattagtgagtcggttttattgtttcttattctaagctttcttttactctttatatttttagatatttaatttcggatccattcttcccatcatgcccaatccaaagactgtcgaaagttttgattgttggtaatgggacattaggtctggggtttctgtttttcttatcctataaattggttatccttcgtttcctctattttgactttattccgtagttaggttagaagaagaaactactgaataatgtttactatacaaacacctcaaaatagccaagcctgtcgaaacacatttagctgataagctagggatgaagagatcaagagatggttagctcagctgtattgcatctcatgggggacgggtgaaacgaaccagagaagtaatatacacgttttttttttaaaaaaaaaaccgaataatttacctgttcttgctacaattacaccgataagttttcaacttgagcaattacaccgtctaatttgcattgctgaagaaattggtctgttccattaccactgttgattaaaaagttctacttgtcagcacagcatgtccatgtgcccagatagttcttgatctttggaaaaagtgctatgtttgcatgcttcggtaagatgtgaggttaaaatgaggaggacataatgttggcatagggaggtcaaaatgtgttaattgagagaaaaaatgtggtggatattggagaggagacatggaagtagagagaaagagatgaggagggaggggtgaaggtaaagggaaatagacatacagaaataaagaactgtgcgagtaatgtgttgcgataagtgaaagagagaaagcaagagaaacagtggtagaaaattgaagtatagagagagatgtagagagggaaaatatggagaactacaagataaaatatctttattctttctctatctaagtatttatctctttagaagttatctctctttgtttctgagtttacccctagtattttcttttttctttctcaagcccttcctctctaacacaatttctctctctctcttctccctctctctctgtatctggctgtggcactttttttgacctcttcctttctgtctttatctcctttgaagacattttgattttcctacacccctcaattggtcttctactcaaactcatctacttgttattatattaaatgcatgaaatcctaatattttaggaagctggagactcattgtgcgtgcatctgcttgcttgtagaaagttttaaattgaaaggcaagccgaaggggcctaattattcaggccaggacaatgatgttggttttagttttttgtttttgaaannnnnnnnnnnnnnnnnnnnnnnnnnnnnnnnnnnnnnnnnnnnttttgaaactaatttttttcttagttttcaagacttggcttggcatttaaaaacattggtagaaaatggataacaaaaccaagaaacttacatgtggaagtagtatttataaagcttacttatgtgtggaagtagtgtttagaagcttaatttttaaaagtctataaccatatggtcatcagtagagtctcatgcaacttatgttgtgacagtggtgtaattgttctaattaaaaattttcgggtacaaatgtaaaaaacattatcgaacagtggtggtttgtgaaatatgcattaactttttgaaaatttgatgtgtcatcatattcattccatgccgtgccttgtttccctcccagctccttatccatgctaattagattcagaccattatccctttggaacagctatgcttaactctgttcttttctccctctgtacaacagtatatcaaaaa

SEQ ID NO: 78 - DNA, 2000 bp, Cucumis melo
  source 1..2000: mol_type = other DNA
tagcttgttaattcttgtgttgaagacgtgtttcaacaaatctgatggggtattcatcttaagtgtccactgaagaatgggggttctgtggcagatctgtatgttatgtagtgaaaacaaatctgtaaagtttttttttacttcgaatttaacgttgcttaagcttctgtgtacagttttatcactgcctcgaggttatgattattattggattaaattacaatttagtttacgtttaccttggaactgtgtatttcttttgattgctcaacttttctcggggatttttcaagaattgtatttttaaaattttaatttatttggaacattaagaagttggttatttacagatgagatataacactgtgattggggtggaaaataaacacagcttcaaacacggagtgagatatagttaattacattacatagtactagagattatataaatcactccactcacatgagttttcatcttaaaagattggaatttacatcttaacagatgcaatcttttaatgtagagttcttaacgtgttctcttacggttgtatcttttcgttttcattattctttggtcaaatcaaaattagactttatagtttttaatgaaatattggacacactacgattcatcaaagtaacccatgatcttataaagttgtgaaatgtatgtatattgtctttgatcaaactttacgtttaattatatcttgaatttataattttgtatttaagagatgaatgaattttagaaaattctaaagttcctaggccaaagttgttatagaagggtaaagaatgctttaaatcatttattccataatcattagttttataatttttattcttcgtaactattttttaacaaaaaaaaaaaaagttatgcatctcttaaatactatcttttaaaagggaaattttcataaataaataaaaaaagacgatagtatacacataaaaaaaactcaaatgatttatagagagtttgatgaattttgctggatttataaatagtttagaaaaataagtattaacctaaaattttgcctatatctcaatggccttctatgtctatgttatttcttaactaaaatcgaaaggatataggcttatggattggcttaagctaaaaaatgtcggtccaaatagttgagatgtcaaaccttaaaagtactacgattatgtgattttcacatgacatagtgttctatggtcaaattttatagcgtacttattccaatccatcactttttatagaactaaaattcatagttcctattttaatatatatatatatattaaaaacacacattaaatgatgattttatctcttctaggttgattgaaaattactaactaaaaaacacggtgcctcaaacctccaacgtaaatacgatttctaagaactgtgttttttgtaaacgccaagtgactgattaaatctctccattctctgtttacttctatttggggttatttatgctaaaggatattattcattcaatagaataaatgtgagatagtcgagttatattcatagatgttacaatgaggtgattcattcctttgtcaaacaatgctttctcgactcgtattttactgtattggatcgaaatccttcttactcgcatggtttgccttcgttgattagttttggtatgaattgatgctttgtttaagggggaaaatgaaaatggttcaattggaggacaattgtccaaatttcgggacattatgggttaaacacaaagaagaagtccaacagtgtaattttgttaaagattgcgttacatttccgaaatataaatgagggtattttggggaaaggaaatcaatataggccttggccgggtgagatgcgaaaaagtctcaaaactgagtgagaagcgtttgagctgggctcgcagctattgaaaaagagagaacaaaccctttcgtcgctcttattttcttcctttgatctgaaatttcctgttccgatctcgctttaggacgca

SEQ ID NO: 79 - DNA, 2000 bp, Cucumis melo
  source 1..2000: mol_type = other DNA
aattcattcgggattgttatgaggtaataaaaaatatctgagtgcgaacatgataattggtaaagtgaaaaaatgttcagctattctgttctagatacagggatggaagtgggaacaatgccaccttgcttattgacaataaaatgaggagtggcaatattttgtttctgaataaatattcactagcataacatattagtgatgattcaaactaaagtgcactaggtcactagtttcttgattcatcgtgtttggtagtaatggtaggtattgtatcttatagtattggacaaagctttaccgaccataaattgtggataatgtgcagagaagaattggcagttgaacgttcctggatattcaagtgatgagtggaagaatcacaacaaaaatgtaagaaaattatattaccctctctaaaacatcattctattctcctccctaaaaaatcattctgtttcaatttaactttcaaaattttgttttagtttaaccatattgagttttttttcttttttaattatcgtagttatcatcaagtgatgtccacaagaaacgtttggacatggtaagttggacttatctcttcaagtgtttgctccatttcttcttttatcatttgtctcaaattttctcttctggggtttcatcagatacgcctattgaaggaagcctcctgtgtcgaaacaaatgtaaacagccctaaagagatggtacgacaaggggttggaatgtcaattggtcccaacactctaacaaggccttcaccgagttcagaacaactattatcacaaacgtctggttcacagttgctgcagcaaatgatgaggttttagtgtattaactacgtttgaaactaatgcttggtagagatcccaactacttggtgaataaccaaccccagtgtcagttcagggatacaacaaataaaatgagatttagaggatgccatatcagagggaacctggactggacatctgtgtggagtggagtgtgatgatttttagtgatacgtctttcggaatcaatttttttaggctgtataatatgaagttgcattatctggaacacgggcgtaatgttaattgtacaaaatatttggcaggtcatattagtataggccttaagtattgttgttgtctaccatgaaggacattttccaatttatgattgataatctttacttacaatctcgagtcatatgaagtttgttgatcaggatcatagcacaattattacaaaaatgaaatagaagatatgatttttcaccccccccccaccccccccccccccccccctcccattcccatccccccttttaaactgttacattacaacttgttaactgttgattttccagatgagagaaagggcctacttgtcttgtacagaaaattcatccatgacgataaatgcagatgacctgaaccaaacgtgacagtaggggtttcttctatgccacaaagctccaagccattcatggtgcgcatgtggtacagagaggcttgatggagcctcttcaccttggtccttagctatctaaaaattggcttcttatgctgatatatctcttcccatgtgcatttggtccactccactttcttcgtcgaatatccttgggttaatcctgaatggtaagcacaacattcttgctaattaatccctctttttatcctacttgccaactgtacaagatgagcagaagaagaattgcccaatcatgaggtcattaactgcaaaaaagagaatttatttctttctttgagaatctgatcttcttgagagttcattgacagccacatgcatcacaaaatgaaatgctgtgtggccctcattcattcattcatcaatcttcctatcctgccatttgagtgaatgttactccaacttgcaggaagctaaattagtacttttttatataaaccctatgaaactcatcaagaaaccacaccatcccaaaaaggaaacgagtgaacaactagacaactcaccccgaaaaa

SEQ ID NO: 80 - DNA, 2000 bp, Cucumis melo
  source 1..2000: mol_type = other DNA
cagcgatcttcgtagaaactaattcaatgctagctcattatttgacttttctcaggcaaggctccgcgaggaagagaaaaggtccaatttcaggaaccaagggcatggacaggttccggtcagaagaagctttttacgtaaaccctttgccagattgtttatgtcaaggagaattaccaaatggaagtacgacttccattttcagatagttcagtagaacatcaaagataaaatgctcttagagagctcaatgtatatgcaggcgaccactcaacgtgtcaccagctttgtacatccaataagccagctacgatggaacgacggagtgtttataacctgagttttggtagttggcggaggcggtgatggtggtatagaaggaaggtcgagggatggcaaaccctttacgccaagtagtggaagggagtagttggagatgaacacattttgagaagtttccaagatcactccatttgggggagaggggatgttggttatttagcacaattgttttcatgttttagtaattttatccaataatgagcgaggcattgaagcaattaaatttatttttaatgattttttcacccttccataggctttttcttttttcttttccttttagtttgcaaactttagctccttttatcggctgtcgaactcatttttgaagttattgaatgaaacacagtttgggctgtgtcagatgggtggtgaaattttatacattataattactacataaaatgaaatcatattgtaattttctatctatgccacaatttttttttattgcatcatgaggattaaattgtacgagtccaaatttgtacagtcatgtttttaaagctttcgagcattgttactaatgcatggaaaggatcgattatcaagtatcctcccaacttcatgaaagttattatttgtcttctaaatttgttttagaaaatgtttaattaattatttgagaagaaagtttaactaaatcctattggtttcctctaaggttgtcatacttatccaataacaattacgtttaaaatcaaaattattctaatggtataagactaatgttttaaaagcataaaattgatgaggaaggattggaagtaatactatttattttgaaggtaaacattcttgaatgtctgtcctaaaatcactaatgttttcttagtttgagactttgagtcgttgaacctctccatctttataaaatataatacgagtccttcacaataacttaaaatatatactaaatcctaattaatgaaaaataaataaataaaaggtacaaaatcattaaagcctaaaaatctattactcctttaaaacttttcaagggtccctacaaccaatgagaaactaccacgtcattttcacaatccgttcagtgtttagaaaagtcaaatcgcaccgtccatttatccactcgtaccaagtacggtaggaatctatctaccgtccgattaagcacaaagaagcacagtaaatgtcaatcgtgtccatccgccgccataccgcacatccttcgtccgaccggaaggccctatataaagtcctttggttttccgaatttctacttcattcgcttttgaaagatttcccaatctcttcgtcggccaaaattctctctcgcttctcaacccttcttcggctttttcatccaggtttgtttctcttctcttttttcttcctttgttgttcttggaatatgtttaatttcatttgtttttccattcaatttcatgctagattttacgattaggttgattttctgttcgtagattgtaattgatggttagggttagctttttctcccattccttctggaatctgtttcttgaccttcgaacttcgttgataaatctttagaaacatttacataaccaaacaataattgaacaactcgtgttgttatgcctatataatagcggttaggaaactggaaacgcccttataattgaaatcgccttagaaatttgttttgattcatacag

SEQ ID NO: 81 - DNA, 2000 bp, Cucumis melo
  source 1..2000: mol_type = other DNA
tgtaatgactaaacatactatagcctatttggaccgggtcgaaaatccaaattaaccaatctcccctcagcctcacaccaaggataaatcatgtcaaccttctccatttgacatgctagctggacaaagagaaatactaactcaaattccatataaatatatctttacgactccttatcaggtaatttagactcaacaattagtaataaatttagtataatgaatgatagtttccatagatcaattatatcatttattgatttgctagatctagagtgaacttattgactaatataccaaatataaaatatatcaatgaacttacccaccaaacataaaaatgtaatatttatatctacatgaattttacaataaaaagtgtatcatataaaatacttatatacataaaccctattatatatatatatatataaaaggaaggtaagatggaaaaaattggaagagaataatttgacctaaaaaaatcgaaagagaaaagagtatttaatatataaataaaaagaaaaagagagaaagaaaaaaatcttgttcgtcgactcctcaaaaaccccagcgtgtagcggttgtgagagaaggagagctcgtttccatcacgataaaaccttatctttctccattcttctatcttctcttccggagctctctccatttctcagccgctccccacaatttcctctaaacacacacatacacgactatttttccattcaaattccttcacttcgttttccattttccttttctttaccccacccactcacccacctctcgtcgatggactccatggacttggcccaacaaccgtcgcaacagaattcagtctcctcaggttcttcttccacttcctcctcctcttttacgtcttctaccgttgattcccatgtcgatactccctctctcgatgaacctgagatgggggttgctgaaattaaaactagtgtagttgccgatgggggtggtagtgatggtgctggttccgaaactgaagggtttttgagtggggaggaggaatttgagtctgcttcagatagaccaattgtgggttatccagaggaagagtccatcgggaagtccgcccaaggggctgatactggtacttcttttgtgggttattctcaactttctgctccggttagtgttaggccaattgcgaaggtttctgttgatagtgacgttgaggaggaggatgaggaggaggaggaggaggaggatgaccttcaggtggatgagaacttgaggggaaaggaggaaattgaggataaagtgggtggagaagatgtttttgttgagagtaagaaggggaaggaagttgaggttccagtggaaaaggaggagactattgttgtatctgatggaaacaagaatttggatgatgtggtgaatgatgatgatgatgccagtcaagtgcaggaaagaacaattgagttgtcggggaactcaaaagagggcaatgtgcctgaaagcttagtagctgaagatgttggctctgtgcccgaggaatctgttgatggtgggaagcaggtgtcagaaggggatgaattgaatgatgtgacagttaaacagtcacaaaatgaggcttcagatggaaaaaagaagcagagttggataaagaaactctggcgtctgggaagcaggctggtaaagggattgacttgagtgagaaggtggttgctgaggatgtagagcaattgaaagaacaggaaacacctggttcttcttctgacgagaaagctgttttgggagaccaagcaagctctaagcttgtgaaactagcagatgaaaaacaagaagaggagacctctgcggctgagaagcaggtagatgtggaggtcaaattgaatgacacggtggctgctgctgaagatggagagcagttaaaaaatttagaaactgattctcctgttgacgacaaaattgttctagctgatgacgaaaactctaaggttttagaaccagcagatggaggacaagaagcagaa

SEQ ID NO: 82 - DNA, 1072 bp, Cucumis melo
  source 1..1072: mol_type = other DNA
tttaatatggtatcagagcaaatggtccagagaggtcttgtgttcaagcccctgcatttacgtttccttcccaattaaaattgtttccacttgttgggcttttcaaatatttcaagcccacaagtgagggggagtgttagtgtatataattaaatttgccttcttcaaccactagctgaagtttgtgggtgaattggtggtttaatagtaactatatcatgcaattagcttttttgagttcaacaatatctgtggtggagatttgaaatcgagattatgatgccttaaccatgtgaactatgcttaggttgacaactatatcatgcaactatcgaaaacatcatctctaatttataggtcttttttaacatagttgaagtttcaatattctatatgaacacagctggctatttaaattaccatattgaaaagcagcacttgaaatgcttctaaaaattaatgccaattagaagtgtttatgattctaattggttaacattactgaacacagattagttatagttattgaaagaataaaaattgtaaaatgccgaactaataccaaatggatgggtagtctgcaaattttaccaaatggtactacagctggtgatgaacttagaaggggtaaaggtatagtgtaactgtctaagttaatgccataaaggtatagtgtaactgtctaagttaatgccattagcagatcaagtccgttgtattatgtactgaacacattttttaatcgtatagttctaaatcctataatctgtcgaccaagttttaggtttgttaggctgaaagttcatgcaaatctaggtgcttttttgtactaattgtttgagattcagaaattgtatctcaatgttctccatgattatgtgcgtgtatttgcaaacagctctttggttttttcttcttcttctgacaaggatagtcaaatcaattacaggacataatttcaagatttaaggagagaaagcaagggaaagattcacgggagtggactgagtttccaagcagagttgcagtgcaattaaatgatactcatccaacccttgcaattcctgaactg

SEQ ID NO: 83 - DNA, 1730 bp, Cucumis melo
  source 1..1730: mol_type = other DNA
gttcaactccacaagtcaaatttttttggaaatctcgtgtgaacacttgtgaaacactttatttttatattaaaagaaacaagaagatttaagatgagaatcccgtatttgtttggttgaaggacaatgaaattggtaaatatatcccatcgaaaaataatcaaatctagacacaaaaatttaaagttaaaacttacttaataatcagctggagcatagtttaatttgaatgaaaataaaaatcctaaactagagaagtttcttatggtattgaaaggccagtttagaaagcccaatagcgtgggtttttcttggacccatgtgtatgtctcactcatgaaattaaattaattggcctccacattcacctctctcctcccaattcccataactcaattttagacctcttaaatgaaacatatcatattttcataaacttcttttttacgttacttatgagattaaaagactttaaataaagtgtcaatttatattatagtagatgagatggagtgtgtgtctttgtgccctccttggggcccaaggactaagtaaggatgaaagggcaaagaaatacaaaatagaagagagtagaaagaaaatgaaatggaatatatagtaagggttatcgtttatggttattatgagggaagggctgaaattgataatgaacctatccttatcttcccttcttcacctctcattttgcttgaaattacaaatgacttttttttcaattattttgtgtgtacatccaaatgtggtatgcacatatgggcctcccattaacttgtgatccaaattaattcttttgcaacctaagttgaaattaaacacttttacctctctttttttccctaacaattttactttcattgttagatggttgattatcttgacatgtaacaaaaagttctctcatgtcaagatagaaaaatcgaatatttgattttgagattgataatattataatatcagttgagctatactcattttaactatcagtaaagcttcattaacatattttttatttagtaaactaagattaatataaatagaatcttactttcattatatactttgacgagacttaaaacctatttagcgcatgatttttaaaagttggtaggattttaacccttgaaaaattggtcattcgggaatcaaaacattagtttccctttgagcatttatttttaaagcacttcaaaagctaaattagtagcattaaaaaaaaaagtcaaatagtatatatatataccaaaactttgtttttcaaaactatattttaaaccaacattcttttttttttattatttattactaattaagtgcagattatagtggttctcttttgtagttggatcaaatatttcattcttttttgacaataacaaaagttaaaatactcattaaatgctaaaaacttccatactaacattattgaaccattaaatatatgagcaacgaaagtataggtaagaatttatattgttgttgtttagtttggaaatagaaaatggaccaatgggtgagcttggtttaagttagggttcttgtggttggatgataatgaaataaaatggccaaaattttaatggagaagaagatccctttaagttcaaccactaatggagtcttttaggatcaattcacaacccctttctccttctgccacgtgtcatctcagctaatctcaactgtgtggttgttgagaaattttgaaactc

SEQ ID NO: 84 - DNA, 2000 bp, Cucumis melo
  source 1..2000: mol_type = other DNA
aactagactagcgagtgcacaaccaaattacaaaatccttaacagagacaaccatctatctcctttaaagcaacaataacatcaaccgaattagaatccacaatcagtaaagacgatgccgacaccaatgaccaaaaccgatcaaatatagcttattacggaccattacttcaacagttacatcaacaaaaaaaaaaaattaaacattgctaataaaatctgaaaatgaggaaaaagagattaaaagttttgaagatagaaagaataaatctgaaatgttctaatttgatatataagaaatatgaggtaatatgacgaaagcattttgatagttttcaccaactccctttgtgaaaggatacatccaaccaattttacaatttctgttcaaattttgtccacctacccttctcttctgccccccaaggctgctttctttcttttattatttgctaaattaccaaaaactattttcgaattaaaccatctatttcaattatatacgtcattcgaattttaacttaattaacattagtatatgtttcggatcaaggatagtggtataaatcatcctaatttcaatttgtatttagaaaagttcaattatacttaaaacttctaaaaattttatattttaaatttggatataaattaaatttaagatttatggaaggtaaataattagagcaaaacaaacttcaaactatatggaaaatagaaaaggaatattttagccaaacaaaaacacttattatatttattttgttttttgttttttttaatttaacaatttttttttttattggttgaatgtgtttctccactggtgagtctccaactttgacctgcaaagggtctatatagcgagtttcacgagcacctaaccaatatctgtgtaataattcccatttttctttcatacccacttcatttgatcatctttttcacaaccccggatctctaattcttgggaatttgcctctttctcgatccatttccaccgtaattgaaaaatattcaggtttgatttcttctgggttttcattcaactgtctaacttcattatgccctttatgtgtttgttgaaagccccccacccaccatcgttcaatgcggtttctttaccttttgttcggtttcaacgatgatttagaagttatagatggatgctaattgtttcgttgttggtttgatccactgatctgcctttgattggcataaaaggagattctagatcttgttttgatgttgtgatttatggatattattgttatagtcgtggaagtttttcttgtcgttctgcggtatatggttgttttattttttgagtggtaaattgagcagattgtgaacttttgggttttatggtgaaagcatgaattagtaaatgtagagctgctgaaacaaaatggaggtttgctagacctctttgtgaattcttaatggtcagcctccatcttaagaggctaagtccaaaaatttaaggcagtcttttgttattgttacaaaggacaagaaataacagaggagttattttaattgaatcaagttggaaagaagtactacttcatgcttctttcaaaagcaggtcaaagtgctttaaagtcttcttatttatttattttttcctgaatcaatttaaactaatgatagaaagaagtgttttttaatgggttattataagtaacatcaatttttaaccattccaaaagttacatcaaattcatcatagtgtgagtttacgaattttggaagttgtaattttaagttaatacttcttttaaggaaatgtacactttgcatgttgtgttcataaggggtatttctttgacaaacgcagcaaccaccccttaatgaaaactacaccacggtggttggttttttcttgttatttttttacttggaatttacaataagttgttatattcggatatatggcaaagcagatatctgtttttatccgaaacctcataaatcttgaatgtgcagcaggtaaaaac

SEQ ID NO: 85 - DNA, 1020 bp, Cucumis melo
  source 1..1020: mol_type = other DNA
tcattgatgaagaaggaaactttaagccaattcgacaacttatccattcaacaactttccaccttcagacattcagattcaactataatataacataaattgatagtcaagtcttttttgagacaaccataaatcatcttagcttcgagaactgtcacttccttaaattggtgaatatatcacattccatccattcaaaactttgttttcgaacttttactgtagttatgaatcaataaattgggagagatattgtttaaaaagagagagcatatttgtttctattatttactctctcctaagagagggttaattagtctataaatgatctattcttctcgtccattgaaattttgttatcctaaatttatgaatacttctacccaaaataaagacttttttttttgaaaagtgtcaaaaaaacataaagaaattgacaaaacattcatttttagtggatttttacggacgtaaatagtttgttttgtttcttttaataatacaatttttttactttaaaaaatatttttgttataaaaccaccgtatttttattcaattttaataaataaataaatgaaagaatataaaaaagaggaaggaaaaagaagccaacgaaccaacggttgccacgtatcaaaggtctaaagtgcgcaaaacgaggccttcggaaaccaaaatgcgtggcttcaattggagcaagtaaacatggaaaccacgtccattgtaacgcttcctgatctcttctttacaaccgttggattcgagtactttttctcaacgattaacgactgagtggacctccacttgcttctgttccacgcgcgtgggattgacgtgtggtccacgcaactcttctcgataggatcattcgagaacatcctttacttaaaccgcctctctctgcctcaatttctcgtcacttccttctccttctttaccctttccactgcggctgattcttcttcgccttttattctctcgtacgccgccatattcttcacttctttttccggcgaca

SEQ ID NO: 86 - DNA, 2000 bp, Cucumis melo
  source 1..2000: mol_type = other DNA
aaatcatcttctcccatttgcatgtgttaacgcctaatgtagtacatttaccatgattcctagaataagaccgattttaccaacgagaagttgctttcaacttgctacaatatacataacatttctttggtacgttattgatgagaagaggtataaagcatttcacagtattctctcagcaactcattagtttaaaaaaaaattaaaggaatatttgaatatcgggggatgaattaagtatagcctcacaatttgccagctccttctccttagcggctgccaacctccgaagctttgcagcctgtgcaaatgtagacggtctacaagaacataaaagcaaatgaatacgatccccatgacagccataacagttgcaaacaatcatatagaatgaatgatttgagccttttttttttgtaagatgatttgagccgaattaacagtgtctaatgctgaatcgagctggaaaatactacttactgagataaggtgctagcctccctcagaagttgctttattgatttgcgcaactccaattccacctggctgttggaacctccctgaaaagtacacgcatgatggaaacatgattgtttcaaaacaaacaagttgacaagattgaacggataacaattataacatagcaaattcccagacattaaaactgaaaatgtcaatagatctccacattaaatgcatcacgtccctaaactaatcaaatcaaatgtcttcaatccaatatcgtaaacttaacgaagcacagttaggcatattgcattctcaagtctgtcaacgaaatactgaaacgcgctacagcccaaacctcaaaattttcaactataaataacaagctttgaattgaaaaacaaacggaatgatagaaaatacaaacacgaaaaaattccgacgggaaaaagaaaatcaaacgaaaaggcgaaccttcttcaggtgctccagccatctagcgagaaactgaaaaccgataacgataaagaaaataaatggagcggcaatggagcttccatgctctacgattccttccgcttccatttccatttccagaggacttttctgccacaacggtgaattaatcaaacaaagaaactccgttcatcgtcgcaattcgacggaggttattctggaagaagttgagatcgtaattgggctacgaatatcatcaaaggggcttcaataaaaggtctctcaaaacccaaggcccaaaaaaacgaaaagcccagcccaattagtggagaatcaaaacgctgcgttgtagatacaaatatcttaggaaagggaaccaagttacgaaaatacccctgagtagtgagatcaatgattacctcaacgacgcgttaatcgttttatcacgtttattgtgataagttccgcactaaggaagggacgagttgtaggaagggaggggtaaactggtgatttcgcattcaaacaacgggctttaactcacgtgtccggatctgttgagagggaacaattcacagcgaggaaattgcaaataacacacaaaggaaacacaaaagagcggaaagcaaatgtgaagagacgaagagtagccaatgagaaaaaaggacgaggatcgatgacatggcaaaagatttttgaaatcccgcctaaacccggagtttcaattgatatcgcgatttatctctccctctctttaacgaaaccgactcccttcatatccctctctctcgctccctcttcacttcaaagggcttttccttctttccacataaacacacgcactcgaagccaatctcaaaaccgcatcacacgaaccaaactaagcctaacccaattttttctcctcatatttcactctcacactctttccttatcttcttcttcccccaaaccctagagttttacaggtaaactcccaatctctccgccgctccctcgctcgattctccttcgtttctccgccttttttcttataatcattacctgttttctccttccctctatctgcaggattcatc

SEQ ID NO: 87 - DNA, 2000 bp, Cucumis melo
  source 1..2000: mol_type = other DNA
gtgtagagtgagtgacggtggccgacagttcgtaacatttagttgttagtgagagacggtgagacgtttggtaacaaactttgtttttagttcaatcattgctttgttttctctttcttttccttaatgtctaatgttttcatcttcctttctttatttcttacccaatttccgaatcaaattttaatttctaaaaaagtatttaaaaaaaaaaaaaaaattagtcgctttattcgagaatttcataatcaacctaattttcaaaattaatcatcaatctggaaacttttttattttttttctcctttggattatcctgtatgaaagtcaacatactttgcactccttgagaatatttttagtggtgttttttttttctcttaataaataaaaaagtttacatctataataatcaagattccttggcaggtgtcactgtcaaaataattcctatttgttgaagttgaaaataatttaactataaactttatttgaacgtcaaaaaaagaaaaaaaaaagatatatgaattcacccattccataatttaactatataactttatttgaatgttgaaaaagaaaaaaatgaagacaaagcaaattcacctgttgccattacgacaaaatttcaaatgcgttttattttgtttttatgtccacaagattctctatttgtattctgcgaaattaaagtcacgggcttcgcacgtgtgtgattaatagtatttgtaaaagggcatgtagtcgaacaggatgggaattaaaggagattatgaatgggttgggtcgggaaggcccatttctataatgaattgatgggccgtcaaggacatttgtctacataaagggcatggaccatgaagttaagcccacttcctaaacgagttccttagtgtgtctacattcatatttaaatcatctttaattcagaattttcaccatcatcaaataatgtcttataaacctcccattttatagtttaattatggattctaataaaaaatctctaacttcaaagtggataatttttttttttttttaagttgaaccatgttcattcatttaattacatggaataaaaataacgtaatttaggttaaaagttgagaggataagatgaagttgaaaaattacaacaagttaagaagggaatatgaagaagaagaattcaaaattgagaacataataaaggaattaggtccaaagctgtaaagactaggagaaacgagtagagaagggaaggactcgtttttcaaagaaaagaaaagtgtggaaaaggaaaaaggttcattaggggtggtgaggaaatggatggatatggaatgatgatgatgagaaagaacagcacgggaagtttccgagtagttgccttttgcatataccaacaagttatctaataaaatgttttgattaattacattaatttattcaattgatttatcggaaatttccatactcttcacgtgatatgcacgtggtcttcccatgttctaatattttttgtttttgaaaatttgaattcctactctgttttgttattctgctcatttaactactcaaatattttagtttgtagatataactttgtaaatttttattataacattttgtaaatattttaaattgtgcccatagattatgagtagataaatttacgaattaaaaaaagtttaattctcacttcaatttaatttttttttattattatccaaatctatttgtcgcagtggggaaaacggggacgtacggccgattggagtccaattagtggatgtgaaacgtggacggtagagatgcaatatgaagctggacatcaactttgcgaaggaattgttccttctttccctctgacgcttgtcccgttattgctcgttttaaagcaattcgagctccgcgttgtctcttccctcacgttttcctttcaatcccactgctcctcctttcaccaataaaacaaaaacgcctcaaagaagaagaagcaacgaccagaaacctcaaaa

SEQ ID NO: 88 - DNA, 2000 bp, Cucumis melo
  source 1..2000: mol_type = other DNA
gttcgagcatgtgaatgtcttctgttgtttgatgttagaaggaaagagatgggttagggagttcctgttgatgtctagtaggttcttttttttttctcttgtgcaatgtaacatagtaacttcgctgcaaagcagctcttatccttagaatacgaaaatcttctgttttttgttatgtttctaactttatcccttcttgattttaacttttgagttaaattccatctctctgactttgctttgtggtattctgtttctgttgtatgataattcttatggaactcctatgctctctctcattgccttctttttcggctgttacttaattactttcttcacttgaaatttatagcttctctcacaaatttgagctcattcaagtatcaaaattacacccatctcataccatatttctatctctgaaggaggatttttccccttttaaggagggtagattgacaaagctgatagggtgagacaatttaataactcaggtcagatgaattatacattgaagaactctcatccagggccagtgctttgtttataacaagatgattaatgtgttgctatcaaaactttgctggttcactaaaaaaaactcttggtccttgaaagtaggcttttactagttttagctttaatgcacatctgtatgtcaaccacgaactccatttttcttacttgatgcatgtgcaactttagcagctttctaagttcatatcaaagcaaatgtacctttattcctattgtaattccttttctgctttcctcttttatgaattgtcaaaaatatggacaggaaagtaagctgagcaccaacaggttgtacccctttttcatgtcttgaaaatgaactaccaggacacaaatcagatgatgattgttgggagaaggaatgtaagattattcgttctgtttgatataagagatgtaagttcacatgtcttacaactttttgaaatttgtgtgtcgcttatgtgcagattcctgtatgtcattagtggcatttgtaagctacaattgttgaatttttgtattattatcttaaaaggaaatgacaaaaggtataatcaaatcaagctgaacctaaaagaaggtacaggtttttagtattatgcatgaagaaggtttttcatgtctcttctgccatttggattttgtctgtgacaagggactaagacactacacatgatgctggaaactgcaagagtgtttttaccctaataagattaaaacgtgaaaagcaattagattttcgtgcatatctatctttttgtgcattccaccaaactgttcgatcataacttgtcaagatcttgctttttccttttttttataaatattttaatatccttctaatgtgaatggtgaaaagagatgcacaaagataagtgatactatagatgtatctaagtattacccttatacctttgccacgtaagattagatacgagaagagaaaaaaatctatgagttagtaatagggcaacaataaaccacagaaaaaccaattaatacctttcctcattgtctaataatatctaaaagaaacttcttttcatgttaatgaaccaaactatgttgtgctatagcatgagcacattatttctaccctttagacaagtgatgagaatggacaatatttcgactgagttcaccagaatgtaaccaacggttttgcatttgtaatatgaatttgaaagtttgagattccttatacgaggaccttttttcatgtatctaacaacacgagaaccaccaaaatgagaagggagttggtccaagccaaaagaattttgacctccatgaaaatccagatagtggggcatccttatctaaacaatcagaacctgaagtccgacgtagccttatccacatttcaacttcaaaaacactccctctaagatcctttcgaaccaccaaaatctaagaaaatttctcttcctcatcctcctccgacacaaaatctagcttcaatttcattcctctgtaaaaac

SEQ ID NO: 89 - DNA, 2000 bp, Cucumis melo
  source 1..2000: mol_type = other DNA
attcgtcttcgcattatcagtaaatttatcattttaagagtttgttcttttttaaaaaaaattaatcatttcgataaagttggagaattcaaaaatttctccaaataatttataaaaactttcggttatatatcgaaaaaattaacatggtattaaaacgatcataactcaattaacataaacactccctctcaactttaataccaaatttctttattaacgcaaaatttaaaatttgtttttaaaattttcacataacataatagaaatacttttctttatggcaaaaatacaataatcaaaattgattgatggtgacaggacaccacacaatatttttaaattttgaatatacgaactatataataagatatttatgagattcccatcctaaagattcctagagatttccttgtgtacaatattacacaagtatcttggaagtccaaagtcctgagaaaaaagctatgtataaagtaatgtgtttgtcgtaggaaatttacttcattcgtgtcattagctttttattgaaaaaaaaaattaggtatatcttagtgaatctcacttaatcgttgtcgatagttattcttttaatatcattatatactaaaatataacaatattgaaaagctaaaactgtatataaaaaaaatgttacctctaaacttttatcgtttatttaaaagataaatatattctttcaaaacttacaatcaacatcctacgactatcattataggtacaaatcttttcatgtttacacaaaaattagatttttaaatggtgtaatgatgatatataacgaaattttgaatgattactatttgaggttaccattgtaattggtcgtgttgtttgaaatttaattttattagaaaatttgtcaaaagtagcaaaaatgaataaactatttaaactttaggataaaatcaagtgttatgagtttttgtctagtttatatatttttatttttattgaaaacccttttcctatcttttcattacttcaaaatagttttaaaatgtctattaaggctaaagttagtataaataaaatttcggaaattttttttcgaaaaaaattgataaattatttatattttatattaaagtcaaaatttattacgcgtagatgtttatcaaattttctttctttttgttgataattttccaaaatttggataattttttaaaatagtaaaattattaaaaaatgaaaacaaactatttataccttaagcaagaaatactaaaaaggcaaaaattcatttacttcatgaagcgtaaaaattaaatattttaccactttttgttattttttaccatctctatcaattatttgtaaaaagaaaactacaaaattagatgttttttcttttttaaggtttaatcaatattaaaatttcttaaattggcagacaagttggtgttggtaattacgaataaatcccgaattgactaaaaataaattcttctccaagtaaaatagacacgtggatgaagaaataagtgaatcaaaggcatccacagttcaataaatggaaaaaactactttctgctgactcattcataagttttcataaaatttcataagaaaggccaaagggcttatgaaagtgaatgtcatagcagtaaatgaagcacagcgccattgaaagacaactcaaattgcatgcaaacccacataattattcaacaaacccacatcaaatttcccataaagatcaattctttagggggttcaattacccaaaagtgaggtagttgaaaaccattaaacaacaagaaatcaacaattttgtaatttgtttgtacagaagtaagagataaaatcatcgttaaccattcctttatttcgtaatacaacccatcaaccatctctctctctctctctctctctctctcggcctttatctttctcttcctcaattaatttaagtactacccaagtgagctaaaagcaagttcagtggacagtgttgtaagaaccactacagaaaa

SEQ ID NO: 90 - DNA, 2000 bp, Cucumis melo
  source 1..2000: mol_type = other DNA
aatcatcaggtctccttccaatgaaaccgacgacaacgacagtgtcggaaaagcgaggaagggatggcgaaggcgaggaaggagaaaacgaagtagagggttccggtaaagcagaatgaggagggagaggagttggggaaggtgaagaggaagaggaagtgggagttgataatggtggcggccggataagtactcggacagaggaggaattgggtacgtccatggatgagagaaaattttgagctttcagatgcaactgaaaactgcttcactgctttcacttccgatgaccgccgaggggaaacttattttttccttgccctttttgcctcctcaatattttccttttaccatttcctttccaaatttatttttctatgttttgattttatgttttgttatatttttgatttacttttacgttatttttaaatatttttgatttaattttgttatatttgaaaacaagatattcattatatactgtaaatcttactttattattgtttaaatgtcgttttggtaattcaaaattaagttgaataaacacaatattttaaatattattttagtaaaataatttttaggttggagaatggcaaaagaaacaaaggattgaaagactgaacccatatttgaggatagaagtcaaagccaatgtcaataagtgaaactcacttggaccaaaataccaattttagttttatatttttaattgttcaatcttagtttccatactttcaatgcatattaaacttatagttcattattctttttcaataaatcttaacattttactacaaatttttaaaatgtttcacatactttatttttttacatgaaaatgattgttattgtttaatccatttcaataaaattaaaatttgaaaagctaaaaattcaagaattatcgatagacaattacaattttgtcccattaaaattatcaaattgaagtggctacacaatggaatggtaaatcctttattcttgtattggtgtgatttggattgagatatgaaacattataatctaaaggaacatgtttaaaccgaacatcacgtattttgtctttcaaaatttcgtaagtttgtaggttgttttttttttgtcattttatatagttacaattatttaagtcagatcggataaattttgttatacaccaataggaaactaaaaattccacaaggagtatgaatgacctcctacgggagcattaatgaaaatgaccaagggttaaaaaatggtaagaaaaatgttcttcactaatgacaattcctcgtgaaagtactaacatgttcttaaaatgcttgcaagcatatatgtcaccaagaattctcattcattcctctggcttctttctctcatttctcatcaacattaatatgacacactttttccttcttctttttgtatgtgtttataatcttactcattccttattctcattgtcactcaacgattccaacaagcaatatgggaacaaacgaaggaagaagagaaaaatacactaagaagaagagatgaacaaagttgcattagaacaaggcgtagaatatcaaagaattcaaaataaaaaggaaaaaaagattactagacgagagagaacgagacttgaaaagaattagaataatttcggtaattttacattggacgacgaaagcaaatgacaaaaacaatttttttttcaaaaacatagctcaaatttcatttagatctttcatcccaaatggcataatttctctaatttcacatacaccacaaatataatgatgactgattaaacgaagtaaattacaataggactaaatatataattaaacttcttaaattgagtttgagataaaacctttgaagccacgaggggtcgggtcgggggcgaaagagacatgccatataagcagttggttgctgtaaagtggcacacgcatatctactggaagcctccatttccaatctcccattatcccattatcatcggcagttccccatagcta

SEQ ID NO: 91 - DNA, 2000 bp, Cucumis melo
  source 1..2000: mol_type = other DNA
ctttcctgacccaataagagatcaaatcactgtctcctgtagcctttcccttgccgctctattattgacatttgggcctaccttccccccccccccttctcccgattcatcacccttgggccttggcccattaaaacattacccagctccttactactttttaataactatcacgtctattccttcgcaagtgggtggaagcgaatatttataccaattatcttttggttgatcatgtagccaaaatttggctcaccaaactcgtacaaagacatttacttgttttccactgtagattttaattttggaagaagagatcagttgccaatagattgaattaatgcatttatgtacactttcatacttaacttttggcaaagagttgaaagcaaggttttaaagaataaaatgaacttactttttttacaaatctcatgatttacgctagctcaaacttaggatttctttcgtttgaaaaattggaccaaatatatatacaatagattgaataggagtcttttaaaatactggcctcaaagaaatagacaagttagctaggtcgggataattgcctcactcattcttcacctcagagatgcctctcctcctaggcatgttttctaccctcataatttaattcactcatttttgcttccttattgattagtaaaagtaccgatttgccttcttttctatgttgacaagttcccactagaaaacaaattagattatgagtttataggaaagaattaaacacaaatacataagtcaaattgtgaagtatcaagataggctgttaggacagaaagttcaaatttggaaaacaaatatatatgttattgagttgtcatcttcttagataatgataaaatgtgaacttttgacacatataataaatagcatgttcttgataaatagttttccattaaaacaataagctattattggatgatagaaactcccctgggactacaagaaaaagctaaaatagaatcagcattaaaacttcctttaataggatcgttatcccaaataacaactccatctcaaaacacttctaaagaagtagttaaagaataacaatgtatattagttatggatgttgatgatagagaacttggattttagctaaatttagaatcttaaaaagggaaggaagaaaaaaggaacaaaataaaaagataacagtatgattactccaacttgtgatgaacagtaccactcatggtatgtcaaacatatacatagaatgagaacaatttagatcaattaatttactcatttatccttcttgctacagattgttgagaaaatagaaaaacaaattaaagtaggaaaaaaaagaataaatggggaattatggaaccaaaatatcaagaaaaaggaggggcaataaattaaagaggaatagtgtaggccttctcacagtggaagtattagcgtttaagtcagtaccttacctttatttgttttcatactaagttctttctctttcatgttaataaattttcaatcgatccatctattcaaaatggtgtgttttattaggaagaaaggtaatttcatacaagaaggctaaaaaatagttgacagctgtgggatttgaacccacgccctttcggaccagagcctaaatctggcgccttagaccactcggccaaactgtcggaattgtgagttgaataactaagatgatcggaaatgtgacgaaataaattgggctaaagaaaagaaaagcccaaacaatgaagaacaattcggcccacttaatttcacgcgcatggcacgtgtaaagaaatcccaatctgttctactaggtggtggtggtggcgaggcgaagcaaagcaaagcaagatcagccttatcaaattgtgtggtgaagaatgaagattgtataatgtagatagaaaaagatccccccattcccattcccattcccttttctgaatccgccattgttatctctctcagacctccataacctccatttctacccagcc

SEQ ID NO: 92 - DNA, 2000 bp, Cucumis melo
  source 1..2000: mol_type = other DNA
cttctaaacatcctcaatgttcgattttgatcaaggtcgtttgcttctaaacatcctcaatgttcgattttgatcaagaggtcgtttctctatagtaaacatctgttacaccttccatttctgttattcaatttttccaattttattgagcagtttatttatttccgtaactactttgcatcggaggcgatcatcagtttttaaggtacaaaactagattatatataattatgaagcacagcaaagtataaaattttgaagatgaaattgattggaccttgtgaacagaactctaaagagaaaatgcatcagatagtctggatcgttagaatttgaaatttaaatttctatcttccactaaagatatctctgttttgcaaactaatgttcctcattctaaacagagaatgccagtggtattttgttcgttttttgcgaatatgattaaattacccattttatttgcatattttatttattctcatatcagctccaaaagaatatgatccctttttcctcgataagaaaaaatatttaatactttcaacttcatgcattgtgagactgcccatttgttttgtttaaagtagcaccaacttctcaattgtataagtttgtgattttttttctatctaaattgacttgaattatttttagatataattaaattaattgcttttaagagcaagttaaattaaggtttcgtaaggatatggattaaatttaattaagaattggcttcttgctctaaatacaaattagagtgagatttgaaataggaggaaaaagagagtatggttacaaaggatatgaaagatcaaatttcaaacctttgccaactgaggcttttcagaactcttaaaccatcacagttttttctttgcccaaatgaaatcaaacattaagaaacagtgataacgaaaacgaattatccctatgccaaccgtgacagatgataggcaagaaacccacgattagtctctcatccggattgttccaacaaatgaaaaagcgttttctgagactacacaaacaacaaacacagagttagatagttcaagcaaatgattctagcagattagaggataaggtttcttattaaatgtttgaatacattctaaccaaaaaccaaaaaccctatttgcaaatcagcttatgtaaaccaaaaacatatttactaagaattcagaatttcgctgcttgaaatttgaaggataccatataaaacaataatagattcccccaatcgtgttcagtagctcaatataggcaccgtgcaaaaggttgtttgttgtaagattaatgaacaaacacccgtgtctgattttaatgccaattcaaactctaattcaaaaaccctacaaagacctaattgcagataatgggattagaaattttaaaaaatgtcgaccgggcattgtatcttaaaactattaagtttcaaggatcttcctccggtaacaaaatatcggctccatgcggcagacggatcgccattaaaacggcgcctgctgctgactcgatgatagagccaattcagaataaccaacccatttcatcgaaatttttaaagagagagaaaataaacgattcaagatatcaaacgcatttcgcttctattgaaggagaagacaatgaaaatcaaaacaaatcggaaattaaagttaaagaagaaggagataatctcaggacggacggaagataattctaaaggtgcgattcggttgaaatttatagaggatttgtgaaggaaccctaaattctgattgtgaattttatcggaaagaccggagaggaagcccattgtgtgaggcccaaagtaactgatctgggccttttttagtttcagcccaaacggaagcgacacgtcgtttctatgtagagccaagagcgtgccacgtcaacagacgacgtcggttagtaggaataataccgatttgtggatttaagaattgttcatttcggtttgtatcggaagttctgaatcttgatccgtggca

SEQ ID NO: 93 - DNA, 2000 bp, Cucumis melo
  misc_feature 1..2000: note = n=g, a, t or c.
  unsure 1..2000: note = unsure at all n locations
  source 1..2000: mol_type = other DNA
aagtagaaattcagcgaaaaatgcagatggtttcatagacaataaaaagcaggaacaagcgcagagaatggttaatcctccagaaaatgtgataaaaggcgccaccaagaccagtaatccctttaccaatcacagaatactcaacaagaaaagcgattccagcaaaaacgaagatgaaactctcacttacaagaagagggtcgacattttcccgcaaaacgatgagaatggcgagtgcccagaagaagaaaatggccagtgattgctgggagaatgcgaatctgtaagtggggtttccggaaaaagcgagaaaaaggaaaatttcagagaaggcgacgatggggaggaggaggatgagggaatataaatcgaaatttttccatttcggttctgataaataccaggtttttgatcggtaaagagatgggttgttgaggtaaatggaggaagaacagaggaggcgacgaaggccaatggggatgaggaaaagggaggcggagagatgcgttgctagtgatgccattgaaagggcttttgaatttgttgaagcattcagattcttctctgtctatggttccgtagattgttctccaattcttccattgggaagacggagttcggtggctgaacgttgaccctaacaagtttgatcacgttgatccgttcaatgttaaacagctcgatgattttcgtctaaaaaagaagtgattttttttttaacctttttattattgaacaaaaaaaagatctgtttataccatagtttacgttcttccacatgagaagttttataatagtttatagaatctatccaaattgtgttttattgggtttcgattttatagaaatgtcatatcaaaaaaaaatttaaaaatgataaaaatcattataattattttatgaaatttttactgtgacttaattagattataaaccgaccattctttaatcattattttggatgtctatcgtatgtgtatttatagatgtcaaacatgagagcatagatttaaaaaacaaatagcttaaacaaacaacaataactttttatctttcagaaaagnnnnnnnnnnnnnnnnnnnnnnnnnnnnnnnaagaaaagaaaagaaaagaagtcttgaaaaaagtattaaatttcacaataaattttttaaaataaaatacattaaatggggatgaggaagaaacaactaagagtccaagaagagaaataaaaaatgagaggtggtgttttttttggtatgttaatcaaattatggtctccacatacaagaaatgaagccacgttaatgacccaacaacactaacacatcaattcttaaaattcaattccttcttttcttcccttccaaaattatgggtcctccaacttacaaattaacaattgactttagctaactatgttttttaaatataaaaaacgaatacaagtcagtttaataggacttgaagattgtataaaccaatattagacaatcaaaacaatcaattttaggttcattcccaacgatacatcaatttggattagattaatttttcattatggtttgatagagtggatttagttttagtggaatgcagggagggaaaagtaatttgaaagaaaaggaatgaggttggtcaattccgaagcctaggtatccaaatacaagaatccatatcaaatttatgaacacctagaaaataatagtaattttaataataaaatggagaaatggggtccggtcgtcctcttcctcgcggcggagatgaagccaccgcgataagagaaagagacccttttcaatacaattcaacaatcacatgaattattccaattcacatctctgcttttgaaactaaactaaacgccaaaaacccttctgtggctcataagtttcctctctcaaatctccgatttccctcacccacatcccacatttcgcatccaaataaaaaagggacacggacaacaagaaggagtttttaattcagtagtgcctctggaagaagctgtttca

SEQ ID NO: 94 - DNA, 2000 bp, Cucumis melo
  source 1..2000: mol_type = other DNA
ttagtgaaagttcaagatgtaattcactctctttaacaaggttgtttctttgcttcactacgcatcaattcaaatatttagatattgatgtttaagcttaatctcctatcttagctcagaacaaaattgtcaaaatctcattcttatttgtctacctggtaactttgctgctatagttatttgtgggagattgtagcaaatgactgtagatcgaaaccatttcagcatcaatttcgacccactcttctcgtcaacaacttgatcggcagcttcgacattcttcaagcgccagcttctattggatctttagctcaaccacatcttcgtctttgaattgcatgtgagctgttgggctcctttcttttgtgcttatcagttgggagattattactataaatacaaagcctcacgggtattttaagacacaacaaaaaattaaaagtctctcctctgaatcaccacttccattttctataaattttgttctgagcaacttttgtttgtttctatttcttattctgaagagtgcatgtttgagtatggggagtaatgttaaccttgaggaacaattggcaacacgattggcacctcggtcaatcatagttgcttttaggacagtggttcgtcacaacacaacaatttattttaagttcaacattctcattcttttcttctacagtattcaaagttatagtgtttatttctcttattgttcctttagttaacaatctaccctttaactaaagtaacaacttaaaagtaaaatggattattctactttttcttaattgttacttttaaaggtttaagaactgaattgttactccgatgaaagtctaaagaccaatagtggtttctatccttaaaaaactattcaatgaaatttatgctaaaaaaataatcactaattcatcgtgagcttccaaaccacttgaaattagctcaatgagattgtaacttggtcgggatctcatcaaagggatggtcttggctagattcttaaagatcattttagaaagtagatcatgaaaggttgcaaagatgctagaaacaactgggttgtcgacgttttggaagctaaagcggtgatgattgacgtaatagatatcactaaacattggcacaatcatacttggaaatagcttctatagatatattccattttgtaaggtcttaaagacaagaacaaagctacctataagcttgtatcttagtttcctcttgcgatcttcttgtcgagagatgactttccggttttgggttgtgtctttgtttgtttttctttataaaaaagtcaaaacaaaataaatttggattaattatcctcgtactgaaatcaattggtttggaactaagtaacaataggatacatgcggcgcaccggatcatgccattctccctctttaaatatcaaagcagatccctaaaccctaacaaagatccaaatatcaaacctcccctcttactacacgctccggcacctccaaaactccatctcgaggtttgtcacttttatgttcttgtttttctttatttagaatatgatgatgattagaccgatggctattttctttaaatgcctttactcctctgactagagtggtctgtactctgaatcagagggttcatttcgaatcttcgaacgttgtatttcgcttcaaaagctagacttttcccaatttacttgaacttattgtaattttagtgctagcccattgatcttggtctccaatgccactctctgttccgaataactgccgattattgaggggttttttttggacttcatgatttcgagttgttgtaaaatgattggggattcatttaaatatgaaatatatccatcgtttatctcaaaagtatatatcttaagataaaccatgaacaagaagtttccgatctaattcccatgggttgtctaacgagttattctcaacagattacgaactgataactagacgtttgaattttggcacagagagaaatcgcatcactttgaa

SEQ ID NO: 95 - DNA, 2000 bp, Cucumis melo
  source 1..2000: mol_type = other DNA
taaatgggaaattggaaactaacttgaaacgaccacaaaccatggggacttaaaaaagtgataatctaacaaaggctttacactcctttttcataataaagaacaaaaagaaagctcaagagcaatcaagtttatcataactaattaaagtcaaacactacatttctcaaaagaatgatataaaatgaccaaacatctagctgctttacagtgtaatgaacacccaccattaaaggaaccaaggcaactgaataaattggtaacttaattgccctccaaatcagagtccccataccaacatcctcttccccattctcttggggcatcgaatcaacctccatcgctttacattccgataacaaacctctaaaacggacatttctgcacaaccccaattgcgttctacgactcccgcaggcaaatttatgagcatcagtcgacaaactcgatgaatttaaacgacccagatgaaagctgtgatagtagaagagtcaagaagataaatggggctaaacgataaggttttgaaagaagatgtagttgccattgtgaagtggtacttgccttggagtaatggtggtgaaggagaggtggtcgttgagtttgttctttagggcgccgagttgggtgggtatgcagactatggaggccattggcatcacatagctgaagatgaaactgcagagtgaagctgcttgttgaagcagaggatggattaattaaagtgggacgattttagttgtgtcttatcttcttcaactttatgtttcctcttggtttgacacggttttaccattatcgctaccattttaagtaacaatagtagtgatgaatgggtaaaatataaatcttattccattgttagaaccttcgacaagttttccattatgtgtggctgtgtttgacccaccaactcgagtagagttgaatttgtttggtctactatatttacaaactaatattaaataacaaaactctattaatttcatcggtgttcactgttgaaatatatacatttagtatgaatctttatctatttctctcttacccttcctctaacatttctagtgcctccatcatcaattgtcatcaacgacgaaatgtgacgataactatagtcaacgagtatttccaccttactttgacaatattcattgccacaatatgctcttgacgacctctagcactccacgtatgataaagactacatttgatgaccaattaaggaaatcgtatttgacaccacattccaatggctatctctagtgatcaatttcgactatcacttgtggttatcgactttcaaccatttctaacgactaacttgacgaccatcttaatcaatcatatactagaaaaacaaaaaaaaaaataactcatcaaatggaaacatttttaaatgcaattttgaaactaccacttctctgtatttaatagtaatttgacattaacaaaaacacttttaagtacataaaaaaccaaacaaacttgtatataaaacacttttgaaaaaaacggatgtaaccaaacacacaagtatttttcttttagattatgttttaaaagatagaaataaaaatattaaaagaaaagcacctttttacaaacatgtaaatccaaatcaaacatgctattttttaatactaaaagaaatagaaaaaacatgttaaacatatccattagcaaaataaagtgaaattccaagaattagaaagatggtttgaaaattgattttataaagcgaagaaaaacctttttccccaaaagaataatattcttattttggaaaaaacagaaaacaaaaaatgtgacaaaaagttacattcctgcggatttgaccctctggtggctgcattcgaatctttgatttcgaataactgaagtaaacattaaccaaagtccgtcgaaatcttcctttttttcatttgggattccctcaatcttcatcaccaccatcaccatcctccactttcactctgtttccctccaaacatcaaaaa

SEQ ID NO: 96 - DNA, 1373 bp, Cucumis melo
  source 1..1373: mol_type = other DNA
tttaaatgttactttgatatgatctatgtttagatttgaagtatttttctcatcattaaaaagaactacacgatcgtattcatttagaagaagaattgtacgtacgcgtgtagccgattaatcacgtgttgagtgaaacattttttatatttttgctaatagacctatatattgttttcatttttaaaattgatatgtaaatattttggtttgttatatatatatattttttttggaaaaaaaactcctttatttatttgtcgttaagtattaatttctttttttagtacttttattaccattgtggccttgttttgctcctcaatttagatatttattatttgtggtttatttatttcttttgttttcgggacaagtgatgtttgggatattaaagtaaaggaaaaaaaagagagatattttgattgtcaaaatgtcagaaatatctaaacccggagcttctgccacgtaggcatcactttcattaccttttataaaaagtacgaattgaaccttcatgacactgctcccctgctcccttatataaaacccaatcctcttccatgctcagtattatcttcactctttgctcgaaccgcgtgtttaacagataagattcaactcacaagcattcatcgctaggttcttccaaacaaaaaccctacatcttttccatttcgcctccttaattctctcatatttctgtatcttaatccattctaaaactacattttaatgcactgccttgtgttctgtattccactatctgttatcgttttattgcgttttctttgatcagatcgctttgttgttgcatgaactgctgagttcgtttgatgattttgtttgcgcttcagttttcatcgtttgccgtccagattgtttgattggcgagagtgaagtgaaaattctgtatgatattggagcgtttcgtgtaaaatctgtcttgtttttctattatctgtattttagtgatttgtttttcgttgacgattttgtatgacgtaaagatattgtccattttaaaggattttcttccactggttactagagatcttagattgagctttcattcggctgtattttgatgatgctttttgtgtttttttttcctttctttctttagcttttgcggactcatggagtctttttctgaacgacatcttaagatgtttaagatgcttatttgcttttttctatttttggtatgacggggtcgagtctgattttgaacgacatgttaatatttatgatatttttgaagctagttgtgcttgattctgaaaattgcttttgatacacgagaaacttttttgttttcttcaatggtaggattttgaccattattattattattttttaaaagatcaaat

SEQ ID NO: 97 - DNA, 2000 bp, Cucumis melo
  source 1..2000: mol_type = other DNA
ccgaattcgctattgggctgcataactttatcacttgctgggagactgcaatttgtttgtttagtgctatgtagttttcaagtttactaggctagtatgtttgtattgcctgagagtgtgcatcatgaggtggataaaattcttaggtcttatttttggaggggtaaggaggatggtagagggggtgttaaggtggcatgagcggaggtgtgtcttccttttgaggagggcaggcttgccatccatgatgggccttcttggaaatattgctatgtctatgaagattctttggtcgctattggcgaattctggttctctttggtggcttaggtggaggcttacattcttaaggggaggtcgttatggacgattgatagtgaggttggttgatattgtgtcttcgggctatcttgtgtaagtgggatagtttgaaagcacttgttcctatggaggtgggggatgggagaaggtgtagagtttggcttgatacgtagttgcatggcggtcctatccttgattaggttggggagagggtgctttatgacgcgacgagtcggagtgaggcttgactttctaattttcttggtcatgatgaggagtggaggtggccacgagtttctttggagttggttaacttatgggatacggttcagactgtttgttcgtgtcttagtgttagtgataggtgagtatgaattcctgacagtcatggtggtttttcgaccgcgaatgtgtgggatactctctgtcctcgaagtagtcaggttccttggactggtttattgtggggtaggggggaattgttttccaaaacatttctttttgagtttgacttgccatcaaagataggttgttctttttgtagttctttcttttggtgctttttgtttctatggatcctgtgagggttttctgctctcgtgccttaaactcaggctgtgaggtcctccttgttatggtataataatattaccttttcaaacaaaaaaaaaacaaattgattcagaatgatttttttttctttcttttgtatttattctatgtttccttattcaggctactagatttgaatatgttatttgttacttccttttctaacaaaattagttataattaattttatttggtttctttaaaaagtgtggggttgaagcttcttgcagaatataggatcacaaatgcctaatacacttctttctacttctttgttttgcagcagggtatgaaaaaacaaattaatatgtattttttatacttctttctcgtatgcattattcttcttttgtttctgttggctttgcattgtagccgttttcttgttcttgtctcattttttctctaccttttgtttcttctctaaattccttttatgttcatttttcataatgcggattttttcaaaaaagaaaattatagttgttagttgtgtttgatgagaaacaagaaaagagagtgaaaagagaaaagaggtagaagagaaaagaaaagaagaatctgagtagaggaaaaaaattgaacaaaaaagttggaattgtgttggatgaagtgagagcaagaactaaattttgtttgagcgtcaagcccccaccccacacgtttctaagaacaagatggtaattttaaatacaactaatataagcaaaatacaatttctcgaggaaataggaaacttcattccaggcttcaaaggaaaaaagaaaaaaaaagaaaaagaaagtaaaacgattagaacgtgaattgcacgtcactagacaaaaccatcttttggtagagaaaaacacgtgattacaaaaaacaaacgaaacccaaataaatatatatagaaaaaaaataaataaaagaaatagaaaaatctaaaaaaattgggttagcgggcaaacaagaaacccttgtttcgatcccccaaaacccccccaccctttctcccatcttctttcttcttcttcccttccccatttttgaagaaccaaccagcacctctgaccaacatttgcttaccc

SEQ ID NO: 98 - DNA, 2000 bp, Cucumis melo
  source 1..2000: mol_type = other DNA
tagtttggttcataggttatagtttccaaatttgttaggctatcattaatcaaacacaatacttctcttgtaggatggctgccccctatagtacttttttaacttaggagaaggatataataattatattccttttagaaaatataataataattgtgtagtgctttgatataccttaaattagctactcacgtttttaggaggaagcttccgttgcttttcatggtgttatgatcttttttattttataaaggactgaactttaaaatttctctttcatctattttggattggattccatctattttatacgggaagtgaactctaagatttctcttcacctattgtgaatcggactccgtcatgtaggtcaagactacgacagataagaatagacttccacgaaagaaagtggtcaatcgagatggctatatttggctctttcagctcaatttcttcttttttccttgcatgttcttccgttggtacatttcttgcactttttttgttctcacatgactaatgtattccaagtttatcattggcattgtgcctcttttaggcttgtaaactctcgatccaaaattatctaggacatatgtttcctagtgaagaaatactagtatattccttatgtcaatatgtcaaaattttcaatttcttaacctttgagtaaatcaatattatatttttatggaggttatttataattggaaaaaagttacacccatctcaaccctaattaacaccaaatgaaattgtaccatgcggcacaatatttttttgtgagttttttgcaaagagaaacaaagtagcagacaaagaacaaacattcccccaaaaacagcagagaatacctaagagagaatgctctctcgtaaaaaataatacccaagaatcttcccaaaaagagggagtaaaagagtccaaaacaaacgaaccgaagattgacaagaagggcactctcgccctccactgcgccgctaaattgtaagaagcatattttcttgagttaacataggaataggtgtaactcaagagaaatgtaattcgtagaattgaactttgtatattaatttatatggtgttgtagatacaatctttagtatttactcatttggtgctttctctcaaatacaatttaaacttagaactttttgatcttcgattttcaggaagttggagttgcaaatcaattcgagtttcaatctctggaatttaataaaagtttgatcttccaagttttcaatctttcagaagacgatgatcttgatatggataaaaaattgcacatcatgagagctttttgaagtttaaatcttcaattctctagagcttaaattcttccttaaaccaaagatcaccaaatgaatgacaaatgtctctatttatcgaaaaatttcatagacttttagatgggcttaggcacattacttgttgggcttggacttgggcttatttgcttggcgggctcatgctcgagcccattatttctttggcctatttttcatgaggggcttgaacttggttgtatacgaaaaaacttgactacctaaatctaatcaaattataatcatcacaattttgacgtgttacgatttaattggccaaaaattcttgttcaacacttgtctctaatcattttcctatataatttaactaaaatatttaactttaagtaacttaaaagatatagtttaattcgaatcaaaatacaaatacaatttcgtctatctattcccatcataaatgttgattgagattcatattataaacttctttcaggaaaagaaagaggaaaattcacctaaaccacgttttcctattttggtaagaatccccaaaccataaatcattccaaaattattttttttagaaaaaagaaattcacatggcgtaaaatttcagccccgtgagatattttcgaacccccagatacaatctacaccgtgaaaacaaaatcggacggtggagattgctataatgtccgtttagaggca

SEQ ID NO: 99 - DNA, 2000 bp, Cucumis melo
  source 1..2000: mol_type = other DNA
acactttgaaagtccatttgagagattagggtaaatttgagtgaggatggcgtgatgacaacgataaaagtgaaaaatgtcagatccaagagagactcaaaagtgaatgacgtgaagacaatcggaatcgaaattgaaaaatcagattttaaattatcttaaaccacatattaattaaatttcgattccagtttcaatttggtttgctgtgataaaactaaattcttaattgtacctaattttctattaaataaataggtaaaaaaagtatagtaaaaatattggcgtcgcccggactcgaaccggagaccttcagtgtgttagactgacgtgataaccaactacaccacgacaccgttttgttacatgagtaaaatgtttcctatttgtctaatattattattactactactacttcttcttcttcttcgagaaaaaccaatttctatgggtttaaatttccaaattgatgttgagtgtatcaataatatagcactcacatgctacttaacaaaaatcaattctttctttttagttaaaaccttttcttttatatttagtgaaaggattaagctatgttctacgttaaattgttataaacaaaatttgattgttacttatcgagattaatttatttaagtggatatgttggaatatgttactaaaatgataattgatagtgatacgtcgagtttatgctaaacacattttgatatggttttctttttcaatataataatttgacattaattacatttttttttcatatactctcaagaatgtttatttttattatgtacttttaaaaattaagattttttatggttttatccataaatttgtttcattttttaatcgaaattttagtattagactttagttgttaaagatcctaaaatatagtcattatattttattaaagagtctccgtcacgtgtataaattaaaatagtcttaaccgttaaaagtatagtgaacaaaatttctaacaagaattggatcggagtagaagggtgattgattcaacatgatccttgtgccattattgttgttactcaagggacgttcatcaatagataacttgaaatcaaaatggcataaactattgctcagttgaaaggttgtttgttgattgaagagttaggtttggatatttgggtggaagccaatggccttgtcgtggttaataaggtgctttcatttaattttgcactctctcctcatggggtttattacactaaagtggttcatttaattgagagcatattggacgaaaataaacaattaagactaaggacgaaagtaatatttaaacattattttaagaaaaagtcattttaattcctaagttcttttttagtataattttcatttgtttgctatattttaaaaggttacgcttttatcaataattctttagtttagttttcatttgacctataaattttaaaatatcacctttttccttttatattttgggtttaattttccttccttgcattttcatattttacactaatacctttaaacaactaaggcttactcctagtctttgaaggttaaacgttgagtttcaactaattgatttaatcatctaaaattttgagatttttttaaaagcaatgattaggtgcagtcttctgcttcccatttatttatcacgtaaaaaaattataaaaaaatcattttttaaaattgttacctgacaattttttgagtgcaactcgaactgcctatcgttgtaacccgactgtacctaaatattttcaatattttaaaacctttgattaaatgataaacaaattaaaactaagggggaaattacattttccttaatttaaaaacaattttgttgataagatggggcctggcccatgaggttttgggctgggccttttcgaatcgtctatttataatgagcaaacgagtctgagcttcgaagaaatcccctttttttcacttgcgaaagagacgaacaaacgcaaaacagtcgaaggaag

SEQ ID NO: 100 - DNA, 2000 bp, Cucumis melo
  source 1..2000: mol_type = other DNA
tgttggcaatgatttctttcagaaacttttgccaccttaatgcttgcgtagtttcaaactaaatgctgattgctgtcagtaactgattaaattttgatttaagtatagtagctgccttattgtgttaacaagtttctccatcattttttgcattgacttgatgatttgacttcttttgggtcatatctttgattctttccatgtttgaaagttctaatttagatgttggtttgtatagccattgagaagtttaattggcaaaacattttatagcgaccttgacatagaagaagatgatatcttcgtttctgatggtgcaaaatgtgacataacacgacttcaggtatgatttgttttagtttggaacatctttcatccatgtaatatttttattttcctcattttttttgaactttaatgttggttactaaccttagttaaatatgtaagatagcctggtaatcgtatctttcatcttgttactatttaacttctcttcccaattttggcagcttgtttttggatccaacgtgtcgatggcagtgcaggacccatcatacccggtgattttctcttctcattaatgaaaactttcgatgattaattggtacactaataatattttgcctgtccacctatatatcagacatttacttaaatgatcatttgaaaaatatcaagctcttgggcaatcattttgtgtgtctcatctttactgttgtgcttgaatgagtgaccacgatggatagactttttgagaaagatccctttgttaatgggtcttttttgttgtattctttgtcggaaagcggaggaaacccagatcatcttatttaggagtcttagtttgtgaggtctatgtggaattttctttcaaaagttttgatgttgtacttgcttgctagagggatgttcatttgatgattagagagtttctcctctagttgcctttcaaagagaaatgacaactattgtgggttggcctagtactaaaataggagacatagtctcaataactaactaagaagtcatgggttctatccatggtggccacctacctaggaattaattttctatgagtttctttgacatccaaatgtagtagggttagacgggttgtcccgtgagattagtttaggtgagtgtaagttggtttggacactcatggatataataaaagagaaatgttgttttctattttgtggtttgtgggtgtgtcatgtgtgctttgttgtggaatctttaaggaaagaggaaccacaaaccctattgaggtttggttcttggtgaagagtgtgaggtttcatgttctgggcttcggtttcaaagactatttgtaattattcactctcacttagttgcaaacactttcttttgagggtttccgtgggcttggttttctgtatgctgttgtgtttttttcactttttccctcaatggatgcaattctttattcaaaagaaaatctttactcttgaatttgcatatgcaccctttgataacttttggtaggttagtcacttcagatcaaaccacaaataataatatattttgttttcgcaaaacttagaaaatatatttttgatatcagtctgttggtccattctcccacttattggtttatgtttttttggtagttatgaagtaacatccaaaggcctgtattgtttaggctgtagaactttatacaaacctctgctaagtcaattcctaatcaagaatttgtggaactgtaggcttatgtggactcgagtgtcatcttggggcagactggacagtaccagaaggatgttgagaaatatggcaatattgaatacatgaggtgtacaccagaaaatggattttttcccgatctatctaaggttcctcgaacagatatcatatttttctgttcaccaaacaatcctactggctcatctgcaactagggaacagttgacccaacttgtgcagtttgactaaaagaatggatcaattatagtctatgattcagcatatgca

SEQ ID NO: 101 - DNA, 1078 bp, Cucumis melo
  unsure 1..1078: note = unsure at all n locations
  source 1..1078: mol_type = other DNA
ataatattaatttcatttaaaaataacttgaattttttcctcctatatttatcatgcatttttacaaatccacgttcgaaaatcccattaatcataggagttaaattgtcatcacttgatttgaatatttatttttttttaaaattaataaataaataatgtcacgaaaatgataaaaatgcaaagtatcgaatttaaaaattaaacagaacaaaatttaaaaattaaatgataaaaataaatataaaatataggtggatgttaaagataataatttaaatctttatctatcatcaaatgacgatcctccaatggaaaaagaaaaaaaaaactttattctttacctcaaactcctcgctaaaaagtaacaatggtaagataaaactttattttaaattattcttccacttgcaagcaaagtaaatagttatttgattcttacacaaaagagaatttttactttttacttttcattagttatatataactttataatacatttccctctcatggaatttaaaactaccatttgagcaaaatattttaaactaaagaaaaatatgaaacttaaaactatgtgacagggatgataatgacgtttactccaaattttcattttaaattaacgtacgttattttataagtatatgtcaaaattttaaggatctattttattagacaattcaaattatatgttgtgctttcatattttgttaaattcaataaatatgcctttggttgattatactatttttctaattaactctggagacatttcaaaagattttttatttatttatttaagaaaatatattaatatggtcaatagatatgtattatgcacatgatataaaaannnnnnnnnnngtaataatattattacataattaaattctttcatcttcctaacagagagagaggatcgtcctctcagcgacgctgatcccaactgttccagtaccaaatctctgtgtcccaatccaacagatccttcttttaagctaaacccaccatttttttttttttctgaaacccatttcttatctctcgccggaccttcagattttacctcaaaacc

SEQ ID NO: 102 - DNA, 2000 bp, Cucumis melo
  misc_feature 1..2000: note = n=g, a, t or c.
  unsure 1..2000: note = unsure at all n locations
  source 1..2000: mol_type = other DNA
cactatctatcatagataaataagtgatagatctaaacgatcatttaccaaagtctcaaagatcatgtaccaatatctaaacgagtttggtacaagattgtataccaaaatcatttgatttgatacaagatcgtgtaccaaaattgtttagatttgatacaatatcatgtacaagatagtgtatcaatatttaaacaattaatcgtctatcctagataaacaaagataaaccactaggaaatcgcacgaagagaaatagaggaagtgaagaaaaaaattactcatataaattgatgaaaaatgttatccttctctaatatggttttaatttttgcactaggaaatcacacattaatgattataatacaaagtcctacaaagagatctgaattgattcatttgtgaaactttacaattttaatcgatacaattattaacttaagagtgtaattgatttaagctacaaggtttaagcaaaaaactaaaacataaacagaagtcaaacttttcttaatttttgagtttagtgagctacttatttattgggtagctttagaaaagtcaaacttgaattgtcatttttaagtatgatcaaacttaatttaacccaaacttctgttgtaggtgaattagcagctagtttgtatatattgactgatttacaaattcttattttaattaattttaaccatccattaaaatggagagttatagttattcaaggattttaactactctcaaaatcatcaagatcacttgcatatttagtataagttcaaggacttaagtccttattgatattttcatcatcatctggaaaactaatcaaataatcatgttgatgcaacttagatgattaagattaaagctaagacttttgaaatgataaagaatataaataaaaaaggaagttttttaaaaatataacaaataggtaaaatatttacattatataaaacaattctagaaacgaaaaaaacccacggtctcacaatgaaaaatacaaaaaataccctagtcaatagcaattaatcagccagcttgcgcgaagaatattcttttaaacgactgtgtactacaatttcaacgaataatccagtattgtttaggtcatgacacgatcatgtagttctattttaacgatgggaaaaaaggttttgaatttaaatgatcgtattgatcatgaaaaacaactatgttgattacgataagcgatcatgtagtccaatgtaaatgaatttcaagtctaacgatcatgttgaccatgctaaacgattgtgttagctatggtaagcaattgtgtagatcatgtcaacacgatcgtttagatcattttaaacgatgtgaaaaagactnnnnnnnnnnnnnnnnnnnnnnnnnnnnnnccatgataaacgattgtgttgacaatggtaaaagattgtgttgacgatgataaacgattgtgttgataatggtaaagatcgtgttgacgatggtaaacgatcggctaaatcatgtcaaaatgatatttagacgatgtagatatttttgaatatgagaaagatgaagtgactttaaagatgaagtagcttttaggtcaaaagcaaataaaaacatataaaaacatacgaggaaaagttaacatatttttagtctattcagactcatccaaattttaattgtgtcatcaaatctcaatccacagctctcaccttgattaaatacataacatatctaagatcttataattaagttcatgaacgtatctaactttttaattcattgatctgccttgcttagttcaagttacataccctcttgcttaaaaaaaaaagttacataccctcttgcttaaaaaaaaaaagttatataccctctttgacaaatatcaaaggagaaaaagacaaaaactgacattggcttcccatcatccagagaaaagaaagaaaagccgcgcgggttgtttatccacttgtttcccttattatcctcatcgattccaagttttgaactcaaca

SEQ ID NO: 103 - DNA, 2000 bp, Cucumis melo
  source 1..2000: mol_type = other DNA
ttcctatttaaattaactggttttcttagaaaataacagaattcctgtgtggaatcccggctctaatccaaatttcatagggatgaaaaatgaaatggggagtagacatggagatggggagtggcattcctgacctcaccccgtccccgtggacatctttggtgacagaatcatcccatccaaatcaatctgtgggcaaatttcaacactcacaacaagttgaaagactttgttttgtaatgtatttcgagttcaactcacatgtggttgtatagtctaccatttcaaacccactccaaataagaaaaaaatataaaaaaacatattttagaaccccacaacattttttttatttgaaacaaacaaatatctccacgtgtttctgtttgatctcaaattgtacaaaagggagacaaacaagagcaacttaatcgtgtggtcgaaagttcataaaaaacgttgtttttcattactattattacatcaaccaatgcgatctcaatcttgtgaagatttttcttccatgtgtgagtcatttcttctcgatcttaattatcttctcacaatccatttattatagcataatctaagttaatttagattcaaaactatacaataataataattaagaaaattacaaatttaaatagcaaaagaaccatttgttctttatagtttctacactaacttttgaaaaggttaaggttattggaaatctttttctggggcatttttctccaattctacaatagacaattttttttaattaattaattaattaaatttaaagtttaccttggagtagtcaataattaatttttatgcacatttgtcttttatatgattgaatgtaacaaacaataacttattcttcttcttttattctattgttttgatgcaaacccacaatatttaatgagctcatagttatgtgtttgctttactaattaattattttcttttcataaaataaaaaaacttgtacaatataaactctattatcattgaatttttagtacttaatttaaacgtactaaaataaaatacatcattctgactgacgatccatgtaaataaaatctaaaaataaaagaaaaatgtcagaaatagcaaattgacaaaatatttacaagccatagcaaaatttcatattctaccgataacaaacatttgatagacattgatattcttctgtcagtggtattggtagacagtgatagaagtctatcaatttctatcatcgatagaattcaaaattttgttatagatcgtaaatattttaatttatttgttacttttaaaaatgtctcaatataaaaattattaaataaacattaattttttatttttcaattttaatatctaagctcataaatattaactttacccattatttatttggtttcttaccgcttaaatgttgcaaaaatattttaaattttatttttgaaatttggttaaattcgtttttacttaaaaatttccgtgataaaaatattcgaattttttaggtttttataagatttaaaagtaaactacataaatgaaatcgttattttctaattctcaatttaacttttttatactttttaattaccaaatggaaacatgaaattttaaatatatttattttaaatcttactcgttacaaacaaaacaataaatttaaaattatttttccgagttttaaattacaagatttaaaattaatttttcaacaagaccaaaagaattgtaagtttcgaataaaaaggtttctttttgggctataaagtccaatttcctataaaagaatttgatcaattggagcccaaagtcagatccattaacttttgggcccaaatagaacaatgaaaagaaagcccaaaagctgacccaccaattaaccttattattagggttttgctctctcttttaacatccgaaaatcaggactctcttgccgcttttctcttcgccgtcgccttcttcgagcttcaagtctcccatcctcttcagcc

SEQ ID NO: 104 - DNA, 1974 bp, Cucumis melo
  source 1..1974: mol_type = other DNA
tttgctattttcgtttcatgtgggaaaaatagtatagtatgtttacgtcttaaattatttcaaattcctagctaggaattaaaactttaatatatccaaaacgtttcttatttattataaagatctgcaatagcacaatgccaatttctcttctttgaaatccaggttcaaatcccggttgcggaataatgttttgctattttcgtttcatgtggaaaaaatagtatagtatgtttacgtcttaaattattacaaattcctagctaggaattaaaactttaatatatccaaaacgttccttgtttattacaaagatctacactagcacaacggtaggtagtttctcttctttgaaatccaaaatctttgctattttcatttcattttcaaattgaatgcatagctttagattgtagtaaacattgtatatatatgtttaggttgtgctaactttaaatgtacaaaattcaaaatgtaatagaattagatgtacatgataaagagttgcaatatttagattaaaatataagaatttaaatgtaagacttgcatatatcaaaaaaagatttctttataaacaatatttttttatacaatttgaaggcaacttattgttactcatgggcttgatccaaacttttgttgtcttcactaaaattcctctaaatagttcaacataaagttgttcatgagaaaactcattaagatatattccaacattatgaattgtttgtccttgtattttgttaattgtcattgcaaagtataaatgaatggagatttgttttcttttgaacttgaatagatatccattatcatttggtgggtttaatggtattcatggaagaaaaatttatttttctgcataatcacccattattatttcagcatgtataatatttttgctaaataattgacatactaatcttgtctcgttacacaatccattagatgaatccaaatttttcaataacaacgttggtaaaaaaaatcaagacagccttttatatagtaaaaaaaatgttacaacaacttttcaacgttcaagtctttaaatttgtattgttgattagaattaataagatatttgatttgcaacaaatttctaaaatgtaaataaaaaaccatttgcattcaaactctttacatccaatactttaattccttcgcatcctatactttaattccactcacttaaatataattaattaaaaatatagtggataaatgaaaaccaatttgcatttaatttttatatatgcatactttaattccactaaacttcgttagaattaattcaaaaagttgtgggagagaatgtgcattttatcatattacaagaaaaataaaattaaaaaagaatttaccataaagtcattaaacaaaattcaaaggttgaatggagagaataaaatttctgcacgctttgatatatacaagatatttaaaattaaaaaaatagttttaaagagaatgtttctaaattattattctaactttaaatataattactcataattatacttatttttttttaaatttagaaactaaaatgatacattctcgaaaactataatcaaacgagttaatgttataaactttgaaaactattttttgtttttaaactctgcatagcaaatagcatatagaggttttttaaaaaataataataattaaaaaaacattaaaggcaaaatctattattccttgatttgtgtatagggtgtaaatattttgttactgtgttatttttaaccatttgcgcactgatacggactaaaaggtaaaaacataattttctcgaattgttattagaaaactggggaagaaaaaggaaatcaaatcgcgcgaggtgggatttgacccgggaacctaagactagctcggtgtggtgttgaaatccacgcgttgttcaccgattttcttcataacaaacgcacccaggctacggcagtcttcgaagctctctcaatc

SEQ ID NO: 105 - DNA, 2000 bp, Cucumis melo
  source 1..2000: mol_type = other DNA
gtcgtcgagcagagctctggcagttaccctacaacccggagcacgataactgcagtgatccctatcctcagcatcagttaaatgggccgattcaaaacttttatgggcctcagcccacttccacttacaactattacaaacatggatacgatagtcacgatcaggcccatcatcttaattactccacacattccaatatcttcggccgccaaactgcctccgtttttagcgacgaaaatgtccataattgctctattatgtaataaggctaaacactaatcatctatccctttaaatcttgaatttttgtaataaaaccaatctatactttttgccatagtttatttctagaaaagtttagaatacattgaagatttgagaaacttgtctacaaggcatcaacaaaactacgtgaaaatgacaaattggaaacaaataaaaatatcttatgtttgagtatatggaatgaagggattgatgtaataaaacttaacgtcaagtgttaatattacgctatagttattttcttgttgtagtaattttctcttagttaatttttttattattgaaataagtgataaattttctaataagaacgtaaagatttaaacctctaattaagttaaaaaaaaaaacttgaattattgtttgagttatgaggtaacgtaaaagacaacttaaattttaaagtcaaaccgaaaggaaaagagttaaatacccacaaatggatcaaagaagttaataacacacacgcacgttgggaagcttaaaaattagcaacaaacaagcaatcattggtgtgggacagtattgaaattccacaaaactacaagggtatattggaaaatccaatttatttatttattttttaataggaattaaatttactgtaaaaaaatgtaagaccgtcgattgacaattggtggactgtgaaacgtggcaaaagttaattggcgaaaaggagaggaaagattttctcttttcattataatgaaaaaaattaatgatagtacacgtggcaaaaaagtattggagagaaatttccgggaattatctctaatacgcggctaatttggatgtcaattttgcaaagaccagaatctttttgaacagcgaagaagaacaaatatatagacatacaataataaataaaaataaaaatatattaagcataagagaaaaagaagatttgaaggttatattgaagtgatattgttggtttctccatttctgtgggtctgactctgcctctctcttttcgagccagaaccaccaaaacgaaaaaacccacacactgtatagcaaaccctaattctttggtctcagatcgcccatggcttccactaaagaacgcgacaacttcgtttacatcgctaagctcgccgagcaggccgagcggtttattgtattggttttcctaccttcctttccactttttttttttgggtttgcttctcatttctattttatgcttttcttaatttgtgttttacttttcactctctctttgctcagatcgtatttcttctggttgtttaattttgtgtttatgttttttgacttcggatttaagccacgatcgcttgcctttttgtgtactattttcagaagtgttgttatgtttatccgtttacacgatctgtttgaaatttatggaaatttagtttgcttataattttgctacatttctattgtttagcttctcgagcagttttttttttttttggccgatccattgatttatactgtttttctgtctgatctgttttatttaatggagaatactctttttttgcgaagcttggtagctcatttttcactcatacttacacagactacttggtcattgtttttatctgtaagcacaaagcaaattcaagtttctgcctgttctttctttgcttgtcaaacgacaaaactatgtttgtagttgcttttggatgatagatggtgattctgattttaatttacgttttcctgctgttttttttttaaaagaa

SEQ ID NO: 106 - DNA, 1643 bp, Cucumis melo
  source 1..1643: mol_type = other DNA
tccattggccctctcaaacctttatgtgcatatcactaatatggttgaatatgtatatcttctttctcgaatagatgattcttggtggtttcaataatcatttagcaaatccagaaattgggacctcaagttcggttgccgtggaaatagctaaattaactctgaaatcctcaaactgaaatgtgagaataatcacgatgaatctgaaccgtcaacggcggaacatagcaacagtaatcagaattaccaaatttcaattgggggaattcctttgtatgatccttccttgggcctaacagggattcttgatttgaacctctcttcttcgtaaaaattacacaaaatatttagctgctagagctagacaaaacaagatttagattggaaaaacaacaatgcagctcccaaattgcaatcctaattccactatttcttttttctttttcttttttttaatcttaggattcaattcatcattcatcaattttattgttactgctcattgatgaccaatgttttggattttgtgtgtcaaatattttagtttatatatggtgaaaagataaaatgaatagtttcaaattttgtgttttatgaattcctcactacctctttctttcactaatacgtatgaaatgtgtatggttgtttataaataagatggatggatgttttgattttgatttgaatgttaatgttacttaaattatagattttaaccatttgaatgaaatatggagagaacagtttttatatgtaaaaacaaattaatgtgagaaagaaataaatagcaatgcctttcttcactaataaatgtatttatattttttattaacaaaataaaatttatattaattattagtgtatgaggtgtgttcttgtacaaaggaaagtattgcaaaattacaaaaatggaaagttgaaattactgcactcatttgctaaaatcaaattagttaattatagaacgaaaaataaataaataagttgtatttgatgatcctagataaataacttttgaagaataaagatcaactatttaaaaaaaatatgtgtatcacaaaaaagaatagagaaaaaaatcacaaaaatcacatcccaaattataataattcatattataataatttatataccaaacataaactataataatcacgtattattataactcatagactataataactcactccacgtcccgtagttattaaataaaagaaagtaacggtaacattaacattataacttcgccctcatttatggcaaggaaaaattggggggattggcaagtattatatttgtttatggaaaacttttgtgaaggtggaaaatagagagagccaaattaacaaaaataataacaaaatcaaagggtgtagaattcatccagtttgagagcggaagattagatgggtgaagaaaggattattctagaaccctagcccacgtgtcataatccaaccctcaccttttcttcaaaaaccctttctttcttctccctcccctatatctccttcttcgaccaccaaactcttttctctcaatttcccagcatcttcttcatttttcattcttaattcaacccatttcttctctcttttcgtttctattttcatcgtttctctataatttctccctta

SEQ ID NO: 107 - DNA, 2000 bp, Cucumis melo
  source 1..2000: mol_type = other DNA
ggatgggcaatcgtgcgacacttgttctactcgattaacaaattagccgtgtaaaatccaaaaattgtggacaatttacggtatgatgtagcccctcttcacgttcttaagaaattttttataaaatgagaaagggaaaggaaatcattgaaaagatcataaaagaaagcattgaagactgttaattgcaaagaaagcttagcttaaaaagagtgcaacaaggcttagttggggatttaactactatgtctcccttattgtacattttgaatatttttatccttggcagacttgcatatgaaaatgtcgaaacgtcacacactaggtcgacaacataaaaatgaaagcaatagagcaatagattaaactaagtagaaaacataaagacaaggtgatttgaaggtatttggatatgtggccataggcaaataacgcgctggacaagcatgttcatgacatatgacactttgcacgcatgctcaatgtggatatatcagcatggcgcacgtgcctcactcggacacataaacatggtatgcgcggcatcatgtgcgcacgccttacacgaccaacgagctaggtgtagtccaagcacacacgcgatgggcaaacgtgcctatggctgcccctggcgcagacagtctcgaaagatgcatgtccatcctaggcccatctagacacgtccaaaagttccaatgacggtccaaaaggatacaatacctttagaagtgtcatggtaggtctagaatgttctagagtcatttgtaaattgttaaactgccttatatcttctagatatacaggtcctcggccgaccttcaaagcacctaggtcggttaggaaagctataaatagatgtaaggtggcttatttgtaatcaccctaaaatcttggcataacctagccaagtaagacaaccttgcctcatcatttgtacacaaggtacctttacaaatggtaataccctggcaaaggactacactcatttgtatacaacttgtacacaagcaatcttggaacgcaaagtactcttccaagaagtgtcaagctaagctccatcattctcacaaaatgatctctcttgcctttcaactatcttaaatcttctactgccatattctttctcatagtgcttagtgcactaacctctcaaaggcttacttggctacgtgggcgttaatattagtcaagtgttgtacgtttggttagttgaaaaatctaaccacgtgacaatagacaaacatcaattttattttattttagagtctcaccaagttcttaaataaaatgtttattgtaagacaaacaaaaatgaaaatatgttattatagtgatatagaattttcactattagtacaagatataaaagcgaaaggaagaatgaatgaacactcaacatttagaaagtgttttgagtaaagaagtaaatagtgagaaataacgagtacaaatgtgtggaaagttataaacttctaagatctacagaacaaaagattgataagatataaaattgatgttaggataggagctacaaactcctttgaccaaatatcgagcaggattcacaagtcatactctcttactctaccaaattcattagaagtacataatgggcatgcatgtgaacgaattaaaaaattggtatttttatttttatattttaaaaaaattggatgaattggcaatggccatgaatgaaccagttgttaaagtttagaggacaaaacccaaaagagagaagtgtacctcataaaaaacaaatccaccaattgagaatcacataaattataggaagacgtgtcactctatcggccgatcctcaaactcttccaccaaatccacatgcacaatctccttctcttcccttccaccatacactcaaaatcccactgatcttcttcttcataaaaacccatataatcataaattaatttcctcaagtttttcttttccaattaaacaaacaactctgcaaaagaggcctttcttccaccatttcc

SEQ ID NO: 108 - DNA, 2000 bp, Cucumis melo
  source 1..2000: mol_type = other DNA
agacgaagaagaagacagggtgtgatcatttaagaatatgcgttttaactctgccctttttagggcttttttcttttatttatttgccttttttctcgctcctagggtttttccctccattgaattagaaggatgactgggccacagacttatgatgggcttcacggtcattatttgaaagtgtgatattctaaaaaaaataaaaactcatttgaattaaaatagggtttccctccatgggagtatgaaagacttttaattgaattggggtttttaaaccctaaattgaactaaatatatttttatgatttttacaaaaattaatactacaaaacaaattatgattaataaaatttgttgatatttttcaaaaaacaattatataataaaacaaactaaatattcaatttggtatttttaaccatgctataggaaaagattcatatgggcatcaaaatgaagcaagaacatggcaaagcaagttgggtgaagataagtattgtcctaaatcgaaggacgaggcaataaactcgatatctcgaagagtctccaggtcaacatcacaacgcctgcacaaaccaaatattattatatatatagccatcgtttactataagactatgtatttacgaaaaattctatattgttttcgacgattacatttatattatataggaataaaatacaaacttttcgaaaagtcatatatcccaccatataaagatcaaacgtggtagattgaaaacattatacagtatattctctatttttttctcataaaacttattacgctttgtcaagttataaagattaatggttttggtatattgtgctaacttcgtccatttgttgtgaaattacattttcactacttttttccacattgcaccatttttcatatgttttatttccattatctcgtagaatatgagcaaagaaaaagattaaagatgaaatttttcaacgtgtgagagaaacatcattaaaggttacttaataaggaattagaaaaaagagcatgaacctagaacaacaagatacaaaatatcaaagacaaaagagttcgatggagagctagaaagataaatcaagattttgtaaaagaaaagtgctcggtggggaactagaaaaatgttatagaagctagaaagataagccgataatttgtaaactataagaggccgtttagaggaagagttgggttgtgaaatgttagtgttatgataaaactattgttatgtttggggaaagagtttaaaaaggtacttttatgataaaatatgtctgggataagagttgaaaaacgtagttttatgggagagttgaagatatagggttatgaagagttaaaaaaggtataagaaaaggagagagagagagggaataggggttatgatcatagtcttaaaacagaattatcataacccaatccaagtgataacccttggaccaaacgacctaaaatatcaaagagaaaactgtttggtgaggaactataaaaatgttatagaagctaaaaatacgaactagaaagataagcggagccaattataagggttggttaagtgtagggtttatttatttgaggggaatgataatttaagatataaattaatagaatggcaagttttgtaagaaaaattaataacaactcgataaacttttgtttgtgttggtagagaaaacatgggccacaaacatgagcccaaatgtggagaagcccagctgataatttaattttaaaaataataaagattagattatttttgttcgcccaaaattcggcgcggctaggaggttgcttataaatggaaataaatggaaagggtgttaggtctcgaacaagtgtgcgacggtattttaaaggtcggccacgttgaggcggcccttttcactcctttttcctcgctcgtattcaatctagggttttaggtttccaacttctcttcctccccttccccttccccttccccttccttctctactcatcactattctca

SEQ ID NO: 109 - DNA, 2000 bp, Cucumis melo
  source 1..2000: mol_type = other DNA
atgggtagttttcaaattaatccgacctttgaagtactttggtttttaaaataattttttatcatctgaaatcactccatagacttatgttaccgtaaatcattattctttacaaatgatttgattttacttaaaagtatattatttcaaacacgttataggtattatgaagttttaccgtcaacaattatagttagtaagccaactatttataaaaatttaaaaaggaatatttgaagcatggtgcatgatgtatgttcttctctctcttaagttgactatcaaaacttaatcatgctcagaataacatacctcacatagcatgtgcaatttaatctaagcaattcaaaattcattaacaataattcatacacactacaaagtcataccacctatgtcacccaagaactactattattgtaacaagtcaaataagaagtccctatcctatccatcctaagatggagtaatttttcttttccttaaatttttggaaagaagaatattgaaattcaggacattaaatcaaagctgttcggagataaatgaaccattcttcaagtaaaattcatatttgtcatcatgcaaacaaatattgaaaacatgatatcaagaaaaagaacaaattatttaaaaacatcataccgcacatcaaacttaaaataaccttttgtgcatatcaaacttaaaataacttttctcaacaaattaaagcgacataaaattgataatttttgttttttttttaaatatatattcaagaaaatcgacaaatccaaatgacaagttgttcacctgtatattaaaaaaaacaataatgaaaatttgaaaggagagatgagaaaaaaaaaatcaatccatcaatccaacttgaatttttgggtcgacagcatatccctaattataataggaagcaccctactttttttacaaaagtatcgaaattattagtcgaaaatcttaattagagtccaaattggatgcagcaaggatagttttaaatccaattaatagcatgcctaatgctattacaaatatattttggattatacataaatagaaaaaaaaaagtgaacttccagactcaaatagattttactctattgttataaaaactatacattaaaattagatgtagagaatgagagctcaaaaccaagaaaagtaaatgataaaagggaaacaggaggtgaaaagaaaaggtgataccgcggatttgatgtggctctcggtttttgcctcccaagcaatccccattgcccatctcctctacaccaacccacttttctccctttctttctttctttctttctaaaacttttgttttccaattttgacctctcttcttgggcccacttactaacaaatcaaaaccaattttcatttttttttcttttctctattcccttccacaaataagaaaaaactttatataaatcaatacaagaatgacatttattataatagtatatactataaggtgggagggatggcaattgccaattgtataagtaactattaatagacagtaaaactttgaaatagaaggtatttagatgtctgagggtaaacttataacattttatgaaatctaaaaactaaaattaaaattattgggacaatataaactttagacataagaagaaaacatatttttgttaataatttaacaaagaacacaacaagaatggtagagtgttgattaagagtgagcataatagacaaaaaaaaatatagtcaatcagccaaaatagacggtggttggtcggagatgaagagagtttcaatctaatcagttggtaaaaaattcaaacatcgtcacattctttaaaacttttaaaggtttaaatctgctaagatttatcgaacaatgacctatttgtactactttatgattgacatcaatttaaatatttaccggtgaatttagtaacgattagggcgagagcggttttaaaaacaggagtggagtagtggacaaggagggggcggaccaaccg

SEQ ID NO: 110 - DNA, 2000 bp, Cucumis melo
  source 1..2000: mol_type = other DNA
ataatactataaaacaaataaattttaattaagttgtttttactttcatattatactaacaagaacagtttgttaagttttatatgtatttataaaagatatatgagttattggttaatctataatatcaatgtcgaatctctaacaaatattttagtgtctagaccttatgtaaaaatcagaagtgacgctcaatatttggaaacaggaatcattgggatacgtggaaatcaatctttctgacattgttacaaacaaaagaataaacgaaaagtatcaccttatagactcaaagaatggaaggattcagattgagttgcaatggaggacttcatcctgaagtacctatatatttttcttcttggttagtttttcagtcttctcttctatggatcaagtggggaatacagcaagagacaagaaagacattttcctatacaaattcattttattattctttcattgtctctataaataaagaggcatttaaatccttttcctaatttaggtttggtatcaatattttgtttgtaacagagtaatagaaccaaaatatttcattatgttacttgaaatgttgatttttttgtgcccattctcttctgagtcgacaagtgagagtagatatgaaagtagcttacatttatattttaagagtttggaatctcttaccttaaatattttctaaaagaatatcgttgtgggaatatgatttttctattttataaatttgacactatcgatcaatttaaacacgacgtataattttagttttatttttagaaaaataagctttttagtttaagtttttttttacgtaattactattgaatccctaaagttttaaaatgctatagctttactcttatactttgagtttagtttgtatatatggtcgataaattttaagattatgtaccgtaattctaagttaaaacattgctcacctcttgtcctcaaagttaatgtaaatgaaattataatactcatacataatagaacttttttttattcttaattatgcaaaaagaatagtgaaggttaatttagttataatcagttctagaaaattaacacaaacattctaaaagtagtttgaaattgagataaaatgaaagtcaaattcaaaacaacgaaataaagttataaatatgaaactttgaaaaatatagataaaattagaactacgcatgaaaactctaagacaaatagacaattctcgagatagaagtttgaaatcgaaatctggggaaggaaaaatctttacatttccattttattcctatatctactaataagttttgtattaaaaaagaacatcaaatagagtaaataactgcacactaaacaacactcacccaaccaccccatatctcaatgagaaatcttaatgtgaactacaaagctagggacagaaaaatgattcattagattccagaacaataataattatgattacattttggattcattagattccaaaataataataattatgattacatttggtgtttgacctatttatttatttattttatataaatattttgtcgaagagatagaaaaaaggatgcatttaaattaaaaaagaaaaattatattgataaagaagaagatggcgggctgacaagagaagaccgggaggctgatgtggcaatgggaattccaattttccaatcaaaaactaaaaacaaaaaagaaaaaaaaaaagcaaaataattttggttcactgaaaattttcatataaatacatgtggcggttgatggcccaaaggatgagctttgaaggtcgcattatcaaaagtttggggaagcagatttttgctaacttcgaggtactctcctctcctctcctctcctcactttcctttctctctatactaactataatttccattcctcctccatcaataatttcttcatcctcttccttagctaatctctctcttctctaccagtcaaacgccctcccttttggtgctctctagcctcctcctccc

SEQ ID NO: 111 - DNA, 2000 bp, Cucumis melo
  source 1..2000: mol_type = other DNA
ttctctctctcttttaatctacaacgtatccaattatatggagaaagttgaggttgttggatttaattcattttttcacattttttagggttaaaatctaaaaacacatttcgattttgcgactgttcaaggcgtatatgtttctttaaatattatagttgaaattacgatcaaattcttacgctggttaagaaagagaaaatcgtaggagagaaattgtgagcatataagtgaaaataacctcctagagttttttggatttttgagcgaaacaaaagtaaggttgtaacgatttatgtctaaaatgaacaatgtcatatcattgtgggaatatgtgtgaatgataaattatcacaacttccaacaatgagtatcacaatacatatcattgatgggttttgagaaaatgagggttgacttggacatgacaacttgatagacttataactgtgtggtgtacttataagaaatcggaagttggtttaaaaggagaatcatttgcgtcgacaagatgattattattgcaaaagatgcaaccaaggtatgtcgatacataggctagataaaaagaagatcaagtaatgatataactatgtctctgttgatatgtttttaagtgaaataaaaaacaaaactattaatcctatacctaaaatgaaccatatcgtactatattagaaaagaataatgtacctcttgatagaaacttatagtaaaagtgattaataaaatatcactagagagatacgtaaatacttcgttatcataatttattttacttataaatgaactataacaaaaagtatttatatccacaaaatcaacgttaagaatattagggcgtcgaagaagacgccaaactattttaatataggttacgtttggtatctcatctacataacaatcttttgctttcaaatacactcaataaagtaaatggaatgattttttgttttctaattttgtcattaaaaacagtgttttacattgtacttgaatttgtgacatataatgatatatttctttttacaatacccaaaatcaacagtaaaaaaacaaatacttacttcttttcattcaaatttttcatatgcttttgaccgttattagcctttagtagtttatcgtaaatagattgtgatatttttatcaagaagttttattttttaaaataaatttcctttttcataaccacaaaaagcacccttgcaaaatcaatatttcattttggaccgggttgacattaggtgctttaaggatcggcccaatctagattcaataatctcagtaaggcccacttgtaaaccacaaaaaggcatggcccaccgagcccactatgccaatagttgggcctttctttcgcaaatgcacgcagctaattaaggcttcattacttaataatcagtaattaattttgctccaaaacgggtcaaagagcgacccgacccgcgaatatgtatctgggccgttgattattttagtagtaatctcaaccgttcagtcggtccttttatatgtctgtcctccctcgtaatcaattcttagggttttctagggtttttagttcttctctacgcttggttggaagtgcccttcctctcattcttcctgctttactacaggttttcaatcttcaacaatttaaatctcaacatttaatttgttttgcacattgattcaagtgtgttttttttctttcgtttgggcttttgttgattgaaattactcaagaaattgcagccacaaggatagtctaaaaatgcatttgatttagtgtaggtgctgctctcttttttgtgattgttcttagcttacttggagctgtatgttaatgctagagttcattgagtatcaatgctcaattacagatagttttgttttgtaatttccacatatattttcgtatttgtgaaattaagctcgtttgttttcattgtttgttggcaatttatgttttatgttatgccaacgattcatgatttgtagcttgactcgaaagg

SEQ ID NO: 112 - DNA, 1027 bp, Cucumis melo
  source 1..1027: mol_type = other DNA
ggggggggttgtcttcctcaaactctgttatcgaaattaggtttacatttagtatctggttgacgttttgattgtattcctgggcctgaaatatgataaataaatatgaccattgaagttggtgtttattctgggtttctatcattaagagggtgtgaacttacgagggaaccaagaaagggatggaaataggaatatttagaatagtaggaagctcaaatgaattatttcgttcgataaggcggagtgaatataaataatatgcaaggagatgcggagaatattacccaccttatgagagagagccacaaatcagaaaacagtaacaaatataacaaatcaaacaacaccatttgcaagcgaattcaaacgtttttcgggtatgttgttccattaccacattcaaacatgaattgaaacctgagctcttgggcactttaattttattttcaacacattacgtttaaattgccgagtggtcaatatcatgtattgcttagtactaggtggatacaaaccttacatataaggtcaaagtattgtgggcatgatataaatgctctagcatattggtctcatagagttttttatacttttacatatccattaatgagataagttaatgtttcaacattaaatttttagttaatatgaattctagatgcatttgttatacaaatggtctgatgtatttgaggttctgaatgtcaaataggattgtagtttattcacgttgaatattgtaaagagttaggacgtttttttaagattagatgatgggtgccatatgctaccccatacgccaacaattataatgaaaattatattttgtcatttggtatttaacaattttttttaaaaaataagctaataacgcatagaattcctgagatttaaacaactttctgtaatttcttttctatgtactaattgttatagaacctgtgatgtgcttgtccatcatgcagattacaacgactttgaacataacttcaaaattgttgataatggtagccgagtttttgcc

SEQ ID NO: 113 - DNA, 2000 bp, Cucumis melo
  source 1..2000: mol_type = other DNA
agccaaagtttaatatgattcaatcttgcacaaatgcaggttacccaaatggttaaggttaagacaggcaacaccactctagcagttggtgatggtgcaaacgatgttggaatgatccaagaagcggatatcgggatcggtattagtggtgtagaagggatgcaggtaaatttaaaacagatcccagctggagtgataaaatatagctttcattcatctcaattttgttttatacttcttatctttctgaatttcaggcggtcatgtcaagtgatattgcaatcgcacagttccgatacttggagcggctgctccttgtgcatggacattggtgttacagaaggatctcttccatggtacattatgatctataaatattactttatattagcttcttagtgagaatcatccagattaatgtgcaactatacagtctcaacatcattttcagcttgaaaatctttgaaatatgtcgaactcatcgcattttatatatggcagatatgctatttcttctacaagaacattgtttttgggttcactctattcttctttgagatgtatgcatcattctccggccaaactgtatacaacgactggttcctttctttgtataacgtcttttttacttctctccctgtgattgctttgggagtgtttgaccaagacgtctcatcccggtactgtcttaaggtaagttcaactttcctttatttcattggtgcaatcttttgccttccttaagtacaatatcaaatggctcattgccctcaacatttttggattttcagttctcacttttataccaagaaggtgtccaaaatgtgttatttagttgggttcgaattttcggatgggtgttcaatgggctactcagttctgtcatcatattcttcttttgtgttggggcaatggaccatcaagctttccgcaacagcggagaggtcgtcgggctggaaattcttggtgccaccatgtacacttgtgttgtttgggttgtaaactgccaaatggcattgtccatcagttacttcacctatattcaacatctcttcatctggggcagcatcattctttggtatttattcctcatggcatatggagctataaacccagccatatccaccacagcatttcaggtattcattgaggcctgcgccccggcaccatcattttggatcctcacactattggctcttggagcttcccttcttccatacttcgtcttttcatcgatccaaatgcgattcttcccaatgtatcatcaaatgattcaatggataaaagctgacggacaatcgaacgatccagaatactgtcaggtagtgagacagaggtcattacgtcacacaaccgtcggttacacagctcggttcgaagcatcaaagcattttgaagaattctcagaaatcaagagtcactaggtttgatgattagatcgtagaaagattcaaaacattttttctacgtaaagtttcttctcagtgtatatatatatatacatttatatatttatacaacatgtgtacataagattcttgtgtagttttgatctccttgtagcttaagtgaccattcccaattcaaatggtcaaaaattttcttcctttcatgaaatttttaggaaataagccaattgtagtattcaatcgtatatttcaaatagtcattgagaagttctaactctactatagttctcaattataagtatgatggttttgtcttattcatcttgtagtagaaacaaaagaataaatttacgaaggatgaagcattgttattttaattataatttgggaaatttggagccacgaaatgaaatccaattttgtgccaagtagatgtgcaacaatgggcaaagaatcactttttctttttcataattttcccttccaacactcaccactaattcatcacctcaatcctcttcttcttcttcttcttcttcttcttcttcttcactcgcctttgggttgaggttggctctgttacagtcatcc

SEQ ID NO: 114 - DNA, 2000 bp, Cucumis melo
  source 1..2000: mol_type = other DNA
aaaagagtcatagtgaaaaaagctgagatcataatagtttcaccctaaacacaacttataataacacatactatcataatatacacaccaaacacagactctatagtcttcactctaaacgcagattacaatagtctgcaccccaaacgtagactattataatcttctgactattataatactcttttcacttatcgccccaaacgtcccctaagagaacaaagataggttataaaagagagatgagggtttatattatgcaacaagtataaggttctagaacgatgtagtcttcaaagtaacgaaagcaataggctacacgagaaaaatatttttaaaatatagtgctttccctaaactagatttcaatgacaaattattataaaaaatagaatcattaatccaacatggcttgcatgtcacaccttggccaaaactgaagacggatgtcatactcgacttcaatatatttttttaattaattttcatgtgacaacacataaatatttaaaatttagattgggttggattttttttcaagtgggtcccaaaatactcttcaaacccaaaccaacccaacttgtttacccatctaataataacccaccaggttcaagaagacgaaccgaaccgaaccgatccggtctaactttgtttcatacttaagtcgaacttagcggtacttttggttcggttctcggtttccccaaacagagccactcaaaattagatttagggttccgttcgcaattttcagcgcatttttatttgaatcggtcgtttgttgaacacgttctctctcagctggtttagggttcatcgttctctcttctcgcgctatatctttctctctctcaggttcgtttctttctcttaggccattttatcagaaagatcctcttcgtttctccgattttctttccgtgttcgccctcggtttctcagcagacgtaggaagtttggtttccgtttagtgaatctgtttggggtattacgaatgatattttgtactgggctttccgcatagtctttttctttctaggaatatatgcatctgagaatttatttgtttggcttttctttataaagtatgaggacatatacatctcgattgctaatccttgattataatctttttttttctatgttgtttgaatctgtttttttttttttaatttctaggttttttgaatctaaaaatgtatttcttggatgaattgcatactgttgaattagaagtttattgattagattgttgatatttgccctaagttccatggataggtttgcgtctttcaccttttcgtttgctttttcttttggctgacgacatcttacatagcctctgctctaaaaggtgccatgattttttttcctggctttatctgagtttgcgcaatttagatttgaagtgatgatttgtctaaatataaatatctatcggccatactattttttgttattttgagtttttcaaggatgactgctagagaatgaaaaatcttgaaaacattgtgttttgaagttcaaggatcttgtagttttgttcttttctagactatctcatttgatatagccctttaaatttaatcaaaatttgttaatattcaaatcctcggacattttaattatttatctaaatagttgtttaggcattactcaggttgcccactattttaagcttagaagcctactctggttgacctaaagtttgcatgctatttgccttatttcgcacgactctaaactgttatagacatcttttttcagccttcaggtaaatgaacacaaaaaggagtgaaagtctgacttctgtgtgatggtcttttaatcaattatagggattaagatggtttttttattcattgtataaatattaaattagaatgatgacaaccaataatattaaaactgacaatggaaggttccttatattatttggagtgtacattacaacagcctgattcttggcttggcaggttcctgatcaccttgtaaac

SEQ ID NO: 115 - DNA, 2000 bp, Cucumis melo
  source 1..2000: mol_type = other DNA
aatgtaaatagtttataaacttaagataaaattggtaattgtttaatacaaatacaaattgttaaatgaaatgacacaccttgagcaattttcttttctaatcttctcttatagattaattttatttaatcatgaaggttagaatttctttagcattatttatttatttatttattagaaaaagatagtttgtgtatattttatatcataaagtttcagaagaaaccataaaattaatggagaataataaaaggtggggatctctaacatttttgccataaacaaatcactaagttaagaatatgacactaaacttcttctaatttaatattatatacaaagattttaaaattataaagtaagagccttgaattgtagctaatttaagaatatgctctaagttttttaaaatcacttttgccctacggttattatttatttttttgttgaaatatgtttaatccaaatcaatttcaatcgaacatagtcaaggatatgactgcggattcgtatattagttgattttgaaacgattaaatgtttgaaatattgtagtttaggaacaattacaattataacaatcagattcaaaattttagtatatacagtaacatttaaaagaataataaatatatcaaaatctatcgacaatagacttctcttcatagataaattatcagggtctgacttctctcatagataaattatcagggtctattagcaatagactaaatccttgatggtttatcattggtagaccaaaagagtttattagtgtgatagactttactacataatttgcaatttgtttaaaatgttgttatacatttggttgctatccttaacattacaatccataacatttgtcgtgtctttaacttgaattgattgttatctgtgataaaaagagatgatcactttttgtcatgagatttgaacaattgatgttaaaagtggtaattaatgtaccattcactaaccaatgtcaatatttattttgtttaataaaaagaaaaaggagattgtgacattagttttatactcttttctaaacataggtttggtttgtgttagatttggcctacacttagctcaaatccactctttataaaattcccttacttattacaagttatattttcactccaatcataatcttttaaaggataatatttgtattagaagatacgacacatgtagaagataattcttttttaaccaaaacaacatacaatttcgaggatatgacaaattaccttttctatttttaactatttgatcttcaagtcccatctaaacatcaaatgaaagttgattaggttaaagaattggacaattagagaaggaatggagaatcaaacctctaacttttaaggaattaggtcattcacattttcattgagctaagctcacattaacaagatcaatattacttgtatgtagttaattcagatgtgaatccttgaggtttcaaaagtgacactttagttcgaggtttaaaaaatatttatatatatacacatgttacaacccaaatttaaggtatatatataaatatatataatttaattatcttgaattataattaccttaaattacttaaagtaaagattggtttatttatgattaagttatgatgaatgttaagtaatttgaaaatttgaagtttagaggattgttaattcacttcattgtgggcctcattaattggcccattaaatctccatatgggcctgtctagggcttcatttccccaagcttccaactgtaatggcggccacagttctctcctccatctcctctcttcttacctacttattatgttaatatctacgttttccagattcattttctttttatttgtattattctaaatctccagaactgcttagctgctctggtttttggggattttagggggctcgatctggtgggtttacggttaaattttgcagcttttcgaggtccttttcggcttccattttgtcggaagttacaaa

SEQ ID NO: 116 - DNA, 2000 bp, Cucumis melo
  source 1..2000: mol_type = other DNA
acacttgtaatgttgagcagggtaacttatggtaaatttgacatgagctggcgcacaaaggcctagcatgctcggagctgtttttccatggagtcaatgcttgatcgcattattggctatattctaaatgaaactaaaattattgatgggttccatctgtttggataccaactttatacacaggtgtttttctatttatgagtgtaaagtttgatttgcttcatcatcgtatattcaacgtagagtttcttagttaatccaatccatatgcctcaactatcatgctcttttccctgtaattgaatgttttttttggtgtccacatggtcatggaggttttgttctgcactagcttcacgatgctactaaacatgatgatgaagcttgagtttatttatttcttagtactttgtgatgaaaaaaaagtagaagaaaacggtagaaaattggaatggatacggtacaatggatgggttgtgctaagtcacgtctcgtggatacaactacaattagttattttgttttgtagatttcatattagcatttccttctgaatagttgaaatcaccatagaatgtgtactgatgttttgtgattttagtgcttcggtataatttgaacgctttacaagtaaaaatttcctcaggtaaacgagtcttccgaagtacttgttcataaaatgttcttgtgtgggagagttgattggagaggatcatggtcaaattcttcttggtgtgttttatataaggttttaatgattctttgaaattgtaatgtttccttagtttttttaagtgatactggtgggttttccttggaataaatattaagggctgaaacttaggaattatatggatttgagggaggtttgtggattctcaaatcaaatcaaaccaaaaccagataattttaaattctagaattttgaagttactatttgtgtttagaaataaaaagaaagaatatcgcttctttgtccttccaatattctttagaaccaaaagagaaccaaaattatatataaaagagtcgataaaatcaaatatatatctataatatagtttattattatttttcatttgctatcaataagaattttgaaatgtaatatttgctccaaattatattaaaaacagctgttgaaatttcaacaaaatgagaatttgtactctggattttgttattagtttttttttcaatatcttaaactatttcttaaatattctcattgcgagtccttccatttacatagaactaaaaatggattgagtttggttagagaataatcccaatcttactcatatttttaggttgattagattggtaatttgattagcggttaagttattgggttgtattgtttcataaattcgatagattacatcgatggcaatgtagtgtggaacataaaaaataatgaaataccagcggaacacaatggagactgaaaaggatagacgatcgaagatgatgaaatgagaagctgacaacaatgaggggcgtgagttgagaagccgagacaagagggagagagtgagtcggaaagagatgtggggcgttacaagttgtgttgaacaaagtgaggtcaaatttaaatttactatttgctaaattaataataaaataaaatataaatataaacatataaatatatatatgattgggttgggttgatacaaaatttctaaccctaactcgataaagcaaaatgcaacccaaattttaaattaaccagatcgggttattcttatcctaaccttaggacagtgattacttaatctgtacgcaggggcaattttgacctttgataaactctcccattttgttttcttttttcggcaattttccctccctctctagtctcttctgttctcagttcagctctctagggttttgtcgaacagccatttctaagtgtacatctcctctcaatttccctcgctttattccattttttcacgtactatcggcggatcctttgagctccaactctctcatcc

SEQ ID NO: 117 - DNA, 1025 bp, Cucumis melo
  source 1..1025: mol_type = other DNA
tttttcttacttcattatcgaacaataatttgatttccaagcgaccctttcaaattcaaacaaacccatttctcctctcagccagagcaagtgattgaactgctgcgctgcgcgtgacctgttatcttctccgtttttcttaccgccgcccgcccctcacggcggagtagtttcaccgccgacccatttcgccggccgccggcggtgtttcgattcctcttgttttgtcccttttcgtcttaccagttttctctctgtctacattgtgtgctcgttaacagccagctgtatagccactgctttttttattgactcttgaaacagagagataggggagattctgtatagtcccactgtttctgctcaactttttcggtttaatgtctgtttctatattcgattcttcgttttatgttcgtgattcgatattgcttttgcttggaatcgtttagaggcaagtgattgtctctgcttttgctatgtagttactctgttttttttccctttctctctctctctctctccccccctctttctcaaaagggggttggtttttttatcgtcggaggatgttgggttgatcttttgatagggtctgttgactaatttagctggtgttcttggtctgctgaatccgaacttctcttagttttagagttttcgatgttgttggtttacactgattcttcttcgtttgtttgggattatttttgacaggactatagtgtttaactgctagctgccatggaacatgcagaatctgcggtgagtttttagaataaacttgttcggttggtgagaaaagcatgggaaagaggagggggaggtttttctttatgtcaaatattttctcaaactcaggttttagaataaaaaagcctttgtttcttaaccaaatagtttatttgataatcagctgttttgttttagctccctcatctcattttcggaaatcttagttatcagtttaatcaactctgtgttctatgatgctcatttgtacttaggcaaaggttataaagaac

SEQ ID NO: 118 - DNA, 2000 bp, Cucumis melo
  source 1..2000: mol_type = other DNA
tgcattttatcagagatgaaattgaaaaaggaagaataaacacgtactgtaaaatcaaaacataagaaacccagctgacttagcttgttaattaaccaaacaaagtttgagcattgtctaaattaaagttgttcaacttgactgttgtagggttattaatttttcttgaaaagaaaacgcagcatataatattaaaggagtattttgtctcgagggggaagattattggttaaaagtatatatggtgtgacataattaaatactttgtaactaaaaaataaaacataatgggaagttatctctaccaatttttttgttaaagggctgaatatataacctccaacattacttagttactgatatatcagtttctctagccgtcaacagtactacatagttgctgatcataaatagaagaaacaagttagaaattttgtgaagagaaaggcgagattatgtgatttttgctttgtataattttgaaaacccttgatataaggaagttccttgttgctgcatgccttcttagagatcagcagttactgtatgtctatatataattctctctctcaatatttttttctgttcttgagcttgattgtttactgcttcagaaatcttctttacaactactactgtatttggaagttttagttccatatatatttctatttttttaatgatttcaaatcttgttgtttcaaacagtactctcctaattacaaatacaataaaattatatctagcattacaattttacaaagtccttttcttgtgaaaaataaattacgtgagactttgtaaatggtattttgaatgtattaaggtactatatgacacttagaattgctttgctttagctctaaccatgggttcaaatgtaaagttaaaaataaaacaatcaactatttaaggttttacttaaaaatgtaattatttgtcaaaataagcataataattgagtagtaatttacatatattgcctccacatttgagatcaaaactagagatgttcattttcttagatatattattaagctaagaatgagagaatgggtgaggggaaaagtgaacggaggcaggaagaccaaatcacccattcctgaaaatggaaggattaaaattgcaattttccttgcaatttaataccaacatgattttgtatatatatatttgaagaggggttttaaaaaaatataacaaactgttaaaatatttacactatatacaacaatcgttaagataaaaaaactcataggtccacaatgaaaaatataacaaatgtcatagtcaacacgcgattaatcagccacactcacgttcgagtaatcttcttctgaatgattgtgtattacagtcaaaatacacaatcgtagagttcttttctaatgatgttgaaaaatacttcaaatttagggtttagggtttagggtttaatgatcgtgttaaccgtgaaaaataatcgtgttaatcaatggaaaacgatcgtgttgattatgataagtgatcgtgtagtccaatgtaaacgatcgtgtttgactatgttaaatgatcactatggtaagtgatcgtttaaatcatataaacacgacgatcatgtagttctttttaaaagatggaaaaagaattcaaatgcaaacgttcgtgttaacaatgacaaatcattgtttagatcatgtcaaaattaatatttaaacgatctattgatattcttaaataggaggaagatgaagtagttctaaagaatactgtcgaaaacaataaagatagaatatgatatttaaattaaaaaataaatgatatcggaagagaagatgaataaatcagagaaacagatataaaaggggaagtgactgatcctccaaatctaaaagataaaaatattttacatgactctgtaaactttggtttcttttgctaggcagtaaatatttgagggttttggtattgtatttgtggcggaatggagtaagtgggcctggcattgggccgtatacgta

SEQ ID NO: 119 - DNA, 2000 bp, Cucumis melo
  source 1..2000: mol_type = other DNA
tcattccagaaaaggtaatctttgattttgagaagttaatttgaattttattttaagggaattcaggcagcaagattaatcatctggcttcctggaaaaaggtcaagttttctcaatcagaaggggggctaggtttgggcagtttaaaaaataaaaaaaataaggccctctttctttactaaataaatggtgttggaggtttttgaaagaagactccacattgtggggtaagttatcaaaagtatccatggcttcaaaaaaatttaattggcagactctaaacaaactagaaaatagccttagaagttcgtggatcatgggaaagttgagttggcaactttcaaaacagagaacgaaaggagagtaactttctggacagattcgtggattagtgatctccctcttaaatatccatttccaaatatattcagattagctcaacaacccaatgattcaattactgcgcactgggattatgtcactaattcttggtcattagtattttgaagattgctaaaagatgaagaaattcaagatttccaaaggcttttaacactcaaatcctagaaagtaatagacttggatgatagaagagtttggtcattaaaaacctcaggccatttttcagttaagtccctttcgaagcacctctctccttcttcacctttggaaaaagattactttaaagcaccttggaaaaccaggagtccaagaagaataaatgttctggtttggattatagcagtgggttctctaaactgttatgagactatataaaggaagcttcctaatatgtgtttactacctttagtgtgctccatttgcttgaaaaacagtgagctcctaatacacttattcattttttgtcccttctcatctacttgttggtttagcatattttctatgctcaaacaacttgggtctttgatggttcattaaacaccaacgttgttcctaattttttagggggtccttatttatatatatatatataaaaaaaacttttctaatttgggttaatttgataaaagcactcctagctgagatttggtttgaatgtaaccaatgcatcttccatgataaaagagagagagagagattgggttgacattgtagacaattctaaaagaaacgtggtagcttggtgttcttcaaatgcagaattcaaatgcaggatatctacttattggactaccttcatatgaagagattcaatgcagtttcccccgactactagtttagaatttgtgtttttgtagttttaatgggctgtaatatgtatttctacctttaagtttttacttttcagtcttgcttctgtctaccataggtagtattgttattttgggtatttacttttgtcttttcatgaccttagtcttgttcttgtattttggatataatgagggtgctatcggggtatcaacctagttgagatgttcgagtgcacctactgatccccttatttgtaggcttctctattattctcaatgtataactctcttgtactttgagtttatcaataataaagaagcttgtctcattctaaaaaaacaaaaaggaaaaggaagataattgctcctaatcgttgaaattactactaattactcttaattactccaaatgatcgtataacatacatttataatttttaactttcttttcctttttaaataccaacattaaattttaaatacatccattaatttgaaattagttttcaaattccaaatcgaaagatttaaagtcctttgaatccaaagggagaatgagcccatccaagcaagtttttgtgtcgtagttgcatattttaagtcgtttcatattagcctcgagtttggcttaatgacttggtggtgtctagtgcaggcttgtggcgactggcgagcgtggttctaaagataaggtttgcattcgctccttctccctccctttcactacttcatatccatttcctttctcgatttctcgtcttcccttctgaattccccattccagcc

SEQ ID NO: 120 - DNA, 2000 bp, Cucumis melo
  source 1..2000: mol_type = other DNA
atttatttgtttagagataagacgcacatgagaatatgagatggattccactccactcacactccaatttctacctatcctattactgtttactattatcattccacccctcgacccctcattcttcttctcaccttacttttttatgatttactactacttcattttggatcacaatctgatcaatgctgggtgggctgccctcggcctgtcaccaggcccagcccacttccaaattaaacctcttggcccaccgcccattgtccccatcccattccatttaatattcccaaccttccctttttctttcccaatgcgatgcttctccaatatacctttcctgccctccatgtttcctttttactgctttcttatatttataacacaccttctacagtcttttggctgggaatgctgcgtatgtgaatgagattcaagatttcgttgatgttatttgagtctctatattcataagttttgttcttagttttctctagaccaactgcaagagttagcgttccatatgctcataagtttcagatttctgctgtgtggtttgaagacagtcatcgatccatgggtgaattcggctttttattattattattattattatttattgttgtcttacttttctatttgaatcttcctatctttttactcattgttggactctaataattcttgctaaacacaatctccatttttattggacattttaaatcccatctcaactcataattttagttaccttccaccatcaccatatccaaatccgaaataaactcaaataaaatccttcacgtgcatgtgctctccatatattttttctacatggtaaaaataaaatgaaaacaatctaaatttaataaaataacatatatggcagacttttattgatgtagagactgggtgttgtacaagaacagtgcagccaagaaaaaaaaaatacttccaatgaatcgtacattttaaggattatgaaactaactagttccaaccattttttcacgaccacgtgcttgttaaacacgcaagtagaatcaaaatgtgggcttcttcgctttatataactgtgaatcattctccaaaaagggaaggggatctcattccctaattcaataaagaaaaagaaaaatgctagcgaacttcatccatctcattccttttacctatttcatgagatgcccattgtatataagtattttttttttttttatttcattttacttagtttactcctcacctctaaaaaaaattaggagagtttgctaaatccattctcaaacttagctttatttttttaattttatttaacctcgtcgtggatgttaacctcaaatgtcagttctttttattctatttattgatgttataatttactttaggattccaattttataaaaataagaatacaaataaagataaagagtgtgaaagccagaaagaaaaaaaggaaatcgtaatatgggtaaaattggtacaaattgggtcccgttaaatattaactcaaaaaatgcgagaaaatggtagaaaaggaaatagggggtaagagcaaagtagtggaaggagagcattgaacatattctctagtttttgcacttggatctaaacacgaggaattataggtttattcatttactaattacataaataggattggattttaaaatttgaccgagtgattatgcatatttgatagagttagaaaatagtggtggggcaggtacaagttacaagtaatgtataagagatatgatgagcatattaggaaactatagatttaaattcgtccgtaaataaataattagaaatataatattcgagtggaagggtattagggttaggcgaaaccaattgcagttgcacctataaaaccccttttacgcctccacccgcttcaacagcggtctcggcgtctacaactacacactacacactacacactacacactacacagttgcagaccagaagcataacgtaacgccggtccacaaaa

SEQ ID NO: 121 - DNA, 2000 bp, Cucumis melo
  source 1..2000: mol_type = other DNA
tgaagagccggaaaagcatggcaaggtcaaggcatttcagcaagaatacgaggatgaattctgggtttgtaagtccggttcttcttcggagttgtggttcgaatttcaaacggccatgaggagccctacagcttaggaagcttcaggtctgagactctgactccgacagaaattgctgatttttgtgtgtgttttgaataaccattgtatgagtatgattggttgtataggtttgaaatgagggaaagtgatccatctccttgttgtctttgcaggaaaggctcatattcgaccaagaacgctttgtcattgctttcgataatcatagaatccacaatggtttggcatattagcaaacaaatcttctttaggcattgcagacagaaaattggagagtaagttattataattaaggattctaaatgagtaagaataataagatcaggcaaagattggaagaactaaagcgtttagtattttgtgtggtacagaagaattgtaattagatacgtagtctagagaagcagatggtgagatttgtgaaagacaaatgttagtggagagtgaagagtgtttctcaacaaccgacatagaaggattctcagaaaatgagaaagatttttattgcgcaaaatagctcccatatcatcatatgccgttgccattccctctggggttgcatgtaatgagtaatggaaagctgtagacaggctaacttcaccctttgtcttgggtatagggtgcatttttggtcactccattttaagttttctaataataaaaggatgaagaaaagatattgaaaaacagctcaggttttaaagttgtcacacttgagaataatgcatttaacagttagaattttgcatcaacgtctttcaaatagaaaagtaaaggagagtctagtttgagctggatagctaaactggtttaatcatatcttctatcaagtggttagagttttagacctcccaactttatatgtcgttgccctaacaatgttgatggatgtttagtcctaagctctaacattgtccccgtatcatatttcataatagaatgtactgagtaatggaaaactagagaggtaggaagttggacgaactttgaatctatattgattttactatagtctttcttccaagtcttaatgagagctttagctaaagtttttcaaaaactcaaaagaagtttttgttttccaattcttcgatccatagattgtcaagatggctataatatccttgaagttaatagccttcaaagtttcatagcttttatcctatgatctttagaaattcaagagttatattctttagaactacagaactttgatcttcgattcttcacctcttccagaacctttatagtagagtttcttgaccttacatgggcttgggattgggcctggctacttatgggcttagagattgaccttgggtttaagcacattcgttttacttggcccaattttcttaaacttctgcaaaatcctaattaactaacacctcaacaaaagtccagtattaaatggggcatataaacaaaagttaaacaaaattgtcgtacagaatcctaatttgctaacctcagcaaattttatgccattcgtccttgtgtatctaattagtgttaatttgaggaaatataataatatagacgtaggacggatattggtatttggtgcaacatcctccgaaccaattcctggaaagtaattggggcaacaagataatgttatcgtcagtttcaagtgcaaaacttgccacgtggaacagcggcaacatgatatctcaaatatggacctctcacccggtcaagcttccaccaccaccaccacctccgtattctaaaataaagtcaggaacaagaacagacacaccttaacaaaaccaatattcttcatctctatctctctctcatttcagcatagaagagagctgagtaaaaggaaaaaacttcaatcaaatttgacagagaagagcccaagagaaaaccaa

SEQ ID NO: 122 - DNA, 2000 bp, Cucumis melo
  source 1..2000: mol_type = other DNA
agatgaaccagaaagatggaaaatctacttggggttcagcagtgagtttggaaaagagagaactatttgaagaaagagcagaaaccatcttgctaatacttaaacaccgcttccctggaattccacaatcttcactagacatcagcaaaattcagttcaaccgggtaaaagaacgctccttccttgtctataatctcatctaaaattatcaacaatccaaacacaatttatacaaactaaaatgaaagcttctcaactttaggctacaaaaacagatgcttattataattctgcccaacaatatcttctcctaaataagatgatatatgttttttgcccatataatcaaataggaaataacaatcctgtgcccatttctttggagtgtgagatcataaaacactgtctaaaacaacatgtccaaacatatcgtaaatacctagtttcatagtgtgatgaaccaccacaaacaaacttactctttggtgaactgcaggacgtggggcacgccgttttagagagctactccagaatactggaaagcttagccttcacagtgatgtcacgaattgaagacgtactccacgccgataggttaactcagaacccatcacaaatagcaacaaggaggaaaccgacgagcgaacccccaatggagaaatcagaagagttgaacaacaacggcccagaaacgccagcttcaatgacgctgttggatttcatggggtggggacaggatcaaaacgagttggagatgaagaaggaatggtttgggaattcagatgatttaaacgcggattcagatctgaaacaagggaataagccagggaatatagtgacgaacaagagggtttcatacctggagaatttgagcgctgtgagaagtccaacggcgcgccattgaagaagaagaatagatagagagatgatttggaggcaaaattccatgatttcagttatatacattccttttgtgtaaataggaagaagaagaaggagaatgagatcaaccccatttttttctctcttctttttttaatttggattttggaatcacaactctttgtgtttgtgtaaaaccaaaattgttctatgtatcatttgtatcaattaatgtagtcattttagattcatacattcaaaaatatcaactccattttccaactactatcttcctccatctcacctctaatcataattcaaagcggatacaaattcatgttagaatgaaagattcgagtatagcctattccattgatcaaatgcatgtatctatactattgacacttttcaactcaagtcatgcttgaacaattgttttttataaatgttaattacaagagtgtacacaaatcgagttgggaaaaaatatgaaccaacccaaaccaaaaactttgagttggaccgaatttgaataaataattcaattttcattatttttatatagtttttcaaccaaattttttatcttttttttctcaaatttcaagtttacaataatgtccattcaaaagtttaaattttcatatttcgaacattgaagttggaaggtccaaacgaaagaactaaatgattatgacacatgtctagggtttatatatattgttgagttgagtaatccaagtttttgaaacaccactagttatttatgttaaataattaactgagtactcgactttcttagttcgagaatattttttagaaaaaagaagagaggatgtgtttagaaataatagcaagttagggtgttggtgagtgagaaatattttgggatcttcttgtaatagttattaagaagatttttcaaagaatttgagagttaaagaaataataataataaataagtaaacatttaatagtaaacgacatgtcgttttatacagcatcgtatttacttaccatgtgctcattcacacacgattcctcctcctcctcctcccgttcatctcttcttatcttcgtcttcttcatttcggataacacaaaaatccctaaaaaaa

SEQ ID NO: 123 - DNA, 2000 bp, Cucumis melo
  source 1..2000: mol_type = other DNA
tcattttcgtttggttaaagaatatatcatcgtttcttttataaaatgtttttgtagaattaatcttcgagtacttctcataaaaacattttttttaattacatagagtcagtaataattagaactatctcaaaccaaagtactataacatttcaaaccataacactgtattttttagaaaagttattgtaaaggatagaattacaaaaatattatagcatatgaaacattattgttatattttataaatattccatatacaatataattgattctagatgtctctaaaaatagggaagcatatgtgttaataactaaatttaaaaattaaaaaattactcgattactgtttatttatttatgtgttgaggctatacatactatattttagtaattattttaaaattaaaaacaaaatcacatggctaatagaaacgatagatatctagtagtaaaattttgttatatttataataagttgtcttattttacttaatgtaactacaaatatctcactgttattttcctttttttttcagcttattggtttatatgtttagaaaatttggtaaaatatttgtgtagctgcggttatcatgtatcaacttaactatgtaatctatgaaaaaatagtcattctttaaaaaaaaaatgaaaagttaaaaaagaaaaaaaggataaatttataacaatattctttaattgaattttatcatttgattcaaagatattcttatacttttaaaagctgcaatgttatttatgaaattgttttaaaattacatttataatgaaaaaatctttaaaaatgtagaaaaatcaaggcttagaattgtattgtcatttccatcaaggagaggatgtaattttttctttatcactttatttgaatcctcaaattttcgataagtatatattttgacatttgagaatatttttgtttactttaaatttaaagttatttttaaaacaaatgaaacaaaatattcataacgtggatcaaatcaccataatttagaaagcgttcttttgaaacatgaccccaaaactttagaagataaattacaatttgaactattttgaaaatggtagcaaggagacaggtaaaaaaagaccacataaatcactttaggctttaaagaaacaatgttaattggagaaagattcattggcatataattttgaaatatgattgtattttatatttcaaatcatattccatgaatttatctatctttgcttgtagtctaaatcatgcaaactttgaaaataacaatgttattgtatcaaaatttaaaagtttaaaacatataattgattaaataaagaaaaatatttagaaatgttgtatgccaataggtattatgtaataaattataaatgatataatattaaaaacaataattcataccattttttaaacataaaaacatgcttagtagattagttataaacagtttcaagtaatatttaaaagagagtcataagtagttttataatttataaaatacaatatcaaacgtacttaaaactaattgcttttaacttcaaatctaaattaagaataagaaaagggagagtgggaaagagcaaaatgagagaaaatgtcgaaaatacgcccaacggttcggaccggtccatttttgtcccgcgcaatggtaaaaatagattaggttacgacaatcaccatgatgatgaggatgatgatgatcatagcaattcaagaagcatagggccccacttttggccctcttattttctcttctcttacttactttaaagaatctaactgtcctccattaccccgccgatcaatgctctatttttctctctcttttttcttttctttattaaacaataataacaaaaaccatcaaattttcaaaattttgaattatattcccttaacacaaaacactctcctcttttcctttctcttataaatacaagtggagctccacacacttgtcattttgtacccttcttccccaacctcccaa

SEQ ID NO: 124 - DNA, 2000 bp, Cucumis melo
  source 1..2000: mol_type = other DNA
gggcttccattggcctccttcccgtcgccgtagtgagagaaaaaagaaagaaaggggagaggcagaagaatttgagagatggatcgaggagaggttttggaatgaatgggaaatttgaaggaagaggtttaaacataaaagtgaggcacgtgcgagaatgcaaatatttacggggctaaaaatgggagagccaacggattcaccccagtaaaaaggtaaattcaaacacgtttatgcctttttacctttttctttctttttttaacacctatagatgtaagatatttcatattcttaactttctctttctcttttcttttttgttttactatttccctttcgttggctaataataaaaattgatggatacagtatatttggtatgtcatcataaatttagagaaggtattaagattttgtgacataaaaacccaatttcttttaatgagattcttagaaattttattgaagagaattataaactttacgtaaattaggtaaagtctttccctccttctcgatagaagttgataataaacatagcatacctagataaaagtttgggaacatttttgttgtttggagggttgaaaaaaattaagaaatttcaatttggttaggatttgatgtcttgattttttgaaatataaactttcaattccaaatggtcggacttggaacctaacaaatcgtgttttcaattttaccttgatattttagatgtgtgagactccattaagtattctcttcgctctcttcttactatttctctgttttgctatcgaacgatattttttttaaaagatttattttttaattggtggaatgtttgtatgagagtatataagttaaggtaaacaaataataattggttatttagcaatcttcctagtcaataagcaaaacagacctaacatgcatcaaagaaacaaaatcaaaaccttaaaatatcatggttgggcgttgattttttttttcttttaatgtttgaaaatgtgggctttgggtgccgcagtcgtatggttgtagggatttcttttaagaaaattattttatattgtattcgttttgatctgaagatatcaattatacaataattggaatataaggagtaatttaactttgttcgtgattgttttctactttattcgatgtgtattttggaattaaatatgatttcaaatgattttgtttatttctttttattgattttgttttgattttactttgtatcaattttgaatatcaatgtagtgatgtgcttgtattaaatgtattggttgataaatttactatgcaaattttttttcaaaatttatgcaattcattgtagtattattaactatatcaacacatcagtaaagtgaatcattatcaagtatatcaattaagttacaaagtgtatatatcaataatgtatcaagtttatcagtagcactttaagcatataaagtgtatttaatcaattaactgtaccagtgaatcttactagatgtatttgcagtacatccgacgtatcaaacatatcatgtgtatcatatgtttaaatttgttgagtatattagtgaaacataacaagtttattagtagtgcatcaagtatatcaaatttatcagttaaacatttaagtctactaagaaaaaatgagtgcaataaaaattatttttcggatatataaaaaaatattgagtgtatcgaagagttccatggtgcatcaaatatataaagataaaaaaatatcaagaaatattaaatgtatatccatatatcaagaaacaaacctaacatgtatttcgtgatccaacaaccggactggaagacaaatttcggcccgggactttcatagtccaaataaaggcccattaaacttaacctgggcccaaattaatttgtaaattttaagtataaaaagaagagaaaccctagggtttccttcattcaccaggccttcctatccccttcccttccccccctccccattcccatttttgccggccgcc

SEQ ID NO: 125 - DNA, 2000 bp, Cucumis melo
  source 1..2000: mol_type = other DNA
ggacttatggggaatgggttcaagtgatggtaactagctacttcagatttaatatcctaaattgccttggcaacccaattcaaatgtattaggattagataggtgttttgtgaggatagttaataaggtgcttgcaagttggtgtcgacattcccaaatgtgaagggaaaaaaaccccaatctttggtctcaactggactttggttcattgcagttgaaaataaattattttagttcaaaccaataaaacacattttttaaaatctttggatatttgtttcttaaagttcctgaaacagcccaccaagtccatagcaattaggaaggcataagttagagctagtatgcttggcatggttgggggtgggttaccttgttatgtaaattcatagaaatattcatatcttgtgctaaaagtcaaatggaaagagggtgattgctgtgatgctgtctaatacaaagtgctagaagccatatggagaaagggtatttctacagtgtctaataagttaattacataataaatttctaggttatgagaatccaatccgcatgaatttaaggactgcacacttgctccatttgcaacatgtgtaccactttagaatcatatttcacctgagttcattattcaactagattaatgtatctcttttggtgttacatgtttttaagaacataattattttagtttactgtcggagagaagcaagtactggttatgcatggttctagtgagcctaatagagtaaggctatggtttgggcatttggaagttttagtggattagaattttgaaggcaaagctaaggatcatacacgcccttcttcccttttgaccagttggagatctatcatgtaactctattgtcttgggcttcggccttattttataaatttcatatatcaatgaaatttatttcctataaaaaaaagaaaaaagaaaaaaagctaaggattttaatatcattgttagtttctttaatttttttctttgggaagtgtgcatgtagagctcctttgaaagagaaaaagcaaagaactcttgaatgtaaaatctctatgtttgagttttatagtagcgtaccacattcacttcatggtgatgtagttatagttttcctatggaatatggctattaatttttgcgaggctcttattttatagttcttttggggtgttctttcctgtaccccctcccctttttgtgagaaggggaggtttctgtggctagctgggttggtttagatttgtggaccttttttgtgagaggaaccatagaaccttttgatgaggacctcgagcactatttgatcatttataagtttccataggcttttgtaattacctttttggtcttattttaattggagtccccttcctccccttttgttggcttttttgttgtatggttgggcattctttcgttagggaagtttgataattcacataataaacatacaataaacaaccatcaatacaatcaacaagcaggattagtgtaatactgtaaatgtcttttattttctttactccttttttcttttgaggtctatgataattgatatccaacagtgtattggccaaaatgatttatcatggtcagtaccttaggggtttgacttccaatccaggatttaaggtttgagaccagatattctgtgcctcaaggccctcaacaaccttctcatggctttttcctgtatacatattattatataaagttataaccaataaaagggacaggtcaaatcctcttaatatatgcgaaaatcaacctaatgtctactgtataccttctcaatcgccaccttcctcctgctgtcatccaaggtagggccttattgtatcagctagctccctttacttatttatttattttttgaagtgcgcagtttgtttgtttaccttgttataggaaattcaatctattctcattttattggtgcattcgtctcagaaattcttgtacggtttcaggttatcatctacccttgtag

SEQ ID NO: 126 - DNA, 1397 bp, Cucumis melo
  source 1..1397: mol_type = other DNA
tatatatattaacttttaaaattttgaaaacgtcatagataaattatatacaaaataaaaagtttgattatttacgaaagttaaaaagtttatccgaaagttgactcaacgataaaaacactaaatatcacttttagagatgatgatattatacataaacatacgaacttacgcgtcaaacttttatactaacacaagatcaaaacaactttgttgagtagtgagaattttatctgctgatatggttgaaacttgggaagcaagcagaggaagttccattcattaccaaaatccattttgtattcatcaaaatatgaagtttagcgacttgataaagtcaagtcaagtggtcctatcgatttgttaatgtcaatgtttggttttgaatttgatacctattagacaatgatatataattttaagtatggtttacactgtgatgctttatatatttttaaatgtaaaatattagaacttgtaatttcaataaattttaaaaatgattttgtgttatttccttttttaaattgaaatatcaatgtatcaatattgcgtcatagagtattgcaacacaaccttatgttaaattgtttattgcttattgctctaattcaactccttcatcaaatgtgcacagaatttaaacaagaaaaagagtaggtgcttttttactaaaatatactaaaagctttttataccaaatcttatgacaaaatcattccaacaaaatgactatttaaatataagatcgaatccctaatttaaaaaaaaaaaatcaaagatgttaatttctattattaaactcactttagcgtagctaacaaaaaaaggaaaaatgagaggctacaaagcttgagccctctgcctccctttattgcattgtttgaaattagatcaatactttgtatttttttcaaaatgaaaaatcgtacatagaattaattctatggacaaaaaatcagagaaggaaataatctagaataaaattcgatttttaacccaaaaaaaaaaaaaaaactcgattctgatttttgtaagcaatcacccaaattaccataaataaatggtattcaattactcaattatggatattttagaaatgataaatttttattcataaactcttttctttctctttcaaaaagaaaaaaattagcataaacttcaatgacatttatttattcttcttcgtttggagtcaaaagtttaaattgagcatcagtccagcccaaaagcccacgaagaagcccaagaatcttcagctttttcgttcaaacgtccctttttggtttataaaattaaagaaaataaaaactaaatttatttgttatttaacaaaacatttttggttaagacattctctttgattatttttcttccattcttcgtcgtcaatc

SEQ ID NO: 127 - DNA, 2000 bp, Cucumis melo
  misc_feature 1..2000: note = n=g, a, c or t.
  unsure 1..2000: note = unsure at all n locations
  source 1..2000: mol_type = other DNA
tttatatttatgaaaatgaagtctctaaacaatttttctactcccaaatttgttgatttttctgcctattctttatcggtgctttaaaaaatgaaaccaaatttcaaaactaaaaaaaccaagcttttaaaaaaatgttaggttatttttgaaattcaactaaatgttgaactcttttacttattaaataggcaaattattgaaataaatttagagcaagtaagcttaatttttaaaactaatatacttaccaaatcgaggactaaaatattcaaatactctttaaaattaagattaacattaatcactttgttatgtttaaaaagttgcagtgtcacttgaacctttttaaattaatataatgaaaatgaatccaactcaatatatataatatctatattattaatctcgatgtcagatgtttgatacgcacatatctcaaaaattatacctcaactaacatcggtgcacgatgtattatttcgtgaggataaaaatcgtttttagtataaattgatggaaagattatttgaattactgaaaaatgcaccggtacattatttgaaacttccccttcatttaaagaggctaatattagaaaaagacacgctgaggctatttttacaattaatgtgggctgttgacttggcccagcccaaaacataaaccctaaagtagcacaaacaaacgcctctttcttcttgaaaccgcatattaagcgttttatcacttctcaccacctctcattcctcctcttccgcacgttgtttcgctcctcaacgggagtgccttccctttgctctccctccaggttcttcttccttctcatctcatttccaagtaatttcattccgtttcttttctcttaatcgtatcttgttcagactctttcgcgtttttttttagttgcgccttaccagatctgtgttttcactcgtttctattcgatacatgcttccaagatccatttcttaatcgcatgtattcggttgattggatgattgtctttttgtaagttttgattacttttttggaatggatcggttgaaccaacggggtttaagtcgatggaagtaggttatgttaaagatttgcttctttttttttatgaagatgtgtgtgttctttttctttgctagatgatgttattatttgattgttttaacagtcgtgttttgtttttctgcagtttatagtcctcggtcttttgaagacttgtcaagatggttagtacacctcttgtcatcgtgattttgattgagtgatgtgttaagtgcttctttaggttacagctaacgcgattttttatattcaattgtgcctgtgcaggtgaagtttacagcagaagagctccgtcggattatggactataagcataacattcgtaatatgtctgttattgctcacgtcgatcatggtaagctacttagtttaagtttatttatgccgagcgtctatttaagaagattaacatcttagctttcatttattgtttatttggtaagcatcgtttctttttctccgaggaactgtacatgtcagttcacatgacaataaaacgatcttccttggacattagtttttgaagttcaattagacgccaaattttgttggttaaaagatgcttgtggagcatatggacctaatggaatcagtactttttgatggatggacttgtcttttgttcttttattttcaaaagaaattgcatgtgcaattacatcatctttgatcgaaagattgggtaattgggtaattggggtaaagacatgttgtaaaaactaatgttaattatcaattaccattatataccttatttagtgcttatttatatcctttttccccatttcagggaagtccactctcacagattctcttgtggctgctgccggtatcattgcacaagaagttgcnnngatgtacgaatgacagatactcgtcaagatgaggcagagcgtggtatcaccattaaatctactggaatctccctctactatgag

SEQ ID NO: 128 - DNA, 1657 bp, Cucumis melo
  source 1..1657: mol_type = other DNA
ggcaaaatggagagaaaaaagtttctccctattgccacatttatatatagtatatagatatatactatagacatgatggagaatcataagataaggtaaggctgaggaagattttgacgatatagaatggaaaattttgaagatataaaatggaagattttgaaaatatagaataagatcatcaaatgatagcaaaaaaatccaaatgagtcagatgaaacactacgccaaattttcatcactccaaaattgttgcaaaggagattgattaatagggtattatacacaatcatatttttcgtagcatgataattggttaataattagacataatggcaatcaattagttaactaatacaacattttaggtagcaatattaaaattggagatccggaaaaaaactaaaaactcagaaaaatcttgggcaaaatgagcacggtttatcaaatttttaggcttttttggtacaattttgtctaggatgaaacgagatccataattttctttgagaagataaaaaaaattaagatttggtgtaagatttgggaagatttgaataatttttttaaaagaaaaaataagatttggaaaatggtagaataacggtctaatgtctcccaagatgcaccgggaaagcaaaaaacaaccaaaacaataaataaattggaaaattttaatattttaggaaaatctcgatgtcaatttcgtctaagattggatcgagaaaaacagttttacgagtttttaaaaaatgtgttatatttaaaaataaaatcaaaattgtgctacttttgtcaatttcccaagataaaaatgtatgcttccacgtaaaaagtaacattactacccttctttcatttaatctctatatttggaaatgtcgcactagttcttggtagctaatatttggatactaattatcttatatgacaaaatatttaatgtactttttttttacaacaaatattgaatgaacttaaataatcttttcactgcaatgaaaaaagataaattagagcatcccaaaaagatgaaaagttcgaaagtctgctaactacattgaaaaacaaagcatttaattcttcaaacttgatagttcaattaaatttctaccaactaactcaagtaaatctattattagtgtttgagtgaggctatgaactctaagactaagcctataagtttggttaaatttaattataccagcccttttgtaagtaatttgatttgaaaggtaagacgtaataccgattacccaacccaaaattactgtgaatgagttaaaaaataaaattagttgaattttaaataaaaagcataccaataagacgatgacacatgtacaaaatcttagaaggagaagcttcatttgaggacaaaaaagagtgtgtggagtgagaagaaagaatagtcacgaatattgctgactgtgcaacaaatgtacatttggcaccaatcaaaacctataaaaccttatccaaaaatcaataatctcatcccttcttcgctgttcttccccaatccaaaccccaaccattctcctccacacacacacacactcacatacacaaatccttccaacattattctatacccacttcccaattctcattgcatttcacaatcattgttctaactcacttacaacctccatca

SEQ ID NO: 129 - DNA, 2000 bp, Cucumis melo
  source 1..2000: mol_type = other DNA
atgaacgaaggagaatatcggataatgaagaggagatccatgaatcacagagaatgaatgaaggagacccacgtgaattaaatagaacgaaggagaatgaagagaaaggatgaatacttcttttctttaattttaacctaatcgggtgaatcaaactcaaatcgaaactggtttagttcgattatgtttggtaccattgtcttttaaaccgatcaaacctgaaccaaacgaatcggtacggttttttgcacccctaatttatatcatgtgaaaggttttaagttaagggtcagctagtgtcgtttagagggaatgatattggttgacttcatgtcgtctcttggatcaagagtaggagattcgggaggggtgtgacgaaatcaaccccgagattgtcctacagatggcatgtaaaatgcatcatatctcgggactccttctacaaactcgagaaaaatgtctcttgagattcttcttctacacagccccaaattgatgaaatgactgagattctttgaaagacaccacatgcattaactgaaactaatgttgtacatctaaaaaactacatcacgccaccaactaaaaagttttccatttgcctgatttcaaactaaaaacaaaagacttaaacgataaactaaaaactaaaccacaaacaatgaaatcgttaaaagtgcaccttgagagatttaagagagtaaatgagttcacatagttttttgaaggaaaaatcactaaaacaagttggattgtaggagcgaaattgttcactccttaaccgaaattagcaaaatgtttggagtttagcgtttttagagaatatgtaacgttatgaataataagggtattttggtaatttgatatatccctttattttcaaatttttaataaaaaacacacatcttggtgacacactcgactgaaaaggaccaagatatttccttgaaagatttttttttttaaattgggaaagaatcttggggtcgatctcgatcgagattgatcgagaaaaatagaattacgagttttctaaaactgtgcttttgaaatatcacaccaaaaaagcgttatttctcaaaatttcccaagtttatatgtgggggttattgcgagttagcttttgatgggtttgcttttgggtgtttgtatataggtttgaaatgtacctttaatgtcgatttttgaagaaaggtacctttattgtttaaaattgacattgtaccttcatatttgatttcagtttaaaattgatattaattatccgcattttaaaaaccaacatcaaacatccatgttcatttcttttcaaatttaagcttgaggatgacttcgtgaaactttttgagcaaacacgtttatcggttgttcaaagtaaatcaccttcacaaatttaagcttgaggacgactttgtgaaatttcggcaagcaaaaatcagacaaatctcttcaatcttttttgagcaaacacactttatctctgctgaaatgagcacaaggtttagggttttgagaatatctagcatttaggctttcaatggtattttggtcatttgagaataccatttattttgaaattttaaaacaaaaacctaccatcttggtgacgatcatttaggccgagatgtattgaaaaattatgttaaaatgagtttttcaaatttgattagaacctcgtgttgaggtcgaccgaaattgaccgagaaaaataaatttacgaattttttttcaaaatgtgctacttttaaaatataaaactaaatgggttacttctcaaaagctaaccgaaactattagttatattgcggaaatatcaatttcgcccaattttagtcatccagagcctgactcatcgaatttaggagattctagacgttgcattcaggagatttttatccgttgtcgccgactctctttactgatctacattgtacttcattgctgaactcaacgagtcaactcaatcgtttctagatttggaagaatctgcttcagcgacg

SEQ ID NO: 130 - DNA, 2000 bp, Cucumis melo
  misc_feature 1..2000: note = n=g, a, t or c.
  unsure 1..2000: note = unsure at all n locations
  source 1..2000: mol_type = other DNA
aaaaggcgaaaaaaaagttagcttcccgagaaggagaagacgaggaagagtttgacttcccggggagataaagtttgtgtctcgagggaatctctaatctggagttgaccgtcgacttatgtgtcgagcctggatttagttgcatggtgcgacaaagcgataaggcggcatatgtaaagtagtaattcaaaactagcggttaaagaaataatcagccaaaaaatttagtacaaatacgggtggaggccctaagtgaagtgctgctattcagaggttttggcaaaagagtgcaaagagttgagttgtgcagagaaagtactaggtgaggagaggcgtttggaaaagaaaaggatcaaacatttgcatgagtgatattcttaaactaaacactcttgtgtgagtgacttgcctaagctaaacactcttgcatgagtaactttcttaaactaaacgttttgtaatgttttcttaatggattcttttcgagtctgagttatgcttaacacgttttgtttctctcgtgttattgttgttgttgtttgaaaagagaaaactattgttttctatgtgctgattgtgatgaatgtgtgcgaaccattagccttaatcctatcaagtgaatagtgattatgtggtgtgtgcacataatgtaaatgacattgtgtggatggccagtgcaacaagaaatgaatcagaaagcttcccaaatactgtgaatggagtgaacatcacactagctcaatggcaagatattggcgatagtgaatcacaataggcttgacaaggggaaggattcatgttcttggttgaaaggaataagagaggctaatgtgagatttctgtgatttgcaaaatgaggcgttggaagacacgtttgagaaatgaaaacgaattagtgcttgacttgtattcctaaaaaagttgtccaatatcttcaatcactaaatatttgatgtgcctaagttttccttccttagttgttgaggcgttgaggccgagtaaggaaagataagataattatgacgttgaaaagctggtcaagttatccatctttggatggtttaaagttattacatgtagggagggttgcattccaattttgtgtgtgagatgagtcttattttcgagatgggttgctaggcgatcaaggagaagtataagaaatgagttcttatactcttgaacaacttgacacgaagaataacatcctagtggatgaaggaaggtgatggaacttaaagtttaggttttattttnnnnnnnnnnnnnnnnnnnaaatgtaattgtaaagtattagatcaagtaataaaacagagttgtgttttctatttttgctgtgttgggttgtgtatctttattgtgcttatggcctagttgctaaagagttaaggttattacctaaatgttttacggtgtgttgagttgtaaagatctcctgagttaaagttggaattttgtattggagattgttttgagaagtttagcttactaattgtttaactcattaggtgtctaagcgacacgcctccttttggtcgcatgaagtggctagcagggtggggcggaccggggtggggtgtgataataaacctaaaaaatcacccagataagcctaaattatacgttgaagttaaacttacaatttgattagaagaagaaggaatatctgatttggacatgaattaattacaaatacggcgccaatcatacaaagcacatgtaagatcaacgcattctacactcaatctcagccgttgattgctttcaatccttcaaaaagaaaaaaagaagggcagttcgggcagagtcatacctacccgttgactataaaagcaactacaaatcgaaaacctccatttctccgttaccattacagagaaaatcaaagaaatttggcgttgagagattgggagagaggtttctctttctagggttgcttcttcttcttcatcctccattgttgcaaatttcacttccttctcctcttgttctcatctccc

SEQ ID NO: 131 - DNA, 2000 bp, Cucumis melo
  source 1..2000: mol_type = other DNA
atagagtaaccaatatgcccttttcagcagccaaagttttctatgggcagacttaatcaattaaggttcctattgaggccccactcttagtgaaaagcctagacccttctttccaacatgtctcaattggtcacctccatcaaaagcttctatcatttaatctaaaagcatactcttttttcctttttaaatttcattttgatggtctatatttgaaaataataatcactacaacgacgacacgttgttttcaaactattattttgtatgaattaataatttttttaatagtatagttgttttacttatggaatctatacgtttaatcgattcggtcacatctatttactttgatgtttttgttattttatttagacgtggttgtaaagagtttaaagcaatggagaagaaattgatgctttccaaagcaatacaaatttatatataccttcaaatgagactaacattagacaatacataaactataataaacattttgaaagtacatagatcaaaatgaaccaaagtcgaaaaagtacaattatcaaattagtttttaaaccttggataaacttcagcattcaaactttgtatttcttttttttttcgatcgatatatatagtgatagaagattttttttttctgtttattatttttgacgatacgttgagtagaagaatcgaacatcaaacctttaaatcaataatatatattttacgactcaatatctagccatcaatattttaaaatagcaattattattcactaaattatgttagagattggatgtcatacaacaattgttaaagattatttgtctagtttgttcaattaatcaagagagcattaagcattaaagtcaattattgtgataagatgcttttgcactatgtaactaaaaatagttggatacaccatttaaggccctacatgcaaaccatgataggcccacaaaaaaaaatctctttttggaaacaatggtcaaataatttctttcaaataataataataattacaacaaataaatacataaaccaaattactaaactaatgtatcaagttctagagaaaacaaaattatgccctttcaagttgcaacatcccctactataatttttcttcaaattttccatttaatataatccaattctaaacatggaaaagaaatgtaacaatatttacattatttcaatctttcctatattcatcgactaattttaataagacgtgaaatcaacatttttctaaactcgttgatgtcataaaaaataaacttaaattatgtacaagatcgtctattaaattatgtataacacgtgtggtgtatgagtaatagaaactttaaactcttgatcaaggacatgtacctataaataaatagatttctttaagtcttgactattaaccaacttgtattcagtaaggttaaagtgatctattatcatactaaatacacaagtttatttcgagtatgaatgcaaagaatcaaagatatatggtttaaacaaaatctattataccaataaaaaaggttaaccatatgcaataaaaactaaaaagtctattgctcaaatctctttcgagaccatattaaaaatgttagtttaattgacgtatgtatttattggatttatctaataacattttaagagattgttgcaaatatagctattagattcaaaataattaagtatatagcaaagtctgtcaaattctatcgatgataggactatgttaaaattgttgttcgatcgttggtaaactataaaaatctacgacaataaactactattcaaaaattttttactacccaaattttaaatccatctcatggatcgagtcaagcccacttctaaattgggccacgaatattgattgtgaagctcaataatcccatacgtatggctgaaaacgcattacgaacgaacgcccttcaactatccaaatccgaacccacccaaattccggttaggcttcttctccgagatcgacgaccgcg

SEQ ID NO: 132 - DNA, 2000 bp, Cucumis melo
  source 1..2000: mol_type = other DNA
tgcagctgcacaaaagattccaaatgatataacataatagtttatgaaaatttaatgcatttaatttccccttccacagaagacactatatttttcaactacccaacaataccaataattatcattattattatacctctaattagtaattagtcacaacataaacagctattctcattaatacatataatcaacaacttcataaattcttaaatttgtatgtgtacttgatgggtgtagatttaagaagtccaagagtttgacaccctttgttaaaatgatatacaaattcctgcaaattaaatttaccattggtatgattgttgttggagtggtcacaacactaatttactaattagcttcgtatttaacatagttggccatgcgaggaggtagcttttgaacttccaataacctggcttggaaggacgtcgataaacagaataacaactatgctaaattttgaataatatactttatatatattatataaagacgacaaagttgaggagcatccgtcccctacatttgttggtgctcatatcatcctattgcatatgccttttaccaatgaaaccctatctccttaattatttctactccacactcataattatcattcatttattttcatgcatgactttcttttaccaaatttagtttccaattaaactccattaactaccaacaatcaactccaataacgtaactcacattcattctaaccaattgtttggattgactcgagaaaaaaaaatgttttttctaactcatttttacttatacatttaaaaattcttttggaagtgatcgtcaaacattttgatatttttttccttttaaaatgacttattttttaaaaaacttaaatattcaaaaaggttttccaaatgaatgtaattaattactcaacatagatctccattaatcattattatatgtaacaatagtaattcaaagtaaaaaaaaaattatgtggagtgcaaagatgaaaattttgacctattttacatgatttgaactatatgtttatgcgtacctatgatttaactcttatatacacatatttttgtctcaatttaatttaattttacgattttcttgaataattttattctctaaccacttttgaaaaacattttttaaactttagaaaagaatatctttaccaaacttaattcaatatatgaaaatagctaaataaaatttaaaaaacagataaccaccctttgataactgtagctgatattattaattaattgtcatatttatatttgcaatatgaaaaaggagatgtcatgagtttttttttttttaatcaatctaatgcaattttcttaaatttaattaatgtgaaggtgagagagagaggcaatttcaaattttaggtaagtattatgaataaggttacttaacattattttaatttaattttacattatgttttatttgaatttttttaaagactctcatttttccattttggaacttttggaaaagaaaattttacttcaatctcttatgcaagcaagttaaaactacatttgtcttttcatgggatttttaaggagatgtgtggggaaatacaataagcctttttttatttgcaatttgctaaatgtgtattcttccaattggctaattattaaagtgaaatttagattgaaaaaagagataaaattgaattgaagttgtatagatgggttaggaatatgaaaattgtttgagatatagtgagtattggttttatccaatgccatgtcataggggtggaatccaaatgaaccaatgagaatcactcaaaagaaaacagatataatgcactatccaaacctaaaactaaaagccacacattgctcatccattcactcccattctcaaaaccacacaaaaataaatatcaaatcaatctctttcccttttccatatataccactttcccctctcttcgcctctttgattattacccaccaaatattcccatatatcttacaacaacc

SEQ ID NO: 133 - DNA, 2000 bp, Cucumis melo
  misc_feature 1..2000: note = n=g, a, t or c.
  unsure 1..2000: note = unsure at all n locations
  source 1..2000: mol_type = other DNA
aagcttgtttgaccctatttttaatgtcttaacacaggattatgaacaaaagaagaaactagtgaatcacagaggaactcacgcaaagactaggtgagaagatcatatcaaaatgagagaataagttcgctagaagataaaagtggtagttgaagttgatgtgacttgaccaagaggcagcttctggtgttgatatattcagaagactagatttcctgcctaaatctacctatataaagaactccatctccattaagaaaatgaggcctgaatggaccacccaagtggtcgactgtgtgaagagccaaatgtttgtgaactgcccatgagtgcctgaaaggcccgatcctagagagtggtgggaaggagcagcctttccaccatctgtaaagtctttcttcatcttctccagttagtttaagagtgaaagtttgaggttgagtgaagaagattccattcctatctttttctaactggtaatgtcatttctattctttccatttttgtatatttctttgtaatgtatttnnncatattgtacagtggcctaagacctatattctttaatacatttcatgtttatatcttttcaatctatcacgtttgttattattcatctgtccttgtgctattggtagcttaagatttatgataagttcttgataagaaggttagcttatatttcttatgtgtgttagttgtgagctattttcatcacctggctagtgtatattgcaaactacctgagagggtaagtagcaaagatatggcttaggcgcacaaggaggagtttggagacaaaatccacattggcaagataacttccatcatttgtgtctcaaaaggagaacaagtgtgggtattaagcattgagatgttgtgacccttaaacgagaagctatataagtcttagtgaaggtcgtttggatctcgagaggtgagcaagtgtggtgtttaaagacaccgagaggtgctcgtcttaatcataagctcgttaactaagttatattgcattagggatattttattgcttaatttcttggtaatgcacgaactttttttcacccattcttttatgccagctagttcacaattccatctcgcatccattttaatccccctttacagattctccggtgtagataagtagatatagtttaaacttacatgctttcacactatatattttattcttttatactacctaaatgcctagtgaagcctagaactaagctttgatatcgattccctgcattcgactctaaatcgcccatataaacctattgtttcgcttacacttgggcaagcaataggaaaacttgtactcaacgaggacttatgagttacatgatgacgagatacatagagagcatctaatatgcattgaccatgatcattgactcttcatgtagatttaaatacctttcagcttaattagatagaagatatataataaagccattccattagtttaaaagaattaagttagaggtagttgaaatgctttataagtgggggttaattctattttagctgtaatgctgagctgatctcaagccaaggttgccttgagatatccccgagtttaaaaacagaagctaaaatggaaactaaaaactaagacatataaactttttagttacttttagggaaatatcttagctataaattaaagaatatgaccaacatggaagttcctccatcacttttccaccaactcattttattgggggttagtcattttaaggccaattagtttaaattaaagttcaatctcagtgatgcactaggccgagagagaccgagataaatcattcaaatatttttttaaatttgggaagaatcttgaggtcgagattgatcctgagaaaaacaaaattacgagttttttaaaactgtgaaatataaaacaaaaaagtgctagttttgtcaattcccatttatcttgctcattgttgatacaagatcattaaaagtttatggataaatgttggttgaga

SEQ ID NO: 134 - DNA, 1696 bp, Cucumis melo
  source 1..1696: mol_type = other DNA
tatatatatatataaaaagaggaatacaattaagacatcccattgttaataaggggtggaataaattgggaaattaccattcgagaaatcattgacgagagcaaatatgtcaaagtagaaaattagtcatctcaaaagaatgtaatcgttacaaaaattaaaagtacgtaaatttaatcatcgttacaaaaattaaaagaatataaattacaccgttacacaataataccaacaatccatttataatatgttgtttttatttcaactttgaataaaatttgaactctttgataaaatttgtttaaaataaatttaaaaccatttcaaaagctatttttatattatccaaatacatatattcttttctttttccaaaatgacttgtttctaaattcgaacatccaaaaattaaaacataacatttttagtatattaagaattataaattaagagataaaatattcaatactattataataaaatcggtgttttcagtaattgtatttgtacaagtaaataaaattaatagtaaaatttttaatatataaacaagttttaaaagaaacttaaagatataaaaaataaattgaaataaaattcaaacccatcaacaaataaagaaaataaagatggttttattgaaatgaatgaactaaaatttgaaggaggcaaaagtaagtacaccaaaaatagaatactaaaatggtagaggacaataattgcatatgtttggtagatttttcattaactatcataccaattaacaataatgaaataaactttctcgttgatattgattacaatcgtaatagggcaacccactgtttaacttgtcaaagttttcttaactttattatttttgactttatttgtttgttttattgattagattgatagattatatattttaatcatattatttatagtacaacaactacgaggtaagtgattgaagctttagtctctaagaacaaaggttcgacctaattttttagtctgtttttatttgacatattttgtccattgatagaattactatcacttaagttaaatgtattattattgcaaaccactaattctacgtaaaatctctaagtagcaagtgttatgtcaataaaatagcaattttttttttaccaattacacacatcatggtgataattattatcatgcacgggtaaatttttaattataaaatttcaactttcaaaattataccaatactaaatttattacaaaagttattttaggtaaattataaaaacttgataacaattacaagtacattctaaaactttcaataataaagattgaatcatccaattcatccaaatgttaaatttataatccgatttcaagaagaaaattaaaaactcaatttttatgaaaatgtaactacaaccacaaccatattaaacaaaaactcacaatttgtccatattttttaagttaaaaatataggtttaggattcaaatatttataaaataaaataaaatgaaactatttgaaaacatagtttaaaaaagaagaagaagaagtgttaaataaagtcccattttttaaaaaaatatcaagaccgatattaatattatatatatatagaaatgtacacaaagttaaaaaaaagtatcctataaatatctaagtttctccccgtctagccttcgccaaccttatctcaaaaactcggaagcc

SEQ ID NO: 135 - DNA, 2000 bp, Cucumis melo
  source 1..2000: mol_type = other DNA
tttacatatttatgaacattttcctatttttgtaaatatcttgattcaagatttttgttcgatatatttaaaaataaacttattttaaattcatacttctttctccttctatatgattatataagtattgtagttactatagattaaactcataacctcctagttagatattgagattattactttcttttattatcgggccagtacagaaacgcttttatgacgattacattcgtcattcgtcacttatttgtgcattaaagttggcattgtaatgtttgtttttacatgattctctattccatagatttcctttatccttttccttgcatttgagtggccctttcctaagatgtattcttcggactttcaaataaataaagattagaagcatttttctcttcaatattgacttcatccttaatccttaagccttaagcggaggctaaaaaggctttatttgcctcgaatcccaactaattctccctctcatgcccatttcaatctcttgcctaattgttaattaatgggtcaaatttcgtattgaatttcaattttggatcaatcctacgattatctcaattaggggtcaaaattaatggttgatgtaggagcaagtggaagacacaattttggtgtagcaattggagcttcatcatcaacaacatgagatttaatcccgtggttgcagttaaatggtgtagaagaagtagtcaacacaacccaaggtgaagaagagggagacaagagaagtggttgaggttgtggctctatttgcctatggcagccttcacctcttctctctcgctccctctccgtttcaatcccttatccccttcctctccccgccattttcttcttctcttcttcttccctccaccaatttcacctcccgattctctgccctaaccatctcttcctcctccttgcactccgcctccgacaatttcgatcatgccaaaagctcccctttttcatctaaggtctgattcatttctgttgtttgtttaactcaatttgtcttagttatattcaatcgggattttgcttgcttgtggaattaattttcgtttattaagtggaagatatgggtatgcttggtgacactgtatttactgttaaatttcaaacaatcctaccaaattttggtttaaattgagtatttttagttccttcttggtaaattggatttgcgaatgattaacttaactatgttggcacttcgttgtaagaccgttaactatttagcttccttacgggtaatgatgtttagaaggggggtgcttggtccactaagtggagttaagtctatggtaaacatgttggcattagtaagtttttggtaaacatgttggcattagtaagtttttggtaaacacgttggcattagtaagtttttggtaaacatgttggcattagtaagtttttgtttgtgatgtagagttgtaagattgagttctttaataatttgagttgtaagattgaattcttcgataactgtgaaaagtatattaagaaagtaagatagagttacttgataaatttgaatagtggagataggggcaagattgagttccttgataaaagtataataaagtaaatgtgcaactcttgcctatatacagcttagcaggaactcttacttttgtgtgtcatgtattcttattggttcgttcttattgcatttagtagatagtggatcccagtgaacttttttaatcgctagaatggcgccttaaaaagttagttggagcttctacttgttggttggtatggtgcggttgcaagtatttttcctttctatgattatgtttttagatctaaattttaaagcactcgatgaatgctgatgcttgatatgttttctgtgttaaattcttttgttgatgaatattatttccatttttcagaaatcagttctttcatctttgatacaagagatagagccgttagatgtaagcttaattcaaaaagatgttccacctactactgtggatgct

SEQ ID NO: 136 - DNA, 2000 bp, Cucumis melo
  source 1..2000: mol_type = other DNA
ttcttgattagcttggtgtgctgttgtatatcatatttggtgcgagcataacttacccttggctaccttgcatctaccctaagtggtttagtcagattgtatgatttgaggtatttcgtttctttgttgctctaagtggctttgagcttctactgagggaacctaggacgtctcttctttttgggatcttttttctcgagtagttggatgcctagttggtttttttgttcctttactcaagtcctttgtttgtcatttgatcgtgtcaaagtccaaatgctttctattgcaattcagtatcttaaaaaactgttctttgttgatttatgtaaatgacatactgtatgtataaaaggacagaatgctaccatttcttgaagtttctggcacttaccctgataatcgttacggtaattattatgtgcagattgacggcaataacgcagctagcacatcatggtatgatatttgtacctcttgggtacacatttgggagtaagatgatggaaatgaatgaggtgaaaggtggctctccttatggtgctggaacctttgcagccgatggaactcgacacccgactgagttggagcttgaacaggctttttaccaaggtaagtatgttgctgagttaaccaagaaactcaaaaactaatgccatgtttgaaatgttgttgggtatttgaaaacgtgttattacactagcacacttttactgtacttccttccaacatctattattcagcttctcacatcatggctatataaataaaggttaatggaagttactaaaaatgatgtaaatctatcacattgttaatactcctgtaattatattgattgatgaacaattcgatcaccatcttttgttatttaaaattaaacttgtaatatgtattcgaacgtttttagctttattgcatgcttattatttcactgttttaaaactatctttagacttcaaatcaaattctgaaaaacaaaattaagttttcacatacattatgtcatgaatataaaattttagatattttagttcattttactatatttaaaaatgttttattattattaattttgtaaaacaaccatgatcgtttattaattgaattgtcacaattaagccattatttttttttttactttcctttttcccatcaatttctttattttctaaaaattattggcctcccagactctttgttatttgcaaataatgagtctaatcataatagaatttcattgataaaaccaatcatagcgagtcttaaaaccaatcatagcgagtcgtaattataaatattattgaattgctcttggtccagtttagctagaattatgaatttgatcaaattttctgttatcattaccgtataacaataaatgataaaattcaaaaaaaaaaaagaaagaaaattgatatgttaacgacaatggtaatgataaccataattgtaatggtaaccgtaactacaatacataatttttgaatccaatgagatgaatcacttacttagttgatttgcgtaccaaattatagaacaccaatcatttttgtaattaggattgatttactagcgttagattagagaaaagcttggcttatttctaattcctcctccctcttccactcattttgtccttaactaaaacatagtgatagttccctttttcttttagagaaaagaaaagaaaagaaaagaaaaagagtgttaattggtaatacataataacatatcacatacataaataaatcatgccgagttcgccttagaaacgacgccgtttaaagtaagtcaacaagtcaacactgacagctaatttccgcaataaatacgtaaaaatgaaaagaaaattaaaaaacgatataatataaatagaagcaagaggctcccatcacaagatcccattcgcaaccacattccggccttgaggcttcaaaaaatcgaaggaaaacactctctgtatctctcccctctacccaccgattccgtcgcggccg

SEQ ID NO: 137 - DNA, 1575 bp, Cucumis melo
  source 1..1575: mol_type = other DNA
atatatatatatataatttaactaaataaacaaatgaaagaaaaaagtgagttcccattcggaaaatgcagatggatccatttcttcaaatattaaaaaataaaaaataaaataaaataacttaaatatgcaaatagaaagaattttaatttctggattatccatatgggacaatttttaaaactcatttattttattttttttatttatttgattttgatatatctatggggaaatttttcgtaataattttcgaaaaaatattgcaatatatcatttgatcagatcggtattattaaatctctatcacatttggtcttaaattatccaaagattcctttaagataatttagataaccatctacagatcactactataatcaacaaaaggaacaacttaaattatttaaacaaattcattaatattagactttgtgcttcattagaaaatgatcttatcacaaccacaaccatagtggtggtttaaaattttattttaaactcttattagtattattttaattcatacttaatcaaactaattactttaaaaaacatatatatataaataagttaaatcattcccccttatctaaataacataaaaaaaaattgtttactctacaagaagtttgtatatatatatgctcggtactatttagcatctttataataaaatttctaaatcaattttttatatctctttattaaatgtatagtcatcaaaaaatttaacgagataatgtgtcaaagatttattttattaacgttcataaatatcaaattatacttagcttataattgaaaacatgttcgataaatataagtaaataaaattttattttttttaaatattacaaaataaactaaataagttataaatatgacaataaacattatatattttattatatttataaatacttaataatttagtcgtttaaaataattttcttaattttcaaaacatgtttcatatgttaataataaataaatggaaaaccttccaaaagaagaaaaaaagatatcttaaaatttaaaaattgagattttgaggatcaataattaataaaagaaggattaataagggtgaaattaaatcccaaaaagaaaattgaaaatgaagaaaagaaaagtgaagaaataattgaacgtgggaagtggattcgatgtctccagagaacaagcgaaaggagacgaaatccacataatttgcacgttacgtgtccctatcaaccgtagacacgtgtcaacatctcaacaccctacgccgaattgcttcgctggatctggacggtcatcggataacagcggcaaccaattaatatttccccttatatttcacagcctggccatgtccaccaatcacgttcaactattaattcatttttcatttcctttttctttttttttttaattcccctcaattattaccgacaacctgttgtagccggttaaccctaccctccaacgttccattataaggcctagaaaatggacgtgaaaatggagtactacaaactacaattaattttaaagaattttaattttaaagttctctaattactattagcc

SEQ ID NO: 138 - DNA, 2000 bp, Cucumis melo
  misc_feature 1..2000: note = n=g, a, t or c.
  unsure 1..2000: note = unsure at all n locations
  source 1..2000: mol_type = other DNA
ccgtcgggaacctctgctctgacataattaatattcatgtatttcctgatacccatgcaagtcgtcgggaaatatgttaccaattttcgacgccagacgagaatcgttaggaacaagtgtcaccatgcccaacttcttgtatggggcatcaggataagttaaatttcttttttagttgtgaactattcccgacgccataaacctagatgtcggaaatgtcttcttgtttttcgacggcttcgtgaatcttcgaaaaaacgtaagattaaaataatgttttcgacgagttccgacctgtgcaaaacgacatcgggaataggtatttattccaacgttctagcttctgacatctagaacccttcaatttcttgtagtgccagtgcaaagattgacactcttaaacgatgggacttgtcaaatagatgttgcgcagatatccataggttatctaaggttttgttttgttacctaagttatcatcaaacttcttcatgaattctcttagctatttctaagtacctaagttctcctctatccactaggattgtctctcttaaagtcaagggtggctgttggtaggatgtagactttgtcggcattggtctaccaatttaatctcttatatccctaaagacctagactccatggtctccacctatttccataaatgtacccataacatcattaaatgaaattattactcaagtacaaaaaaattgtttaattttattgataaaaaccatatgtgaaaaaatagatgacatttttaaaagcttgtaaacagtgtgtgaaataagtatcctaagtgaaggctattaatttaacttaaacacaataattattattgttttaatgatgaaaataattaacttatataaccaattttcatcaacacatacataccttttgtataaacatttatttgaacacaaatgagagacaaatagacatttttatttggtaattttctcagcattattaattatcattttcagatatcttaattgaaatttctgaataattttttatttttcggattttcacattataatattttgaattagttagttgaaaaccaaagccagcatcagtgaaaactcattaatacatgtaaaatactaaaattgtttttttaaacttctcaaagaaaaaaagtcttaatttttattttcttaacttgacataaaaatcattggtgttgtttttaataaagtaaatgttaaagtagactcagttaaaaacgaaaaaaaaagttaaagtggactcaacacttggagtaaacattttttttaaaaaaaattaatcctaaaattatgattataatttttatttggcttaaatatttcaaaatgtgttacacatggtttagtttcaatttagttgttacaaaatttattattgtatttgaatttttgatagactaattaaaatttgaaaatcaatttatttatacagttgtttttcttttaatgatgtaaatagaggtctaatgattttaacttgtaagggttaatttttcttatgatctaatgtaattcaatgagcattaattttagaagaaaatgtgtacttattttgtgtaaaaataaattataataacaattttttcattttggtataacgtatgattaagttccatgaaaaaacaaaataaaaaagaataaaatatttttccatttaaagaaaaacaataataaaaatggagggattcaataggaatttcggagggcccacttcccaattccaactccccactcactcactcactcacnnnnnnnnnnnnnnnnnnnnnnnnnnnnnnnnnnnnnnnnnttttttttattattatattagaaattaataattattgtttatttcgctgtcaaataaaaataaaattgtggggcaggtgcagctcacgtgcctcctcacattgacaccacatttaaacactttcattttcaaaggctgctgctttatattcttcacaaaaacttcctcttccctttctcacactacta

SEQ ID NO: 139 - DNA, 1006 bp, Cucumis melo
  source 1..1006: mol_type = other DNA
ataataataataaatacataaaataaaaaaataataatagtaatgaaaatcaatagaataattttaaaatcgggaaggaagtcgtgtacaatccttgcacgttggagagtcaaatggcctaagtggtgatgtggaagtcgtgtaccgggtacacgattttcctacaagtcaataataataatatggttattttttttctagtttagggttcatgacaaaagattgttcagtcgactggatgtagacaaatctaaaaaataaattaaaatctaatatgaaaactagttttaatttccaaattattaagggttgaattcgaccaataaataataataatacggttattttgaaatttaggaaattgaataaagttgttaaaatcttcaagcaaattgttaagccccgagatattaagaagaggtaataatagaggattctatatttataacatgttaaaattaattgcaaactcataaatgcatcacacagattaacaacataggagggacttccgataaaagtgcaaatattgaaataattacagttcgcgaacatgagtattttaatattttataaaatagtatgcacgtgtatttttgccaaaagaaaaaaagaatagattttgccatttttcaaagtgactctcggttatatcttttatggcgattgtattttatagcgtatgttgtttgtagttaacccatttctcattggcaaattcaatcgtgggccacaacgtttgggcatagcttcaatttggattaactcaattatgtctgaatgggttggactagttcggactcttcggctgggccagaatcagattcgggccgcaatctgttcatttcacacctatatccaaacacccccaaaatcgatacccatcaaaccctaactctcaataacccccatatataaattccttctttagggtttttcatcctcatacactctcaaacctccggtcattctcattttccctgccgcttcttcaataaccctaatc

SEQ ID NO: 140 - DNA, 2000 bp, Cucumis melo
  source 1..2000: mol_type = other DNA
aaggagtagactctcaagtccactattctaacttcttacccgaaagagccaaaacttttcattcaaattcaactagaaagttattattgatctatcaatttgattttaatctacaggcgtgcgttgcaatttgggaagggattgagtttgtaactggagtacgggcaacctcattgaattctcttcgatcaacgtggggatgaagttctttcaccagttggagtctggaaaaacttttgctagactaacctattgctactgccttttggtgaaatctttgtgctctaatattaaaaagactccaactttgaatcgttaattataaactagtgttatttgcttgtaaatcttacttatagtttgaaatgagtgcttggcgaaagtgttgttcaaatcggtacgtgtaagtttaaagattcttatttcagctttgaatcagatcagagtcttttaaacttaatcaaccgacaccaccacaccccactcttgttcttctccacgtgggagttcccaaattggttgatttgttatctctttgaatcatctcaaatcaagaaatttcagaacaggtttggggaaatttgataaactacactctcttgctcgaactttgcaaggtttttactgtttgttatatgattcaatattcccatttcttctaattggatgaactgttgaaaattggaaatgctcagctgccaagtttttttccgaaataggtataaattcaaagattcaatcagtgtgggtttacccaaaaaaccaatggggtaagtccattttggactcatgtggagggcacatgtttaggcaaagccttatctctttgccagtgggctcacaatcaatacggacaagacaagaaatgcttcctaacaccgtcattgtcagcgaccatgtgagctttcagcaaattggatccttcaagtaactcacgtgaaagatatttagtgattgacttaattactctccccttcctgtttatctaaattaggcgaatagatccaaagtgggtatttttggagatcatttatctgtttcctgttcttgtttatcgtttataattattgattgtttttctggctcaagtaaaacgaggactttgacatttcaatacccccttttttgttttctggtaggtagcgctaagtgggtttctgatatcgtactgaaaaagttatagttttgctagaacactcgatagattttagcttttgtattgatttttttgttgatatttcctggtttcagtgaatgaatgatattcttttatgacggttgttgtgaagactcataagtttgtctcagatcttcagttatactcttgaagcttcttcgttcatacttcaacagttcttgtacattttaccccctctgttcctctttccatcggcttgtgaatctgtgattgtaaattgtgctgatgattgtttttaagctgttgagatggcgttggggttgtgtcctaatttgagactggtcaacttgatcatttggggtagtgatggccttcttttctatatcattctgtgaagagtactttctaaccgattttgttaaaaacacatgtcggattgcttgcttgttttgtggtgtttctgatttgtgatatgatttgattaatctctgatcgagttgttatgaatttgattgacagcaattgggggaccatggaatcattgtggttcctctcatagattttgatttctgaggtgttgagaaggctttaacctttttgtcactgaaatggatggtggaagctctgaatccccagatatgggttgtaacaagaccatagtatggtttcgtaggacctcaggattgaggacaaccctgctttagctgctgctgctaggaatggttttgtatatcctgtgtacatatggtgtcctaaagaagagggacaattctatcctggtcgggtatcgaggtggtggttgaagcaatcccttgcccatttgaaacagtctcttaaatcacttggtgctgacctagtgctg

SEQ ID NO: 141 - DNA, 1556 bp, Cucumis melo
  source 1..1556: mol_type = other DNA
ttttagtcattatacttcaacatctcgttggttttaggtttttggaaagcaaacctacaaaacacactctttcattcattggttttaagttttgttgacaactttttaggagtgctttgactaagatttcaaagtcttgtacttaaaatgatgcatactatcgtaaaattagtataagagactagatttttaaaaaagaagaagatcggtggaagtatgttctaatttctaagtttttcaacacttacaaatttattgaaaaacagctgtcggtacatgcacacatactatttatggatctacaattccaagcatagaagagtttagtatatatccaaattcttatttttaaggggaaaaaatgaacgaaagaatgcattgtattctcgcttttgtcgtgataacgtatgattttcaagctctttcgtcgaaaaacatcaacaaacaaacaagctaagtgtaatctaaataatcttcaacatccttggaaatttattgaaaaataaagatggctagcaatgcatactttttatggatctatatcccatttcaaccgtagaagattcaaagtattcgaattcttaaaaaaacaaaacaaactgccttgttaagataaaatggaattagaatgaaattttcaaaattgaagtggggccttgtaaaagaataaactttgtttgaaaattaatttccatcgttggttggtagatgtgtccttaattgaaaaagtggaagaaatgaaggatgaatatgaaagttctgaaaagaatatggacggaattggaaaaaacaaaaaacctaatttcataaattaaccagaatctaaacattgggggatgaagggagcggaggccattcatgtaattggccgtacagattcatggtttaacaaaagccacaacgactcccattcttccaccacagaaatttcctctcctcctaaattcacttatctctttctatataattgcttcgttccccaactttctatcttcgtgcagccccattcaatcccccattttacccacttcgtcttctcctttctccttcgtcttccagttccgttttccccatctgggttctcctgatttctctttaaaatcaactacccatgttcgactttgaggaactggtgcgttggaattgagctttcgaaggagatttattgtttttatcacaacccatctgctcgaggtaaggggtaaaacccgggttcgtcaggctgtagacatcacggctatacacgtagtttcccggtcgttctttcatgtccgggctgtacgacggaagggttgtataactccgacaaacccttcgccgcacggcggacgtggtgctttgccttccgaaggtggtagtccttctgatcttctttttctcgccggcggtggattctcttgcttcttctcttcttcgtattagctttgcaacgagtccgtttgtgttttagctctaccggtttaggatttgacatcagcaagtttctgttttgcgtttctttgttttgggtggggagattttggtgttgggtttggtttgaattagaagcagacgat

SEQ ID NO: 142 - DNA, 2000 bp, Cucumis melo
  source 1..2000: mol_type = other DNA
gagtacctaatctaaactaattaactcgctcaccctcttatttactgccccatactaatgatcctaatagattgtttggttgggttgataaattctctttaaaattatcaagttttccaatttttgccacctaagttgttttcttacaaaaaataaaaaataaaaaaaggcaatgttatttctcgtatgcattaattgattgattttctcaactaacccttcaatttgactttatatgtaataatagtgtaaaatatatacgcacatacctacatatgaccaacaataaaaacgataacattaaattcagacagaaataaaaattacgattatgattttaataaatataaatgcacataaataaaatttacagttcatagaaaaatccgatgtaatgaagtttaaatcgttagttattttatttcgtaaaataccaatttatgatttgcatgacaaatttttaaaatataacttatgaaattaaaagttggttttgagaaaacattcaagactttattacaaccaaacaaaaattttattgagttttgtttcattaaaaaaattattaaattacaaatatttggacttacgtaatttgttttctttctttttagggtagaaaaatatgatagattaaaaggattcgaaatcaaactttatatcaatttccttttaaataattatttctttccaaatttagtttttatatgatagcctaagtctccatcataagaaacaacgttaattataataaaaaatggatgtagattcaccaatattttccaactatattattactttcacgtttacattaaaattaaatccacacaataatataatagttttctttgtttgattcaaagtttctcttggttaaaattaaatttcgaaatgataataaataaactcgtgattaataaactttaatttaaatttcaaacttaggtgtctaataaattcctatattttgtatcacaacttttcaattatgtgcaataaattttctaatgatttattattttttttaagaatgtaaagttgattatattcatattaaacataagattgaaaagagagagttgattatataccgagtagccgacagtcattggaagcattaacccattatcatctccggcgagcaaaagcaaggatctacaaacaaacatgacaattaatatgaaactcatcaatccacgtatccaaacattccatatgttagacatggaagagcaataattacaaagctctctcatcgtctccgatcactccatttatcgtacaaatccgtctttcttcaccttaatcattttccccgaaattcatcccactgtttcgcaacaaaatccaagtttggaaagatgagtttgtttttagtgatcaaggaaaggacaaagaatgtagcattggcaatgacgggcaaacaagagaggtgtggctaaacttatacatgcttttgtttggtgaaaggttaaagcgaagaacgccaaagacagaggaaaccgtataaaatatgagtaaatgtcaatgctaatgaatgggcagaggtgaagcggtcgtctatggctggagaagggcagatgtgaaacaatatgaggtagacgaaggtggagacaaaacaatttagtaaagtcaaaacaattcatccatatcctaatccaattatatttctttaaaaagtttaagtatcaaaattggactgcttgatcatctatcaagttatttttgaactttattttaaaaagtttaagattattaataaaaatgtaatgtttaaagtggttagtgctttggaagccattacgtcctatggattatgtggtgtgttgggctactctctatttggacatgttttgacgtaccgtgcgaagtcctgactctatttgtaaaacgtcacccggcaaaaacccaacttaaaaaacagaactttatttcatttaatttgcggggtttatccggaaagaattgtgagagctctcttgtgtttggtttgcttatct

SEQ ID NO: 143 - DNA, 2000 bp, Cucumis melo
  source 1..2000: mol_type = other DNA
gtaatgcaatattagcaattattttggagcaatacaaacaactaggtttggatcaaatatcacgaaatacaggagcaataacattaacaacaaataaatgcacgaagtttttttttttgaacaaacacttaactctctccaaaccaaaacgagctaagttagacctaaaaaaacaaagtatcggaatacaatatagcttaaacaaaaatcatgtttagattattggttaggttcatctaaactagtggttagccatttttcaaaagaaaaatatgatttgtccttgctaattttccaaatctatattttaaaagtatcactctcgtcataattttccatagctcaattaatactaatctcacggtagcttttaattgttcttgacaagtaatggattaacttaaaacatttatataactttgtaggtattattttatagaaaaattagtttatacgtgaaaacttcttaaatatctaactacaatcaaatacctagattacataatgtatttttcataatatttatacattatatttgaaaaaggactctcatttcttttattggtatctacgcagaaattaagattttcgagttgcgacatctcaatcaacgaaccagctaagaagaccggcaaattccaaacgtatccttcgggaagcactgagtgtttccacgtcaataacaaaatattgacccaataaatttcagccacgtagaaacaaagcaatgaaagccgtcggattctccacatcggctaccgtatgccgttaagatcatcaagtagacttctaattcccatgtcttccgtgggggccagaaatggaaaattgaaatcgctttatccacgtcaagctaacaaaaaacaaccaataataattcgccacgttttctcattagaaaagtgcaccgttggatcatccacgttggcaacatagatcgatccgatggacttatataaatttgggtagctcgtcgagaaatcagatcagtgatcgaagctactggaagtttttgctaagaaccatgaggaagtggacgatcgcttctgctcttctccttctttgcattctctctctcgttcccgatgaaggtgtgatttcgtttcttccttcagcagtttgatttatttgttggaatgtaaactgaatgcattgcattatcttaatcacgagggctgatgctttaatttttgggggttcgaggagaaatttggatgagattcgagcttcgtttgaactgcgaaggtttgatggtgatatttctattgtgtttgaattttcaggtcctagatttcatgccaaggccgacggtgatgccgacgaggttgtagatccaccaaaggttgaggaaaaaatcggcgccgttccacatggtctttccactgattctgatgttgttaagaggttcgtgaatgtctaatctcgttgatacacgcttcaagtatagatttgtccacttcgggaaaaaaaattatcgaaccttcttttgaatgttgattcagagagtcggagtcaatctcgaagagatctcttcgcagtagcggggagaaatttgagttccaagctgaggtgtctcggctcatggatattatcatcaattccttatatagtaacaaagacattttcctaagagaattgatctccaacgcttctgatgtaagttcactctgcctcttctcacttcattagatctagtaatctcattgttagatttgtgttagttaataatggcgtctctgcatttcaggcgttggataagattaggttcctttccctaaccgacaaagagatattgggtgagggagacaactcgaagctggagattcaagtgagttcgaccttcatactgacatattgttttcttattacctcgctgaaaaaagctgctcgttctggttgatgaaccttgcatacttttattgttgtccataaatcaaatatcgcagattaagttggacaaagcaaacaaaatcctttcaattcgcgacagaggtattggt

SEQ ID NO: 144 - DNA, 1337 bp, Cucumis melo
  source 1..1337: mol_type = other DNA
ttttttttaattttctttttgcagattgtggggctgatcgtccacgatatgattccactttggctacgaggggtgtcgggcaccttgtccgtaagggcactggtgggagatcgtctgttaggtaacctagccctagctttttcgtgtttggattcttctatttaattgttggcttgatgttgtagatgtaatgctgggtttgagtgctttgaaatgttgagggaaatttaagaaatttaatgggatgaagatgaacagtggtacttcaagcctcaaattgaattaaaattattttaaacatcctaaattggtatgactaagtattgctaaacatgatagtcatataaaagcgcaaaagaaaagaaaaatcacccctctactaggattggtttattctatggatttttgccttcagtgttcttgaagtcacaataataaaagtagtaatagttgcagtcacaactcaaacctttatatgttttttaagattgtggtaaatattgttttgatcattagacaagacatagagattttaagtctctgggccttttcacgaagccataagcctcttatggttcagcaaaggcatactcaaggctagaagttaaaaaagccttgccttgagatgtaattctgaatacctttttaaaacatttggtacttcaaatttataagtttattagtggaaaatataatctttcagtctcttttttagctgaaatacttataccttttttccccattgtcattgatttcttaattcatatgcagaggaaaggactaattagatatactttgttttattgagtaatctaaaagatgtggcactacccactatgaacattttgacgtcattccagcttttatgggatattgaagcaggcaattttaatctgagctggtttctctgtcgctgtcagataatccttgtttgtgcttatgtgttctctttcaagcatgcacattaggattctcaggcagatcagatcattgatatttaattcaatttgtggatttagtttgtagtgaatacactaaattctgtctctggtttctctgatcttactgttttattacaaaattgttttgcagtgggattgttgctactgtcttcggagctactggattccttggccgatatgttgtacagcaactaggtaataggtgaacataaatggtactagcattcgactttctttttgcttagatatgtaatttattacgtttctctataccttctactactagtgggttttggcagctttggctctattcttgatttttatatcaattttatgctaagcatgattttggaaatgaattgtgtttcagctaaa

SEQ ID NO: 145 - DNA, 2000 bp, Cucumis melo
  source 1..2000: mol_type = other DNA
atatgtgacgattaattacctaaaaattaattatttacatagggttagtcaagttgtcccgtgagactagttgaggtgagcataagttgatccgaaagctcacaaaaatataaaatacgtcaatctccatgctttcataaaaataacaatttgattctcatgactactcattcacttatcgtaaactcttttaaagaatattaagagcgtattagtgtagtgggctagtttgttacaaaagttggcgacaaatagatgaaattagagttatctcgagattcgacgagggttaaaaagagcatttgctttaccctgtattttcatcgtagttcatatttatttatattcaaattctatcaagttaaggccacgtatattccaagaaaacataatccattaatggtaatatgaaaaatgagttttaatttgatcatgttgtcggcattatgtaatcacaaagatatctaaagctcaatgttaaatctaattaatggaggccgataatccaattatatttgaaaattaagtggaacctacggtgagatatttgtactatcacaattacaattactcttacttgttcggaaaagaaattttgtaaacatgtcaaaattatcgttactattccaaatattgtcactgacctgaacattgtcaaaaagaaataaataaataaaataatattagataatgtaaaataaaccacctaaactttaatctattatggtcgcaaatgctttgataacacataaaccgattgatccgtcaatgaaattttaccataatctttattatggatcgataaatatgacttaattttcttttaaaaaagtgttttttaatttaaaaaaaaaaaaggaaaggaaagggggaggggcaaaggttctagagtgttccaaataggacaatggaggagggtctccaatggagggaggagccaaatccaacggccaacaattgctggaagcttcaggagcctacatgattcttgggttcgtttttctctcctcttcctatccatccttttgaaatttgctataaagaaacctacttctcttctccttacaaaaaatccattttacactctctgtaatacccccagttttgcctcactcgcagcgctcatttctcaccctcttatccaaatcaatccttctccctctaaaccctaaaacccctttgcacctccgccgttttcttgtaagattccccctctcttttcattctgttggactttcttatccttttactttactgggtcatgcttacatttctatttgggttttgtttttgcttgccgattcagtcttctgtattgtgttttgagctttctgactgttttggctttctgggtttcaattgttggtgtagacttatcgattgattcgtttgttttgtgtcctttcatttctgggttttgatttctttaacattttcttcatgggttttggattttgggtcttcttcttgtgtgcatctctgtagcttgctgattcatttgtatctcgtgtttatctatttgtttgagttcctgacatgtgggtttttgttgttgtctgagaattatgtgtcaaatgtcaattgtcaattcctatgttcttgaatttgtttatgtcatttcctttctgggttttctctgttcaatcttgctacatgggttttgggttttcttacccttgttgtgtgtagttttagctgatttttgtttatgcttactgattcggttctgtattctcgatgatttgcttacctggttttttatgtcgtttgagaattgtgtgtcaattcctttgttgttgattttgtttgtcatttctggtttgacattccatccaatcctctctgctctaagtctacttggttttcaattcatgaatttccatcagacgcattgtcggccccctgctctatttgtttacaattctggttgtgaagttgtttcagtttgaactaattgatggtctggtgattacgttctgtatcagtttggaagagggtaa

SEQ ID NO: 146 - DNA, 1212 bp, Cucumis melo
  source 1..1212: mol_type = other DNA
atatatatatatataatggaataggctatttgatttagatgaaagctattacgtcctggggtttacatcataatctctattataatgttaatcgagaaactttataaaggttaactcattatctctcttgtcttcagtttattattgttgtttttatatcggtggaattccacctttcaccaactctcaagctgtggtgtgaatctatgggattaatctagggcgaataagggagctgagtattttctatttgtggaattaaatctatagtacacaaaacatttgctcaactactaaggatatgaaaacccttggctctgccaacatggcttatagaaagtatctgaaaacgttcaccactttgcaatttcaacaataagtgtaaattcttttcctattgttgttatttagtcgatttgatcgttgtacaatatttgctgtaacatgtttgatttttggccattttagtgttcacaagaagatattgtttgttataagaatctacctgatccttttcaattgttattcaatatattgcctactccgttgacagcaggtccatgcagaggaacaagttctaaagttcaaactcgatgctgatattcttcaggtactacttttctgttttcacaagtttgttgtttcaatagttctaagacagtgacactcatccctttatctccgtaacccaattcattaacgatgacttttgatcggtttgaagaaaaaatttataacactttctcatctcgttccctttggattttcagtttttaaaattgcatctatatgtattcttttgttatcaaattttacttgataatgacttttaaattgtactaactcatttagatgtgaatattaataattttaaacttcatttctgacgtctaatactaataaaataataataacaattatccttcttaattaaatatggtttacctaccggtctattgttctgaactggatatattcaatttgttttatctgaataatcttttgaggttgagttatcaagagcctgtttaacttacctaaagcatttctaacctgaactatgccccatatgaatacttcattttctttattctattgtaaaacattgttgttattataatttgaaacgcctgtaatagtttttacgatgtcttgcaggagtctatcgttcggcatgtaaacgaacacccacaggctggctggaaagctacc

SEQ ID NO: 147 - DNA, 2000 bp, Cucumis melo
  misc_feature 1..2000: note = n=g, a, t or c.
  unsure 1..2000: note = unsure at all n locations
  source 1..2000: mol_type = other DNA
acatagtattaataaattagggaatgacttagttatttaatttaagcggtagtaaatattattaacttttgttcgttgtgttattttactttcaaaacgttcatcttgatctttatcctttctaatatttatttattttagttaatatcaaaaaactaaatttaatttatacgttaagttacaacttcatttatttcaatctaaaacttttagaattacactttattcactaaaaaattactcgtaaatgcaaccattccaaaaaggtttcaatattatataaaatatcataatttttcgaacattcttaaaataaattaaacaaaatagtagttttcatatacataaaattcgaataaatcctcatacaaaaattttaaatttgaatcatcacattgttttattttagataatcaatcaaataatttaggaaaagagaagaaagaaaagtaaaaggaagttgaaggtattttatttagtgatagaattataaaatagggtattttagaaataaaaacacaaatatataaaaatacagaaattgatgcatttaatggaacactatttgacaatcaataagaaagaaaaaaaagaannnnnnnnaaaaaaagaaaaaagagaaaaggtttggtattgggtttgtgggattttattaataaatgaaataaaaaaaaaagaaagaaaaatttaattgattaatttggtgggagaatattacaatgaaaccccactttgtgaacaaatacattgcatttgggttgtaatcaagtgtacatgcatctacccaaacctttcttgaactcaccataaatccttcttttagaccgcttcgacttcccaatttttcttcactttttttcccccttctctctcttcctccgtttcccccccccttttttttccctatctcatagggtttccatccaccttcttcttcttccgttctctcatgcattgtcattcacaatctcattctgaattcctcttgatcttcttcatcttcatttcctccttattttttgctctctttcgagggtttttcggttcatttccgtccagattccaccacctcccgtggttttttcacccatactcatgtcgaagctcttcgccttttccggtaagtttatggatttttactgattttttttttttgtttgttttgcctttctttggatttgacttagattgggtagctggtagggttaagcgtcgtgttttgtatgggtgtttggattgttatttggatcgtagggaaagatttggaattattggttttagtttttgggggtttcttgattcgccaggtggcggatcatggcttggtatgaattgtgagggaatatggatttgggtttctttctattaggattgttttattgtgttgattgattggctattttattgtcttgaacagtccatgccagatgtaagtttcttgaaaagagatatcgtagtttgaagatgggtttaccttttaagtgatgtgtatgtgttgttgatctgtcgttcccgtacagatttagatttgaggtttagaataagagagcacatcaatagtaaatattaaagggtcaaatatagttttgcagagattgcttcttgtttttctctgttgataaattttcgatcttttgatctagaagttgaggggtattttggtctgaggatttatttgtgatgttggatgatgtatctaacttgtagttcttgttgttgaaatttcaggtagtgaagatttttgcactggagggtcaatatacccaaatcccaaggactccagtttattcttgtcccttcctcaccacgttgatgtctattttcctcctcgaaagaggtctcgcatcactgctccatttgtgtttggtggagaagaagttgaatcaaaagcaaatgtttctatcgagattcttccggatgagtgcctgtttgagattttcagacggttgtctggtggcaaagaaaggagtgcctgcgcaaccgtttctaaacgatggcta

SEQ ID NO: 148 - DNA, 1254 bp, Cucumis melo
  misc_feature 1..1254: note = n=g, a, t or c.
  unsure 1..1254: note = unsure at all n locations
  source 1..1254: mol_type = other DNA
tcataaatatatatataaaaaaacaaatattataacctaccttttgcaaatgataaaattgtaaagtctcgtgccgataatgtgttataaaataaaagaacaaagaaactaaataagaacaatgcaacaannnnnnnnnnnnnaatagagaagagaggaagaaggggaaacaattaaaaactcaattgtagtgtgacttacacaaatgcaacacatatatctatttataggacatatcatggtatatgttatattatgaaattcaatgaaatgaatgttacaataaagaattgaatgagagttgtatgaaaattgtaaccttcataaattatggatatctactcttataatatatcattatatttataatgtatactatatgtttgtattttaataagaaaattatcccattggatttgcgatcttagatctaacctactaaacaaatattccaacgaagaggaacgagatgagaacgccgttctaacctacgcaatatcaatcgtttcttcgctgctactttacgcctcaagttcctacccttcaagtttcatcttcaacgatcaacccaacgattaacccactgcaccaccttatctcttgttggtgtcatctaatccatcttcttcctgcatcttctgcaaatgctctcaggttctttcctctctcttgtgcacaaactgatcacccatgttgttcgccggaaaatgattcagattcttcgtatcttgcctgcattgtctttgactataatatgattgaaattcacttgttgattggttttcaattgttaattaccgttggttttgctgtttagtgatagtatattatgaggtttttgttcgttttcgggtttttggatgtgatttcatcctatagaatgaagagtatgcaacgtatgctgtcaccttgcgggggaaatggtacacgtggacccgaaatggagctaggttttgatacgtgcagtttgagttttggttttgggaggatttggcattcgttatatgaattttgtaattaactatgccgtttgattgttatttataacggtgcattgctttttgaggtttagaatttggacttaacgcctctttctattcatggttattggttttatttcttcctttttgttgactgagattggtcgtagaactcgttgcctgtctatgttttaatgttggcctgattttgaatttctaatccatgactaagtatttctttattgtcttgatatagttgattgaatcatcaatc

SEQ ID NO: 149 - DNA, 2000 bp, Cucumis melo
  source 1..2000: mol_type = other DNA
cattttaaattgacctttcatgaaaaatcgtatgtttttggtgtgattttgagtataataaaaatgattttaaccatttgaaaatcactttaaattacacctaatgggtgactgaggttttagctttcgtctttgtttagctctaaatttgcatggcaagttttccattccaatgattgatgtggcttgtaatagttgaaatatatatatatatatatgaggtatcaaaatccccagccttgtgttaggttgaatatggagggagtggggagttatttttcctgctcttaccccgttcctaattcccaccttgtttactatgtgttattgttattgccatatttactatgtacataatatttcgattagaaattttattgtttaaccattagacaattttatatgtctaaaccataggtttgaacaaaccatttagattatatatatgttgacaattagattgatagggcaattattttgtttatcctaaaaatggtaaataatgttcttaaacttggttctttgtgaaataccttcaactttcaaagtttttaataatattcttacgcttataaaaagaaaaaaaggataagttgaaaaaagaatacttctatgataagttttagatggaaactatttactttttcatttaaaaaatacttttcaaatttatgaagttccaaaagtatgacttaaagaaatagttatacccttattgataatatacgacaaaaacaacgcaatatttcgttacaaaaataaatctagctgcattactatcttactttaaagatactcttatcgtctatctaaactaccttactctagaattaataattaagttccttttactttataaatataacttattcctactattagtatatatttatattggtatctaatagctaattttgaattttgttccaaaaaaaaaatatcgctgagttttgttttgaagtctttttttttttttaaatatatattttcgattaaagctagatgttgcagttgatatgtagatttaaaagaaatgtgtgagatcgtttataactatatagaagattaagcatttattacttcaaaatatatcgttaaaattattcacataaccaatttttactcatcaaatattatgtcagagaaaagaaaaacgaaaaagaaaacctacttcaacggacaaagaagtccttagttcaaatcttcaaacctttatttgtattaaaaaatggcatataaattttttcaatttttacgcattacctgttgcgtgaaaaacattgatttaatagaaaagaactgtcctttcagttttgtttttttaaaaccaatttcgaaattcaagaatagaaacaaaactttaagtctagaggatcactaaaatctatcataaggctagaaatacatcttgtaatctgcagtaggcatttgccgggatgacaattttctggtgcttggattaagaaaaaagaaaaaaagaaaaaagaaaaaaaaatggtgaggacttagaggccataatgagtttggcattgggcccacagtaggatgagtaaattataattgggagaaaatgagcatagggtgtggaggggaaaaggagaaggctaaaacactatcacaaatcacacagtagaagatacacagaagaagtaaccacagccattcattgagtgagaggctatccataatctcatcctcttacccttctcatcattcattcaaagccattcaactcaacatcccactcttagttaaccaacaaaatatatatacatccttctcaatttcccttctctctactgctttaatcttttgcttcttcttcttcttcttcttcttcttctgctttctcaataccctcaaccatggctacggctactctatcagtagccaaaccatctattcaggttcctccattactaaacaccatcctctttcccttccactcttctttaattttttgtatctgataaacattactgcattttcttgcatagcag

SEQ ID NO: 150 - DNA, 1680 bp, Cucumis melo
  source 1..1680: mol_type = other DNA
tttttatgaagggagttgttattttcctttgggatttggagggatatgatatatatcctttttttgcaatttgatgacagaattctgcttttagagacttttcaaactgtttcgtaatgaatttgatgggttgggggtggcttagttcaatactttgtgggttgaaaattttgatttgcaataaatgaaagccaaaaatgtggggaagctttcagttcaagtaagttaagggaaaactgcagaatatctggcttgaaataagagatgtcttcgaaggttaatagttttacattgacttttttaaaaaaaagattatattataagtacaaatatgggtggatgtgaacttatattattcaaagagactaatataagttttgggcgcttaatattttatattttcatttagcagtcaaagatgtataagaaaactttggtaatgcattttatactagtttatttatgtaggatgtaggatctatcgaataatacaacatatttttaaatgatgtgtacaattgtgaaaaaaaaaggaacatacagtattgtagaaactaaaatattttctaagatatatcgagatgtaaaaaaaatgaatggatgtcaattccagcataacttaattgttgaactaaaaacaaaaagaagaaataaagggggcaatggtttgatcctcatgccccacatgaaagtcaaagttatgtaaaggttccgtgtaggatatccttcctcctaataaggggagataggattttatgagggtgccaacagctcagaattccaaattcccaaaataccctcttgcttgaaaatttcaaactcttctgtttttgccttgtgtaccattcactattccgatgcgtacagttcattaaccacacaagttctccttttgcaggcaggtttagctaaacttattggacttgctggagagaccaatgttcaggtaagatcttatttgttataatgaactcacaaactaatttagattagccaaagaattctgtttctgaagaaagagaggatgaaaatcatctcataccaaatttctttctttttttggaattatgtcttcacatttattcattttccttgtcaacagggtgaagagcaaaagaaactggatgtgctctcaaatgaagtctttatcaaagctttggtcagcagtggcagaactgtaagctgctatctaatcatacaaatgacacgacaaaaatatctggtgacttactctaatagttgacaaattggtggcagtgtattcttgtttctgaagaagatgaagagccaacatatgtcgagccatctcggcgtggaaggtttgttttccattcttgatgatttttgtctaatgcttacaattatcatcagtatcaactcctcttactttgttttaattttaatgttatttcttcttattttccaatgacaaaggtattctgtggtgttcgatccactggatggttcctccaacattgattgtggtgtttccattggaacggtaacatccctatgctaccttctgaatgagatttcaaatatttttggtataatttctttccaataagctgagtgtatgattgtttgaatatctactttttcatgtagatttttggaatttatcacttgaacgacagccacgaacctaacctagaagacgtcttgcaacctggaaagaat

SEQ ID NO: 151 - DNA, 1524 bp, Cucumis melo
  source 1..1524: mol_type = other DNA
tatatatatatatataggtaatgagtaaagaaatgaaaaagaatgagttgaagaatcacacccttaccattctatttgaaactcgtgagtcttgtagacttttacatgtcttctccttcacttaatatcattctggattttgattatatgtatctttatttctaaacagcttggacagatttattattgttagaataccttgaatatgttttctggtgcttagaacgatcatacatgggtttttctagggttagaggagtgcgctatacataaactttctagttctagaggcattgctgtaatcttaagtttaacagtttctctttaataacaaaaactgctcttcccctacggtttaagttttctccttatcttaacagttataattatgaaaaatgatggaaccaaaacaaagttctgttaaaatttgactaattgattgaatgaacttttgtttccaagattcttaatttgtaaagtaataatgttcttacaaatcattattttgatgtctgagttataacccttaagcttggtggttcatattccattcaggtgaagaagattgtgagtgaaagctgttcccaagaggttttagaagtggcgttaaactccatctcatccctaattaccatcctctcctccatgtcatcgtctaccaaactccattcttcactttgatggtataagaaagtgaattagatttgggattgagcttcaaaacatgtatgatgatgtgaatatttactcgtgtaaataatataacatgttgtattcttgcttgtttctctttgctcatcttcgttttgttaagagcaaagaaaagcttacgagcatgaacatgtgcaaatttatgaaggtcaatgggcttcgtaattttttttccccattgatttaacgatttatggaagatggatatagtaaatttaggttaagctgtacaaaaccagagaattttcattatagtaaatactttacaattttcaattagctacaataaacaccgtttcaaaatctccctcatttgctaccatatttactattcgatatttatcattttttttattcctgttgtaatgtctactatttttcttttaaactattacaccacaaacacatactattataattcaaattaaaataatcactagtataactcaactataataactcagatgatttcattccatgaaagtggtaattataaatatttaatatcttatatgataaggataactatctatttggtgaaaccaaatcacaatgatgcagtggtaagtgctttggactttgaatctcttttttatagtatttcattcttttttcaacgaagcagcatcatgggccttgaatggaggccagctagaacgagcccattacatttgacagagcatctcttcggcccatgagcccaaacactattcatcttgttaaaccacgaacaaatcgagactgccgagagtgtaagagaattgagtaatttttttcgagacacagggagtttagagagtaagtcggagaaca

SEQ ID NO: 152 - DNA, 1851 bp, Cucumis melo
  source 1..1851: mol_type = other DNA
ttgggtcgttacaatatcactgtttaaacttaagtttatttttatttatttttttattttttaatctttttcccttcttcctttcatcttccattcatttatacaaaaataaataatgagaaaattacttttcacttttgagtttaattatttttaagttctaaaatctacattttaatctttaaatttaaaaaaaaaaggatttacaagattcttgagtaatttattattattattattttgaacgtaaatataaccttttacaaaatctaaatgagtgtttgggacaatgagttgattattataagtattgaattataataattttttgtggggtatagactattttaatttgaagaataataggtacgtgtttgaaatataaattatgttagttgggaaagaaaatagtaaatatcgtagaaaaaaataaaataaatgaacaataagaatataaaatatggtaataaattgggactttgaaataatggtaataattaattaattaattgaaagctacaaaacaatgttcacttcattgctatagttctaaacagactaacaatctcaatcaatgacctaatgggtcaggccattatattgggctcaaatagattttggcaaaacgaatcgaaagcccaatggggcctatattatgtagggccgaaatgaatttcaacgaaaggaacccaaagcccaataggcccaaattgagacttacaaaggcgcatgttagcatgaagagagaattgaaagcttaaacagcgccatcacaaaacatttgcattttcgtgttgaaatcgcatttgggccgtaaaccaatgaaacacaaaacaaacaaatcctggaatagcctcaacggttctggaagaagaagaatcttctggaacctccaatcccacaataaaaatcaaaccctaaactcttacattcagctctttgcttaccttatcccaacaaaccttcaccaacgctctaccggaactaaaacccctccgacctcccacttccgacttacgacctctgttgcctgaacatggcgtctgccaatgctctttcttccgcttctattctatgttcttctcacaaggtacttcacttataaccccctcatttcttccttgtatttttcacaattcctctttggaaatgatgatatctagattgtagtagttgggattgtatgttaggtagagattttgtggagttagctgagagcggctgagaatactaatatatcgtttccagtagcttacgttgcgtttttctaatgttgcagagcttgagaaaggtgaatcaaacgcagaacaacagagtaaattacagacaggctggtagtagatttgttgtgagagccactgcaaaggagatagcattcgaccagagttctagaactgcacttcagtctgggattgataagcttgctaatgcagttggtttgactcttggacctaggggtaactttctgtttatatttatttatgaattggttagtattggatgttgttctaatattgaaatccctacaggatatattcatcacatttatagattcgtgttatggttatgttgagaaatttgggttcttcacataattctcaatcttgttgtgatattttgtatttgaagggaggaatgtggtgttggatgagtttggtagtcccaaagtggttaatgatggtgtgacaattgctcgggcaattgagttacctgatcccatggaaaatgctggtgcagctttaattagagaggttggttttttatactttgttatgaagcaaaattttctcatctatcgattattgaagtcttattagttcttacattgcgttgacaagtattctatatgtc

SEQ ID NO: 153 - DNA, 2000 bp, Cucumis melo
  source 1..2000: mol_type = other DNA
actaattaatagtaatttgtatgggatatatgtatatgtgtgtataacaggaactacagagatagagattcactttctagaaataaagttgactgccattggagtttatttggagccttcagttgtggagcatttgcaacaatggaagggaaaagctgctaaggacttagtggaagatgatgacttctttcaggctattgtttctggtatctccctagttatcctatttttaactatactatctcatcacattcctaaatgtgaattacttgacgatctgttcaaacatatatatttcattgtttgatcgtaatgtttcatatttatgatgtttcatatactacctcgtcacacgtgcaaaggatttagatccgttcaaacatatttcattattggatcgtaatgtttcatatctatgatgtttcttatactatcgcatcacacatgagatccattcaaacatatctcattgttagaaagattatacattatttcaattcaaatagctctaaccaatgacaaaattagattcgtcccgtttagcttattctatatatatagatagatagatagatagatagtatggatatgcttgtgataagtgtttttttcttcttttttttttctttttttgttttttttctttttttgtcactttctaaattatctatctcacagttagctagttggcggggtgatgacttttggtgtgtcagtctagtgagaagtttgggggttatttttattttcgaaagcttcctaattgaatgacttgtaaaggttaatgtttatgtttttgtacatgtttttcatgaactattggttttacaagagttacaattctatttatttgtgtaagaaagatcatatcacatttttacccctggtgtgttcgttttatgttcttgatttgctttttgtttttcaataatttacggggaaagagagaataaaattttctttctccgatctccgcattcaatttttttttttttgaaaggtgcattcaatttttttgtgcttattaaatattcacttacatcttttgttttgtttatttttttattttcatctttcttatatgaaaataaaatattttttagtacaacaatagaacctcttgttaccattgaaatgaattacaggaaattaaaacttttactttttatttgagagaattaaaagagtagtttttaaatataacaaaacgactttcgcaatagatccagatgatcatttattaacaattttctaattaaaattgttactaaattttaacaattattaaaaaatattaattgaaaaacacgtgtatatatataggaacattttcaattatagccaaaagttataattatttactctataaaattctttagagtctatttaacctttttgttaaattttgttaatagttttactttgccattcataaaaatttctcatattatatacagtgagaattttataagtctcaaaagtcaaagatttgattaaaaaaaaaagaaatgaaagcatatctaaatatattatttatactttgaaaattacttccgaagcaaaatgtaaaaccgttataagtgaacttagaatccaaaaacatatattaaattaagtttaaattatataacaacacctttggattttgtcattttctaaaataccttttatcatttcaataattgtaaaatgagtcctaaattttcacaaatgtttcaaaaatatttggaggagacaattccttgagaatttcaaagatatattaaagaggacgtattgacccaaatcttttgttctatgtcactatgatcacccttttatatcacaatttatttccatctacaattctaaagaatttataatttaaaagtagtttcaaaatgtttctaaattttcgagggtaatattttaacttttggaagtacggaaagttaatcaaatctttgtctcaaaatctcaactaataactggaattgggaaagctaaagtctagaccttaa

SEQ ID NO: 154 - DNA, 1288 bp, Cucumis melo
  misc_feature 1..1288: note = n=g, a, t or c.
  unsure 1..1288: note = unsure at all n locations
  source 1..1288: mol_type = other DNA
cgagaagtacccggcgttggtcaccggatttttcttcttcatgtggtgggtttaattgttggtcacgtgttttgcacggcgaaggccgggtggtaattattacgttgcggcaagtttgagcttggttgtgtgaaattaccgtgttgtcctttctgttttgtaggtactttttgaacgtgattttcaatatcctcaataagaagatatataattacttcccctatccatagtatgtatttccaatttacattttcatccctgtatttttcttcttcttcttcttnnnnttttttttttaatattgttattaatatttgtttacgttccagttttgtgtcggtgatccatttagttgttggggttgtgtactgtttgataagctgggcagtgggtcttcctaagcgagcagtaagtcaactctttctatagcccaatatgccaattttgtctttttctttcattaaaattgttatttttaactttttcatacccaatttagtttttttagtctgtttattagtcttgttttcttcaaatttagtagtattggtagtctaattggtagggctgttttgaaagtaattacctaatataatgagtatttagattgagacagtactatagtctaaacgatgtcattgcagttttgattgaaattttttctcctttatttatttcgaaaatgacaatataacttctgtaatctttgtaaccatgtttatttgaagctacgttgtaaaggggaaaaagaaaaggaaagtgtaaaatggtcaaataaattatatttttaagtgaatagattatataatgtgcggtaaaatatagcactcacaagtaaatgcaacttagtaatctaaagattgaactatcaattcatgaatttttttataattagcatggttttctatagtttttgggagtctgtttttcaatgaaaatattgccagtatggtaatcttgtatgacaatgtattttctaaagtatggatataattaaattttctttaatttatcggcttaaacttttcgttgtactaaaaatctaggataggacgtttaatatttgaacctttgtaatgccatttaatcaccgattaatatagatctaactattgaaacttcttcaaaagttttaatccaacggatggctaagagtgttaaaatattgatacaattaaatttatcgtagcttaagctttgacagtgtcaaaagctaattcagttattttctctgcccttggtataagggtaactctgttctctctatttcacacaagtgattgctaac

SEQ ID NO: 155 - DNA, 2000 bp, Cucumis melo
  source 1..2000: mol_type = other DNA
ttatgttttattaactccatagttttactaaccccatttcacgggaaagtacaataaaacatttgtgttaaaaaggagttgtttgtatagatcgaataaacattttgtactaattccaatcatattaccaaatgttttaagagcatgcgttcttgtgtgcttgaataggggtgatcatcaattgagtggcgtcagatttaaatttaaagtggcaccaatcatcgacttgttggtttagatcgatcggtagttgttgtttgtgggacaatcatagttatcatttttctccttctatatgaataatagtcaactagatagaattgacatttcttagtattaaaaaaacgaccactgacctgtctatatcactaaactgcttgacctaagtgagtttggttggacttgattgcttcgttgtggtctaattcacttaaccctacttgaaagtaaaggtagaatataacatgattctttccaaattggcaagttgtgacttgatttatgcatgcacgaagattcttccactctccacctaactagtactcgatcacattggaaaatggatctgtcccgtgaaggatcgcaatattacatgccttcctacttttttcttttcttccaccaaagaaaaagaaaacgggacacacaataactatacattatcaataataattaaacgaatcatcccaccaaatgtaaaccatgaatattgaaatcatcatgttttaagaatcattttaataattatgttatttcattgttttatatagaacacaccgttcatgaaatcaaacaaagagagagaaattataattttgtaacaaattaccaacattctttttctttctatttttcataaatgagcatatgtttgtgtatatatacatactgttatttgatctccacattgttgaacaaaaaagttggtgttcttgaaaatagctatcaccgaaaatacgtcatatactgggttgttatgtaccaaggcccagaagaaagcccaaaatcaccggcccatgagcagtgaacaaataattgggctaaaagcccaatatacgtgatgatgggccaacccagagaagtttatagttatgttattatagaattccagatcagggagtatcgaaacaaaagcctccattgtcctcgttctcttctccttgtgctctctctctctctctcttgctcttttctctttctctttctctccgacgacaggttcctgaagctcgaccagccaagggcattgatctaggtgagtccgctttcacttttccactttcctctgccgtttttcttgtcatttccaattctccattctttgttctggatttcacttctttacttcgtcgttgattagaagataatagtgagatcgaattctatgtctcgcataccttcagtttcaaggaacaagacaatgattcaaccgcgccgtccacgttatggatagagggttttgattctcacctttatagctgcataacaccgttcttagggttcggacctttgaatctgcgatatttctcacactgttttggacgtttttaccgttttcctatggttctttagccttaccttatcttgccttcagatcttcgattgcggatctgattcgttcatttctacttgttactttttcttggaagtcgaggattataaatcaacaacaaagcattcaaaatctctagtgcaattagtgttttccatctagttattggagatcgtttgtagctttgattttgtccactttcttattttgaacgtctggaagacgttttatacatgttctttgggtaaagttgcgtttgggcactgttcttcacctctgggttttcgttcttatgctatgtttcatgatttcttttgatatctttgttattgtttccccatcatcgagtatctgattcttattcggaagccgtcttcttgaagctgcgaaccggttttctttttctccctcatcaagtctttaattttacaggaaagcgctgaataag

SEQ ID NO: 156 - DNA, 2011 bp, Cucumis melo
  source 1..2011: mol_type = other DNA
ttgttagaggagttagcttttcagggagtcggttacaacttacaagacagacaaccatactgtacaatcaatcactactgcctcaaagtcgaaaccatttaataccagttgagcctcattgtgactgcataattttgacccctaccacgaggtaatttcagttcaaatcaattgtatctctcttctggatatcagtcaagaatctcatgttctcaagttatagtacattgataattactgtgcatttttattaatttatgagttaaaatcctgctgattaattcaactaaaggaataaaatagttattggcatttggatgagaatagaatgtgaatcccatcattcatcgctagattggaccgtaattataagtgagagggagaaacttctgttgctattccctttttatttcttaattcatttataaattgtttttaggccttttatatatatatatttctaccatttttacatttaaaattcttttaactttattatgtatggactcaaactaacaagctttatttgataaaattgttcaaactattatattagttttatatttgtaaaccataaaacaaatccataaaattccacctgcatcactcactcatgttgttgaatggtacgaaataaacaatacatgtgaaagatgaaaataagaattgttctcttattaaatctaaaatctagattttctttttagtacatttaacacttcaatgaaaggtctaaaacattattgaatgacgtcacgaactattacaaaagattattccgatttatctcaaaaggggtctatttcactaattttggtgtcccacatctgtaaagagaattttcgtgatatgtgtagatatttaaatataattgaattcgatgaaagcaaagcaagaatcgatatccgtagttattttgatatagatcggtgataaataaaagacaatatgcataaagtttgtgggtacagagtcggctagttgcaatgaggggtatggccccaagacttttccccaaccccaacggtcaattaatcaccccaatggggcatcgaatcttccccaccattttccttttcttcgccgactcttctacccatctcttttgccgactctttctcacaggtttgattaaatcccattcatattcagatacactatttcaaaatactcgcaaattaatttgtttttttaaatattggtataataataaaattaattataaattgtgacctaaaaagtactttgtggaagaggggatatagtctgtctaatatattattgattaaatatataatagaaccataaatgcaaaccactagaattgttaataaaaatcaacgctcttttaagtctttccatagaaagaaaggcaaagacgcgcaacgtctagaattttctttataacggaagctaactctgttataacggccgtccacataatatggtagatttaaaatgacgtcagcatgtcgcttctaaatttgggtccaaaggggggattcatttatagggaagggaaacggcaaatgcaagcatagtgagtaaatacgtggcggcaaagtaatggataattctgcctctgccgtgacgacattgcccttccatttcactataaatacacctcctctatccctcgatttcttcgcaattgaatttctcttctcatctctgtcgtagcaaaccaaatcgatttcttcaaaggtatttcttcctttcctttttttttttttttttttttttttaaatcatgttgttcaaactttgagagatgaaatgattaggggctttcaaagtggttttcgtttgatatgtttcttagatcgatagggtttagaatcgagcatccttgtaggtatcctgaggtttggtggttggatctgcttaatttttatgtggttgcatggaaaattgggattttttttttctaattacgtgattctggaaatattgatctgtggttcagatggaattgaatctgatctttctgttttgttctgtataggtgggc

SEQ ID NO: 157 - DNA, 1698 bp, Cucumis melo
  source 1..1698: mol_type = other DNA
ttgttagaggagttagcttttcagggagtcggttacaacttacaagacagacaaccatactgtacaatcaatcactactgcctcaaagtcgaaaccatttaataccagttgagcctcattgtgactgcataattttgacccctaccacgaggtaatttcagttcaaatcaattgtatctctcttctggatatcagtcaagaatctcatgttctcaagttatagtacattgataattactgtgcatttttattaatttatgagttaaaatcctgctgattaattcaactaaaggaataaaatagttattggcatttggatgagaatagaatgtgaatcccatcattcatcgctagattggaccgtaattataagtgagagggagaaacttctgttgctattccctttttatttcttaattcatttataaattgtttttaggccttttatatatatatatttctaccatttttacatttaaaattcttttaactttattatgtatggactcaaactaacaagctttatttgataaaattgttcaaactattatattagttttatatttgtaaaccataaaacaaatccataaaattccacctgcatcactcactcatgttgttgaatggtacgaaataaacaatacatgtgaaagatgaaaataagaattgttctcttattaaatctaaaatctagattttctttttagtacatttaacacttcaatgaaaggtctaaaacattattgaatgacgtcacgaactattacaaaagattattccgatttatctcaaaaggggtctatttcactaattttggtgtcccacatctgtaaagagaattttcgtgatatgtgtagatatttaaatataattgaattcgatgaaagcaaagcaagaatcgatatccgtagttattttgatatagatcggtgataaataaaagacaatatgcataaagtttgtgggtacagagtcggctagttgcaatgaggggtatggccccaagacttttccccaaccccaacggtcaattaatcaccccaatggggcatcgaatcttccccaccattttccttttcttcgccgactcttctacccatctcttttgccgactctttctcacaggtttgattaaatcccattcatattcagatacactatttcaaaatactcgcaaattaatttgtttttttaaatattggtataataataaaattaattataaattgtgacctaaaaagtactttgtggaagaggggatatagtctgtctaatatattattgattaaatatataatagaaccataaatgcaaaccactagaattgttaataaaaatcaacgctcttttaagtctttccatagaaagaaaggcaaagacgcgcaacgtctagaattttctttataacggaagctaactctgttataacggccgtccacataatatggtagatttaaaatgacgtcagcatgtcgcttctaaatttgggtccaaaggggggattcatttatagggaagggaaacggcaaatgcaagcatagtgagtaaatacgtggcggcaaagtaatggataattctgcctctgccgtgacgacattgcccttccatttcactataaatacacctcctctatccctcgatttcttcgcaattgaatttctcttctcatctctgtcgtagcaaaccaaatcgatttct

SEQ ID NO: 158 - DNA, 313 bp, Cucumis melo
  source 1..313: mol_type = other DNA
tcaaaggtatttcttcctttcctttttttttttttttttttttttttaaatcatgttgttcaaactttgagagatgaaatgattaggggctttcaaagtggttttcgtttgatatgtttcttagatcgatagggtttagaatcgagcatccttgtaggtatcctgaggtttggtggttggatctgcttaatttttatgtggttgcatggaaaattgggattttttttttctaattacgtgattctggaaatattgatctgtggttcagatggaattgaatctgatctttctgttttgttctgtataggtgggc

SEQ ID NO: 159 - DNA, 2010 bp, Cucumis melo
  source 1..2010: mol_type = other DNA
tagaaaaaaattgaagatcttcttaatgctaataataaaagcatatataaaaaggcttcatattacacaagcatcttaaaaccaaaccgaacttgatttgaaattatcccactaattctgtagatttcaccaaagtccttaacctttatactaacatctgcatttgactctttcatttgacctccaacatattctttctcattttccttccattcaccacaaaaaccaacaaatacaaaaaaccacaaatacatagaaaattaataaaaaaatcaaaatttcgagatgaaatcattataaactcatccgataactttgagatttgaaaccttacactatataaagaaactcatccgataactttgaattcgcatcgaaattacgtaagtgaagacgaaaatgtaaatgattagatgcgaataacaaaaaaaacataatttctaaacgtaaaacactatattcaccttattatacttgattattttggaaaagtatgaaatttgagtgtgggagaggagccaaagaattggaaacttgttattaggagtcgttatgaaacattttcaacaagccaatattctttcacatactataatgatatacatagaaataatacaataatatttttgaaattgaggcatttttgtcgtaatttatctaaaaatgtcagggtagattcatcatgtatacaaatctctcgctatcaaaactatataaaaatcttgtgaatgatttcaatcgaaatggaccgagaaaaaacatcgtaaccacctctaaaatcgataaatttgtttcaatttcaaatccctaaaactaaaggtgctactttgtacaatttcccctgattagggtgctaaagttaaaccctaaataaaggtgtgtacgtttccggaagtttctagaatccccagcgaagttctccaaatcgtggcttgcagaccaaggacccccattaaaattcgtttcttcctctaaacctcctcccttaattttggcattttggtattttggctcctataaattcaccccctccttatccctaatcctttgtcttccaaattttccttcaaagcctgcttttcccatttcgtcgtgctttttcttcatctaaaggtatatttcagttctagttttctttctctgttgatctcttggatttgagggacgtttgaagttggctttgtttaattctttgttattcaatctctttttttgttagagttgttgtttaatcgtttcccttgttgtttttctcccttctagttcgattttagaacgctttttgtgggttgattttaatttctccgttttcttacatctttcacaaagaaacgattgaaatcgtgtttgttttttttcccacggcatacgttattagatcttgtagataatgatctcaatctattgtttagtttttgcaaataagaagttggttttttatctccaacttttatatattcgattcgatgagatgttctacaccgttaggatggaaccaagaagtgaggtaagggtgtttgattgaaaaattgaactgagaagttaaagttccttcctaactttttaatggattgtataattcgttcaattccttgtcgttccatttttatttctgtttcgtttttcgtgttgctgcgtatcgcttcccttgttgttttcctcccctattgattttgcgtttcttggagtttctctgttttctctcttcatttttctacaaaaatcaattctatttttattcgttttcaattcccgagctccttggaatgttatccttttctcctgtgtaaataagaacccgtattcaatcccagttcatagtttggctttcccaaataagagcaaaaagattgtactgagaagttgaagatttcaaaattttgtacatgatttcttctaatttatcaatttgattggactttttgtatatagatttggttcttgagctatttatgttatgacgttttcatattgaggccatgcgttgaattggtttcttaacaggtgggc

SEQ ID NO: 160 - DNA, 1107 bp, Cucumis melo
  source 1..1107: mol_type = other DNA
tagaaaaaaattgaagatcttcttaatgctaataataaaagcatatataaaaaggcttcatattacacaagcatcttaaaaccaaaccgaacttgatttgaaattatcccactaattctgtagatttcaccaaagtccttaacctttatactaacatctgcatttgactctttcatttgacctccaacatattctttctcattttccttccattcaccacaaaaaccaacaaatacaaaaaaccacaaatacatagaaaattaataaaaaaatcaaaatttcgagatgaaatcattataaactcatccgataactttgagatttgaaaccttacactatataaagaaactcatccgataactttgaattcgcatcgaaattacgtaagtgaagacgaaaatgtaaatgattagatgcgaataacaaaaaaaacataatttctaaacgtaaaacactatattcaccttattatacttgattattttggaaaagtatgaaatttgagtgtgggagaggagccaaagaattggaaacttgttattaggagtcgttatgaaacattttcaacaagccaatattctttcacatactataatgatatacatagaaataatacaataatatttttgaaattgaggcatttttgtcgtaatttatctaaaaatgtcagggtagattcatcatgtatacaaatctctcgctatcaaaactatataaaaatcttgtgaatgatttcaatcgaaatggaccgagaaaaaacatcgtaaccacctctaaaatcgataaatttgtttcaatttcaaatccctaaaactaaaggtgctactttgtacaatttcccctgattagggtgctaaagttaaaccctaaataaaggtgtgtacgtttccggaagtttctagaatccccagcgaagttctccaaatcgtggcttgcagaccaaggacccccattaaaattcgtttcttcctctaaacctcctcccttaattttggcattttggtattttggctcctataaattcaccccctccttatccctaatcctttgtcttccaaattttccttcaaagcctgcttttcccatttcgtcgtgctttttcttcat

SEQ ID NO: 161 - DNA, 903 bp, Cucumis melo
  source 1..903: mol_type = other DNA
ctaaaggtatatttcagttctagttttctttctctgttgatctcttggatttgagggacgtttgaagttggctttgtttaattctttgttattcaatctctttttttgttagagttgttgtttaatcgtttcccttgttgtttttctcccttctagttcgattttagaacgctttttgtgggttgattttaatttctccgttttcttacatctttcacaaagaaacgattgaaatcgtgtttgttttttttcccacggcatacgttattagatcttgtagataatgatctcaatctattgtttagtttttgcaaataagaagttggttttttatctccaacttttatatattcgattcgatgagatgttctacaccgttaggatggaaccaagaagtgaggtaagggtgtttgattgaaaaattgaactgagaagttaaagttccttcctaactttttaatggattgtataattcgttcaattccttgtcgttccatttttatttctgtttcgtttttcgtgttgctgcgtatcgcttcccttgttgttttcctcccctattgattttgcgtttcttggagtttctctgttttctctcttcatttttctacaaaaatcaattctatttttattcgttttcaattcccgagctccttggaatgttatccttttctcctgtgtaaataagaacccgtattcaatcccagttcatagtttggctttcccaaataagagcaaaaagattgtactgagaagttgaagatttcaaaattttgtacatgatttcttctaatttatcaatttgattggactttttgtatatagatttggttcttgagctatttatgttatgacgttttcatattgaggccatgcgttgaattggtttcttaacaggtgggc

SEQ ID NO: 162 - DNA, 1235 bp, Cucumis melo; identical to SEQ ID NO: 22
  source 1..1235: mol_type = other DNA

SEQ ID NO: 163 - DNA, 617 bp, Cucumis melo
  source 1..617: mol_type = other DNA
aaattttaataattaaaatgaacaatttttcaagagtaatagagtttgagagatgtcagagaagtttgaggaagaagataacaagtgggagaagagaataagtttgttgtgtgaaagagaaggggaaatttcattcaagggtatattgaactttttactcaaattttgtaagtctattttttccgatcaatcctaaaatcacacacacccttaaaaaatggattatatttggcaattttccatgataaactcatttttaatttagagttattttttcaacgagatattaacagttttagttcatatactaattgtaagaatagtttcttttaagttgaatagaatttttgaaacttttaatagttcaaaaggtatttttgaaacaaaataagaatgtttttgaactttttataaaaagaattgagatttttttgaaatttttgataaagagaaaagaaaagaagaaagaaaaaagaaaaacaagtttgtagaactccgtgggaaaatcgtcgagggccctgtgaaggaattttgaaattataatgagggtattttcgtcaacaagggaatttagacatcgtatataagcatcctcaaaccctataattaagcccttc

SEQ ID NO: 164 - DNA, 54 bp, Cucumis melo
  source 1..54: mol_type = other DNA
aatccaattgccattctccatctctcgccgcaagggtttaagagcagcttctct

SEQ ID NO: 165 - DNA, 545 bp, Cucumis melo
  source 1..545: mol_type = other DNA
cctcaggttggggtttccccctatcttcttcattcttcctcttctcgatttctttcttctatttgctcgatagtctcttatttcttgagcttttgctgtttttctcctgtacatcctaacatgaattataacttggttttgattttgtcttttacttctgtattaaacaacttttcttacccttttattcttctcttcttcttcgtgtccctgcccttttgtttttatgctaattttatgtttctgtttatcaatctatcgaggcgtgacctgtcgttcttccaatagcgtagatctgcacttaatctattctagctgattggattggtcgtttttcgtttttttaatttattttctctgttctagttccgataaatttttttatatataattaacaagttctccagccaaaagggttaatattgcgttggatattttaatttttacgttatttagatgtgtgaatctaataaaattagggttattcataaatttcagtaatgatattttggttatctgttcttgctgttcctgtttcgcagttc

SEQ ID NO: 166 - DNA, 19 bp, Cucumis melo
  source 1..19: mol_type = other DNA
ttttacctaatattcaagc

SEQ ID NO: 167 - DNA, 2003 bp, Cucumis melo
  source 1..2003: mol_type = other DNA
cagtgtgctggaattcgcccttatccaaggagattaatgtcgagagattattatcgaggtttgaatttattttgtccaatcatatgattccaagagctgaccatcaattcaacagaacatgaaccggaacctcatacctattgtaatggttcacagcatcctaatacagaacatgaaccgaaacctcttacccattgtaatggttcacagcatctttatacgtattataggtagtaccattgaagatgcatttaaatgctgtccatgctctgttctctaaaaagttggacttggacttggacgtcagctgaaagtatgaaatgcactgtagccaacgaagctatgttttcaggcttcaacatggttttaggaaagtggaggctctttggttgaagggttgaatgaatgcttttctaattccagcatgatcttcaaatttcgacacaaaaagcttaagtattttgttccgttattcttttaatccttgtattgttatatattcttttctctgaactgaatgtacgatgattgcaggggtcgagagcaagtccgatataatgaaacacgtaaggacgtgattgaatgaaaaactatgagcagagatacaaagtctaacttacgggatgaacgatgagaggtttgaccaagagctgtgacgcctgtatatttcaacaaaagttgatgactaacatcacatgtcagagtaatcaaagaaatgcagccgcacatatatatatctatatatatatcgagttttttttttttttttttttttttttttttttttatctaatatattttaatctattttcctctgccctcctccccctcctcttcccccacccttcttctgcacatagtagccaaggattgatcggtttcttttgattcggggggaaaatgttgtacaatttttgcttccatagaagcttgaaagttttgcagattatgttgtaaaattacccttgtgtactcacactagttcttctcgtggaaacttatattacaatggttgagttttaaggggcatattcacactggtaactaccattttctaatttatgaatgccgagtttctctccatgaaagacctttcaaatgccctttcctccgcggtgcgtttgttgttgtaaatgtgcagtgtcgttggatacacgattgtgtgaaagggaaaagggaatacgattaactcttaaattcaacccctatctccatcagtatcaatcacatttcagcaactagctcttgaataacattgagattcttgtttaatccacgtactactactactattactactatttgacagttgatatctcaaataacatccatatttatcaaattggtattttaaggacttttaatttcttcgtacatatttcattataatttaactactctgaccatcattgaaaatttcacaaagaagacattttaaattgaattgagttgaattaagttgatataatggttgaacgttggatttaatttataatttagtggtgtatgggtccattgtaataattcttaaaaaaaatatcatattctgaattctaaagaaccatctaagaccaaaactaaggggtcaccaatgagtatggtaaagtcaacaaagtttgtctacttttcttatccttatcatcaagagtgcaatatgatatcaaagataaattgtacgtgggcgtcatccattgggtaagaccaagaagcaaaatatcatagagaagttgttttagtagccataggaaggaaggaagcaaaataataatatagatttgaaattgtggatgataaactgccaaatgggaattcaaaataaactaaataaataaaataaaaagagaaatcttgggagtttccattttagccaatgaggaaacagatagagatctcatcaagataaggaccctattctcttcttcatctataaaacaaaaacaaatcaaaccctcatttcactcattcaaaacaaaaagtactccaaagtcaaactaacaaatacg

SEQ ID NO: 168 - DNA, 2004 bp, Cucumis melo
  source 1..2004: mol_type = other DNA
tggatcgaccatgacattcaaaaacctttaagatatggatcttataaaataaatgtaaagggtaaacaattcttccttgcttaacccaagctatatattttatgcactaatttaggtattagagtatattcagctgaacaccacctaccaatgctagtactttaatcagtcaattctaacttcgataatatatctcaaccaaattagtgaaaaagagtcgtaaatgaaaaactatgtaccaagatattctatttgttttttttatgtttaaatatctcaaagataatacctaaaacgttttctcctcgtacaaagattcctcatttactttttattgtcgtaaactctaatacaataaactaaaacaagtacaaatacactagctttagaaatctactttttattgaaaccaaaaccaataattcaacatttcattttcaccgacaaacctttgtaaacaattgaagtaatttttgttggtactatgaatagtaacatcaagtcttcaagtgcatcatatcaaccaagacatgttcttaaaagcgacactaaaagatttaaaaccaaaagcatttatgaaatccgaacttaatcaaatcctaaatatttttcacttaaaaaaaaaaaaataggaagaaaaattgacataaatgggatattttcgttttcaaactggcaagccagcatgcaccacgttgttgacgtgtccttccacgtcggaaaaaaaaatattaccacagtaaaaagagaataaaatgaaagtcgttgactctcccttagtcggaggaagcgcgtgaagctgaagccggattagaaatcggcaataaccccgacacgtcatcgaaatgctagtatcaaatattgtccgttggatcttccttcaccaactctatttgaacggccacgatcttccaggtccaacggttcggaagaatcttttcgaaattccatggctagtccctacactcctccctattggctccctagggcatcccgaccggttattccggttgccgggaaggtggctggacgctataaatacccgctttgttcatctcgtagtccttgtaccgttgagcttcgccttctaatagagctctggttcggttggcgtattagctcgaattctttctctcttccagatctacgctgccgatttcatcaggtttgcgagctctgttccaccatttttcttttcctgaagctttgagcatgcttgtgattcttcatttcctcatttctttgatggtttatgaaagaatttaggggaattttctctttttgtattctagtggtactggtagatttgtttgaagtttgtttctcttcttctgagaagtgaattcttccagatctgacagttgcttttgattttttctttgggaattagtgaatgatacttcgatactgttttttgctctctgagattctggatctcgggccttggggttttctattgtcttttggtagctatgtttcgtttgtcagcttgtatttgtcattgttgaatggttcgatccggtttgtaaataaaataaattttgtaggcgcacttgttttccacggttttcgtgttacggtttcatgattccctagatctctggttagaactaagttttttgtcggtaattggatttggtaagggactgttactgtggttgaattgtagatccagtcatcttctacatgagtgtagggttccttagggcagatcttgtgttttataattttaattttgttgtttccctgattttgaacctgtttggttgttcagattcgtcgagtcatttccattcattaaaagtttctataattttatttgaatcttctgaatctgtgcttgtattacccagatttctataaacctatcttgatttcaagtgtgctatgtggtaactgttgatattttcaagcttaagcaatactgatgtgactaaaacttaactaatgaactgaatgttttttgtacacgaactaatatggtgttttgttatgtttcagagg

SEQ ID NO: 169 - DNA, 1067 bp, Cucumis melo
  source 1..1067: mol_type = other DNA
tggatcgaccatgacattcaaaaacctttaagatatggatcttataaaataaatgtaaagggtaaacaattcttccttgcttaacccaagctatatattttatgcactaatttaggtattagagtatattcagctgaacaccacctaccaatgctagtactttaatcagtcaattctaacttcgataatatatctcaaccaaattagtgaaaaagagtcgtaaatgaaaaactatgtaccaagatattctatttgttttttttatgtttaaatatctcaaagataatacctaaaacgttttctcctcgtacaaagattcctcatttactttttattgtcgtaaactctaatacaataaactaaaacaagtacaaatacactagctttagaaatctactttttattgaaaccaaaaccaataattcaacatttcattttcaccgacaaacctttgtaaacaattgaagtaatttttgttggtactatgaatagtaacatcaagtcttcaagtgcatcatatcaaccaagacatgttcttaaaagcgacactaaaagatttaaaaccaaaagcatttatgaaatccgaacttaatcaaatcctaaatatttttcacttaaaaaaaaaaaaataggaagaaaaattgacataaatgggatattttcgttttcaaactggcaagccagcatgcaccacgttgttgacgtgtccttccacgtcggaaaaaaaaatattaccacagtaaaaagagaataaaatgaaagtcgttgactctcccttagtcggaggaagcgcgtgaagctgaagccggattagaaatcggcaataaccccgacacgtcatcgaaatgctagtatcaaatattgtccgttggatcttccttcaccaactctatttgaacggccacgatcttccaggtccaacggttcggaagaatcttttcgaaattccatggctagtccctacactcctccctattggctccctagggcatcccgaccggttattccggttgccgggaaggtggctggacgctataaatacccgctttgttcatctcgtagtcctt

SEQ ID NO: 170 - DNA, 92 bp, Cucumis melo
  source 1..92: mol_type = other DNA
gtaccgttgagcttcgccttctaatagagctctggttcggttggcgtattagctcgaattctttctctcttccagatctacgctgccgattt

SEQ ID NO: 171 - DNA, 845 bp, Cucumis melo
  source 1..845: mol_type = other DNA
catcaggtttgcgagctctgttccaccatttttcttttcctgaagctttgagcatgcttgtgattcttcatttcctcatttctttgatggtttatgaaagaatttaggggaattttctctttttgtattctagtggtactggtagatttgtttgaagtttgtttctcttcttctgagaagtgaattcttccagatctgacagttgcttttgattttttctttgggaattagtgaatgatacttcgatactgttttttgctctctgagattctggatctcgggccttggggttttctattgtcttttggtagctatgtttcgtttgtcagcttgtatttgtcattgttgaatggttcgatccggtttgtaaataaaataaattttgtaggcgcacttgttttccacggttttcgtgttacggtttcatgattccctagatctctggttagaactaagttttttgtcggtaattggatttggtaagggactgttactgtggttgaattgtagatccagtcatcttctacatgagtgtagggttccttagggcagatcttgtgttttataattttaattttgttgtttccctgattttgaacctgtttggttgttcagattcgtcgagtcatttccattcattaaaagtttctataattttatttgaatcttctgaatctgtgcttgtattacccagatttctataaacctatcttgatttcaagtgtgctatgtggtaactgttgatattttcaagcttaagcaatactgatgtgactaaaacttaactaatgaactgaatgttttttgtacacgaactaatatggtgttttgttatgtttcagagg

SEQ ID NO: 172 - DNA, 2018 bp, Cucumis melo
  source 1..2018: mol_type = other DNA
actattggagacgacgaaggaaaactctaatgtgagcttagaattgaagatggtgaacaattgggagtcttttttaaaaatctttcgtcggtatattgaaatttccttttacactcaaataaccccccttttcacgcgttcaacgtcttcaaaccttcctttttcaattattttttcgtttacattaatgacatttaggtaataagataaattagtggattcttttgtgaaaaatgttagcccatttaagacttttatgaaatatattagaaaaaaatcatatagcaatttatattattctagttaaaagcccataatagaaactaacccaacctaaagtaacgtaaacattcaataagagagacaaattttaaaataatttctaattaaaaaaaaaattgtcaagaccgtccgggtcggatccaaaatataacccgaaccggccggtttagcatctatataaatacacctttagggtttttattctctcaagacttcaccgcatttccacttctctgaggccacggtcagccattggagcagctcaataatcctttgactccctactacggtaagtcgaccttactgctttcggcttctagttttttcaatcctgtcattagtcctttggagttcttctgtacatttatgacgttttcggctcgtgttttgtttcgcctgtatgtagtgggtttttcgagttttgtttttacttttttttatacttgcaggaattagttgaaatctatgtacttcatgccttggataatactcttgatctgttgtgttattcaaaaatgaattgttttaagatggtatttgagaatggtcatgtgagttttgcctacttggttattaaaatgaattgttttaggatggtatttgagaatggtcttctgggtatttggttggaacctttgtgctctgctatgaattagggtgttctccccgtttttttttttttttttcttttggttattaatatatcttttatgactacttattcatatatgatatcttttactcgtaaattttgactcatttgaaagttttatccttagtcctttctcattcagggtgtaaaggtatgttgttagggttaaaatagcctatgcaggaaagttctgtatttgttctaattattgcatttgtgtgcatttgtatctagtttatttcttgctgagagtatgcttcattttttagtacacatcacttgtgccactttattatagttgcacatttttgtttatggagaggatgaatagcatttagggatgtcaattttttattgagaaaaccctctctcctacttaagcttggggaatttttgttctaaatgtggtaaacataatacttcttcttattttaatttgaatggaaggggaagacgaatactaatattttcaacgaaccttcacaacttttttttcttatttaggaagccatgtttttcaaaattgtactgtgtgatccacatatttatcgattattagtgaatcgaataataattagagttttattggtataattttgaagttcagacttattacatttgtggaaagtttggttacaattttcaattttattggaatcctaagaactttgtgttaacatatattgagttttcttctctttttttttactcattaagttctctattaggaatgtttggttcaatgtcacatagtcgatagctaagaccagtgacccacaaagctatgattgaacgaaaaacaagcctttcacatcttggtaggaatttgttatttctcaatagatttacagagctgtttcatgtgatcacaatttttttctatttttctgaagttctctattaggaatgggctatctggttagttgcttttgagagaacatgtggattggtgttgctcggtttccttgcctttgtaattttgtccttggaaaaagcaaaatgattaggtatcctgatatgcataacatgtttaagccaactagttctcacttttttagtgcaaataattgatcttcaggaatcg

SEQ ID NO: 173 - DNA, 565 bp, Cucumis melo
  source 1..565: mol_type = other DNA
actattggagacgacgaaggaaaactctaatgtgagcttagaattgaagatggtgaacaattgggagtcttttttaaaaatctttcgtcggtatattgaaatttccttttacactcaaataaccccccttttcacgcgttcaacgtcttcaaaccttcctttttcaattattttttcgtttacattaatgacatttaggtaataagataaattagtggattcttttgtgaaaaatgttagcccatttaagacttttatgaaatatattagaaaaaaatcatatagcaatttatattattctagttaaaagcccataatagaaactaacccaacctaaagtaacgtaaacattcaataagagagacaaattttaaaataatttctaattaaaaaaaaaattgtcaagaccgtccgggtcggatccaaaatataacccgaaccggccggtttagcatctatataaatacacctttagggtttttattctctcaagacttcaccgcatttccacttctctgaggccacggtcagccattggagcagctcaataatcctttgactccct

SEQ ID NO: 174 - DNA, 1453 bp, Cucumis melo
  source 1..1453: mol_type = other DNA
actacggtaagtcgaccttactgctttcggcttctagttttttcaatcctgtcattagtcctttggagttcttctgtacatttatgacgttttcggctcgtgttttgtttcgcctgtatgtagtgggtttttcgagttttgtttttacttttttttatacttgcaggaattagttgaaatctatgtacttcatgccttggataatactcttgatctgttgtgttattcaaaaatgaattgttttaagatggtatttgagaatggtcatgtgagttttgcctacttggttattaaaatgaattgttttaggatggtatttgagaatggtcttctgggtatttggttggaacctttgtgctctgctatgaattagggtgttctccccgtttttttttttttttttcttttggttattaatatatcttttatgactacttattcatatatgatatcttttactcgtaaattttgactcatttgaaagttttatccttagtcctttctcattcagggtgtaaaggtatgttgttagggttaaaatagcctatgcaggaaagttctgtatttgttctaattattgcatttgtgtgcatttgtatctagtttatttcttgctgagagtatgcttcattttttagtacacatcacttgtgccactttattatagttgcacatttttgtttatggagaggatgaatagcatttagggatgtcaattttttattgagaaaaccctctctcctacttaagcttggggaatttttgttctaaatgtggtaaacataatacttcttcttattttaatttgaatggaaggggaagacgaatactaatattttcaacgaaccttcacaacttttttttcttatttaggaagccatgtttttcaaaattgtactgtgtgatccacatatttatcgattattagtgaatcgaataataattagagttttattggtataattttgaagttcagacttattacatttgtggaaagtttggttacaattttcaattttattggaatcctaagaactttgtgttaacatatattgagttttcttctctttttttttactcattaagttctctattaggaatgtttggttcaatgtcacatagtcgatagctaagaccagtgacccacaaagctatgattgaacgaaaaacaagcctttcacatcttggtaggaatttgttatttctcaatagatttacagagctgtttcatgtgatcacaatttttttctatttttctgaagttctctattaggaatgggctatctggttagttgcttttgagagaacatgtggattggtgttgctcggtttccttgcctttgtaattttgtccttggaaaaagcaaaatgattaggtatcctgatatgcataacatgtttaagccaactagttctcacttttttagtgcaaataattgatcttcaggaatcg

SEQ ID NO: 175 - DNA, 1999 bp, Cucumis melo
  source 1..1999: mol_type = other DNA
ggtctcagacccataggaatagatcatttattgccttatgaattagtttatgagtacataataattgtcaaccgtatacaaatcaacatgaaagaatataatgttgtacatagtcattccaagtttactaatattatattttaggagtgttctacaccgaacctgtcacatgtacactgggtatgctacccctgaattcaatatcataaagcaactttaattgtcaagcattctcttgaccatttgtgacccatttgctcctactttttcaatcaataactatcacaaaaagctagataccacatgtgataaactcactgaaatcaggtatatggttacctgtgcttggtcagcactcaatcagattcgaaggcctagtctttgtatttccccccctctgcacactacaaatagtcctccacgtaaagacccataacaaaacgcaaaccaagtacagaaaatctagccgaaatccagaccactcaaacataacaaatcttctggtaagtttgaataaaatataaaactaacctatttaatcaaataatacaataaaatggaagcaactaacataacatatctaaatatgatcacgtagtaggaaaaaaaaaaacattccaaaactattaacaatcattcttaatggtatgggtcaatccccattatttaggactataacaagaattcctcatacctaatgccacatcctatgtccaaccctcgagattacctcgtgagtaatcaatcttattcatccttatttcaaattatgtgaaatttctcatcaggttgatcatattgactttcaatacaacttatgattaatctttcccttgatataatttcgtatgaaaaggaagttgacattatgtgattttctcataaggtaaaccaagtaaacttgacatgacgtcttaacaagtcttggtttctaagtgtaatttactgcagaaaaaatcctaaattctatgacttttcctatgagattgaccaaatcaactttacgagaaatcttgggaagccatacctacaaagtcttcccccaagaaattacaatttctagtaaagattgttgaaatttaccctccaatttttccgtgaaaatttgacaaacttgtaagaatatcaaatttgggttggatattgacattccaaaataagtagttttaaaaaggatttatccaacaataatagaagaaaaaagataggaaataacatacccacgtaaatggaatgtaaatatttatatattaggtgtcttgaacgaccgtcaaacgaaaataaattgttcatccgaagttgaaactctttaagtgtacatttatcttttcgtaagaataaaatgtaaaattaacgtgtgaaaggttgggttaaataagttatgtagagataatattgaagatgatagaataatcacgatcgatgaattagtatagtcccagagcggatttaaacctctctcactttcatgctttctatatatatcaaaataatttcaagtagttggtttagtcgtaaaaaagtcaaccaatctcttttagataaaccttgagttattaaaaaattagatcaaagataatcgttgaaattgaaattttaagagtataattataacaaattggaaagttctaaagtagtttttgcaatattctccatcaaaatagagtagaaaaatattttagtaattttcttatcttaattttagttttgtaatagttattaggatggtcctaagttctcaatccgcttttagtccataaaaagaaagaagagagagaaaaaaagtccccgatccgcgacacataccaatccaaccaattatgcacaatccatgtgatatcgaacggtcacaagaataaatgctttctacacacggatcaccatccaacggctttccttccatctcatcctctatataatctaccaactctgtcatcttcgacacacttcaattatctcagcttttatttcatcggattttccatcaaacaaggcaaca

SEQ ID NO: 176 - DNA, 2004 bp, Cucumis melo
  source 1..2004: mol_type = other DNA
tatagtttgtaacaatctactctatgttctttcaattttgatacatttgaatcttaaactttattgagttacacaatatagtccttgtatttttaaaatttataatgactctatttatattaatattatagaaatttttgttaaggtttaataaaaatttttctgtataaataaatcgaacacgaagtctatatttagactgcaatatagtaaaacctgacatctaagtttggtgaattttgttttgctttaaaaactaaactattacaattttaaaaatattttaatttagttaatgcacattaactttacggagtaaatttttacaagattgaatatacatagattaaatagttataaaaccaaagattagagtaaaaaacatttaaatagaaagaactaagatttttttaaaacgaaaatgatactagatacatatatatgtatctatattataattactcattttaacatatagttttgaaagaacaaagattagttgcatgtgttgattgtttttaagaaggaaataatttttgaatggaaaattttcaaaagttttaaatttgacaataaactcatatttaaagtgtactacaaattttaacttttggttaaactccttgtttagttcaatcatgtaataaattctcattccaagaatcgttttagaaaattttattgtgcatttaataaaatatagaacatatatggcatataaaaattgattacttttttctttttttgggacgaaaaacacattagatataatcttttttgaaagtttatgaactttaaaaatgggttattttatacggtggtcaactttattttattgaaattattgagtttataaagattgttatatcattttcttcttctctttcactagaatacaatcaaacctatcaaactctctatgacttatttagaattctttttgttatatttttgaaattaataaatgaaaagcttagagtctaaattataacaattaaaattgaaaattttgcaataattttatttttagcaaaatgacgtttggtttttggggattgggaatggatcgatactatcccgattccggacaaagaaaccgacccgagattcgaattttttccattcccaaacagagcacttaaaatttaagcaacgttataacggcgtcaccgaactaaacggaaaaatatgaagaaaattagaaaaagaaaaacggaacagtcaaacgttacttcacgtcaatggcaatattcatttttttttttgtttaaataattgaatttaattaatttggtttataaaaatagagtcctcatatatcgcgaatgcgcatttgatcgtgaaggacagcttctcccttgtgttcaagagagagagatctatcattcttatttggggccgatctctctattctcctctcttctattccgtaagtttttctcattcattctcctctctcatttctctccgagatctgtttacaatccttttgattttcatttttcctgcttcgatctgtgctcctggtgattcccttttcctgttttatcttttgttgatcttggaattgattgttcttttgtgggttttcattgatttgtattttctgatctgggtttctgttttctcgccttgatgttttgtatttggatctgatctgacgacccttttttttttttttttttatttgaattgcttttccaatgtttatacctggatttttattgatgcatgggtttaaccgattggttggatgcgttttctttgtgctggatctaggtgtccttgtttttaatttgaattgtgggtaaaaatggcattattgtaatgtgtttggagtttgattttgaatcttggctagttgatttttgaattacaaagatcggatcctcttcttttttgggttgtcttaagatttttggctggtttaagtatttgatgtcgttgtattttaaggggtaactgatgccggcttgttgtgtttgtattcagtttacttgaaaa

SEQ ID NO: 177 - DNA, 2005 bp, Cucumis melo
  source 1..2005: mol_type = other DNA
aattagcaaattgtatgtaacaacgtcatgaagaggcatttcatcgaacaatttaatagcagagtcaagatggcccagttttataagtttattgatttctcgattcttaaggtaaatgagatcgcgagcatggaaatgcagacccaaacgagaatatgggtgtggtaaatggaccggtgatgttgtggctacaaattcggattttacagcagtaatagttctgacgaaggaagcgaatttagtgacctttcgcatcacagtttaagcttatcagagacctgaacaagggctctagctctacaacttagaaaggtttgatatggtccgtgatcgggagggaccgaataacaggcgcttaaattgttgttcataaagaagaggattgtcgttgatgtattttaaccaagagatgattagttatccacatccacagagagaacagaagacggctttctaaatctacaccgataaaaataaccctaccactttgtttctttagaaaagggtcacattctttaaaaacattagcgtcgaggattaatagggtatattgactaatgctctgtttggatttcgagaaataccaatttacaattgatttcaaattaattatgttttgttgttgcacgaaagataaaaagaatttaaaattcaaaaggatctcaaatcttatttttaacttaaaaacttttatgacccaaacggtttatgtatgatttaaaagtagaatacctctgtgaattcttaatttttttttctttccaattaccacataaatatgaaattttaaatacatttattttaaattttatatccgaaacaaaataataatttaaaactatttctcatatatgaagtgtgattcgatctaaattataaaataataaaaatttacatctagttttgattatttttttttcgttagatactaaattgttaagaaaataacatttttaatccaaagttttgaagaatatatgacttttaaaatggtatttatctttttagtgtctgatttttaaaaaatggatttcaaaagttcatcaaatagcattgtatttttattttaaataattttgacatttaaaattagagtaatggtttataaaagacacttgatctctaaaactattttcttagatataaatacgtatgattatttttaaaaatcaatcaaaataggtaaattgtaaaaaaaaaaaaaaaatcataaaacatgatagtagttgtaattatgctctcaaactttcggttatgaaaaataaacattttaacttttagacgtgtcaaagttgagtcaagttggaccttcaaagttatgtagttatataaattgtaatatatgtataagcttgtggattcaattttatcatttatgggtccaatctctacaattatcgtaagtctatgggtcaattgtaacacatgtggagtttaagagctcaattttggacgtggatgtgttttgcaaccaactccacaccttaaaaaggtgtttttttttaatttatcaaaaaacaagaatttagaatctttaagtttatctttaaaaatcaacggacattttgaaaaccaattgaaactactgttataaacctaacaactaaaagtatattttttaagaccgaaagcataaatccataaaaaaaaaatccagaactgaaaatgtaacttttatagttgaaaatttagctaaattatacatattaaaattcaaggaccatataaaattaaagtacctgattaaataataacgaattaatgtttggtatttttaacctacattagaaaaaaaaaacaaaagaaaaacggcatactatttgtcaagcgtccgatgggaagaaaatccaacggtgagtgttagtattgaaatacgcagttctcgtgaatgagcctggcttagatttgggaacaagagccaacccctttcgaccgagaagccgtcgtcttcaccatattcgcctcaaccattcgatagccacgtttgaagaagaataggattgcc

SEQ ID NO: 178 - DNA, 1978 bp, Cucumis melo
  source 1..1978: mol_type = other DNA
aattctaacaactccggaacaaataatttagcatggattgaaatataaatcttcttgacttgcaaaaaaatcattgtaatggtcttatgttggttatagttagggtatcgaaacgccatacaggaatatgggattaaagttaacttttgttcatcaatttcagcttatgaacttctaaaatatcaattttacctttgaacttatatgttattacccctttcgattgtggtatgttaattaatatctgaatctcagtccttatgaaacttttttatactgtcacaaacatatgaagttttattgtaagttcttagaaatcatctaaaaagagtagtttgttggactatttattttattttttcttattaagttgttttcacgccatttcagtaaaataactatagtgaatagagaatcaaacttctaatcttaagttaaggtagtagggtatatgctaattcaataagataatccgtgatgcttgacatctgacttaattgttataagttttaaattttttattgtaatatttaaaatactagtttttggtttctaataaagaaataattgaacaattacaaatatttatacaaaattaaactagaatatatgatcattttccttcgtgttagaaaaagggaaatatatgtgtgtatttatacatattagatattgttttactatattccattttcctcacgggaaatggaggattgagtgggagataaacattgtccccaagagaattgggaatggaaatgcaaatgacatggccctccacaaaattgttcgcctaaaaatgggctttctcacttctcactccgcaagaaaaatatcgtttcccttcgaattcgggcaagatctcaaaaccacatgtttttctttctttatttttcaagcctacattatttataaaaatataacttaagcagagaattatgtaaattcaagtccatttttcgcttcacttagctaaatcattaacaaatctgtaattttgttcataaattagctcaccaattatgttttagcccactaaggcccattagacatttttattagaaaaacatgaaccgttggatcaagatgtgtgttttcttttctttttctttttattttttttgggttttggtggatcaattcgtagctttagcaacctattattatatggagggaaagggcgtattaatctgttagcgccgtccgggagtttagctttcttccccgagcctcggtcttatcccctaactccaaaaccctagcccaaaggtaatccactccttccccctccgctcttcatctttttctattcatcatctttaatctgttctcccttttggttcttagattcttcttttgttggattcttttaatctttactcatggttggccttgtaagtttagacgacgtttttatacattggttaatcctgcttctctatctattcgcacgctagggttttcctattgttttctattctgctctacttctgcaaggttgtgttcttcttcgttcaggtccctttttttaaccgaaattaaattaatgcaaattcgtttgtgcttctaattaggaagccttttggaacatctcgacattttgattgctgcatttcatttcgggtatatttctatgattgaaggatgtgggtctgttcactgcatggtcattacttatgcagctatgcttatcgagtccattatgtttgtgcaatctgtttccggattcataattttttagtaattgatcagtagatgaaaaaagatattgtaatattccttgagtgttgcaccagtcttggtgggtatctgctcctgctctttgcttgtggattttacttttattatatctgtattattcgaaatgttctgttcttgttataacttatacccgaagatgtgttcctccccgcgtctagcgttgtgggttacttatgatggacatggttttgattctgtttggtttgtgcagggtacc

SEQ ID NO: 179 - DNA, 1263 bp, Cucumis melo
  source 1..1263: mol_type = other DNA
aattctaacaactccggaacaaataatttagcatggattgaaatataaatcttcttgacttgcaaaaaaatcattgtaatggtcttatgttggttatagttagggtatcgaaacgccatacaggaatatgggattaaagttaacttttgttcatcaatttcagcttatgaacttctaaaatatcaattttacctttgaacttatatgttattacccctttcgattgtggtatgttaattaatatctgaatctcagtccttatgaaacttttttatactgtcacaaacatatgaagttttattgtaagttcttagaaatcatctaaaaagagtagtttgttggactatttattttattttttcttattaagttgttttcacgccatttcagtaaaataactatagtgaatagagaatcaaacttctaatcttaagttaaggtagtagggtatatgctaattcaataagataatccgtgatgcttgacatctgacttaattgttataagttttaaattttttattgtaatatttaaaatactagtttttggtttctaataaagaaataattgaacaattacaaatatttatacaaaattaaactagaatatatgatcattttccttcgtgttagaaaaagggaaatatatgtgtgtatttatacatattagatattgttttactatattccattttcctcacgggaaatggaggattgagtgggagataaacattgtccccaagagaattgggaatggaaatgcaaatgacatggccctccacaaaattgttcgcctaaaaatgggctttctcacttctcactccgcaagaaaaatatcgtttcccttcgaattcgggcaagatctcaaaaccacatgtttttctttctttatttttcaagcctacattatttataaaaatataacttaagcagagaattatgtaaattcaagtccatttttcgcttcacttagctaaatcattaacaaatctgtaattttgttcataaattagctcaccaattatgttttagcccactaaggcccattagacatttttattagaaaaacatgaaccgttggatcaagatgtgtgttttcttttctttttctttttattttttttgggttttggtggatcaattcgtagctttagcaacctattattatatggagggaaagggcgtattaatctgttagcgccgtccgggagtttagctttcttccccgagcctcggtcttatcccctaactccaaaaccctagc

SEQ ID NO: 180 - DNA, 715 bp, Cucumis melo
  source 1..715: mol_type = other DNA
ccaaaggtaatccactccttccccctccgctcttcatctttttctattcatcatctttaatctgttctcccttttggttcttagattcttcttttgttggattcttttaatctttactcatggttggccttgtaagtttagacgacgtttttatacattggttaatcctgcttctctatctattcgcacgctagggttttcctattgttttctattctgctctacttctgcaaggttgtgttcttcttcgttcaggtccctttttttaaccgaaattaaattaatgcaaattcgtttgtgcttctaattaggaagccttttggaacatctcgacattttgattgctgcatttcatttcgggtatatttctatgattgaaggatgtgggtctgttcactgcatggtcattacttatgcagctatgcttatcgagtccattatgtttgtgcaatctgtttccggattcataattttttagtaattgatcagtagatgaaaaaagatattgtaatattccttgagtgttgcaccagtcttggtgggtatctgctcctgctctttgcttgtggattttacttttattatatctgtattattcgaaatgttctgttcttgttataacttatacccgaagatgtgttcctccccgcgtctagcgttgtgggttacttatgatggacatggttttgattctgtttggtttgtgcagggtacc

SEQ ID NO: 181 - DNA, 2000 bp, Cucumis melo
  source 1..2000: mol_type = other DNA
aaataatttgtggattttatcatattatgtaccttagactttgtaaggtttataacacaagatgtggagaaatcccatgatgaacattggacgttattatatcctttgaaactaaaaacaaaggaaaaaagacaaatggctgagtataagaaaaagagaagaaacaaccaaaaagctaaaatgtcatgctctcatatgtaacatatttgaattgggattgatttcaagatgtattttaaaataatttaacacacgataaaataattctaacaaactcaaaattactcttaaacatttacttgatatcttcgacataatgacttttgttttaatacaactcaaaacataattaaggttggttttaaatgacaacaaacgaaaaactcgattctaatttcaatactagtctttgaaagccctaaggagcgtggttttgaattgtatagcaaggtttcgaaaattttaatcatcaaacaataggtatatttacctgttcctcaagtacagttaattcatagctacttgtcgtgcttcctacgacaacattgtaagacttgccacacactaattgaagccgttgttgaaggtagttttccatgtatagcttgaatcgacggatgaccaaagaggttgaagaaggtttgaaaaataggggaagggatatacaaagtttgagagtgagagagggagagaaatagaaatagaagagactgaaaaatgtaaaagaaaggatgaaaaaatgtggggtaaacgcaaattggatttttatagtagtattttgaaaatgctatagaaaggctatgtatagtagtgcttccaaagttctatatgaatgagacaaatcaaaatatattttttttgattaattaaccccaaaaagactcataaaaaaatcttataaatcccactaagatattgcatgttatatgtagtaaaatttatcgttcaaataaaccttaaacataattcaaacgaagaaagtaaaaatttgaatttcttatcttacatcattcaaccaaacaatttccatataagagattaaacttctaactttaagagagagatatccagcatatgcaacctaaaccaacagtgactttgctatatatttgcacaaaatgtgggggacaaagttgtaatttcggaatatcaatgattaaagaaaaggtaaaatttaaaattcggaagcttgacgtggcaacacggaatggtgatgatatttccaactcctcgcgacttttagaagttggcctcaccaaccgcatatccgcccctttgccacgtgtcagactacaacaacttccaacaatttcctttaagaacaccaaattatatcaataaatatttaacttaaattaagaatatatttgttacaattttcctactgagttagatagatagacagacttgtcaattaactaataagtccaaagtcaatttactcaacatagatacaattctaatttgagtgtgaaatacatattcaaatcaaaattattattaagaggaaaaactgatttgctttctcaatttaaaatataatattttgaaaaagaaacacacatgtattatggttttcaatatatttactttcttagtcacctaatctcaaactaatttttgaagaaattaaatatatatattatcatttttattttcttggttatgatattggtatagaatcaacaaaactacaagtgtcctctcctctgctatcgatggggattagactctaaacttgtttagcgattagtaattatatattagaaaaagtttatgttaatgtggacccgacaatctcaccaataggctcttcacttcaccaacccccgacccattccctctaataattcgacacggctcatccccggttcgaaccgggccgacgtcttcctatttaacacacctccatttcctcttccctccgcaacacaaacagagacctcaccggaaaatcaagttaaagcaaaaccaaagagaagcttcatcactctccggaa

SEQ ID NO: 182 - DNA, 2000 bp, Cucumis melo
  source 1..2000: mol_type = other DNA
gcatcttatggatgtagtcacaacatatttatatggattttctgataatgatatttatatgaaagtcccaaaaggatttaagatacctaaaacatataaatcaaattcccataaactatgttcaataaagttacagagatcattgtatggattgaaaaaatcatgacgaatgtgatacaatcgcctgagtgaatatttgttaaaaaaataatatcaatataattcaatatgtccatgcgtttttataaagaaatcaccgtcaggatttgctattataactgtatatgttgatgatttaaatataattgaaattttgaagagttttcaaaggcaatagaatattaagaaagaatttgagatgaaagatctcagaaaaataaaattttgtcttgattttcaaatcgagcatctagtaaaagggatatttgttcatcaattaacttatacagagaaaattttaaaaagattttatatagataaaacacattcattgaacattctaatgcaagttcattcattaaatgtgaagaaagatatttttcgacgtcgagatgataatgaagaactccttagtccagaagtaccataccttaatacaattggtgcacttattttgtcaataatcaagaccagatattgcattttctataaatttattagctagattcagttctccaacaaaacaacattggaatgaagttaaacatatacttcgttattttcgaggaacaattaatataagattattttattcaaataaatcaaattttaacctagttagttttgcatattcttgatttttatctgatccacataaatctagatctcaaacaggttatctattcacatgtggaggaactgctatatcttaacgatcagtgaaacaaattaccataacagtcaactcttcaaaccgtgctgaaattcttacaattcttgaggcattcatgaggctagcggagaatgaatatggttaaggtcgatgactcaacacattcgaaaattatgtggtttgtcttctagtaaactccttccaacaacattatacgaagacaacacaacttgtatagctcaaataaaatgaggttatattaaaagtgatagaacaaaacacatctcaccgaagtttttctatactcatgatcttgaagaaaatggtgacatcacagtacaaaaaatttgttcaaaagataatttggtagatttatttacaaaattattacctactgcaacctttgaaaaattggtgcacaacattggaacgcgacgacttagatatctcaagtaatgttacatcttacttgccaagttaactatacatagtgacatttggtggagttgtaagaaacactaatattggagaaaaatcgaaagaaattggaaaatatggagaattgaattttttttagatttttcttattttctaattttaggtttccgtattctgattatgcctcattttcacaacattaataactttaataagatgatttcttgggttaagggaaaaaaatcatttttttagagttgcacgtacaaaaatattatcataacatatcgattataataaaccaattcaccgtcaacctaacctaggtagagtttgagttaaatgttaaaagaatatccacccctcaacattgtaatcccaactaataaatcagcaacctaaagttttttttaaaaaactaaaaagaagagcaatatattttttttactattatttttttaaagagtggatttatttattaaattaaaaaatgaaaagaagaaaatttgttagtttgggtaatccgaaaacccgattatttgggcccgagaaaccgacgttttgtttattgttcctcacggcaataagtaatggcgtgaatcgaccgcgtgcgcttcaagctatctagacatttttatatcctccgattagaaaccctaattcagattctccgtattacccaccctggaacatctttgaaacgcgaaaaggtgacccgaagaaacttgaa

SEQ ID NO: 183 - DNA, 1989 bp, Cucumis melo
  source 1..1989: mol_type = other DNA
attacttgaacttaatccacatttatgtctttatataaagttcgaatactcataatatagccaagaaaccttgtttattggattttgagttttatcataagcaaatctcttatccaataacaaattattaaacaacacttcaacaataactttattcaacaatatattagtttaacattcacaaatcacgagtattagaacataaaacgcaacaaagaatggactaaggtactatattctaacttaggttgtttaggatttccatatgtcaatgcttttgtgatttttgaactagattttcttgttagattaattcaattctatttttaaatggcttaatatcttattttcggatgcttggggattgctagactaccgctttgttgaagcaataagttaaatttgtttgttacaggtattgatcaatctaacatagaattgaatttgtatgaatatttagttagacgcttgaaaactaattattctaccaatgagccgtagatcttaatgcaattgttattaatttgaactttgtatgcttctcatcgattaaatttatatcaagtagttaattaggacaaatctattggctttttcatttaattttgttaagtaaaagcaacttagaattttgaaaatgatgaacccatgatccaatacattgaaagagaattttgtttaactcaaactaggattcttctcacattgatttcgtataatttaactttttcaatttatatcaatccccccagggtgaaaaaaatttgtttgaagaattcatgtgctttctaaatctgatctagacttgccactaaaattaacttttgatatgtaatttggttaaatatttgattcggatttcgacgacaaacaattgatcaatgtggtattaaattctgatctccatgtaagaaatttacacattttcataagttcaatgttgacacaaagagagtaagagcattttaaaaaaaaagatacttttaatcttttctaaaaaaacaccaaaatgccattatgtaaatgtaacctaaataataaacatttaaacttagaattcatgcaattaggctttgtatgggacattgaattgattattaaaatcagtagttatagaccgtgagttataatggtttgtattagaagcataaattattttaattttgatcgtaatagcatgtatttgagatataaattaatttagtttgggtggcaaatagtaaacagtaaagcaaaatataaaaaaatgaatttaaaatagtaagatttgtaacaaatgattaatactataacaaacgtggttttaaaataacgttgatcgtagctaattgaacattatttattgtaaaattgagtgtttttaatatttggagcctcaaacttcgggtggatcaccacaatataatcatattcaaatttaaaattttatttttattataaatattgttaatagatgctcattatgggccatctgtcactccctccgtgcatatcctacctgaaacatcatatatcttaaacaatgtccattgccatgtgtcactatttttacatcccatccacttgacaaatatgttgaagatgcctacttttttagggatcatgtaatctatctcatgcttgtcaaattgttcgataatagtgttacaaaaaatttagtaattattattattatatttcttcgatatttatgcttcatatgccattgtgctctccatttttaccatacttaaaaaaatttcttattataaattttttcaaaaaaaaatttactatatagtcatcatctttattaaaattaaaattgagaacctgatatttttgatattaataatttaaaatttgaattaatccactttaaaattattaataatttattcgaatttgggccttaaggaagagatacggaaacaaaccctagatcccatctatatataaatcgccacaaaaccctacctttctctcagtttctcgttttagccggcaaaa

SEQ ID NO: 184 - DNA, 1463 bp, Cucumis melo
  source 1..1463: mol_type = other DNA
ttttcttcttgatttgaaattcttcctccttcctgttgcaaacaaacccagatgaataatcagacaaaaaaagcagcaaatttgaagatatgcatatacgaagaagaagaagaaaaagagagggaaggataaggtaggagatagcttgagattacagcgtagaaaccgatcgaaccggagatcaacggcgcgaattaggtcaagaagaagtgagggtttttatgaagaagaagtgagggtttttatgtgccgatgaaaaaccctacttctgtgttggtgatctaacgttgtttgatcggttcggtttttttgagaatcgagtaccctcattattattattattattgttattattataagtttgttgtaagaattaataaattatttcaaaaattacaatttttatttatatatagtttaaaaaattttataatttttttaaataaatttcgaaatataaggttggatttcttaaaaatatatgaaaaaagagatgaagtttataaattaaaaatgaaataaaaatagtaagtttgtactcttattcttatttacaatttaattttccattaaaattttaaattaaatagaaatataattaaaatcttaaattagatagaaatataattaaaattttcagaatgtaaatttaaattagcttagtgtatatttaaaatatataagattgaaataattgattttgtttatctaaatattttatattattatttattgaataaatataattatatatggtaaattgttttggataataagaaagtaaagatggtatttatatatataattaaccaaaatttaagtttgttaaaaagaaaagttttcaaaaatatttttttacgagtaattaggaaaaacccacattttacatcgaagtcatagactgggtctatgtcttcattgccttgtcgtgtacccgatccacgataacgcattatgaaccgagtagatgacttaactttttgtaatagcttttcttctaccatatttttgacatttttttaaaagtaacattatttataaaaaaaaaatcgtagtttgatctcacatgaaactattattacatcattaactaatatatctatatttaatgtagttttcttgacatgattttaatgctaattgaaatagttacaatttttgtgtcccattttgtttagatcaatatgacttcacgtattatgacatatggggccatcttaccagaaattggtgccaatgagaaaatgaatgtaccttaaccaatggagcaacccatgtgagccattgatgaacccaactttcttggtttcccatcttctattcatatgtcacaataccttctcttttctcattctatatatagactctaaacaaacaactaatctccaacttcaaatctttcacatattctcattcaagcattgaagtttaccacttccaaaaagattcaatccaatttagcc

SEQ ID NO: 185 - DNA, 2006 bp, Cucumis melo
  source 1..2006: mol_type = other DNA
cagcgatcttcgtagaaactaattcaatgctagctcattatttgacttttctcaggcaaggctccgcgaggaagagaaaaggtccaatttcaggaaccaagggcatggacaggttccggtcagaagaagctttttacgtaaaccctttgccagattgtttatgtcaaggagaattaccaaatggaagtacgacttccattttcagatagttcagtagaacatcaaagataaaatgctcttagagagctcaatgtatatgcaggcgaccactcaacgtgtcaccagctttgtacatccaataagccagctacgatggaacgacggagtgtttataacctgagttttggtagttggcggaggcggtgatggtggtatagaaggaaggtcgagggatggcaaaccctttacgccaagtagtggaagggagtagttggagatgaacacattttgagaagtttccaagatcactccatttgggggagaggggatgttggttatttagcacaattgttttcatgttttagtaattttatccaataatgagcgaggcattgaagcaattaaatttatttttaatgattttttcacccttccataggctttttcttttttcttttccttttagtttgcaaactttagctccttttatcggctgtcgaactcatttttgaagttattgaatgaaacacagtttgggctgtgtcagatgggtggtgaaattttatacattataattactacataaaatgaaatcatattgtaattttctatctatgccacaatttttttttattgcatcatgaggattaaattgtacgagtccaaatttgtacagtcatgtttttaaagctttcgagcattgttactaatgcatggaaaggatcgattatcaagtatcctcccaacttcatgaaagttattatttgtcttctaaatttgttttagaaaatgtttaattaattatttgagaagaaagtttaactaaatcctattggtttcctctaaggttgtcatacttatccaataacaattacgtttaaaatcaaaattattctaatggtataagactaatgttttaaaagcataaaattgatgaggaaggattggaagtaatactatttattttgaaggtaaacattcttgaatgtctgtcctaaaatcactaatgttttcttagtttgagactttgagtcgttgaacctctccatctttataaaatataatacgagtccttcacaataacttaaaatatatactaaatcctaattaatgaaaaataaataaataaaaggtacaaaatcattaaagcctaaaaatctattactcctttaaaacttttcaagggtccctacaaccaatgagaaactaccacgtcattttcacaatccgttcagtgtttagaaaagtcaaatcgcaccgtccatttatccactcgtaccaagtacggtaggaatctatctaccgtccgattaagcacaaagaagcacagtaaatgtcaatcgtgtccatccgccgccataccgcacatccttcgtccgaccggaaggccctatataaagtcctttggttttccgaatttctacttcattcgcttttgaaagatttcccaatctcttcgtcggccaaaattctctctcgcttctcaacccttcttcggctttttcatccaggtttgtttctcttctcttttttcttcctttgttgttcttggaatatgtttaatttcatttgtttttccattcaatttcatgctagattttacgattaggttgattttctgttcgtagattgtaattgatggttagggttagctttttctcccattccttctggaatctgtttcttgaccttcgaacttcgttgataaatctttagaaacatttacataaccaaacaataattgaacaactcgtgttgttatgcctatataatagcggttaggaaactggaaacgcccttataattgaaatcgccttagaaatttgttttgattcatacagggtacc

SEQ ID NO: 186 - DNA, 1664 bp, Cucumis melo
  source 1..1664: mol_type = other DNA
cagcgatcttcgtagaaactaattcaatgctagctcattatttgacttttctcaggcaaggctccgcgaggaagagaaaaggtccaatttcaggaaccaagggcatggacaggttccggtcagaagaagctttttacgtaaaccctttgccagattgtttatgtcaaggagaattaccaaatggaagtacgacttccattttcagatagttcagtagaacatcaaagataaaatgctcttagagagctcaatgtatatgcaggcgaccactcaacgtgtcaccagctttgtacatccaataagccagctacgatggaacgacggagtgtttataacctgagttttggtagttggcggaggcggtgatggtggtatagaaggaaggtcgagggatggcaaaccctttacgccaagtagtggaagggagtagttggagatgaacacattttgagaagtttccaagatcactccatttgggggagaggggatgttggttatttagcacaattgttttcatgttttagtaattttatccaataatgagcgaggcattgaagcaattaaatttatttttaatgattttttcacccttccataggctttttcttttttcttttccttttagtttgcaaactttagctccttttatcggctgtcgaactcatttttgaagttattgaatgaaacacagtttgggctgtgtcagatgggtggtgaaattttatacattataattactacataaaatgaaatcatattgtaattttctatctatgccacaatttttttttattgcatcatgaggattaaattgtacgagtccaaatttgtacagtcatgtttttaaagctttcgagcattgttactaatgcatggaaaggatcgattatcaagtatcctcccaacttcatgaaagttattatttgtcttctaaatttgttttagaaaatgtttaattaattatttgagaagaaagtttaactaaatcctattggtttcctctaaggttgtcatacttatccaataacaattacgtttaaaatcaaaattattctaatggtataagactaatgttttaaaagcataaaattgatgaggaaggattggaagtaatactatttattttgaaggtaaacattcttgaatgtctgtcctaaaatcactaatgttttcttagtttgagactttgagtcgttgaacctctccatctttataaaatataatacgagtccttcacaataacttaaaatatatactaaatcctaattaatgaaaaataaataaataaaaggtacaaaatcattaaagcctaaaaatctattactcctttaaaacttttcaagggtccctacaaccaatgagaaactaccacgtcattttcacaatccgttcagtgtttagaaaagtcaaatcgcaccgtccatttatccactcgtaccaagtacggtaggaatctatctaccgtccgattaagcacaaagaagcacagtaaatgtcaatcgtgtccatccgccgccataccgcacatccttcgtccgaccggaaggccctatataaagtcctttggttttccgaatttctacttcattcgcttttgaaagatttcccaatctcttcgtcggccaaaattctctctcgcttctcaacccttcttcggctttttc

SEQ ID NO: 187 - DNA, 342 bp, Cucumis melo
  source 1..342: mol_type = other DNA
atccaggtttgtttctcttctcttttttcttcctttgttgttcttggaatatgtttaatttcatttgtttttccattcaatttcatgctagattttacgattaggttgattttctgttcgtagattgtaattgatggttagggttagctttttctcccattccttctggaatctgtttcttgaccttcgaacttcgttgataaatctttagaaacatttacataaccaaacaataattgaacaactcgtgttgttatgcctatataatagcggttaggaaactggaaacgcccttataattgaaatcgccttagaaatttgttttgattcatacagggtacc

SEQ ID NO: 188 - DNA, 2003 bp, Cucumis melo
  source 1..2003: mol_type = other DNA
aactagactagcgagtgcacaaccaaattacaaaatccttaacagagacaaccatctatctcctttaaagcaacaataacatcaaccgaattagaatccacaatcagtaaagacgatgccgacaccaatgaccaaaaccgatcaaatatagcttattacggaccattacttcaacagttacatcaacaaaaaaaaaaaaattaaacattgctaataaaatctgaaaatgaggaaaaagagattaaaagttttgaagatagaaagaataaatctgaaatgttctaatttgatatataagaaatatgaggtaatatgacgaaagcattttgatagttttcaccaactccctttgtgaaaggatacatccaaccaattttacaatttctgttcaaattttgtccacctacccttctcttctgccccccaaggctgctttctttcttttattatttgctaaattaccaaaaactattttcgaattaaaccatctatttcaattatatacgtcattcgaattttaacttaattaacattagtatatgtttcggatcaaggatagtggtataaatcatcctaatttcaatttgtatttagaaaagttcaattatacttaaaacttctaaaaattttatattttaaatttggatataaattaaatttaagatttatggaaggtaaataattagagcaaaacaaacttcaaactatatggaaaatagaaaaggaatattttagccaaacaaaaacacttattattttattttgtttttttgttttttttttaatttaacaatttttttttttattggttgaatgtgtttctccactggtgagtctccaactttgacctgcaaagggtctatatagcgagtttcacgagcacctaaccaatatctgtgtaataattcccatttttctttcatacccacttcatttgatcatctttttcacaaccccggatctctaattcttgggaatttgcctctttctcgatccatttccaccgtaattgaaaaatattcaggtttgatttcttctgggttttcattcaactgtctaacttcattatgccctttatgtgtttgttgaaagccccccacccaccatcgttcaatgcggtttctttaccttttgttcggtttcaacgatgatttagaagttatagatggatgctaattgtttcgttgttggtttgatccactgatctgcctttgattggcataaaaggagattctagatcttgttttgatgttgtgatttatggatattattgttatagtcgtggaagtttttcttgtcgttctgcggtatatggttgttttattttttgagtggtaaattgagcagattgtgaacttttgggttttatggtgaaagcatgaattagtaaatgtagagctgctgaaacaaaatggaggtttgctagacctctttgtgaattcttaatggtcagcctccatcttaagaggctaagtccaaaaatttaaggcagtcttttgttattgttacaaaggacaagaaataacagaggagttattttaattgaatcaagttggaaagaagtactacttcatgcttctttcaaaagcaggtcaaagtgctttaaagtcttcttatttatttattttttcctgaatcaatttaaactaatgatagaaagaagtgttttttaatgggttattataagtaacatcaatttttaaccattccaaaagttacatcaaattcatcatagtgtgagtttacgaattttggaagttgtaattttaagttaatacttcttttaaggaaatgtacactttgcatgttgtgttcataaggggtatttctttgacaaacgcagcaaccaccccttaatgaaaactacaccacggtggttggttttttcttgttatttttttacttggaatttacaataagttgttatattcggatatatggcaaagcagatatctgtttttatccgaaacctcataaatcttgaatgtgcagcaggtaaaaac

SEQ ID NO: 189 - DNA, 1024 bp, Cucumis melo
  source 1..1024: mol_type = other DNA
tcattgatgaagaaggaaactttaagccaattcgacaacttatccattcaacaactttccaccttcagacattcagattcaactataatataacataaattgatagtcaagtcttttttgagacaaccataaatcatcttagcttcgagaactgtcacttccttaaattggtgaatatatcacattccatccattcaaaactttgtttcgaactttactgtagttatgaatcaataaattgggagagatattgttaaaaagagagagcatatttgtttctattatttactctctcctaagagagggttaattagtctataaatgatctattcttctcgtccattgaaattttgttatcctaaatttatgaatacttctacccaaaataaagactttttttttttttgaaaagtgtcaaaaaaacataaagaaattgacaaaacattcatttttagtggattttttacggacgtaaatagtttgtttttgtttcttttaataatacaatttttttttactttaaaaaatatttttgttataaaaccaccgtatttttattcaattttaataaataaataaatgaaagaatataaaaaagaggaaggaaaaagaagccaacgaaccaacggttgccacgtatcaaaggtctaaagtgcgcaaaacgaggccttcggaaaccaaaatgcgtggcttcaattggagcaagtaaacatggaaaccacgtccattgtaacgcttcctgatctcttctttacaaccgttggattcgagtactttttctcaacgattaacgactgagtggacctccacttgcttctgttccacgcgcgtgggattgacgtgtggtccacgcaactcttctcgataggatcattcgagaacatcctttacttaaaccgcctctctctgcctcaatttctcgtcacttccttctccttctttaccctttccactgcggctgattcttcttcgccttttattctctcgtacgccgccatattcttcacttctttttccggcgaca

SEQ ID NO: 190 - DNA, 2001 bp, Cucumis melo
  source 1..2001: mol_type = other DNA
attcgtcttcgcattatcagtaaatttatcattttaagagtttgttcttttttaaaaaaaattaatcatttcgataaagttggagaattcaaaaatttctccaaataatttataaaaactttcggttatatatcgaaaaaattaacatggtattaaaacgatcataactcaattaacataaacactccctctcaactttaataccaaatttctttattaacgcaaaatttaaaatttgtttttaaaattttcacataacataatagaaatacttttctttatggcaaaaatacaataatcaaaattgattgatggtgacaggacaccacacaatatttttaaattttgaatatacgaactatataataagatatttatgagattcccatcctaaagattcctagagatttccttgtgtacaatattacacaagtatcttggaagtccaaagtcctgagaaaaaagctatgtataaagtaatagtgtttgtcgtaggaaatttacttcattcgtgtcattagctttttattgaaaaaaaaaattaggtatatcttagtgaatctcacttaatcgttgtcgatagttattcttttaatatcattatatactaaaatataacaatattgaaaagctaaaactgtatataaaaaaaatgttacctctaaacttttatcgtttatttaaaagataaatatattctttcaaaacttacaatcaacatcctacgactatcattataggtacaaatcttttcatgtttacacaaaaattagatttttaaatggtgtaatgatgatatataacgaaattttgaatgattactatttgaggttaccattgtaattggtcgtgttgtttgaaatttaattttattagaaaatttgtcaaaagtagcaaaaatgaataaactatttaaactttaggataaaatcaagtgttatgagtttttgtctagtttatatatttttatttttattgaaaacccttttcctatcttttcattacttcaaaatagttttaaaatgtctattaaggctaaagttagtataaataaaatttcggaaattttttttcgaaaaaaattgataaattatttatattttatattaaagtcaaaatttattacgcgtagatgtttatcaaattttctttctttttgttgataattttccaaaatttggataattttttaaaatagtaaaattattataaaaatgaaaacaaactatttataccttaagcaagaaatactaaaaaggcaaaaattcatttacttcatgaagcgtaaaaattaaatattttaccactttttgttattttttaccatctctatcaattatttgtaaaaagaaaactacaaaattagatgttttttcttttttaaggtttaatcaatattaaaatttcttaaattggcagacaagttggtgttggtaattacgaataaatcccgaattgactaaaaataaattcttctccaagtaaaatagacacgtggatgaagaaataagtgaatcaaaggcatccacagttcaataaatggaaaaaactactttctgctgactcattcataagttttcataaaatttcataagaaaggccaaagggcttatgaaagtgaatgtcatagcagtaaatgaagcacagcgccattgaaagacaactcaaattgcatgcaaacccacataattattcaacaaacccacatcaaatttcccataaagatcaattctttagggggttcaattacccaaaagtgaggtagttgaaaaccattaaacaacaagaaatcaacaattttgtaatttgtttgtacagaagtaagagataaaatcatcgttaaccattcctttatttcgtaatacaacccatcaaccatctctctctctctctctctctctctctcggcctttatctttctcttcctcaattatttaagtactacccaagtgagctaaaagcaagttcagtggacagtgttgtaagaaccactacagaaaa

SEQ ID NO: 191 - DNA, 4175 bp, Cucumis melo
  source 1..4175: mol_type = other DNA
tagtttggttcataggttatagtttccaaatttgttaggctatcattaatcaaacacaatacttctcttgtaggatggctgccccctatagtacttttttaacttaggagaaggatataataattatattccttttagaaaatataataataattgtgtagtgctttgatataccttaaattagctactcacgtttttaggaggaagcttccgttgcttttcatggtgttatgatcttttttattttataaaggactgaactttaaaatttctctttcatctattttggattggattccatctattttatacgggaagtgaactctaagatttctcttcacctattgtgaatcggactccgtcatgtaggtcaagactacgacagataagaatagacttccacgaaagaaagtggtcaatcgagatggctatatttggctctttcagctcaatttcttcttttttccttgcatgttcttccgttggtacatttcttgcactttttttgttctcacatgactaatgtattccaagtttatcattggcattgtgcctcttttaggcttgtaaactctcgatccaaaattatctaggacatatgtttcctagtgaagaaatactagtatattccttatgtcaatatgtcaaaattttcaatttcttaacctttgagtaaatcaatattatatttttatggaggttatttataattggaaaaaagttacacccatctcaaccctaattaacaccaaatgaaattgtaccatgcggcacaatatttttttgtgagttttttgcaaagagaaacaaagtagcagacaaagaacaaacattcccccaaaaacagcagagaatacctaagagagaatgctctctcgtaaaaaataatacccaagaatcttcccaaaaagagggagtaaaagagtccaaaacaaacgaaccgaagattgacaagaagggcactctcgccctccactgcgccgctaaattgtaagaagcatattttcttgagttaacataggaataggtgtaactcaagagaaatgtaattcgtagaattgaactttgtatattaatttatatggtgttgtagatacaatctttagtatttactcatttggtgctttctctcaaatacaatttaaatttagaactttttgatcttcgattttcaggaagttggagttgcaaatcaattcgagtttcaatctctggaatttaataaaagtttgatcttccaagttttcaatctttcagaagacgatgatcttgatatggataaaaaattgcacatcatgagagctttttgaagtttaaatcttcaattctctagagcttaaattcttccttaaaccaaagatcaccaaatgaatgacaaatgtctctatttatcgaaaaatttcatagacttttagatgggcttaggcacattacttgttgggcttggacttgggcttatttgcttggcgggctcatgctcgagcccattatttctttggcctatttttcatgaggggcttgaacttggttgtatacgaaaaaacttgactacctaaatctaatcaaattataatcatcacaattttgacgtgttacgatttaattggccaaaaattcttgttcaacacttgtctctaatcattttcctatataatttaactaaaatatttaactttaagtaacttaaaagatatagtttaattcgaatcaaaatacaaatacaatttcgtctatctattcccatcataaatgttgattgagattcatattataaacttctttcaggaaaagaaagaggaaaattcacctaaaccacgttttcctattttggtaagaatccccaaaccataaatcattccaaaattattttttttagattagaaaagaaaaaagaaaaaaagaaattcacatggcgtaaaatttcagccccgtgagatattttcgaacccccagatacaatctacaccgtgaaaacaaaatcggacggtggttgctataatgtccgtttagaggcaatggcagggatgaaattgccaacgcaagataaggaacgaataagagaaggacacgtaagtacaagtttaggatgggcgggcccacagccacaagtgccgttcgtgcttatatacaagtcgctcatattcctagaagtgtctccaaataaaggaaagaaaagttcactcatagagagaaagagaaaaataaagcttcgttgccggcgatctgaaggcggcggccatttctctcgggagagagaaagagagagattgatagagcggagagttcgaggctctctcaaacttcggtcctcttcttctctttcaggtatcgttcttctctatcccttcgtattctgtttcctcttttctctttcttcgccatcatgctctttctcttgttttgtactcactcaatgtgattgactttatgttgtttttctgttttatttttccattaatgctcgttgtaatgtgtagatctatgataagatttgaattattgctcattaatgtgttgcatgcttttgatttcattttaaaaacagagattactttctctatattgattaaatcgttggattttaggttcttacagagtttgtaaacagtgatgttaaggattgctgagatttatgactgatgagagttagtgtttgtcttttagcttgtcgttttcctctttgaaatcacatggattcgatctggatatctgggtttggctcgtctgaaatggctacactatagcatatttgagtttgtgatgttgaagatttgttaatttcttggaaaatcgggagttcgttttgtttttcctctttttacaggttttattgattggtttattgatcggcgatatctcgttttcaacttccgaaatgctatttttcataagaagaaattgtggatgtctttttctactcgattagagatccttgaaactatgccaaaaaaaattggttctttcaccaaattgttttttgtcgtttgtgatattaatgcattttcttattcttaattaagttcaagtattcttttattattttttaatgatggttgttgtaatggttttttcccttttactaaaagctttttccatgtgattcaaaggtgtacttggggtttcccggtctttgttcccaagtcaattaggatgggcgccaattcgattttagcttctgtatcattggtgtatattctgttctggggaggaaaaaaaaaaagaaaaaaatcttccgtcctacagtgtgctgagtaacaatttgaccagccttttctgccgaaaactttttgaaattattttttaattgtgatttggtgaacttaaattgttttaataaataaggtggattgaatcttaacagaaacatcaaataaaatcgagttttaaaaaaaaaacatatttttagtgaatgtttattttatttaaaagatctccatcagtcctgatgtttcctagaaaacttatacatcataggtcttgattaacaaatttggaggaagtcaataggttattctttttttctttttccattctagtttgaaacaattttcttttcttttttaacttagaaaataatgggtagctagaaatatggaaatcaatgtattttgggcttctccttgaaactggagcagcggtcaatttctctttcgtttgtatagatgtgatagaaatagaatgtttccttcgcttacggcatcagagagttggaattggtctttctcaacctcaatatcaattaaatcaagtttcgtcataaacaggttttttttttcttcgtttcaaatgtttggtagggtcaaataatttgtaaaatacctagccgtccaatatgatacaaactggaggatttcacttgctcttttaaattacaaaaaatattttatcattgatgttgcctgtctgtgtttatcttttctctttccgcctcaagtaggcgtctaattgtcttggcaagttggttttttgtacttccgccccttgtcctttggcccttttgattaagtttttcatttaattttctggtcggcgtacgttgaattattaggtttgcatttaatgtggtacctggtgctttgactcttatttgataaggtattttgaagtctaaaacgttaaaccctttgtttgatgtttatttttttatcgttccaggacaatatcctttggaaaaa

SEQ ID NO: 192 - DNA, 1999 bp, Cucumis melo
  source 1..1999: mol_type = other DNA
aaaagagtcatagtgaaaaaagctgagatcataatagtttcaccctaaacacaacttataataacacatactatcataatatacacaccaaacacagactctatagtcttcactctaaacgcagattacaatagtctgcaccccaaacgtagactattataatcttctgactattataatactcttttcacttatcgccccaaacgtcccctaagagaacaaagataggttataaaagagagatgagggtttatattatgcaacaagtataaggttctagaacgatgtagtcttcaaagtaacgaaagcaataggctacacgagaaaaatatttttaaaatatagtgctttccctaaactagatttcaatgacaaattattataaaaaatagaatcattaatccaacatggcttgcatgtcacaccttggccaaaactgaagacggatgtcatactcgacttcaatatatttttttaattaattttcatgtgacaacacataaatatttaaaatttagattgggttggattttttttcaagtgggtcccaaaatactcttcaaacccaaaccaacccaacttgtttacccatctaataataacccaccaggttcaagaagacgaaccgaaccgaaccgatccggtctaactttgtttcatacttaagtcgaacttagcggtacttttggttcggttctcggtttccccaaacagagccactcaaaattagatttagggttccgttcgcaattttcagcgcatttttatttgaatcggtcgtttgttgaacacgttctctctcagctggtttagggttcatcgttctctcttctcgcgctatatctttctctctctcaggttcgtttctttctcttaggccattttatcagaagatcctcttcgttctccgattttctttccgtgttcgccctcggtttctcagcagacgtaggaagtttggtttccgtttagtgaatctgtttggggtattacgaatgatattttgtactgggctttccgcatagtctttttctttctaggaatatatgcatctgagaatttatttgtttggcttttctttataaagtatgaggacatatacatctcgattgctaatccttgattataatcttttttttttctatgttgtttgaatctgtttttttttttttaatttcaataggttttttgaatctaaaaatgtatttcttggatgaattgcatactgttgaattagaagtttattgattagattgttgatatttgccctaagttccatggataggtttgcgtctttcaccttttcgtttgctttttcttttggctgacgacatcttacatagcctctgctctaaaaggtgccatgattttttttcctggctttatctgagtttgcgcaatttagatttgaagtgatgatttgtctaaatataaatatctatcggccatactattttttgttattttgagtttttcaggatgactgctagagaatgaaaaatcttgaaacattgtgttttgaagttcaaggatcttgtagttttgttcttttctagactatctcatttgatatagccctttaaatttaatcaaaatttgttaatattcaaatcctcggacattttaattatttatctaaatagttgtttaggcattactcaggttgcccactattttaagcttagaagcctactctggttgacctaaagtttgcatgctatttgccttatttcgcacgactctaaactgttatagacatcttttttcagccttcaggtaaatgaacacaaaaaggagtgaaagtctgacttctgtgtgatggtcttttaatcaattatagggattaagatggtttttttattcattgtataaatattaaattagaatgatgacaaccaataatattaaaactgacaatggaaggttccttatattatttggagtgtacattacaacagcctgattcttggcttggcaggttcctgatcaccttgtaaac

SEQ ID NO: 193 - DNA, 2000 bp, Cucumis melo
  source 1..2000: mol_type = other DNA
atttatttgtttagagataagacgcacatgagaatatgagatggattccactccactcacactccaatttctacctatcctattactgtttactattatcattccacccctcgacccctcattcttcttctcaccttacttttttatgatttactactacttcattttggatcacaatctgatcaatgctgggtgggctgccctcggcctgtcaccaggcccagcccacttccaaattaaacctcttggcccaccgcccattgtccccatcccattccatttaatattcccaaccttccctttttctttcccaatgcgatgcttctccaatatacctttcctgccctccatgtttcctttttactgctttcttatatttataacacaccttctacagtcttttggctgggaatgctgcgtatgtgaatgagattcaagatttcgttgatgttatttgagtctctatattcataagttttgttcttagttttctctagaccaactgcaagagttagcgttccatatgctcataagtttcagatttctgctgtgtggtttgaagacagtcatcgatccatgggtgaattcggctttttattattattattattattatttattgttgtcttacttttctatttgaatcttcctatcttttttactcattgttggactctaataattcttgctaaacacaatctccatttttattggacattttaaatcccatctcaactcataattttagttaccttccaccatcaccatatccaaatccgaaataaactcaaataaaatccttcacgtgcatgtgctctccatatattttttctacatggtaaaaataaaatgaaaacaatctaaatttaataaaataacatatatggcagacttttattgatgtagagactgggtgttgtacaagaacagtgcagccaagaaaaaaaaaatacttccaatgaatcgtacattttaaggattatgaaactaactagttccaaccattttttcacgaccacgtgcttgttaaacacgcaagtagaatcaaaatgtgggcttcttcgctttatataactgtgaatcattctccaaaaagggaaggggatctcattccctaattcaataaagaaaaagaaaaatgctagcgaacttcatccatctcattccttttacctatttcatgagatgcccattgtatataagtatttttttttttatttcattttacttagtttactcctcacctctaaaaaaaattaggagagtttgctaaatccattctcaaacttagctttattttttttaattttatttaacctcgtcgtggatgttaacctcaaatgtcagttctttttattctatttattgatgttataatttactttaggattccaattttataaaaataagaatacaaataaagataaagagtgtgaaagccagaaagaaaaaaaaggaaatcgtaatatgggtaaaattggtacaaattgggtcccgttaaatattaactcaaaaaatgcgagaaaatggtagaaaaggaaatagggggtaagagcaaagtagtggaaggagagcattgaacatattctctagtttttgcacttggatctaaacacgaggaattataggtttattcatttactaattacataaataggattggattttaaaatttgaccgagtgattatgcatatttgatagagttagaaaatagtggtggggcaggtacaagttacaagtaatgtataagagatatgatgagcatattaggaaactatagatttaaattcgtccgtaaataaataattagaaatataatattcgagtggaagggtattagggttaggcgaaaccaattgcagttgcacctataaaaccccttttacgcctccacccgcttcaacagcggtctcggcgtctacaactacacactacacactacacactacacactacacagttgcagaccagaagcataacgtaacgccggtccacaaaa

SEQ ID NO: 194 - DNA, 2000 bp, Cucumis melo; identical to SEQ ID NO: 121
  source 1..2000: mol_type = other DNA

SEQ ID NO: 195 - DNA, 1400 bp, Cucumis melo
  source 1..1400: mol_type = other DNA
tatatatattaacttttaaaattttgaaaacgtcatagataaattatatacaaaataaaaagtttgattatttacgaaagttaaaaagtttatccgaaagttgactcaacgataaaaacactaaatatcacttttagagatgatgatattatacataaacatacgaacttacgcgtcaaacttttatactaacacaagatcaaaacaactttgttgagtagtgagaattttatctgctgatatggttgaaacttgggaagcaagcagaggaagttccattcattaccaaaatccattttgtattcatcaaaatatgaagtttagcgacttgataaagtcaagtcaagtggtcctatcgatttgttaatgtcaatgtttggttttgaatttgatacctattagacaatgatatataattttaagtatggtttacactgtgatgctttatatatttttaaatgtaaaatattagaacttgtaatttcaataaattttaaaaatgattttgtgttatttccttttttaaattgaaatatcaatgtatcaatattgcgtcatagagtattgcaacacaaccttatgttaaattgtttattgcttattgctctaattcaactccttcatcaaatgtgcacagaatttaaacaagaaaaagagtaggtgcttttttactaaaatatactaaaagctttttataccaaatcttatgacaaaatcattccaacaaaatgactatttaaatataagatcgaatccctaatttaaaaaaaaaaaaaaatcaaagatgttaatttctattattaaactcactttagcgtagctaacaaaaaaaggaaaatgagaggctacaaagcttgagccctctgcctccctttattgcattgtttgaaattagatcaatactttgtatttttttcaaaatgaaaaatcgtacatagaattaattctatggacaaaaaatcagagaaggaaataatctagaataaaattcgatttttaacccaaaaaaaaaaaaaaaaactcgattctgatttttgtaagcaatcacccaaattaccataaataaatggtattcaattactcaattatggatattttagaaatgataaatttttattcataaactcttttctttctctttcaaaaagaaaaaaattagcataaacttcaatgacatttatttattcttcttcgtttggagtcaaaagtttaaattgagcatcagtccagcccaaaagcccacgaagaagcccaagaatcttcagctttttcgttcaaacgtccctttttggtttataaaattaaagaaaataaaaactaaatttatttgttatttaacaaaacatttttggttaagacattctctttgattatttttcttccattcttcgtcgtcaatc

SEQ ID NO: 196 - DNA, 2019 bp, Cucumis melo
  source 1..2019: mol_type = other DNA
tttatatttatgaaaatgaagtctctaaacaatttttctactcccaaatttgttgatttttctgcctattctttatcggtgctttaaaaaatgaaaccaaatttcaaaactaaaaaaaccaagcttttaaaaaaatgttaggttatttttgaaattcaactaaatgttgaactcttttacttattaaataggcaaattattgaaataaatttagagcaagtaagcttaatttttaaaactaatatacttaccaaatcgaggactaaaatattcaaatactctttaaaattaagattaacattaatcactttgttatgtttaaaaagttgcagtgtcacttgaacctttttaaattaatataatgaaaatgaatccaactcaatatatataatatctatattattaatctcgatgtcagatgtttgatacgcacatatctcaaaaattatacctcaactaacatcggtgcacgatgtattatttcgtgaggataaaaatcgtttttagtataaattgatggaaagattatttgaattactgaaaaatgcaccggtacattatttgaaacttccccttcatttaaagaggctaatattagaaaaagacacgctgaggctatttttacaattaatgtgggctgttgacttggcccagcccaaaacataaaccctaaagtagcacaaacaaacgcctctttcttcttgaaaccgcatattaagcgttttatcacttctcaccacctctcattcctcctcttccgcacgttgtttcgctcctcaacgggagtgccttccctttgctctccctccaggttcttcttccttctcatctcatttccaagtaatttcattccgtttcttttctcttaatcgtatcttgttcagactctttcgcgtttttttttagttgcgccttaccagatctgtgttttcactcgtttctattcgatacatgcttccaagatccatttcttaatcgcatgtattcggttgattggatgattgtctttttgtaagttttgattacttttttggaatggatcggttgaaccaacggggtttaagtcgatggaagtaggttatgttaaagatttgcttcttttttatgaagatgtgtgtgttcttttttctttgctagatgatgttattatttgattgttttaacagtcgtgttttgtttttctgcagtttatagtcctcggtcttttgaagacttgtcaagatggttagtacacctcttgtcatcgtgattttgattgagtgatgtgttaagtgcttctttaggttacagctaacgcgattttttatattcaattgtgcctgtgcaggtgaagtttacagcagaagagctccgtcggattatggactataagcataacattcgtaatatgtctgttattgctcacgtcgatcatggtaagctacttagtttaagtttatttatgccgagcgtctatttaagaagattaacatcttagctttcatttattgtttatttggtaagcatcgtttctttttctccgaggaactgtacatgtcagttcacatgacaataaaacgatcttccttggacattagtttttgaagttcaattagacgccaaattttgttggttaaaagatgcttgtggagcatatggacctaatggaatcagtactttttgatggatggacttgtcttttgttcttttattttcaaaagaaattgcatgtgcaattacatcatctttgatcgaaagattgggtaattgggtaattggggtaaagacatgttgtaaaaactaatgttaattatcaattaccattatataccttatttagtgcttatttatatcctttttccccatttcagggaagtccactctcacagattctcttgtggctgctgccggtatcattgcacaagaagttgctggtgatgtacgaatgacagatactcgtcaagatgaggcagagcgtggtatcaccattaaatctactggaatctccctctactatgagcagaagagctccgtcggatt

SEQ ID NO: 197 - DNA, 1999 bp, Cucumis melo
  source 1..1999: mol_type = other DNA
aaaaggcgaaaaaaaagttagcttcccgagaaggagaagacgaggaagagtttgacttcccggggagataaagtttgtgtctcgagggaatctctaatctggagttgaccgtcgacttatgtgtcgagcctggatttagttgcatggtgcgacaaagcgataaggcggcatatgtaaagtagtaattcaaaactagcggttaaagaaataatcagccaaaaaatttagtacaaatacgggtggaggccctaagtgaagtgctgctattcagaggttttggcaaaagagtgcaaagagttgagttgtgcagagaaagtactaggtgaggagaggcgtttggaaaagaaaaggatcaaacatttgcatgagtgatattcttaaactaaacactcttgtgtgagtgacttgcctaagctaaacactcttgcatgagtaactttcttaaactaaacgttttgtaatgttttcttaatggattcttttcgagtctgagttatgcttaacacgttttgtttctctcgtgttattgttgttgttgtttgaaaagagaaaactattgttttctatgtgctgattgtgatgaatgtgtgcgaaccattagccttaatcctatcaagtgaatagtgattatgtggtgtgtgcacataatgtaaatgacattgtgtggatggccagtgcaacaagaaatgaatcagaaagcttcccaaatactgtgaatggagtgaacatcacactagctcaatggcaagatattggcgatagtgaatcacaataggcttgacaaggggaaggattcatgttcttggttgaaaggaataagagaggctaatgtgagatttctgtgatttgcaaaatgaggcgttggaagacacgtttgagaaatgaaaacgaattagtgcttgacttgtattcctaaaaaagttgtccaatatcttcaatcactaaatatttgatgtgcctaagttttccttccttagttgttgaggcgttgaggccgagtaaggaaagataagataattatgacgttgaaaagctggtcaagttatccatctttggatggtttaaagttattacatgtagggagggttgcattccaattttgtgtgtgagatgagtcttattttcgagatgggttgctaggcgatcaaggagaagtataagaaatgagttcttatactcttgaacaacttgacacgaagaataacatcctagtggatgaaggaaggtgatggaacttaaagtttaggttttatttttggccttgtgataaaaaaaatgtaattgtaaagtattagatcaagtaataaaaacagagttgtgttttctatttttgctgtgttgggttgtgtatctttattgtgcttatggcctagttgctaaagagttaaggttattacctaaatgttttacggtgtgttgagttgtaaagatctcctgagttaaagttggaattttgtattggagattgttttgagaagtttagcttactaattgtttaactcattaggtgtctaagcgacacgcctccttttggtcgcatgaagtggctagcagggtggggcggaccggggtggggtgtgataataaacctaaaaaatcacccagataagcctaaattatacgttgaagttaaacttacaatttgattagaagaagaaggaatatctgatttggacatgaattaattacaaatacggcgccaatcatacaaagcacatgtaagatcaacgcattctacactcaatctcagccgttgattgctttcaatccttcaaaaagaaaaaaagaagggcagttcgggcagagtcatacctacccgttgactataaaagcaactacaaatcgaaaacctccatttctccgttaccattacagagaaaatcaaagaaatttggcgttgagagattgggagagaggtttctctttctagggttgcttcttcttcttcatcctccattgttgcaaatttcacttccttctcctcttgttctcatctccc

SEQ ID NO: 198 - DNA, 1578 bp, Cucumis melo
  source 1..1578: mol_type = other DNA
atatatatatatataatttaactaaataaacaaatgaaagaaaaaagtgagttcccattcggaaaatgcagatggatccatttcttcaaatattaaaaaataaaaaaataaaataaaataacttaaatatgcaaatagaaagaattttaatttctggattatccatatgggacaatttttaaaactcatttattttattttttttatttatttgattttgatatatctatggggaaatttttcgtaataattttcgaaaaaatattgcaatatatcatttgatcagatcggtattattaaatctctatcacatttggtcttaaattatccaaagattcctttaagataatttagataaccatctacagatcactactataatcaacaaaaggaacaacttaaattatttaaacaaattcattaatattagactttgtgcttcattagaaaatgatcttatcacaaccacaaccatagtggtggtttaaaattttattttaaactcttattagtattattttaattcatacttaatcaaactaattactttaaaaaacatatatatataaataagttaaatcattcccccttatatctaaataacataaaaaaaaattgtttactctacaagaagtttgtatatatatatgctcggtactatttagcatctttataataaaatttctaaatcaattttttatatctctttattaaatgtatagtcatcaaaaaatttaacgagataatgtgtcaaagatttattttattaacgttcataaatatcaaattatacttagcttataattgaaaacatgttcgataaatataagtaaataaaattttattttttttaaatattacaaaataaactaaataagttataaatatgacaataaacattatatattttattatatttataaatacttaataatttagtcgtttaaaataattttcttaattttcaaaacatgtttcatatgttaataataaataaatggaaaaccttccaaaagaagaaaaaaagatatcttaaaatttaaaaattgagattttgaggatcaataattaataaaagaaggattaataagggtgaaattaaatcccaaaaagaaaattgaaaatgaagaaaagaaaagtgaagaaataattgaacgtgggaagtggattcgatgtctccagagaacaagcgaaaggagacgaaatccacataatttgcacgttacgtgtccctatcaaccgtagacacgtgtcaacatctcaacaccctacgccgaattgcttcgctggatctggacggtcatcggataacagcggcaaccaattaatatttccccttatatttcacagcctggccatgtccaccaatcacgttcaactattaattcatttttcatttcctttttctttttttttttaattcccctcaattattaccgacaacctgttgtagccggttaaccctaccctccaacgttccattataaggcctagaaaatggacgtgaaaatggagtactacaaactacaattaattttaaagaattttaattttaaagttctctaattactattagcc

SEQ ID NO: 199 - DNA, 1023 bp, Cucumis melo
  source 1..1023: mol_type = other DNA
ataataataataaatacataatagtaataataataaaaaaaataaaaaaataataatagtaatgaaaatcaatagaataattttaaaatcgggaaggaagtcgtgtacaatccttgcacgttggagagtcaaatggcctaagtggtgatgtggaagtcgtgtaccgggtacacgattttcctacaagtcaataataataatatggttatttttctagtttagggttcatgacaaaagattgttcagtcgactggatgtagacaaatctaaaaaataaattaaaatctaatatgaaaactagttttaatttccaaattattaagggttgaattcgaccaataaataataataatacggttattttgaaatttaggaaattgaataaagttgttaaaatcttcaagcaaattgttaagccccgagatattaagaagaggtaataatagaggattctatatttataacatgttaaaattaattgcaaactcataaatgcatcacacagattaacaacataggagggacttccgataaaagtgcaaatattgaaataattacagttcgcgaacatgagtattttaatattttataaaatagtatgcacgtgtatttttgccaaaagaaaaaaagaatagattttgccatttttcaaagtgactctcggttatatcttttatggcgattgtattttatagcgtatgttgtttgtagttaacccatttctcattggcaaattcaatcgtgggccacaacgtttgggcatagcttcaatttggattaactcaattatgtctgaatgggttggactagttcggactcttcggctgggccagaatcagattcgggccgcaatctgttcatttcacacctatatccaaacacccccaaaatcgatacccatcaaaccctaactctcaataacccccatatataaattccttctttagggttttttcatcctcatacactctcaaacctccggtcattctcattttccctgccgcttcttcaataaccctaatc

SEQ ID NO: 200 - DNA, 1654 bp, Arabidopsis thaliana
  source 1..1654: mol_type = other DNA
tgatgattcttgttgttgtagttctttttaaaagtcccacctgagcctctatagactctgattctcttttaagttactattttcaccgctctctaataaggctcgtgattttttgggagccatactgtatactcgccggccctctcacgatgttgttcaattcacagactaaatttgatttatctatttcgccaaaacataacttcattaaaaaatgttctccaaataactaaacgaattaaataaaagaaacctttcatgtaaagttaaaggtatgagactttaagggcagttgctgaacattcgtaacacatgggagaacaatagagaaagttgaaaagaaacgtagcatatagaaaaattatctttgtaaccaagttgatttagaaaaatatcactatttgtgaaaaatactagatcagtttattattacttttttttttttgtatattcacaaatatcatattcatatagaagaaaataaacaaagttgtaaaaatctggcatttaaaataaaattgaacacttcaatttatttcctttcataataataattttggcataagatatttgcaaattgatctggttcggtatggtcgacaaaataattttccacgctacccttccagccgtccattcactatttgccctcaacgttaccaaataacggtccagattcctagggcaagatctaacggttagcaagtaaagtcgtaccatcagaaagaataacaattctttcacaaagtaaacataaccaacggttaacaagttcttagggttaaatcagtaagatccaacggatattaaattgcaaggcccaaatagtttttttgcagcagataataactcgtccccactggcgagtgacgaccgagactctgtgaccctatttttcgagacgataaaagggcaaacaatcgctcttttcaaagctcgcctcttcaccacagagaaaacttcgtctctcttctctgcttcgccctctcatttcctgtgagataaaggcggagtctctctccagttattttgctcatccatcgattcttaggtatgactcgtttctctcagatctgtgattctttataatctcgtcgttcttcaaatcattgttatattcgtttcttcgatctgtgttttttagatctgtaaggtaaatgagacgtttcgatctgtagatctgattgttatattgatagattatgttatctgctttgcttaaagtccgatcggaatgttttgtgctcattgtcgaatatctgatgtatcggtttcatagatctgcttctttttgtgcgtttcgttgatctgataatcttctagtgatcaaaatcgtttggatctgttgactttagtttaaaatgtatccgatctgatgtcgaggcttcattattggaagttgttattgttgtaatcctgatttaagttgctgttcttaaatttatatgatctttgcgttataatatgacatggtagatcttggttcatggttcactgttttccaataaacttggtttgtttggttggatagcgttctgtgatacgaccatgtcttgtgttggataagaattctctgaatttccttggctggtttgtagtatgttattcacgtctggtttctcatcaatgattatgtgattttgcagagttcacc

SEQ ID NO: 201 - DNA, 712 bp, synthetic construct
  misc_feature 1..712: note = Chimeric transcriptional regulatory expression element.
  source 1..712: mol_type = other DNA
ggtccgatgtgagacttttcaacaaagggtaatatccggaaacctcctcggattccattgcccagctatctgtcactttattgtgaagatagtggaaaaggaaggtggctcctacaaatgccatcattgcgataaaggaaaggccatcgttgaagatgcctctgccgacagtggtcccaaagatggacccccacccacgaggagcatcgtggaaaaagaagacgttccaaccacgtcttcaaagcaagtggattgatgtgatggtccgattgagacttttcaacaaagggtaatatccggaaacctcctcggattccattgcccagctatctgtcactttattgtgaagatagtggaaaaggaaggtggctcctacaaatgccatcattgcgataaaggaaaggccatcgttgaagatgcctctgccgacagtggtcccaaagatggacccccacccacgaggagcatcgtggaaaaagaagacgttccaaccacgtcttcaaagcaagtggattgatgtgatatctccactgacgtaagggatgacgcacaatcccactatccttcgcaagacccttcctctatataaggaagttcatttcatttggagaggacactctagacagaaaaatttgctacattgtttcacaaacttcaaatattattcatttatttgtcagctttcaaactctttgtttcttgtttgttgatt

SEQ ID NO: 202 - DNA, 938 bp, Arabidopsis thaliana
  source 1..938: mol_type = other DNA
caaaagccgagccgataaatcctaagccgagcctaactttagccgtaaccatcagtcacggctcccgggctaattcatttgaaccgaatcataatcaacggtttagatcaaactcaaaacaatctaacggcaacatagacgcgtcggtgagctaaaaagagtgtgaaagccaggtcaccatagcattgtctctcccagattttttatttgggaaataatagaagaaatagaaaaaaataaaagagtgagaaaaatcgtagagctatatattcgcacatgtactcgtttcgctttccttagtgttagctgctgccgctgttgtttctcctccatttctctatctttctctctcgctgcttctcgaatcttctgtatcatcttcttcttcttcaaggtgagtctctagatccgttcgcttgattttgctgctcgttagtcgttattgttgattctctatgccgatttcgctagatctgtttagcatgcgttgtggttttatgagaaaatctttgttttgggggttgcttgttatgtgattcgatccgtgcttgttggatcgatctgagctaattcttaaggtttatgtgttagatctatggagtttgaggattcttctcgcttctgtcgatctctcgctgttatttttgtttttttcagtgaagtgaagttgtttagttcgaaatgacttcgtgtatgctcgattgatctggttttaatcttcgatctgttaggtgttgatgtttacaagtgaattctagtgttttctcgttgagatctgtgaagtttgaacctagttttctcaataatcaacatatgaagcgatgtttgagtttcaataaacgctgctaatcttcgaaactaagttgtgatctgattcatgtttacttcatgagcttatccaattcatttcggtttcattttactttttttttagtgaa

SEQ ID NO: 203 - DNA, 633 bp, Pisum sativum
  source 1..633: mol_type = other DNA
agctttcgttcgtatcatcggtttcgacaacgttcgtcaagttcaatgcatcagtttcattgcgcacacaccagaatcctactgagtttgagtattatggcattgggaaaactgtttttcttgtaccatttgttgtgcttgtaatttactgtgttttttattcggttttcgctatcgaactgtgaaatggaaatggatggagaagagttaatgaatgatatggtccttttgttcattctcaaattaatattatttgttttttctcttatttgttgtgtgttgaatttgaaattataagagatatgcaaacattttgttttgagtaaaaatgtgtcaaatcgtggcctctaatgaccgaagttaatatgaggagtaaaacacttgtagttgtaccattatgcttattcactaggcaacaaatatattttcagacctagaaaagctgcaaatgttactgaatacaagtatgtcctcttgtgttttagacatttatgaactttcctttatgtaattttccagaatccttgtcagattctaatcattgctttataattatagttatactcatggatttgtagttgagtatgaaaatattttttaatgcattttatgacttgccaattgattgacaac

SEQ ID NO: 204 - DNA, 315 bp, Gossypium barbadense
  source 1..315: mol_type = other DNA
tgatcacctgtcgtacagtatttctacatttgatgtgtgatttgtgaagaacatcaaacaaaacaagcactggctttaatatgatgataagtattatggtaattaattaattggcaaaaacaacaatgaagctaaaattttatttattgagccttgcggttaatttcttgtgatgatctttttttttattttctaattatatatagtttcctttgctttgaaatgctaaaggtttgagagagttatgctctttttttcttcctctttcttttttaactttatcatacaaattttgaataaaaatgtgagtacatt

SEQ ID NO: 205 - DNA, 315 bp, Gossypium barbadense
  source 1..315: mol_type = other DNA
accatatgacactggtgcatgtgccatcatcatgcagtaatttcatggtatatcttaattatatggttaataaaaaaaagatggtgagtgaataatgtgcgtgcattcctccatgcaccaatggtgaatctctttgcatacatagagattctgaatgattatagtttatgttgtagtgaaattaattttgaatgttgtttttaaattttaatgtcacttggcttgatttatgttttaacgaagcttatgttatgtattttactttaatgatattgcatgtattgttaatttaacattgcttgatcagtatactct

SEQ ID NO: 206 - DNA, 2001 bp, synthetic construct
  misc_feature 1..2001: note = Codon redesigned coding sequence.
  source 1..2001: mol_type = other DNA
atggtccgtcctgtagaaaccccaacccgtgaaatcaaaaaactcgacggcctgtgggcattcagtctggatcgcgaaaactgtggaattgatcagcgttggtgggaaagcgcgttacaagaaagccgggcaattgctgtgccaggcagttttaacgatcagttcgccgatgcagatattcgtaattatgcgggcaacgtctggtatcagcgcgaagtctttataccgaaaggttgggcaggccagcgtatcgtgctgcgtttcgatgcggtcactcattacggcaaagtgtgggtcaataatcaggaagtgatggagcatcagggcggctatacgccatttgaagccgatgtcacgccgtatgttattgccgggaaaagtgtacgtaagtttctgcttctacctttgatatatatataataattatcattaattagtagtaatataatatttcaaatatttttttcaaaataaaagaatgtagtatatagcaattgcttttctgtagtttataagtgtgtatattttaatttataacttttctaatatatgaccaaaatttgttgatgtgcaggtatcaccgtttgtgtgaacaacgaactgaactggcagactatcccgccgggaatggtgattaccgacgaaaacggcaagaaaaagcagtcttacttccatgatttctttaactatgccggaatccatcgcagcgtaatgctctacaccacgccgaacacctgggtggacgatatcaccgtggtgacgcatgtcgcgcaagactgtaaccacgcgtctgttgactggcaggtggtggccaatggtgatgtcagcgttgaactgcgtgatgcggatcaacaggtggttgcaactggacaaggcactagcgggactttgcaagtggtgaatccgcacctctggcaaccgggtgaaggttatctctatgaactgtgcgtcacagccaaaagccagacagagtgtgatatctacccgcttcgcgtcggcatccggtcagtggcagtgaagggcgaacagttcctgattaaccacaaaccgttctactttactggctttggtcgtcatgaagatgcggacttgcgtggcaaaggattcgataacgtgctgatggtgcacgaccacgcattaatggactggattggggccaactcctaccgtacctcgcattacccttacgctgaagagatgctcgactgggcagatgaacatggcatcgtggtgattgatgaaactgctgctgtcggctttaacctctctttaggcattggtttcgaagcgggcaacaagccgaaagaactgtacagcgaagaggcagtcaacggggaaactcagcaagcgcacttacaggcgattaaagagctgatagcgcgtgacaaaaaccacccaagcgtggtgatgtggagtattgccaacgaaccggatacccgtccgcaaggtgcacgggaatatttcgcgccactggcggaagcaacgcgtaaactcgacccgacgcgtccgatcacctgcgtcaatgtaatgttctgcgacgctcacaccgataccatcagcgatctctttgatgtgctgtgcctgaaccgttattacggatggtatgtccaaagcggcgatttggaaacggcagagaaggtactggaaaaagaacttctggcctggcaggagaaactgcatcagccgattatcatcaccgaatacggcgtggatacgttagccgggctgcactcaatgtacaccgacatgtggagtgaagagtatcagtgtgcatggctggatatgtatcaccgcgtctttgatcgcgtcagcgccgtcgtcggtgaacaggtatggaatttcgccgattttgcgacctcgcaaggcatattgcgcgttggcggtaacaagaaagggatcttcactcgcgaccgcaaaccgaagtcggcggcttttctgctgcaaaaacgctggactggcatgaacttcggtgaaaaaccgcagcagggaggcaaacaatga

SEQ ID NO: 207 - DNA, 1653 bp, synthetic construct
  misc_feature 1..1653: note = Codon redesinged coding sequence.
  source 1..1653: mol_type = other DNA
atggaagacgccaaaaacataaagaaaggcccggcgccattctatcctctagaggatggaaccgctggagagcaactgcataaggctatgaagagatacgccctggttcctggaacaattgcttttacagatgcacatatcgaggtgaacatcacgtacgcggaatacttcgaaatgtccgttcggttggcagaagctatgaaacgatatgggctgaatacaaatcacagaatcgtcgtatgcagtgaaaactctcttcaattctttatgccggtgttgggcgcgttatttatcggagttgcagttgcgcccgcgaacgacatttataatgaacgtgaattgctcaacagtatgaacatttcgcagcctaccgtagtgtttgtttccaaaaaggggttgcaaaaaattttgaacgtgcaaaaaaaattaccaataatccagaaaattattatcatggattctaaaacggattaccagggatttcagtcgatgtacacgttcgtcacatctcatctacctcccggttttaatgaatacgattttgtaccagagtcctttgatcgtgacaaaacaattgcactgataatgaattcctctggatctactgggttacctaagggtgtggcccttccgcatagaactgcctgcgtcagattctcgcatgccagagatcctatttttggcaatcaaatcattccggatactgcgattttaagtgttgttccattccatcacggttttggaatgtttactacactcggatatttgatatgtggatttcgagtcgtcttaatgtatagatttgaagaagagctgtttttacgatcccttcaggattacaaaattcaaagtgcgttgctagtaccaaccctattttcattcttcgccaaaagcactctgattgacaaatacgatttatctaatttacacgaaattgcttctgggggcgcacctctttcgaaagaagtcggggaagcggttgcaaaacgcttccatcttccagggatacgacaaggatatgggctcactgagactacatcagctattctgattacacccgagggggatgataaaccgggcgcggtcggtaaagttgttccattttttgaagcgaaggttgtggatctggataccgggaaaacgctgggcgttaatcagagaggcgaattatgtgtcagaggacctatgattatgtccggttatgtaaacaatccggaagcgaccaacgccttgattgacaaggatggatggctacattctggagacatagcttactgggacgaagacgaacacttcttcatagttgaccgcttgaagtctttaattaaatacaaaggatatcaggtggcccccgctgaattggaatcgatattgttacaacaccccaacatcttcgacgcgggcgtggcaggtcttcccgacgatgacgccggtgaacttcccgccgccgttgttgttttggagcacggaaagacgatgacggaaaaagagatcgtggattacgtcgccagtcaagtaacaaccgcgaaaaagttgcgcggaggagttgtgtttgtggacgaagtaccgaaaggtcttaccggaaaactcgacgcaagaaaaatcagagagatcctcataaaggccaagaagggcggaaagtccaaattgtaa

SEQ ID NO: 208 - DNA, 936 bp, synthetic construct
  misc_feature 1..936: note = Codon redesigned coding sequence.
  source 1..936: mol_type = other DNA
atggcttccaaggtgtacgaccccgagcaacgcaaacgcatgatcactgggcctcagtggtgggctcgctgcaagcaaatgaacgtgctggactccttcatcaactactatgattccgagaagcacgccgagaacgccgtgatttttctgcatggtaacgctgcctccagctacctgtggaggcacgtcgtgcctcacatcgagcccgtggctagatgcatcatccctgatctgatcggaatgggtaagtccggcaagagcgggaatggctcatatcgcctcctggatcactacaagtacctcaccgcttggttcgagctgctgaaccttccaaagaaaatcatctttgtgggccacgactggggggcttgtctggcctttcactactcctacgagcaccaagacaagatcaaggccatcgtccatgctgagagtgtcgtggacgtgatcgagtcctgggacgagtggcctgacatcgaggaggatatcgccctgatcaagagcgaagagggcgagaaaatggtgcttgagaataacttcttcgtcgagaccatgctcccaagcaagatcatgcggaaactggagcctgaggagttcgctgcctacctggagccattcaaggagaagggcgaggttagacggcctaccctctcctggcctcgcgagatccctctcgttaagggaggcaagcccgacgtcgtccagattgtccgcaactacaacgcctaccttcgggccagcgacgatctgcctaagatgttcatcgagtccgaccctgggttcttttccaacgctattgtcgagggagctaagaagttccctaacaccgagttcgtgaaggtgaagggcctccacttcagccaggaggacgctccagatgaaatgggtaagtacatcaagagcttcgtggagcgcgtgctgaagaacgagcagtaa

SEQ ID NO: 209 - DNA, 253 bp, Agrobacterium tumefaciens
  source 1..253: mol_type = other DNA
gatcgttcaaacatttggcaataaagtttcttaagattgaatcctgttgccggtcttgcgatgattatcatataatttctgttgaattacgttaagcatgtaataattaacatgtaatgcatgacgttatttatgagatgggtttttatgattagagtcccgcaattatacatttaatacgcgatagaaaacaaaatatagcgcgcaaactaggataaattatcgcgcgcggtgtcatctatgttactagatc

SEQ ID NO: 210 - DNA, 622 bp, Cauliflower mosaic virus
  source 1..622: mol_type = other DNA
ggtccgattgagacttttcaacaaagggtaatatccggaaacctcctcggattccattgcccagctatctgtcactttattgtgaagatagtggaaaaggaaggtggctcctacaaatgccatcattgcgataaaggaaaggccatcgttgaagatgcctctgccgacagtggtcccaaagatggacccccacccacgaggagcatcgtggaaaaagaagacgttccaaccacgtcttcaaagcaagtggattgatgtgatggtccgattgagacttttcaacaaagggtaatatccggaaacctcctcggattccattgcccagctatctgtcactttattgtgaagatagtggaaaaggaaggtggctcctacaaatgccatcattgcgataaaggaaaggccatcgttgaagatgcctctgccgacagtggtcccaaagatggacccccacccacgaggagcatcgtggaaaaagaagacgttccaaccacgtcttcaaagcaagtggattgatgtgatatctccactgacgtaagggatgacgcacaatcccactatctagacgcaagacccttcctctatataaggaagttcatttcatttggagaggacacgctga

SEQ ID NO: 211 - DNA, 1446 bp, Cucumis melo
  source 1..1446: mol_type = other DNA
tcccttcagccacttaacacttaaaaatcttaggaaactccatgggctcctctttctccaatgaaattttgacatctgtgttgttgatagctcctatatcctttgagaatttgatatacacctgtcatttgctgatttgtggataactgttagccttttgatattgatacgttcctttttttatgaatttttgtaaatccattcaattttaatgctgtcgtaaatgaaaagccctttcattaatgttgtttatatacatattttaaaattaattcaataacaagtttagttctgttagcttctaggtttgtatctattttatctattaaaggtatgtttgggcttcaggttggaatggagtagaattgaatgggttggggagtaaattttccattcaacaagttcaatttcaaaatggctaataagttttgaactcaattttattttcaataaattccttaattttttgttccttgtttgtaaactattgacttattcgatatattttaaaattgaggtattttaaaaaaataatacaatattaaaattatttataaaatataacaaaatttatgtatagtttatttgaaaattttactatagtttcatttttatattattcctaaccatttccatttaaaattatttcaattatttcttttattaatataattgaaatttcatggatttattagacacatgatttgaaattttatgggtttattaagtattttctaacacaaaatcgcttccgcatcgttttcaattcattcagtaatagaagtaattttttaaaagaaccaaatttgccaaattttgagttccataaggactctgaaaactcattatgtctattactcttcactaattgtagagacttaaattcaagataagagacactaattgatgataattgcccaaaaaataaaaataaaaatgtttcttccccatcctcaacctccatgaattcacagagcccaaagattaattattgggccccaattcctactcatatataccttacagtccctcaaagaaatcttaggaagtaatcaatttctgtttattcaagatgtagcctcccaaaagaaaaatacatcacatcaaattcaaacaaaaatatctacagctagcaaaacctcaaaccgttaaaatttcaagccacataaatgaaattttcatctgaaaaaaggacaatctatctagacgttagatttcagccctaatatgaatctgaagcatttggtggacgagaaagagccatgtaggaatgcatcaaacaaaggaaaaatctttgaactccaatgggattgaagatacagataccaatggataagaatctgttctctttgcccactatttaaactcaccaaacccaccagtatcttcctcaccacaaaatacattccaccgttgatcacaagccttattccaccacctccaaca

SEQ ID NO: 212 - DNA, 2018 bp, Cucumis melo
  source 1..2018: mol_type = other DNA
actattggagacgacgaaggaaaactctaatgtgagcttagaattgaagatggtgaacaattgggagtcttttttaaaaatctttcgtcggtatattgaaatttccttttacactcaaataaccccccttttcacgcgttcaacgtcttcaaaccttcctttttcaattattttttcgtttacattaatgacatttaggtaataagataaattagtggattcttttgtgaaaaatgttagcccatttaagacttttatgaaatatattagaaaaaaatcatatagcaatttatattattctagttaaaagcccataatagaaactaacccaacctaaagtaacgtaaacattcaataagagagacaaattttaaaataatttctaattaaaaaaaaaattgtcaagaccgtccgggtcggatccaaaatataacccgaaccggccggtttagcatctatataaatacacctttagggtttttattctctcaagacttcaccgcatttccacttctctgaggccacggtcagccattggagcagctcaataatcctttgactccctactacggtaagtcgaccttactgctttcggcttctagttttttcaatcctgtcattagtcctttggagttcttctgtacatttatgacgttttcggctcgtgttttgtttcgcctgtatgtagtgggtttttcgagttttgtttttacttttttttatacttgcaggaattagttgaaatctatgtacttcatgccttggataatactcttgatctgttgtgttattcaaaatgaattgttttaagatggtatttgagaatggtcatgtgagttttgcctacttggttattaaaatgaattgttttaggatggtatttgagaatggtcttctgggtatttggttggaacctttgtgctctgctatgaattagggtgttctccccgtttttttttttttttttcttttggttattaatatatcttttatgactacttattcatatatgatatcttttactcgtaaattttgactcatttgaaagttttatccttagtcctttctcattcagggtgtaaaggtatgttgttagggttaaaatagcctatgcaggaaagttctgtatttgttctaattattgcatttgtgtgcatttgtatctagtttatttcttgctgagagtatgcttcattttttagtacacatcacttgtgccactttattatagttgcacatttttgtttatggagaggatgaatagcatttagggatgtcaattttttattgagaaaaccctctctcctacttaagcttggggaatttttgttctaaatgtggtaaacataatacttcttcttattttaatttgaatggaaggggaagacgaatactaatattttcaacgaaccttcacaactttttttttcttatttaggaagccatgtttttcaaaattgtactgtgtgatccacatatttatcgattattagtgaatcgaataataattagagttttattggtataattttgaagttcagacttattacatttgtggaaagtttggttacaattttcaattttattggaatcctaagaactttgtgttaacatatattgagttttcttctctttttttttactcattaagttctctattaggaatgtttggttcaatgtcacatagtcgatagctaagaccagtgacccacaaagctatgattgaacgaaaaacaagcctttcacatcttggtaggaatttgttatttctcaatagatttacagagctgtttcatgtgatcacaatttttttctatttttctgaagttctctattaggaatgggctatctggttagttgcttttgagagaacatgtggattggtgttgctcggtttccttgcctttgtaattttgtccttggaaaaagcaaaatgattaggtatcctgatatgcataacatgtttaagccaactagttctcacttttttagtgcaaataattgatcttcaggaatcg